European Patent Application EP 4 428 233 A1, published September 11, 2024. Title: C2C9 NUCLEASE-BASED NOVEL GENOME EDITING SYSTEM AND USE THEREOF. Applicant: ShanghaiTech University. Application WO. The sequence listing filed with the application follows.

SEQUENCE LISTING (308 sequences)

SEQ ID NO: 1 - protein, 76 aa, synthetic construct
LHQITKRLTTGFAVVALEDLNVAGMTRSARGTVAAPGKNVRQKAGLNRVILDSAPAELRRQVNYKATWYGSELAVA

SEQ ID NO: 2 - protein, 67 aa, synthetic construct
AELRRQVNYKATWYGSELAVADRWFPSSKTCSGCGWQNPHLKLSDRVFRCTDCGLVMDRDMNAARNI

SEQ ID NO: 3 - protein, 506 aa, synthetic construct
MVQTEILKAFRFALDPTSVQVAALSRHAGAARWAFNHALAAKVGAHERWRAEVAKLVGDGVPEEQARRQVRVPVPMKPAIQKALNAVKGDSRKGLDGACPWWHEVNTYAFQSAFIDADQAWKNWLDSLSGKRVGRRVGYPRFKKKGRARDSFRLHHDVKKPSIRLAGYRRLRLPRIGEVRLHDSGKRLARLIDRGDAVVQSVTVSRGGHRWYASVLCKVTVQVPDRPSRRQRERGAVGVDLGVKVLAALSKPLVVDDPSSALVRNPQHLRQAERRLLKAQRALARTQKGSARREKAKRRVGRAHHEVAVRRHAALHQITKRLTTGFAVVALEDLNVAGMTRSARGTVAAPGKNVRQKAGLNRVILDSAPAELRRQVNYKATWYGSELAVADRWFPSSKTCSGCGWQNPHLKLSDRVFRCTDCGLVMDRDMNAARNIERHAVLIDRNVACDRRETLNARGASIRPTTSRGGRHDASKREGSGARPESPQQSDLLTLPTLNNETATPP

SEQ ID NO: 4 - protein, 493 aa, synthetic construct
MSGAIQRSHATETREVLRAYRVTLDPTPDQESMLAQHAGAARWAFNHALAAKVDAHERWKTAVAELVAAGVPEEAARKKIKVLVPGKQVIQKALNAVKGDDRKGIDGACPWWHTVSTYAFQSAFLDADMAWKAWLDSLTGRRKGRRVGYPRFKKKGRSRDSFRLHHDVKRPTIRPATTRRLLLPRIGEVRTHDSLKRLKAALGRRSGVIQSVTIARGGHRWYASVLVREQMLMPAPTRAQQAAGTVGVDLGVHSMAALSTGEIIPNPRVKARHAPALAKASRAYARTVKGSRRREQARRRLARLHHREATRRSTGLHHLTKRLATGWAVVAVEDLDVAGLIRSAKGTVDKPGRRVRQKSGLNRSILDVSPGEVRRQLDYKTGWYGSTIAILDRFYPSSKTCSGCGGRKPNLTLSERVFICTICGLSMDCDVNAAVNIARFAVASDRGETLNARGASVRPSHLQVGRPDALMREDPPEGGPPQHSDALASSTPT

SEQ ID NO: 5 - protein, 537 aa, synthetic construct
MTSTTLAPEEPLMVFRGARFRLDPTGEQQGILSQQAGAARVAYNMMCTLNKDILEARSQLYSTLIKDGKTKDKAKKELKAAAKEDPSLAIVWARDFDKNYITPERNRHKHAAQRIAAGENPVDVWNPDEERFNEPWLHTANRRVLRSGQKQYEQALDNFFKSQNGSRAGQKMGKPRFKTKIRSTDSFTIDAVDVSSSTTLIRDIGPKDHARYKTGEASTGIIADYRHVRLSHLGTFRVFGSTKALVRQLDRGGRIKSCTVSRSADRWYVSFLVELPIEIARSTPTKKQYKAGAVGIDLGVKSLAALSTGEIIPNPRFLRTADKKIKKLQRKIARCQKGSKNSIRLKRRLARCHHELALQRAGYLNELTSMLASSFSAIALEDLNVAGMTSSARGTVENPGKNVKQKAGLNRSILDISPGRIRTLLEYKCTDRGVELQVIDRFFPSSQLCSSCGSKTTIPLAQRIYHCDVCGGVIDRDVNAAINIVYEAKRLVEQKCSEHSAPEGAEDKRPWSVHLPSTQYVDGLYTRKRQGPSGHSS

SEQ ID NO: 6 - protein, 537 aa, synthetic construct
MTTREILRAYRVPLDPTDAQTAALASHAGASRAAFNWALGAKVHAHRMWSACVADLTYTRYGHLDADQALAAAKKDASRYYRIPTSQTNEKAFDRDPDYAWRTEVNRRSWVSGMRQADTAWQNWLDSLTGRRAGRRVGYPRFKSKGRCRDSFTLAHDVKRPSIRPDGYRRLTLPKKISVTGSIRLKGNIRHLARRIRRGVARIQSATISRAGNGWSVSILALETLDIPDHPTPRQQAAGAVGVDVGVHHLMAFSDATIIDNPRHLRAAQKRLTRAQRALSRSKWRLPNGDLIDTPKRGQRVTPTTGRVKARARLAREHAAVAQHRASTLHAITKQLATSHAVVAVDDLNVAVMTRSARGSIDKPGRNVAAKAGLNRSILDASFAEMRRQLTHKTSWYRSQLLPSGCFVPTSRTCSTCGAEKANLPLSERVYHCENCATVLDRDVNAAKNVLRAALASHDAPGMEESQNARGGRGETSVARRSAKREDPPRGGPPRPCNRVRSSPPDGEAKVRANASPTNCKARKHSTPQGSAPRTRR

SEQ ID NO: 7 - protein, 492 aa, synthetic construct
VAQVETLRAYRFALDPTAAQLADLNRHAGAARWAFNHALGVKVAAHRQWRAQVDALVSGGMPEAQARKSVKVPVPGSQAIKKALNTLKGDSRAETELPDGFHGLHRPCPWWHEVSTYAFQSAFIDADRAWGNWLDSLTGRRAGGPVGYPRFKRKGRARDSFRLHHDVKKPTIRLDGYRRLQLPRLGSIRVHDSGKRLARLVAKGQAVIQSVTVSRGGNRWYASVLAKVVQEVPGKPTRAQTGRGTVGVDWGISHLASLSQPLDPADPGSIHIANPRHLDQWTRQLAKAQRALSRTERGSRRRVKAARKVGAIQHRIAQRRASTVHLLTKKLATGFATVAVEDLNVRGMSASARGTVEKPGRRVRQKAGLNRAILDAAPGELRRQLTYKTSWYGSALAVLDRWHPSSKTCSSCGTARPKLTLSERVFHCTTCGLAIDRDHNAAINIARHAAVPLVEGDVNARRSPPPADNGRHGRAARQKREGPPPGGPPRRE

SEQ ID NO: 8 - protein, 553 aa, synthetic construct
MSETTASSDVRAYKFRLDPNKAQVVRLSQCAGAARVGYNMLIAHNREIHQEARRRRDALIASGVDPAAADAKLREQRRTDPAVRMLSYQQFSTTHLTPEIARHRAASDAIKAGADPAEVWADERYAEPWLHTVPRRVLVSGLHNAWDAFTNWMTSFTGQRAGRRVGYPRFKRKGRSRDSFTIPAETTGGKGTRYHHSDPHKGVIGDYKHLRLGPLGTIRTHQHTRRLVRACEHGGRITSFTVSRAADYWYVSVLVETPAAEPPAPSRAQRSRGAVGVDVGVHSLAALSTGELIANPRHGQATREKLTRAQRAFARTEKGSRGRQRAAVRVARIQHKLALQRATTLHKLTKALATGYETVAIEDLNVAGMTRSAKGTVENPGKNVAAKAGLNRSILDAALGELRRQLDYKTRWHGSTVTTIGRYDPSSKACSSCGTVKPKLPLSVRVYDCDQCGMSLDRDVNAARNILAWASNGRDSFTVPQTEVGADGRGGPTPPSPRGEGTLVRDQRSVKTGRRRRPATSAEQSAGHLATPREQTAPPERETPSSGASLHVR

SEQ ID NO: 9 - protein, 539 aa, synthetic construct
MSQDKKDETVDHRAFKFRLDPTDAQLSLLAQSAGAARVGYNMLLGHNVAAYQARQELHASLLDSGHNEHDAKSAVTDRKTHDPSLQTLSYQSFSTHYLTPEITRHRIASDAIKAGADPSKVWNDPRYETPWMHTIPRRVFISGLQHANTAYTNWFASMRGDRAGARVGRPRFKKKGRCRDSFTIPAPEAMGAKGAPYKRGEPRSGVIEDYRHVRLAFLGVLRTHNSTKRLVRACQRGGKIKSFTVSRNADRWYVSFLVASPARAAVTTKRQRANGAVGVDVGVHSLAALSNGEVFSNPRHGQLAQKKLKRAQRKLARTQKGSKGRARAAQRVGRLQHLVTLQRETTAHHLTKYLATHYCAVAIEDLNVSGMTRSAKGTMEHPGKNVKAKSGLNRSILDASFGRIHQQLRYKMGWSGADLQIIGRFVPSSKMCSECGTVKSKLPLSERVYECEHCGLKIDRDVNAAINILHAGAGSITPSNSPLTRGSLNGRGDQTCLSPSGERITRGDSRSVKADPIWCRSPQTSNRCSSLTVRGTALK

SEQ ID NO: 10 - protein, 552 aa, synthetic construct
MSVATDAPTQRLRAFKHRLDPNASQLELLGQYAGAARVAFNMLTAHNRAALQAGWDRRRQLAEAGVPAEELVGRMKAERAADPALKVAGYQQFATAHLTPMVRAHREAAEAIAAGADPGQVWADERYAQPWMHTVPRRVLVSGLQNAAKATENWMASACGARAGRRVGLPRFKKKGRSRDSFTIPAPEVIGAAGTAYKRGEARGGVITDHRHLRLASLGTIRTMDKTTRLVRSCRRGAVVRSVTISQAGGHWYASVLVAEPVTLRRGPSRRQRANGVVGVDLGVKHLAALSTGELIPNARAGQAQARRLARLQRALARTERGSRRRERVRRQISALHHQVALRRTGMLHEVSTRLARDYAIVALEDLNVAGMTGSAAGTIEHPGKNVAAKAGLNRAILDAGLGTLRAQLHYKTSWAGSQVKMIDRFAPSSKTCSRCGAVKATLSLRERVYECEVCALVIDRDVNAAINIRAWAVQEGTGHRVELAQGNGESQNGRRAAGRTPPSGGPTGWQRRSVKPAPRGAGRSSRATGWSSHTPHIEREHAEADVFGPVR

SEQ ID NO: 11 - protein, 485 aa, synthetic construct
MVRSVGDDLRAYRFALDLRPAQLRAVAEHAGAARWAYNHALGVKFAALKQRQTVIAELVTAGVDAQAAARRAPRIPTRPQIQKDLNATKGDSRSGVDGLCPWWWTASTYAFQSAMIDADRAWHNWMSSVTGQRAGRRVGRPRFKSKHRCRDSFRIHHNVKQPTIRPDTSGYRRLIVPRLGSLRTHDSTKRLRRALDRGAVIQSVTISRGGHRWYASVLVKTPDAPAVGPSRAQRKAGIVGVDIGVHSLAALSTGELVVNPRHLNSSCDRLGAAQRALARCQKGSNRRRRAARLLGRRHHELAERRATALHQLTKRLATCWSVVAVEDLHVAGMIRSARGTVDKPGRNVRAKSALNRAILDVAPGELRRQLAYKTVWYGSSLVVCDRFYPSTQTCSACGAKAKLTLADRVFRCTACGFGPTDRDINAARNIAANAAVASGAGETLNARRADQQHLPQVGPCRRPAMKREGHHQSKTDSGHLSRATG

SEQ ID NO: 12 - protein, 569 aa, synthetic construct
MPLNGWTMLAQEEVRAMTTTTGTDLAPRLRAFKHRLDPNPAQATLLAQYAGAARVAYNMLIAHNRAALAAGAARRTELAESGLAGPELAARMKAERAADPTLRVASYQSYSTAHLTPLIRRHREAAAAIAAGADPAEAWTDERYAEPWMHTVPRRVLVSGLQNAAKATENWMASASGTRAGARVGLPRFKKKGRSRDSFTIPAPEVIGAAGTPYKRGEHRRGVITDHRHLRLASLGTIRTYDKTSRLVRACRRGAQIRSMTISQAGGRWYASILVADPTPIRTGPSRRQRANGAVGVDLGVKHLAALSTGEVIDNGRPGARQAARLTRLQRAYARTQPGSNRRERVRRQIAALHHGIALRRAGLLHQVSTRLAMDFAVVALEDLNVAGMTRSARGTLEAPGRNVAAKSGLNRAILDAGLGMLRRQLDYKTSWAGSQVKMIDRFAPSSKACSRCGTVKSTLSLAERTFECEACHLVIDRDVNAAINIRAWAVQEERRAGVELARGRRESRNGRGAAVSGPPSGGAAGQGRGSVKPAPQGVGMSSRATGWSSQPPSTEGESAERGASALAR

SEQ ID NO: 13 - protein, 505 aa, synthetic construct
MGEQLRAYRYALDLTDAQASVVAQHAGAARWAYNHAIATKFKALDERQAAIREAVDAGVDPAVAANLAPKIPSKFDIQKALNKVKGDDRTGREGECPWWHSVSTFAFQSAFSDADRAWKNWLDSITGNRKGRRVGRPRFKAKRRSHDSFRIHHDVKNPTIRPDVGCYRRIRVPRLGSLRVHSSTKQLCRALDRGAVIQSVTISRGGHRWYASILTKQEIVSEVLPTRRQRLAGTVGVDLGVHTLAALSTGETVSNPRHANMARTRLTKAQGALSRTKKGSNRRRRAARLVGRRHHEVAERRASTLHAVTKALATRWATVAVEDLNVAGMTASARGTVDKPGRNVRAKAGLNRAILDVSPGEFRRQLEYKTAWYGSALAVIDRFYPSSQTCSACGARAKLTLAERIYRCAACGFTADRDVNAAINIAAQAAVAPGKGETINARRAVSDHPQPAGTRSLTAMKREGHRDNAVVTPTRQRVGHPIRCGMRLDERIGAGQEASAPHAYG

SEQ ID NO: 14 - protein, 561 aa, synthetic construct
MKELAADGIPVAVTCRVLKLARQPYYRWLAQPVTDAELVEAHRANALFDAHRDDPEFGYRYLAEEAREAGEPMAERTAWRICSQNRLWSVFGKRKRGKNGKTGPPVHDDLVERDFTAEAPNQLWLADITEHRTGEGKLYLCAIKDAFSNRIVGYSIDSRMKSRLATTALSSAVARRGDVAGCILHSDRGSQFRSRRFVQALNHHAMVGSMGRVGAAGDNAAMESFFSLLQKNVLDRRRWDTREQLRIAIVTWIERTYHRRRRQAGPRTIDPHRIRSDYERTGQSGRVTETVTYSCSRPAGRVGVDLGVHHLAALSTGELIDNPRHHRQARRALTKAQQALSRTEKGSQRRRKACATLARRHHLLAERRATTVHGITKRLATGWSEVAIEDLNVAGMTRSARGTVESPGVNVAAKAGLNRSILDAAPDELRRQLTYKTQWYGSRLAVCDRWFPSTQACSACGAKAKLTLADRVFHCPACGFGPINRDHNAARNIAAHAVIVAPGTGETENARRADAGPPPRVETTPPSVMKREDHPTRVATSAEQSADHPKPADQHTLPLVN

SEQ ID NO: 15 - protein, 496 aa, synthetic construct
MAQVLRAFRYALDPSPPQLETLQRCAGNARLAFNFALAMKKDAHQRWRDEVDILITTGLSEKDARTRLKGTSKIPNKPDVYKAFQHLRGDAAQGIDGIAPWHAEIPTYVFQSAFQDADRAWKNWLDSYTGKRAGRRVGYPRFKKKFRSRDSFRLHHDAKKPKPALRLEGYRRLRLGGALKTVRLHGSAKPLHRLVSSGRAVVQSVTVSRGGTRWYASVLCKVETDVPDPTHRQKANGRIGLDWGLNHLAALSTPLDGHHLVDNPRHLRHASKRLTKAQRALSRTQKGSARRRRAAARVGKLHHLVAEQRATFLHTLTKRLTTTFACVAIEDLNVAGMTRSARGTVQLPGKNVSSKAGLNRSILDAAPAELRRQLEYKTSWYGSHIAILDRWFPSSKTCSGCGWRNPSLPLSEREFVCAECGLRLDRDLNAARNIAAHAEVPASGTGAPGRGESVNARGGCVSPRLLRESGQHPSKREDAAPSGPAPPRRSNPPTFP

SEQ ID NO: 16 - protein, 499 aa, synthetic construct
MAEVLRTFKFALDPTSTQLQTLGRYSGNARLAYNFALAMKKEAHQQWRDRVDTLVATGVDEKAARDRLKGTVKVPKKPQVYKAFQLLRGDAAKGIEGLAPWHAEIPTHVFQSAWINADRAWQNWIDSYRGTRAGRRVGYPKFKKKFRSRDSFRLHQSSGRPVLRLEGYRRLHLSGQLGTVRLHGSAKRLHRLVSSSQAKVQSVTISRGGSRWYANVLCKVDSNLPGPTRRQRANNRVGLDWGVHHLAALSTPIEGTTLVDNPKHLAKATTRLRKAQRALSRTQKGSKRRHTAASRVGKLHHQVAEQRATFLHALTKRLCTTFAFVAVEDLNVAGMTHSARGTKDKPGTNVRAKAGLNRSILDAAPGELRRQLEYKTSWYGSQLALCDRWFPSSKTCSACGWQNPSLSLSERVFVCAECGLRVDRDLNAARNIAAHAEVPSGTGAPGRGESVNARGGRVSPPLSRERGQRPSKREDAGLKGPAPPRRSNPPTSLTRVSRT

SEQ ID NO: 17 - protein, 560 aa, synthetic construct
MLIAHKIKLLPTPEQAALFRRCETVAKATYNQALRMWQEDYQRYLREMVALCGSRGISALTDSPRCLWPRFKKRSDLEKELIAAGVAKDDIPATSGFRWISKHYANRPAHWEDLGYWPGAGKITNLKDAANHFFKDGFGYPRPIKEDDVCGFLVLSSAEKCGGKKDANGRHNGPFARHVDRPVWQRPLEFNVPKIGKVRMAEPLRFEKFETQKKISPRGKNEGQEIETFPVASVTISRNKAGDWFASILCSVPEIEPNAPVRDYKVGVDLGIKTLAKLSDEVPGQPDRFPARKALSNAERRLLRLERKMSRQQAQAARRKRKLSECKNYQKTKRLHALAWKKVGHRRESYSHQLTTVLVRDYPVIGIEDLGVKGMMRKGKPGNKPKKARLNRAIGDAGFGRFRIQLEYKAKWHRREVHYTPQFEPTSKVCNQCGWKNEKLKLSDRQWRCGGCETIHDRDLNAALNICRKSVPKSSDDPSVAGKDEKDVKSGSAKSRRGRFVSRKSEGDSSSPFDPGAVDTEQSVVGAPNGQKALEEATGHRRNNADFSRSSGFKSRLDGY

SEQ ID NO: 18 - protein, 532 aa, synthetic construct
MSYLCARGRFNLSGFSTGSMGVLPVRASLFALLFTTLHGARISAHWYGMSKENDHTVTCIKICLEPNKAQRAQFASFAGSARWAYNFALAIKIGYQKRWFEARKQFIESGLDEKAAGKKASEQVGRMPNYMSIATNEWTQLRDEVCPWYPEVPRRVFVGGFQRADAAFKNWFDSKSGRRSGAAMGWPKFKSKSKSRESFVIANDVQPAFVANLNRYIKTGELADMDYRHIKVPKCGEVRLTPGSAGQLRQLGRTMLAEAKTGELITRITSGTISRLGDRWYVSLVISGPFVPDAISTKRQRRNGVVGVDLGSGRFYATTSEGLSIINPKFVSKYEQELARANRALAKTAKGSAARKKALARLRRVHARSALARDGFSHQVSAWLTSQFAGVAVEKFDLASMLASAKGTVEKPGKNVDVKARFNAHLADVGIASTIDKLLYKGKRDGCRVQVVNTLDNSSTTCAKCGHTCVCGPEQKTFTCPDCGYNAPRQLNSAQYIRQLATVGFDELGLDMTASLTPDTGKRPIAFMTSAH

SEQ ID NO: 19 - protein, 579 aa, synthetic construct
MTGAKQKTPIRVVRFSIDHSALTPAQVVAFARHAGAARQTWNWALGRWMDWRNNTKFYVDYKVFKAAGMGPGLSTDDLIQVIERAVSIRQDDKWMDAAWDEARQIHGEWDQFQKASTLQSLYLAGAQEPFDPSRDDGINPYHWWVTEGDKSGLPKAERHNVNSGATYTAPLRAFEEAVGRFYKLPGKKGTPKFKSKHDDEQGFCIQRLTETGLSPWRAIEGGHRIKVPSIGSIRVVQSTKRLRQLIKRGGKTTSARFTRRGGKWFVSVSVAFDLSAPRVQRPARLSRRQRAGGSTGVDLGVNRLATLSSGDQFPNRRLLRKSMAEIKRLQRKFDRQHRAGSPECFNEDGTHKKRCRWGREDGPAMSRSAQTTKRQLRRIHDLTARRRAGVLHEITKDLATRFELIGVEDLNVAGMTAKSKPKPDPDRPGHFLPNRRAAKAGLNRAILDVGFYEFKRQLGYKTEWYGSTMQMVHRYAATSKTCSGCGWVKPKLTLAERTFNCTQCGLAMDRDHNAAVNIRALALEGAAPMEREQPAPVGAAEKRHRDPVSHRRRPKSLAPCESTRPVRDLSPPATQEETA

SEQ ID NO: 20 - protein, 540 aa, synthetic construct
MATTDKKDEENLRAYKFRLDPNQAQTTALYQAVGAARYTYNMLTAYNLEVNRLRDDYWKRRHDEDISDADIKKELNALAKEDKRYKQLNYGAFGTQYLTPEKKRHEQAEHRIENGEDPSVVWNQETERSANPWLHTANQRVLVSGLQNASDAWDNFWASRTGKRAGRLVGTPRFKKKGVSRDSFTVPAPEKMGAYGTAYLRGEPAYKQGRRKITDYRHVRLSYLGTIRTFNSTKPLVKAVVAGAKIRSYTVSRNADRWYVSFLVKFSEPIRRSATKRARAAGSVGVDLGVKYLASLSDSEAPQRFPNLKFVEGLPSLENPRWSEASSRRLHKLQRALARSQKGSNRRSRLVKQIARLHHMTALRRESNLHQLTKKLATEYTLVGFEDLNVSGMTASAKGTVENPGKNVAQKSGLNRVVLDAAFGVFRNQLEYKAVWYGSAFEKVDRYFASSQTCSECGRKAKTKLTLRDRVFDCAYCGNMMDRDLNAAVNICREAQRLFDEKLASEDRESLNGRGSRGALRGAETVEASRPPASHRRGSP

SEQ ID NO: 21 - protein, 549 aa, synthetic construct
MAAAECSTQKAHRAYKFRLAPNQKQLTALYQAAGAARYAYNQLTAYNLDALRRRQQYWGTRQDEGASESEIKAELRAIAREDASYRLLGYIPYATEYLTPERRRHQDAAAQIAAGAQAHLIWGADEHFEHPWLHTASRRVLVSGLQSADKAWKNFWDSRTGARAGRLMGTPRFKKKGFSRDSFTIPAPEAMGAYGAAYLRGEPAYVRGRRTITDYRHVRLSHLGVLRTYDSTKPLVKAVAAGAHIKSYTVSRHAERWYVSFLVELSQSPRRQASKRARAAGTVGVDLGVRYLASLSDPQAPQRLTQLDFLADTPSIKNPRWADRAARRLHRLQRALARSQKGSVRRARIRQQIARLHHKTALRRESNLHQLTKRLATGYTLIGVEDLNVAGMTASARGTVEHPGRRVAQKSGLNRVVLDAGFGVFRRQLEYKSTWYGSAVQEIDRYYPSSQICSQCQRKAKTKLSLRERVFECALCGYKADRDFNAAVNIAVQAQRVFEEKLASESGESLNGRGGGRTHKGAVVIEASRPPAGYGSGSPQVSNHLPIRT

SEQ ID NO: 22 - protein, 541 aa, synthetic construct
MTATAAAETVMDLRAYKFRLDPNIAQTQALSQAAGAARVAYNMVIAHNRAAHDEGRRRVEELTASGVDPEEAAARVRAQRTTDPALAMVFTKMGFNAILTAERRRHQEAAEAIAAGADPAQVWAGQRYERPWLHDANRRVMVSGVEHATAAFTNWVNSYTGQRAGRRVGYPRFKKKTVSRDSFTIPAPELMGGKGAPYKRGEARKGLITDYRHLRLGFLGTIRTHQHTRRLVRACQRGAVMRSFTVSRAADRWYVSILVATPRETAPEPTRAQRARGGVGVDLGVNNLAALSTGELVDNPRYGRRGAAKLRRAQRAYARTKKGSQGRARAARRVARLHHLVALQRSTVVNTLTKRLATGYAVVAIEDLNVSGMTRSAKGTVENPGKNVAAKSGLNRSVLDAAFGELRRQLEYKTAWYGSSVATIGRYEPSSKACSSCGAVKPKLSLGERVYDCDQCGMRLDRDVNAARNILAWATGGRDQPPAPGTGADGRGEPAPPSPPGEGPPAPVQRSAKTGYVPHPATAAEQSAAHPHQSRTPIPPS

SEQ ID NO: 23 - protein, 558 aa, synthetic construct
MAEKTGTDAGTMNRAYKFRLDPNQAQKAELMRCVGAARYTYNLLNAYNLQILRNEQEYRNTRNAEGADYETINGEIRKLRKKDPAYKFLGHAEYEKRYLTPEKQRHEAIAQAIADGADPAIVWPETERFTEPWLHTIARRVLVSGIKNADKAWDNYNKSRMKQRAGARIGIPRFKRKGVSRDSFTVPHETTGAYGAYYHKKDPEYARRKAQLKRRGISVKPTITDYRHVRLASLGVIRTHNTTRPLVKAVRAGAEIKSFTVSRAADRWYVSILVELTRPSTAPTRAQRAAGAVGVDLGVRYLAALSDEQAPQRFARYPDLEFTGDGDPTLANPRWARTAEKRLVRLQRALARAQKGSNRRARIVQQIARHHHLVALRRESGLHQVSKRLTTGYTLIGLEDLAVAGMTASAAGTIEAPGKNVRQKAGLNRSILDAALSALRRQLEYKSSWYGSQVQIIDRFFASSQTCSACGARAKTKLGLHVRVFECAACGARIDRDVNAARNIRAEAVRMYEAQLAPGTGESLNGRGATDSDAAGSVVLGDAALDASRPAATGGGSP

SEQ ID NO: 24 - protein, 559 aa, synthetic construct
MAKKISTDADTTLRAYKFRLDPTQTQKIALAQCAGAARYAYNLLTAHNLEVSRVRADYWHTRIDAGAEETTVKAELKALAKSDAAYKSIGYAAYGTQYLTPEINRHRAASNAITDGADPAAVWPETERSSEPWMHTIPRRVLVSGLQSADKAWKNFFDSRTGARAGRLVGTPRFKRKGASRDSFTIPAPETIGAYGTAYLRGEPEYARRKAQLKHRGIKTAPTIEDYRHVRLSHLGVIRTHNTTKPLVKAVRAGAQIRSYTVSRAADRWYVSILVELTRPSATPTRAQRSAGAVGVDLGVRYLAALSDEQAPQRFARFPSLEFTGDGAPTLANPRWARAAEKRLVRLQRALSRAQKGSNRRARIVQQIARHHHLVALRRESGLHQVSKRLSTGYTLIGLEDLAVAGMTASAAGTIEAPGKNVRQKAGLNRSILDAAFSTLRRQLEYKASWYGSQVQIIDRFFASSQTCSACGARAKTKLDLRVRVFECAACGVRIDRDVNAARNIRAEAVRMYEAQLAPGTGESLNGRGVAGSDAAGLVVLGDVALDASRPAATGGGSP

SEQ ID NO: 25 - protein, 559 aa, synthetic construct
MAKKTSTDAETMNRAYKFRLDPTQAQKAELMRCAGAARCTYNLLNEYNLQILRNEQEYRRTRAAEGIDHKTITSELKKLGKKDPEYKFLGQAEYEKRYLTPEKQRHEAIAQAIADGADPAIVWPETERFTEPWLHTIARRVLVSGIKNADKAWDNYNKSRMKQRAGARMGVPRRKRKGVSRDSFTIPAPEAIGAYGTYYHKKDPEYARRKAQLKRRGINAAPTIEDYRHVRLSHLGVIRTHNTTKPLVKAVRAGAQIRSYTVSRTADRWYVSILVELTRPSATPTRAQRAAGAVGVDLGVRYLAALSDEWAPQRFARYPSLEFTGDGAPILANPCWARAAERRLVRLQRALARAQKGSRRRARLVQQIARHHHLVALRRESGLHQVSKRLSTGYTLIGLEDLAVTGMTASAAGTVEAPGKNVRQKAGLNRSILDAAFSTLRRQLEYKSGWYGSQVQIIDRFFASSQTCSACGARAKTKLDLRVRVFECAACGVRIDRDVNAARNIRAEAVRMYEAQLAPGTGESLNGRGAAGSDAAGSVVLGDVALDASRPAATGGGSP

SEQ ID NO: 26 - protein, 485 aa, synthetic construct
MTTEIAHKAFKYRLKPTQTQENAFRQAVGAARVAYNMLTALNRDVLRRGWEIRNQLIEQGLSEAEASAQMKKLRKEDLSLKIMSSFAWQKDVLTPEIARHKQAAARIAAGDPIESVWSGERFAEPWFHAVPRRAFVSGADQAATAISNWMKSVAGQRAGNKMGLPRFKKAGRSHDSITIPVVDGSSPAGGYGASYKRGEPRKGFIQDHHRLRLAMFGTVVTYNSTAPLTQLVTQGGTIKSFTISRDAQYWYVSLLVEAPINLLHRPGPTKAQEKAGVIGVDLGVKAKAALSNGEIINNPRHLQLSLKRLAKLQVKLSRTQKGSKNREHLKKQISRLQHKIALQRAASNHQMTKELSTTYVGVGIEDLNVAGMTKSASGTLENPGKNVAAKSGLNRNILDVSFGQIRNQLEYKTKMYGSALTVIGRYEPTSKRCSQCGAMKSDLSLKERTYICVECNYQDDRDINAAKNIRNLAEKELGMVSSISS

SEQ ID NO: 27 - protein, 562 aa, synthetic construct
MAKKTSTDDGALYRAYKFRLDPNQAQKAKLMQCVGAARYTYNLFTDHNRKVSRACAEYVDTRISEGATEVIAKAELDDIKEENPAYKYIGHFEYGKRYLTPERQRHEAIAQAIADGADPAVVWPETERSSEPWMHTIDRRVLVSGIKNAHAAWGNYFESLKGLRAGPRMGVPRFKRKGISHDSFTVDRDPRNDELGGYGTPYKKGTPEYARRTAQLKRRGIKTIPTIEDYRHVRLASLGVIRTHNSTKPLVKAVRAGADVKSFTVSRAADRWYVSILVKLSRTPVTPTRAQRAAGAVGVDLGVRYLAALSDEQAPQRFAQYPSLEFTGDGSPTLANPRWARAAEKRLVRLQRALARAQKGSNRRARIVQKIARHHHLVALRRESGLHQVSKRLATGYTLIGLEDLAVAGMTASAAGTIEAPGKNVRQKAGLNRSILDAAFSTLRRQLEYKASWYGSQVQIIDRFFASSQTCSACGARVKTKLGLHVRVFECAACGVRIDRDVNAARNIRAEAVRMCEAQLAPGTGESLNGRGVADSNVAGSVVLGDAALDASRPAATGGGSP

SEQ ID NO: 28 - protein, 494 aa, synthetic construct
MSSGTTARRMRAYRFTLDPTRTQLDTLAQHAGAARWAYNHALATKLDALRRRQLQIDELVTLGLTEQQARRDATVTVPSKPQVQKRWNQLKGDTTRGGDGICPWWRAVSTYAFQSAFLDADRAWKNWMDSLTGKRAGRRVGAPRFKKKGRCRDSFRLHHAVNDPTIRLEGYRRLRMPRLGSIRLHDSGKRLARALARGGRVQSVTVSRGGHRWYASVLVDEPDHTPGRETQHRPSRAQHTAGGVGVDVGVHHLAALSTGETLDNPRHLHHAHTRLVKAQRALARTQKGSHRRRRAAERVGRLHHQLAERRASHLHTITKRLATQHALVAVEDLNVQGMTRTARGTLTQPGRNVRAKAGLNRAILDAAPGELRRQLEYKASWYGSTLAVCDRWAPTSKTCSTCGTVKTKLPLSTRVYRCDTCGMVCDRDINAARNILKDADPVAPGRGETLNACGGPVSPSAPHAPTARPSEAGRPGHPARSPRGNDPPSTPKTE

SEQ ID NO: 29 - protein, 606 aa, synthetic construct
MAQAEAPRRLRAYKFALDPTEAQLREFEQHAGSARWAYNHANAILSRYSDTLRNRWNAWIAQHHGLSREQLYALPDRERTAIQAAARAAVKAENAQLAAELRIIDDHRKRVTHKGKPSVEPGEQPAEDAPERAYQLWRERVELARLHAEDPQAYRAERKRILDEIRPLVNATKRKLIEQGAYRPTAMDISTLWREIRDLPPDEGGSPWWPEVSIYAFTSGFAHAETAWKNYLESLAGRRAGRPVGKPRFKKKRRSRRSFTLYGSVKLVTYRRIQVPSIGSVRLHGSAKRLHRALERRGGIIKSITISQGGHRWYASVLVDELDITPGRETQRGPSRRQRDRGAVGVDLGVHHLVALSDPNEKTLDNPRHLRKARKRLLKAQRAMSRRRGPDKRTGQEPSRRWVKARNRVARLHHELAVRRAGHLHEITKRLATSYELVAIEDLNVAGMTRSARGTIDQPGRGVRAKAGLNRSILDTSPAEFRRQLQYKASWYGATVAVIDRWAPTSRTCSSCGAVKAKLSLAERTFFCEHCGMELDRDINAARNILAFAQSAYPGEGKALNACGGSVSPGSQSVVQAGADEAGRPARKPRRSSRGSDPPATPTTRA

SEQ ID NO: 30 - protein, 459 aa, synthetic construct
MSCVTKTQVVRAYRFALDATPSQVEILRRYANASRAAFNFALGMKTASHERWKRGRDPLVAADMDMAEAKKKAPKVRIPRKPQVHRHFIATKGKGPIGPLRQGEERRTPYPWWEGVNANSFQEAFFDADAAWKNWLDSMTGKRAGAPVGYPRFKRKGSRESFRLTNTAVRFAGYRRLWIGGGGGQAAFTVRLHEPARRLVRLLDAGQARILRATIARDGHRWFAAVVVEEIAVLPNRPTRRQANAGRVGVDLGVKSAAAFSDPVVLAHGAPGVLELANPRHVRNTEKKLARAQRVASRRFVKGAQKQSKGYHEAKARVAKLHAQLAARRASTQHLLTRRLVEQYAEVALEKLMVKNMTRSAKGSAENPGKNVRQKAGLNRAILDVGFGEIRRQIEYKAAWYGSSTRYVGTYFPSSKTCSNCHWKNKELTLADRVFKCTQCGMIMDRDANAAQMIKKHAQ

SEQ ID NO: 31 - protein, 517 aa, synthetic construct
MQQEILKAFRFALDPTPSQLEGLAQHAGAARWAFNHALGMKVAAHQQWRSAVQELVDNGMSEAQARKEVRVPVPTKAVVQKHLNQIKGDSRGDALPDGSLGPERPCPWWHEVNTHAFQSAFIDADRAWKNWLDSLKGTRAGRRVGYPRFKKKGRAREAFRLHHNVKQPTVRLESYRRLRLPTIGSVRLHDTAKRMSRSIGRGDAVIQSVTVSRAGQRWYASVLCKVNADLPDQPTRRQWDRGRVGVDLGVKHLAVLSQPLETDAATTAFVSNPRHIRKAEQQLAKAQRALSRTQKGSARRAKARRRVGRVHHEVAVRRSTVLHALTKQLATRFAEVAIEDLHVSGMTRSSSGTPDKPGRHVKQKAGLNRAILDTAPGELRRQLTYKTRWYGSTLAVLDRWFPSSKTCSACGWQNPRLTLADRTFHCTNCSTTIDRDLNAARNIAQHAVLADQLLAPGRGETQNARGAPIRPPGPRAGGQEAMKREDTSPARPVPPQRSDPLTLFTLDDTGHETAKRA

SEQ ID NO: 32 - protein, 469 aa, synthetic construct
MSETVTIVVKEALDPTPAQVVILQRYADASRCSFNYALGLKRGAQQTWSQGRDRLVAQGQTPAEAARNAPKVRIPGQFDIQKIFLAKRDEPLPGPLLPGQEPRLLYPWWKGVNAIVCQQAFRDADAAFANWKSSARRKGGPVGFPRFKRRGRCRDSFRMFSIRLVEEDLRHVRIGGERGGQPAFTVRLHRPARRLARLLAEGGETKSVTVAREGHRWFVAFNVRVPAGPPPRPTRRQRGAGTVGVDLGVKVFAATSDPLLINGTGLQLFENPRLLDNARRQLRKWQRRMARRHVRGLRADEQSSGWKEARDQVARLHALVAARRSSTQHLLTKRIVTQYEHVALEDLRVKNMTASARGTAQSPGRNVKAKAGLNRAILDVGFGEIRRQIEYKALLYGTTVTVVDPAYTSQTCNRCGHVDAKSRRTRDLFTCTRCGHATHADIGAAINIKARAQHSHPAQERPEGTTDVP

SEQ ID NO: 33 - protein, 583 aa, synthetic construct
MFERTTTKAAFLSPLDLRPTQATDLERFAGTTRWAFNWANALLEAHHQAYEGRRQQAARHLFGLGPEQLDELRVLANGTRDENGKKAKGDPVKRREYESIQKATKKAVSEENKALGAEMKLWDEHRSLVVHKGRPLLTPGDEPALDAPPLAHRLYARRVELAGIQKTDPDYYAEQRKKEREAITPNVVAMKRDLMAKGAYFPSEYDLQYIWRTVRDLPKEEGGSPWWPECPTILFYDGINRARTAWKNWMDSASGARKGPPVGMPRFKSKYKAKDTFTITNPNRSVIKFETYRRIAITGIGSMRLHRGAKLLARRIAAGQAEITSATISRSGTAWYVSVLCTVHTTARTAPSKAQRSRGAVGVDWGVRALATTSKPIALTPGKPASRTVPAEKYGAAMSQKIARAQRQLARMPKGSSRRRKAARHVADLQHLVAQRRASSVHQLSKALAQSFEIVAIEGLNVRGMTKSAKGTVENPGKNIRQKAGLNRAILDATPGELKRQLEYKTKKYGSRLVELDTWYPSSKTCSRCGWVHPKLKLSMRTFRCQQCGLVEDRDFNAAVNIERQGITHIVKENEGTDDREEG

SEQ ID NO: 34 - protein, 466 aa, synthetic construct
MDEALSPRQVTRVVRLPLDPTPVEQAILQRYADCSRACYNFAFSLKDAAQRRWAAERDRLIADGMQEKAARKAATARFAVPRQFDLQKIFLAVRDRPFTGPERAGEPFPRYRYRWWAGVNAMVCQQAFRDADRAWSNWLSRSREGHGYPRPKQRGRCKDSFRLPGVSLAAEDLRHIRISGERRPGGQKAFRVRLHRPAYRLARLLQQGGQVKMVTVSRSGPRWFAAFNVRLPAPPAVVATRAQRRRGAVGVDLGVEVIAATSQPVLLQGAVTQLVANPRYLANARRALAKWERRKARRWVKGLPAGQQSRGWHEAKDHVAKLHALIAAHRASTQHHLTKALVTQFAQVVIEDLQVKNMSKSAKGTLEDPGSRVRQKAGLNRALLDVGFGEIRRQLAYKAPWYGSVLSAVNPAYTSQTCHRCGHVDSKSRRTRSVFECTACGTQVHADIGAAHNILARGQQTPAALF

SEQ ID NO: 35 - protein, 463 aa, synthetic construct
MTENTVTVVVREALDPTPEQRLILHRYADASRCSFNFAFGIKHAAQQRWSHGRDLLLAQGLTSAEAAKRAPRVHMPSQPDIQRVFLAVRERPLPGPCRVGEEPHSLYPWWKGVNAIVCQQAFRDADKAFANWKSASRRGAGPVGYPRPKRRGRCRDSFRMFSVRLVSEDLRHVRIGGERDPHGQRSFVVRLHRPARRLARLLARGGVAKSVTVAREGHRWFAAFNVRLPAPPAVRATRRQREAGTVGVDLGVAVFAATSDPLVIGDDKVQLFANPRHLDNARRQLRKWQRRMSRRHVRGVPAHRQSKGWKEARDQVARLQGLVAARRSSTQHLLTKRLVTQYAQVVLEDLRVRNMTSSARGSVEAPGRNVVAKAGLNRAILDVGFGEIRRQIEYKAPWHGTTVSVVNPAYTSQTCNRCGHTDAKSRRTRSLFVCTRCRHTTHADTGAAVNIKRRAQSAAPKPG

SEQ ID NO: 36 - protein, 511 aa, synthetic construct
MGRAEVLRAFRFALDPTDTQLASLNQHAGAARWAYNHAIGVKSGAHARRRAEVEALVAAGMTEKDARKAVNVPIPMKPAIQTSLNAIKGDPRVQEVLPGAMGPHRPCPWWRDVATHAFQSAFRDADTAFKNWMDSLRGQRAGRPVGYPRFKRKGRARDSFRLHHDVKAPTIRLDGYRRLLLPRIGSVRLHESGKRLARLVGRGEAVVQSVTVARGGSRWYASVLCKVWQELPEQPTHAQRARGTIGVDLGVKVLAAVSKPVSMTRGGPQLDLVPNARHGKAARRRLTRAQQTYARTAKGSKRRAKAARRIGRIQHLTAERRATSLHTLTKRLVTAFATVAVEDLNVAGMTASARGTVDNPGRKVRQKAGLNRSVLDASFGELRRQLTYKAHWYGAAIAVCGRWVPSSQTCSVCGWQNPRRLTLADREFECTPCGLTMDRDLNAARNIERLAQHVASGREETENARGGGVSPPVRLGGRQSPVKREDPAHRAGPPRRSDPPATLTARRKRAA

SEQ ID NO: 37 - protein, 519 aa, synthetic construct
MAETAVLRAFRFALDATAAQEEGFLRHAGASRWAFNHALGMKVAAHRQWQREVKALVEGGMLEAQARKTVKVPVPTRPTIQKHLNRIKGDSRSPDHPEGAQGPQRPCPWFHEVSTYAFQCAFEDADRAWDNWQASLSGRRAGRKVGYPRFKKKGRTKDSFRICHDAKKPTIRPDGYRRLRIPVLGSVRLHDTAKPLARLVDRGASVKSVTVSRSGARWYASVLVSVLQDLPERPTRRQRQAGTVGVDFGVKTLAALSAPVTLPNLGTLTMVPNPRHLASDTRRLTKAQQTLSRTTKGSARRRKAAQRVGIVHHRIASRRATYLHTLTKQLATGYAVVAVEHLNVAGMTSSARGTVEEPGSKVRQKSGLNRSILDASPAEMRRQLDYKTRWNGSQLAVCDRWFPSSRTCSACGWQKPRLTLAERVFNCGQCGLVIDRDLNAARNIAAHAVLVPHGTAAPGSGEASNARGAATRPATPRGGRQAALKREDTGPPRPVPPQRSDPLTLFTLDVPDQQTAKRP

SEQ ID NO: 38 - protein, 515 aa, synthetic construct
MEQEVLKAFRFALDPRPAQVEVLLRHAGAARWAFNLALGMKVAAHKEWRSQVQALVDQGVPEAEARRRVKVPVPSKLQIQKHLNLIKGDSREGGLPEGVLGPERPCPWWHEVSTYAFQSAFIDADRAWQNWLASLAGKRAGRAVGYPRFKKKGRCRDAFRLHHDVKRPGIRPVGYRRLRLPTVGEVRLHGSAKRLVRLLGRGCAQVQSVTVSRGGHRWYASVLCKVVVELPGKPTKAQARRGTIGVDLGVKYLAALSQPLDVKVPESRFVDNPRHLVRAEKQLAKAQRALSRTQKGSARRHKARCRVGRLHHEVAVRRATVLHAMTKQLATRFSTVAVEDLYVAGMTRSARGTVEAPGKRVRQKAGLNRAILDAAPGEVRRQLAYKTRWYGSKLAVLDRWFPSSKTCFACGWQNPRLTLADRTFHCGGCGLSTDRDENAARNIAHHAVVADDSPVAPGKEETRNARGAPNLAGLKARRQGASKREGTGPPGTVPPQRSNPLTLPDPHGQQPAKHP

SEQ ID NO: 39 - protein, 518 aa, synthetic construct
MEQQVLKAFKFALDPTSSQVEELTRHAGASRWAFNHALGMKIAAHRDWRTQVQELIDAGVQEKAARQQVRVPAPTKPTIQKHLNSIKGDSRSDDLPPGAMGPQRPCPWWHEVNTHAFQSAFIDADTAWKNWLDSLRGTRAGRKVGYPRFKKKGRSRDSFRLHHDVNKPGIRLATYRRLRLPKIGEVRLHDSGKRLARLIGRGDAVIQSVTVSRAGHRWYASVLAKVTVTLPTRPTARQVSAGKVGVDLGVKSLAVLSRPLVPGDDTTAFVPNPRHLRHAETRLTKAQRALSRTTKGSARREKARRRVARLHHEVSVRRAGQLHALTKLLTTTFSEVAVEDLNVAGMTRSARGTTERPGRRVRQKAGLNRAILDTSPGELRRQLTYKASWYGSKLLVLDRWYPSSKTCSACGWQNPRLTLADRTFHCGNCHLVIDRDLNAARNIAQQTHGAPHHPVAPGKGETQNARRATGRPPSPRAGRQEAQKREDTGPPRSVPPQRSDPLTSPPPGSPGQESAKSL

SEQ ID NO: 40 - protein, 532 aa, synthetic construct
MGQQVLKAFKFALDPTPGQTEELTRHVGASRWAYNHALGMKIAAHREWRTQVQSLVEEGLPEKDARQRVRVPVPTKPTIQKHLNSIKGDSRADDLPPRALGPHRPCPWWHEVNTYAFQSAFIDADTAWKNWLDSLRGARAGRKVGYPRFKKKGRSRDSFRLHHDVNKPGIRLATHRRLRLPKIGEVRLHDSGKRLARLIGRGDAVVQSVTVSRAGHRWYASVLAKVTVTLPERPTARQTSAGKVGVDLGVKNLAVLSRPLLPGDDTTAFVPNPRHLRHAEARLTKAQRALSRTTKGSARREKARRRVARLHHEVSVRRDGQLHALTKLLTTSFSEVAVEDLNVAGMTRSARGTIERPGRRVRQKAGLNRAILDASPGELRRQLTYKASWYGSKLLVLDRWYPSSKTCSACGWQNPRLTLANRTFHCANCHLAIDRDLNAARNIAQQTHGAPHHPVPPGRGDAKRPPSHRKTAQPTGWTAGGAEAGRHRPTQVGATSAERSADIPTTRATWSRKGKAGLTSQARKCPARTCRG

SEQ ID NO: 41 - protein, 513 aa, synthetic construct
MSSERAPKLRNVVTQQAYKYALEPTPRQQCAFSSHAGAARFAYNWGIARVADSLDAYAEQKAAGIDEPDVKFPGHFDLCKMWTAWKNTAEWTDRHTGQTTTGVPWVASNFVGTYQAALRDAAGAWQRFFRARKTGARAGRPRFKKRGRARDSFQLHGDGLRIVDAKHVNLPKIGTVKTFEATRKLARRLAKGSVPCPTCRATGKITDSASGKVKKCSDCKAAGSRPAARIVRGTVARDSAGRWYLALTVELVREVRTAPTPRQLAGGPVGVDFGVRQVATLSTGQLVDNPRHLESHLRRVKTAQQALSRCPPGSRRRAKAQQRLGRLHARVRHLRENSLQQATSALIHQHSVIAVEGWDVQQTAQHASPKNLPKQIRRNRNRALLDTGIGAARWQLQSKGAWYGTTVVVTDRHAPTGRQCSACGTVKATPIPPTQDEYRCPACGTSLDRRTNTARVLAAVAAQHHDAPSGGESKNARGENTRPTAPRRNGQFSAKREPRSRPPGRGQTGTPGT

SEQ ID NO: 42 - protein, 522 aa, synthetic construct
MSEGVSGMAEVLRAFKFTLDPTRAQVGALQQHAGAARWAFNWALGEKVAAHREWRRQVGALLAEGVAEEQARKQVRVPVPTKPTIQKRLNSFKGDSRVQDLPDGVLGPRRPCPWWWEVKTYCFQAAMADADTAWKNWLSSLTGARAGQRVGYPRFKKKGRARDSFRLHHDVKKPGIRLAGYRRLRLPTIGEVRLHDFGKRLARLIDRGRAVVQSVTVARCGHRWYASVLCKVDQSVPQRSTRAQRRRGRVGVDLGVKHLAALSQPLHPYDRASLYVENPRHLRRAAQRLAKAQRALARTQKGSKRRAKAVRRVGRLHHEVAVRRESTLHQLTKRLATGFAEVAVEDLHVAGMTRSAKGTIDAPSRNVRAKAGLNRSILDTAPGELRRQLTYKTCWYGSRLAVLDRWWPSSKTCSACGRQNPRLTLADRTFHCTGCGLRIDRDLNASRNIATHAALADTAPPVAPDRGETQNARRAGTRPTGPRAGRHPATKREDTAPAVPPQRSNPLALPPPPTGYEQVTLF

SEQ ID NO: 43 - protein, 519 aa, synthetic construct
MAETEVLRAFRFALDATAAQEEGFLRHAGASRWAFNHALGMKVAAHRQWQREVKALVEGGMPEAQARKTVKVPVPTRPTIRKHLNRIKGDSRSPDLPEGAQGPQRPCPWFHEVSTYAFQSAFEDADRAWGNWQASLSGRRAGRKVGYPRFKKKGRTKDSFRICHDAKKPTIRPDGYRRLRIPALGSVRLHDTAKPLARLMDRGAIVKSVMVSRSGARWYASVLVSVLQDIPERPTRRQRQAGTVGVDFGVKTLAALSAPVTLPNLGTLTMVPNPRHLASDTRRLTKAQRALSRTTKGSARRRKAARRVGVVHHRIAERRATYLHTLTSQLATGYAVVAVEHLNVAGMTSSARGTVEEPGSKVRQKSGLNRSILDASPAEMRRQLDYKTRWNGSQLAVCERWFPSSRTCSACGWQKPRLTLAERVFACGQCGLVIDRDLNAARNIAAHAVLVPHGTAAPGSGEASNARGAATRPATPRGGRQAALKREDTGPPRPVPPQRSDPLTLFTLDVPDQQTAKRP

SEQ ID NO: 44 - protein, 518 aa, synthetic construct
MQTEVLRAFRFTLDPTPAQQEDLLRHAGAARWAFNHALGVKIAAHQQWRTKVQALVDSGVAESIARKQVRVPVPMKPEIQKHLNRIKGDSQKQPWPAGSIGPARPCPWWREVSTYAFQSAFIDADQAWKNWLDSLAGRRAGRKVGYPRFKKKARSKDSFRLHHTVTQPTIRLDGYRRLTLPRLGTIRVHDSGKRLARLITRGHAVVQSVTVSRSANRWYAAVLVKVRQNLPDRPTRRQQSNGTVGVDLGVKTLAALTQPVTLPGATDTLLVPNPRHLAADTRRLTRAQRALSRTTKGSTRRRKVARRVAQLHHRIAERRATYLHTLTKQLTTRYAAVAVEDLNVSGMSASARGTVEEPGRKVRQKAGLNRAILDMAPAEIRRQLGYKTRWNGSRLAVCDRYYPSSKTCSACGWQNPRLTLADRTFICGQCGLTIDRDLNAARNIAAHAVPTPLHSTVAPGTEETQNARRAATRPTTPRGGRQTAKKREDTGRQPPVPPQRSDPLTLQPPQHQEVAKGP

SEQ ID NO: 45 - protein, 506 aa, synthetic construct
MASTKTVVLRAFKFTLAPTATQDQQLLRWCGNARLAFNYALASKRAAHTEWRAQVDALVTSGVKEPVARKRVTGPKTPTKPAVYKAFIAERGDTREGLDGVCPWAHEINTHVFQSAFIDADRAWKNWLDSFKGTRKGRRVGYPRFKKRGRARDAFRLHHTVTKPTIRFSTHRRLRLPTFGEVRLHDSARTLVRQIDRGTAVVQSVTVSRAGHRWYASVLCKVEMDLPSGPTRSQQAAGTVGIDFGVKALAALSKPLVPDRPESTLLPNPRHLAKAAHRLKRAQQTLSRRQKGSARREKARRRVARLHHEVAVRRQSALHQITKRLTTRFATIAVEDLHVSGMTRSARGTMDKPGRKVRQKAGLNRAILDASMAEARRQITYKTSWYGSRLAVLDRWWPSSKTCSACGWQNPSLTLADRVFECAQCGLTLDRDLNAARNIEQHAVQVASGTGETQNARGEPVRLPRPRAEKQGSTKREDTGPPGPVPPRRSDPPTPPNPRQGQAKLF

SEQ ID NO: 46 - protein, 477 aa, synthetic construct
MSVAHVSLLNMTTTENTTTIVVREPLDPTPEQVLVLKRYANASRASFNFAYGLKHEAQQRWVRGRDRLLSKGLGREEANRRAPKVLVPRGSDVQRIFLAVREQPLAGPLREGESEHRRMFRWWAGVNAIVCQQAFRDADTAFANWRSSGRRAGEGVGYPRPKRVGRCRDSFRMTSVRLVGTDLRHVRIGGEKDPAGQRALIVRLHRPGRRLARAMARGGVVKMVTVAREGSQWWASFNVRIVLPPPAQPSRRQREAGTVGVDLGVAVFAATSEPVLTAAGKEQLFDNPRHLDNARRQLHKWQRRMARRHVKGLPVHRQSAGWREARDQVAHLMGLVAQRRASTQHLLTKQLVTQFEHVALEDLRVKNMTRTARGTVEAPGRNVAAKAGLNRAILDVGFGEIRRQIEYKAKWHGVTVTAVNPAYTSQTCHRCGHVDRKSRRTRSVFECTRCGHVTHADIGAAHNIKHRALAPDANDAR

SEQ ID NO: 47 - protein, 509 aa, synthetic construct
MHTEVLRAYRFALDPTRGQLEDLARHAGAARWAFNHALAAKVAAHKEWRAKVAALVEAGTAEAEARKQVRVPIPTKPGIQKALNAAKGDSRTGTDGLCPWWHEVNTYCFQSAFADADRAWKNWLDSLKGVRAGRKVGYPRFKEKGRARDSFRLHHDVKKPGIRMVGYRRLRLPKVGEVRLHGSGRELARAVDRGRAVVQSVTVARDGHRWYASVLCAVAMDVREKPTQRQTMRGTVGVDLGVKYLAALSQPLTEGDEASKFVANPRHLKAAEKRLVKAQRAFSRTQKGSGRRDKARRRVARLHHQVARQRAGAMHQFTKRLATGFAVVAVEDLNVAGMTRSSRGTVEAPGRRVRQKAGLNRAILDVAPGELRRQLAYKTSWYGSKLAVVDRWFPSSKTCSNCGWQNPSLTLSDRTFHCSNCESAMDRDWNAARNIARHAVLGDSQVACDRRETENARGALVSPGASRGGRRRAVKREDTGPPPVPPQRSDPLALPTPTRKVTGIQASLF

SEQ ID NO: 48 - protein, 468 aa, synthetic construct
MTTTSTTETLRAYRYALDPTPAQIEILQRYATAARCGYNFALGYMVAVHQKWARGRDALIAAGMDKAVANKAAPKVKVPNAFRAQAFFRETKGHPFTGPLPEGAERTTPYPWWEGVSNRAYYTAMEDAATAWKNWMDSASGRRAGGPVGYPRFKRRGRARERFRLVHNVKKPEIRFETSRRLRIPGGGGQSAFTVRLHQDARDLLRLIADGRAVVNSLTVSRDGHRWHASVLCRVEQHIPSGPSHRQAAAGRIGADLGVKALAALSDPLTLTPAAGPTVLIPNPRHLAATERKLARAQRVMSRRFVRGAAQQSKGYSEARARVAKLHAQLAARRTSALHLISKRLVQQYAEIALESLNTKGMTSSAKGTLQSPGRNVRQKAGLNRAILDASFGELNRQIAYKAAWHGATLARVPTFFPSSKTCSACGWINTELTLADREFACRSCGIVLDRDANAARNIKNHAIPVQP

SEQ ID NO: 49 - protein, 462 aa, synthetic construct
MTDTIIKAFRYALDPTEAQIEILHRYATASRCGFNFALGMKTTVYDRWRRGRDALVAAGMDKAEANKKAPKVRVPNRNRTQAYWRETRGQGFIGPLREGQEPRAPFAWWEGVNNRAYYTAFEDADTAWKNWLDSLAGRRPAMGFPKFKRRGASRESFRIVHSLKNPDIRFDGPRRLRIPGGGGQPAFTVRLLQSPRALTSLIASGQAVITSVTVSREGHRWHASVLARIEQDLPTRPTRRQQAAGRIGIDLGVKTALTLSDPLTLHRGQAPVLAIDNPRLLENTARKLARAQRVMARRHVKGAAQQSQGYLEAKARVAKLHALLAARRSTAQHLVTKRLVEQYAEIALETLNTKGMTRSAKGTVDKPGRNVRQKSGLNRALLDVGFAEINRQIEYKAGWRAVTIARVPGLFPSSKSCHRCGWIHTNLTLADREFRCDACGMIIDRDVNAAQNIKNHATPDRP

SEQ ID NO: 50 - protein, 530 aa, synthetic construct
MALQRIQQAFKYALDPTPAQARMLTSHAGAARYAFNWGLATFATALDAYSAEKTAGVKKPVTKLPGHFDLCKLWTAHKDNPTSDLGWVGQNFSGTYQAALRDAHAAWKAFLDSKNGRRRGRQVGRPRFKSRHRTTAAFQTHGTGLRVADHRHINLPKIGPVRSYEKTKKLRRLLTRPDVTCTTCDGTKEAPAPAPATKSCGDCKGTGHAPHTRIVRGNITRTPSGRWHISLTVETHRDIRTRPSQRQREGGIVGVDWGVRDLATLSTGEVIGNPRHLERNLARLRRAQQDLARKADGSAGREAARLRVARLHGRVANLRRDHLEKVTSRLVHSHTRIVVEGWDVQHAMQHSGDGAPKWVRRDRNRALSDTGIGAARWMLGRKAAWYGSAIVETGPHEPTGRTCSACATARTKPVAPADERFTCPSCGYSGDRRVNTARVLVRLAHTSDAPSSGESLNARGGDVRPAAPSTRPGGQTPTRPSGHIAVHALGKDEEGRDKGKDKEFRGRRSPMKREARSRPPGRGKAGTPDP

SEQ ID NO: 51 - protein, 512 aa, synthetic construct
GTDRYGKPQKPDWEAARQVFIDGGIEDEVADTILSEWQQRYRREPSDTKPGNDPLVDGIAPWLAEVPNALVQRAESDCEEAWKRFYKMLREGTATPSKRSRPRKTARPDGSFDYDPPGLPRYKRRSPGRGSFYLTNTEVRLVPNASRRIRLGGKIGDVRTLEGRTMRRIRRSIAKRDGVIQSVTVSRGASRWYASVLVKETFTPPKPTRRQLEAGRVGVDVGVKHAFVVAGPSTTAGGLIVDRPARCGSEKALNDARKTLRETAPRSKARMKARITVSRLEDREQWAIEQAGRAVSRKKLRSKNWYKAVARLAELKHRQAVRRKTFIHEATKRLATGYAEIVIEDLQVKGMSASAKGSAEAPGRRVRQKAGLNRRILASSFGEFRRQLEYKQQWYGSHVLTADRWYASSKICAHCGATKAKLPLSARQYVCDSCGYTADRDVNAARNLARCAKVASTRKGVASEVGETVNDRRGRYGRRRSTVSADAAAVPAGRPAIDAGHRGGSDSATYPL

SEQ ID NO: 52 - protein, 758 aa, synthetic construct
MAAMETQMIQQAYLFALDPTQAQAATLASHAGARRYAFNWAHAMIAAAADARQAQKDAGLEPDIAIPGQFEVGPAWTRWRDAAVGCKTCRRLLARDPAVPASLWADSRTGEITCDPGALQRLGLDYGAPPLHDPADVGCRRCWKVLRETPAGEWADSSGSAACPEARRPGPPHEPSGTCQDGCDGAARACGGPHEPSSDFLAWTGDVFSGTIQAAQRDADVAWKKFLSGKARRPRFKKRGKSAESFQVHGDGLKMDGPTRIVMPKIGAVTVMSDDSMHPAMRRSRSRAGAGRRHMGNRRRSRSLRKHLARSGPKAAALAPLLRRAREDAGLTPAAALAALNFEAGIYAAEAKAVRAVRAAKQEQQLLGMLDAEERTLPVPVPGAPQAEFAAIEGIAARRKKTQARLRSAQKRAGESPDAEALRTAAWTAPKLAALEKTGDTAGLAQLEVAAIFCAAYLVTGPLRDRVTGLFAQARITRATVTLGADGLWWCSAGAEIPMEIRTRPSRRQREGGVIGLDFGVREIATASNGVRIPNPRHYETALAELRAAQKQLSRSAPGSKRREKDKRAAGLIHADVARLRADAIHRATTVLVRQHDVIAIEGWNVQQVMRDGSRNLPRQVRRRRNRALADTGIGIGRQQLTYKGPRNGAVIMITSPDARTGTTCSVDGKARTTPLPPDQEMFTSDRCGHTLDRRLNTALAVQAWAVQELKRGPSPGGPAKPRGGDVRPGTSRARQSPGKRAATSSRPRRGETGTPGG

SEQ ID NO: 53 - protein, 669 aa, synthetic construct
MAAVGRPRHHHLHRRARSPSRWHRGARLRLLHLPLGTRDRRRTPLHARYGPGHRALRRQRGHDPRRHARHLPGPVPPQPHRQGPHLLPRPRPARVHRAPHGRLHRQAPRRRLTTACQRPPLPCVDMGTEGALTHRVVRVCLDDAALTPDQRTLLDRHAGTARAVWNWGLAARNAQQDALMAHVRAVALEQAASDETAAAELLDDRDWRTATIKAAPDELRRPLRAATLGRAFTAETRDPDSRFAWWAVERHGVNRFAVSSSLQALDAAFDRYYRDTGGHRSARRARPRKDGRPAAWPRFKKRGRATDAFALFNLVVAGQDPWRVIEGAHRIKVPSLGSLRVHENTKRLRRLIARGGRPTSARFTRTGGRWYMSVVVALPATAASTVLSPAGAPRAAAPTRAQTRAGLVGVDLGIKTLATMSDGTLVANARHGRAAARRLARLQRRAARQQGPRKGAAPSKGWVATQRTITRLQHDTAARRRGLVYELTKTLAAGYAAVAIEDLNVAGMTATPAARPDPDRPGVYLANGRAAKSGLNRAILDVGFGEFRRQLTYKTPMYGAQLLEIARFAPTSKTCSTCGAVRAKLRLDERTYRCEHCGLVIDRDLNAARNIAALGHQALGTSPADAGDAKRRDHKEGDRERSVILVSQDLGPPRSAERVTDSSPPTRAA

SEQ ID NO: 54 - protein, 531 aa, synthetic construct
MADMTCSRAVLLHLDAAALTDRQQLLLERSAGTSRAVYNWGLAAINEWETRQYAWLRERAHAVTSAEDQAQTLLGDVDWRRGALLQTPGDVRRRPNTASLDRRFTELTRDPNSRFHWWHVENHGVPRHAMSTALGNLDTAIDRYRNHVGPSSRPPRKPRKDGRPAGWPRFKKKGRSKDSFAIFNLSVTGRRTDPWKVIDKGHRIRVPNLGSLRVHENTRRLRRWIQRGAIPKSARFVRRGTGWTVSITLDVPAEVISAPATTRRQRAAGAVGVDVGVHSLVALSTDELIAGCPSADFWRRLRRLQRRAARQRGPTHEQGPSAGWVETTRRIARLQRVDAVRRRGRLHEVTKRIATRFETVGIEDLAVAGMTAAPHPKPDPDHPGSFLPNGRRSKAGLNRSIRRAAFGEIRRQLLYKTSWYGARLVIVDRFAPTSKTCSGCSAVNATLRLSERVYHCEQCGLVLDRDLNAARNIRSLALTPSPVDTADVKRCDTPTPSRSRPARCWGPADLPKGRPQRPAMDLPSPLRDSGN

SEQ ID NO: 55 - protein, 527 aa, synthetic construct
MADMTCSRAVLLHLDAAALTDRQQLLLERSAGTSRAVYNWGLATINEWEARQYAWLRERARAVTRTEGEAQTLLGDVDWRRGSLLQAPQDLRRRPNRTSLGRRFTELTRDPNSRFHWWHAENHGVPRHAMSTALGNLDTAIVRYWDRARSPDRPPRKPRKDGRPAGWPRFKKKGRSKDSFAIFNLSVTGRRTDPWKVIEQGHRIRVPNLGSLRVHENTRRLRRWIQRGAIPKSVRFVRRGTGWTVSIVLDVPAEVISAPVTTRRQRTAGAVGVDVGVHSLVALSTDELTAGYPSAAFWQRLRRLQRRAARQRGPTHEQGPSAGWVETTRRIARLQRVDAVRRRGRLHEVTKRIAIGFETVGIEDLAVAGMTAAPHPKPDPDHPGSFLPNSRRSKAGLNRSIRRAGFRELRRQLHYKTSWYGACLVIVDRFVPTSKTCSGCGAVKATLRLSERVYHCEQCGLVLDRDLNAARNIRSLALTPSPVDTADVKRCDTPTPSRSRPARCWGPADLPKGRPTEASNGPPAPTP

SEQ ID NO: 56 - protein, 560 aa, synthetic construct
MAKKTSTDADTMNRAYKFRLDPDQAQKAELMRCVGAARYTYNLLTTHNLEVSRARDDYWHARIEAGVDEATVKAELKKLEKKDPTYKILYKSGYRPLYLTPEVKRHRAAGEAIVAGADPAVVWPETERFSEPWLHTIKCRVLDSGLMNAEKAWKNFFESRAGARAGAQMGLPRRKRKSSGRDSFTIHAPEVIGAYGTPYKKSEPEYVRRKKQLKCRGISADPTIEDYRHVRLSHLGVIRTHNTTKPLVKAMRAGAQIRSYTVSRAADRWYVSILVELTRPSTNPTRAQRSAGAVGVDLGVRYLAALSDEQAPQRFAQYPSLEFTGDGAPTLANPRWARTAEKRLVRLQRALARAQKGSNRRTRIVQQIARHHHLVALRRESGLHQVSKRLSTGYTLIGLEDLAVAGMTASAAGTIEAPGKNVRQKAGLNRSILDAAFSTLRRQLEYKASWYGSQVRIIDRFFASSQTCSACGARAKTKLGLHVRVFECAACGVRIDRDVNAARNIRAEAVRMHEAQQLAPGTGESLNGRGVADSDAAVSVVLGDVALDVSRPAATGGGSP

SEQ ID NO: 57 - protein, 496 aa, synthetic construct
MAQVLKAFRYALDPTSAQVELLRRWAGNSRLAFNFALAMKQDAHQRWRDELDTLLAQGLEAKEARARLKGTHKIPTKPAVYKAFQHVRGDEAKGIDGIAPWHAEVSTYVFQSAFDDADRAWKNWLDSYTGKRAGRRVGYPRFKKKFRSRDSFRLHHDAKKPKPALRLEGYRRLRLGGALQTVRLHGSAKTLHRLVSSGRAVVQSVTVSRGGSRWYASVLCKVEVDPSTPTRRQKANGRVGLDWGLGHLAALSKPLDGSRLVDNPRHLRKASERLLKAQRALSRTQKGSARRRKAAVRVGRLHHRVAEQRATFLHTLSKRLTTTFACVAIEDLNVSGMTRSARGTVRKPGRNVRSKAGLNRSILDAAPAELRRQLEYKASWYGSEVAILDRWFPSSKTCSGCGWRNPSLALSEREFVCAECGLRMDRDLNAADNIAAHAVAPDSGAGAPGRGESVNARGGGVTPGLLREPGPLPLKREGAVSSGTAPPRRGDPPTFP

SEQ ID NO: 58 - protein, 500 aa, synthetic construct
MARQEVLRAFRFALDPTPAQEETLRRYAGAARWAFNHALAAKVAAHEEWRNQIAAIVETGVPEDVARKQVKVPIPTKPAIQKAWNQVKGDSRTGEDGCCPWWHEVNTYCFQSAFVDADAAWKNWLDSLTGRRAGRRVGYPRFKKKGRSRDSFRIHHDVKKPGIRLVTYRRLRIPKLGEVRLHDSAKRLARLIDRSEAIVQSVTVSRGGHRWYASVLCKVTVELPDRPTRRQAAAGTIGVDLGVTHLMALSQEVDLGQGPTQLVDNPRYLKATLRRLRRAQQALSRTEKGSARREKAKRRVARLHGQVAERRATFLHGITKRLATGFHTVAIEDLNVTGMTRSAKGTIEAPGKNVRAKAGLNRAILDASPGEIRRQLTYKTSWYGSALAICDRWFPSSRTCSACGEQNPRLTLADRVFVCPSCGLAMNRDINAARNIAVHAVIAPTSGAVASGKGETLNARGASVSPSIPQGRGREAVKREDAGSSGSAPPRRSNPPALPP

SEQ ID NO: 59 - protein, 539 aa, synthetic construct
MARREVLKAFRFTLDPTRAQETELRRYAGAARWAFNHALAAKVAAHQERKQRIAALIGGGLAEEAARKQIKVSVLGKGVIQKAWVRARGSSRNGAEGICPWSHEVNNYCFQSAFDDADAAWKNWLDSITGKRVGRWVGYPRFKKKGRTRDSFRIPHNVNKPGIRLVTHRRLRIPKLGEVRLHDSARRLVRLIKCGQAVVRSVTVSRGGHRWYASVLCKVTVELPDKPTRRQAAAGTIGLDLGVTHLIALSQPADLGKGPTQLLDNPRYLRATTKRLRRAQQALSRTQKGSTRREKAKRRVARLHNQVAARRATFLHGVTKRLATGFHIVAVEDLNVAGMTRSARGTVQNPGRKVRQKAGLNRPILDASPAEIRRQLQHKTSWYSSTIAVADRWFPSSKTCSACGRQNPRLTLADRVSTCSSCGLTMNRDINAARNIAVCAVARPGVQPTGAGSDPRNVNVKAPATGAFTTMAIFQSLSAHGLSTDRANASIMSIPGVMPRARSSIPAPACAIPARSATCGLRPRACRSSCTSLTSRAAS

SEQ ID NO: 60 - protein, 595 aa, synthetic construct
MATAETEAPAPVLRAYRFALDPTQAQLADFARHAGATRWATNRGIAWMSQAQLAWEARRDEVITRIAGPMPQPPDGLDEKSTAAWTAQVRGERIKQWDKQARPILKAEAAELAADTKRLDDERKALMAAVKDKTRPDLLEIKERLAAVRREVLQFKKARFERGDAIPSAMDCTTMWREIRDQDAADGGSPWHPEVSVYCFTNGFDRAQAAMQNWMASRTGARVGRAMGRPRFKKKGRSTDSFTLFHDVHNPSIRPDGHRRLNVPRIGSVRLFESCKPLARLIDRGHAVVKSVTISRGGSRWYASVLCELSPEAMRHREEVSRARQKVSKERQRMRPAVGVEWGVRTLVALSDETAYENPRYGKRHKRALVKASQAVARKPFVRGQAQSANRAKAVRRLGRVHHRTAEARRGTLNQISASIAINYPEIAVRDLNVRQMTGSAKGTVEAPGSDVKVKAGFNRAILDTAPAELRRQLEYKAAQWGTRFRAAAGDLPSSQTCCKCGWRDPSIPLTQVVFRCGNIKCGMKLDREVNAARNILHHAVPLASDIGESLNACGGGQSPSGDRRLSTPLSKQEGQSRRRGGSSRGSDPPASLDS

SEQ ID NO: 61 - protein, 631 aa, synthetic construct
MATCGPAQRLGTGGTPRVAAKSNPAGPGPGPGPAAVTMPGTEVLRAYRFTLDPSDAERAALSRYAGACRWAYNYAVAKKTQAHQAWADRRAAYLEAGLSEAEAKERIKADGAELTDRIKVWDHHRKSLTLILAGKPPLPAMQPPAGQEALVRQLAAARADAAGTSRERELLTEGRATVNALKAKAFSAGFRTPNATDTSALWRMERDLPKEEGGSPWWREVNVYCFTSGFDRAQVAWKYWQDSLAGRRAGQRHGYPRFKKKGHAESFALFHDVKRPIIRLEGYRRLVMPGLGSIRIHDSGKRLARLVERGQAVIQSVTVTRGGHRWYASVLAKVQQDAPVLWEHVHDDGIRTPYLSRAQAEKAAENGGRVEQIGRPTARQRAGGLVGVDLGSRNLAALSSPLDPADPADPALVQYPRLLADSLAKLSKAQRAMSRCQQGSGRWRKATARVSRVHQQITVRRASFLHGLSKKLATGFTHVAIEDLDLTALTTSAKGTRDKPGKNVKAKARLNRHLLDAGLGSLRKKLAYKTAWYGSQLVVLDQGEPVIATCAKCKERNPSSDPSCSQFHCPSCGAAVHRHENSAANIVDAARRQLKTVASDRGETQNARRAPASPRVRKAPGQGALKREDTG

SEQ ID NO: 62 - protein, 505 aa, synthetic construct
MATVLRAFKFALDPTADQRTKLKRYAGAARRGYNFALGMKIQAHQQWRERVDALVAERMEESEARRHCGIAIPRKPAVYKEFIATRGDDRTGEDGIAPWHHQIPSYCFQSAFNDADQAWKNWLDSLTGKRAGRRVGYPRFKSKHRSRDSFRLHNKKGATPMLRLEGYRRLNLHTKLGSVRLHDSGKRMHRLVASGAAVVKSVTVSRGGSRWYASVLCEVETDLPAPTRRQRRNGRVGVDLGTHHLAALSKPVEGAVLIDNPRHVRAAAKRLAKAQRALARTEKGSARRKKAAVRVGRLYHAVALKRATTLHALSKRLVTTFACVAVEDLNVGGMTRSARGTVEAPGSNVAAKAGLNRSLLDAALAELRRQLDYKTSWYGSRLAVVDRWFPSSKTCSACGWRHPSQTLADRVFVCAECGMRVDRDLNAARNIAAHAEPVPGPGTVAPGRGETINARGGRGSPAALRGSRRRPVNREDAGLIGPAPPRRSNPPTSSARRPQDDNGSE

SEQ ID NO: 63 - protein, 566 aa, synthetic construct
MATWQPGRPLPVLVRPGHTLSSAFDFAGVTFMPALEVTRSFRFALDPTEAQRESFLKSAGACRWAYNYALEKKTRSHQAWVSRRDSLIAKGMSRPQWKAQLRRETADLKASCAAWDHHRRALIRMARSAEPEVAVAPQEPADLVARLAREREEARPGGSGEEYARALARARRMVARHKEELFARGDQIPNQHDMAAMWRTERDLPKEQGGTPWWNEVNVYCFTSGFDRAQAAWNNWMTSASGERGGRRVGYPRFKKKGGCLDSFTLYHDVQKPRIRLDGYRHLIIPTTGRIRIHGSAKRLARLVALGEARVQSVTVTRRAHRWYASVSCKITQRFPAEPTLRQRAGGTVGVDLGSRYLAVLSNGPGTAGGRESVIPHPQFLLRDLPRINCINRRMRRMQPGSREYRRLSARAARRHHLVALRRAGTLHDITKRLSRGYACIAVEDFDLVSLVTSAKGSRSRPGTKVKVKSLFNRRLLDASIGEFRRQLAYKCPQYGSRLIKIDRGEPVATTCSRCGDRNPNAKPSQEKFTCPSCRYTADRHANAAACIYMAALRKMSAVASGSGET

SEQ ID NO: 64 - protein, 715 aa, synthetic construct
MEQASLIMCHAVGFRWAAEADCVFVICLTTGTTRRSTRCDRTQARVFASHVSKGSCLARAEAIASVRVFFDCPTNTTVWRVTGSLYPMATCGPAQRLGTGGTPRVAARSNPAGPGHGPAAVTMPVTEVLRAYRFTLDPSDRERAALSRYSGACRWAYNYAVAKKTQAHRAWADRRTAYVEAGLTEAEAKERIKADGAELTDRIKVWDHHRKSLTLTVVGKPPPAAMRSPAGQEALVRRLATARADAAGTSRERALLAEGRAMVNALKAQAFRAGFRTPTATDTSNLWRMERDLPKEEGGSPWWSEVNVYCFTSGFDRAQVAWKYWQDSLSGRHAGQRHGYPRFKKKGHAESFSLFHDVMRPIIRLEGYRRLVMPGLGSIRIHDSGKRLARLVDRGQAVIQSVTVSRGGHRWYASVLAKVQQDVPVLWEHVHDDGTRTPYLSRIQAEKASENGGRVEQIGRPTARQRAGGLVGVDLGSHHLATLSSPLDPADPATAVVHLPRLLADSLARLSKAQRAMSRCQQGSGRWRKATARVSRAHQQVRVRRASFLHGLSKKLATGFTHVAIEDPDITALTTSTEGTRDKPRKNATAKARLNQHLLDAGLGSLRKKLAYKTAWYGSQLVVLDHGEPVTASCATCKERNPSSDPSCSKVHCPSCGAVVHRHVNSTASIVDAAHRKLKTVASDRGETQNARRAPGSPGARKAPGQGASKREDTG

SEQ ID NO: 65 - protein, 529 aa, synthetic construct
MGEQTTTRVVRLCLDTRALSEEQAVLLARHAGTARAVWNWALAAVNAHEDAVRAHVQNQAAGAAASSTALMDDSAWRRRAYAAARAELGRTPRAIALGRAFTAETRDPESRFAWWQTERHGVNRFAVSSALRALDASVDRYHQRLTAPARRTRRDGRPAGWPRFKRKGRDRDAFSLYNLVIADQDPWRVIDGAHRIKVPSLGSLRVHENTRQLRRLIHRGGRPTAAHFSRHGDRWYVSINVAIATTSLPAPVTTRAQRTAGVVGVDLGVKHLAVLSDGTVHDNPRAAAAAERRLTRAQRAAARRAGPRRGVGPSEGWKEAQRAVARLRHRTALRRQGVVHELTKALATGWAVVAIEDLNVRGMTAAPLAVPDPDRPGSFLSNGSAAKSGLNRAILDVGFGELRRQLTYKAERYGSVVVAVARFAPTSKTCSGCGAVRAKLLLSERTYRCDECGLVIDRDLNAARNIRDLASAIVATSPADAGDAKRPDERRRPRATGEQAGPARPRTAGPPERVTDSPSPQRTAPSLVA

SEQ ID NO: 66 - protein, 449 aa, synthetic construct
MGPLRHYRENPMQQTVLRAYRYALDPTPAQADMLASHAGAARWAYNHALAVKITAHKQWKQLVAELVETGIPKAEARKQANQQVKIPTKPEIQKALNQVKGDSRKGIDGLCPWHHEVSTYAFQSAFEDADAAWKNWLASTKGERKGPQVGYPKFKVKGKSRDSFRLYGTIRLVGYRRLFLPRIKEVRLHGSGKELARLVERGDAVIQSVTVSRGGHRWYASVLAKVTMVIPDTPTKKQQTRGMVGVDLGVKALAALSKPLNPDDPATALVPNARHLAAAERRLKKADRALSRKTKGSNRRIKAERRVAKLRHQVAVRRASTIHQVTKRLATEFATIAIEDLNIAGMTRSAKGTIDAPGKNVRAKAGLNRNILDAALGEFRRQLEYKTAWYGSQLVVVDRWLPSSKTCSACGTVKETLRLSDRVFVCDACGMRLDRDLNAARNIEAAARL

SEQ ID NO: 67 - protein, 577 aa, synthetic construct
MIQQAYRFALDPTPRQERMLRSHAGAARFAYNWGNAQIIAALDAREAEKAAGTEPGTPVPSHFDLCKMWTAWKDAHAADPEPPEGERRTSTAWVSENFVGTYQAALRDAAKAWSDYFKSARGERKGRRLGRPRFKKRGRARDSFQVHGTTLRPVAASGDGVAFRARHLSPGSHRDVIVLPKIGPILLHESARKLRRRLGKGEVPCPECCQAGVVPATGSTRRKDEVPCPAGMHAGAGCLVCDGGGRVRPCPACGGRLAVPAARIIRGTVARDSDGRWYISLTAEIAREVRTRTVREVQPAGTVTRTAVPAPTARQRAGGVVGADFGVRDIATLSDGTAIANPRHLEAALGKLAKAQQEVARCEKDSAGRRQAAARVGRLHARVKHLRLDALHKATSTLVQSRAVIAVEGFDVQETARYRRGGKVDRGKAEGREKVPGKVRQARNRALADTGIGIARWQLQSKGAWYGCQVLVMDKHAPTGRTCSACGTAKAKPVPPAEEMFTCEACGGVMPRRVNTARALASRARVSVSVAPSTGETLNARGGDVRPAAARRGGQSPLKREASTRPPGRGEPGSPGG

SEQ ID NO: 68 - protein, 582 aa, synthetic construct
MKETVTRVVRYRVDVNALTPTQAQLLDRHAGTARQAWNWATARWLDWQASIEHTVWAQAAHAVGLDHATTTTRLGDALLAARALLRGHEPEQRAWQSTAYTTARATHGHHATFEDAYTLAHLYRLTAAQPHDPTSPDGLERLHWWAAQGTSSGLPRTQQHGVSTFAYQTALADFAKTAQAYWARPRYSPRTGRRLGAPRFKRRGEHDAFAIMNLTTTASGPWKCILDGHRLLVPNLGSLRLTRNTRELRRLIQRGGRPTSVRFTRTGGRWHLAVNVSFEATNPAVLPPPRPNRVQIAGGAVGVDLGITHLATLSTGTHIPNPRHLTAAAARLENLQQRRDRQHRAASPTCFTPDGTHKRGRCTWGRADGAPLSRRARTTQAQITRLHALLATQRASTLHQLTKHLATRHERVAIENLNPASMTRRPYPKPDPAQPGAYLPNQRRAKAGLNRALLDAGFGEFRRQLTYKTTRYGSTLTLVPPAGTSQTCHHCGHRAPQNRETQADFVCVSCGHVANADINAACNIRDHHVAAPTESQHPAGAGAATHHPPVAVAEQTPPGVNETRKGSPVQHTRTADPARVPA

SEQ ID NO: 69 - protein, 509 aa, synthetic construct
MKTEILRAFRFTLAPTPAQEQRLLRWCGNSRLAFNYALAAKKAAHEDWRTQVVALVDAGVEEATARKRVKVPTPTKPTVYKRFVAERGDDRRGVEGIAPWWHEMNTYVFQSAFLDADAAWKNWLDSFKGKRAGRRVGYPRFKKRGLARDSFRLHHDVKKPGIRLTTYRRLRLPAFGEIRLHDNARRLGRLISREEARIQSVTVSRSGHRWYASVLCKVQVDLPEKPTRAQQTAGTVGVDLGVKMLAALSRPLDPKSPDREGHFVTNPRHLARVAKRLRQAQRALSRKQKGSARRDKARRRVARLHHEVTVRRRAALHQVTKKLATRYATIHIEDLHVAGMTATARGTLKRPGRSVRQKAGLNRAILDTAMAETRRQLTYKTSWYGSQLAVLDRWWPSSKTCSDCGWRNPSLTLNERVFHCAHCGLVLDRDLNAARNIERHTAARPTPQQVASGKGETQNARGESVRLPRPRAEKQDPVKREDARPSPAPPRRSNPPTSPPTYNGQAKSS

SEQ ID NO: 70 - protein, 509 aa, synthetic construct
MKTEVLRAYRFTLAPSPAQEQKLLRWCGNARLAFNYALAAKKQAHEQWRAQVDELVAGGMPEAQARKQTKVPIPSKPAVQKAFNAERGDTRADVEGVCPWWHEVNTYVFQSAFIDADRAWKNWLDSFAGKRAGRRVGYPRFKKRGRARDSFRLHHDVKKPGIRLATHRRLRLGSFGEVRLHDSGKRLFRQIDRGEAVVQSVTVSRGGHRWYASVLCKVTTDVPDHPTRRQAERGKVGVDLGVKVLAALSKPLPTSGAVKVSGGGLLVDNPRPLRAAAQRLVKAQRALSRTQKGSARREKAQRRVGRLHHQVAVRRDAALHQVTKALATRFAVVAVENLNVAGMTRSARGSVEAPGRRVRQKAGLNRAILDSAPGELRRQLAYKTSWYGSQLAVLDRWWPSSKTCSNCGWQHPSLTLNDRTFHCTTCGLTMDRDLNAALNIERHTETPNVASDTGETKNARRASISLPGLRAEKQDATKREDADPTGPAPPRRSNPPTLPPQRHEQAKLF

SEQ ID NO: 71 - protein, 760 aa, synthetic construct
MMAVLVVGALCCADHMRPSSDRVGRWRTVRLTLDPTRRQIKVMEMYCLLDRRAYERALPDGPCPNGDSSHASVSRQPDVAAVLASIEPPSTPGDLETKWAVVSSAHHYAAAVSGRRALRVPPRSARRPAPRKRPQTSTRTMFGLYERGGRPHFEIQSYRRVRIGPLASIRIHNSAKGLAAELKDPAVRLVMTTVHRKAHRWYASILIEDSRPLPAPTARQKRNGPVGVDLGVLHLATLSTGETIPNPKVFERGRKQVAKASQAVARSAEGSRRHQKSVERLHRRHHEIAEHRKTVLHTITRRLATSWSHIAIEDLNVRGMTTSARGTIENPGRNIKAKSGLNRALRDVSPWKFREQISYKSGWYGSELVICSRWFPSSKRCSQCGTIRRALPLTQRIFRCATCQLTIDRDLNAAVNLASRVGVAWGTWETENARKESIITNTAGVSHDAASTGRPRADSSATLDEQSSSHPTRSNRQGGPKTLRGPGPLTSRKQPDWTRYHTQWLLNCLALAAQQPPTTRARWEAVTQSLAENSQRSGNVEHGMPVVAVGSRALAIGAQYLCESVIQRCLLQLSAISPDPPIALVRRGRGLGADRWALLPVTSPTEIATGIKPMHPAWHIVGPAHMPTYELVQKHGPTSPVEIISAATHIGKSAAYNSFNVLQQWGLITRRPRYIALGPTTLDDILDQHDHAAAKDAMLDRHRRQRAGWRKTLNLIEYARTSHDIAELAPDSPQLTAGDSEDEQQYRIAVMAGPPPPEAP

SEQ ID NO: 72 - protein, 494 aa, synthetic construct
MNERRLRRLRTYRFTLDPTRAQVDVLVQHAGAARWAYNHALAAKFDALRRRQLQIDELVTLGLTETQARREATVKVPSKPQIQRRWNQLKGDATRDIDGICPWWRAVSTYAFQSAFLDADQAWKNWMDSLSGKRAGRRMGLPKFKKKGRSRDSFRLHHDVKNPTIRLDSYRRLRMPRLGSIRLHDSGKRLARALDRGGRVQSVTVARGGHRWYASVLVDEPDITPGRETQHGPSPAQRAAGGVGVDIGVLHLAALSTGEVVENPRHVRRAHARLVKAQRALSRTVKGSRRRRRAAARVARIHHQLAERRATHLHGITKRLATRHSLVAIEDLNVAGMTRSARGTVAEPGRNVRAKARLNRAILDVAPGELRRQLEYKTSWYGSTLAVCDRWAPTSKTCSNCGTVKTKLSLSTRVFQCDDCGMVLDRDVNAARNVLAVAVPHVASGGGETLNARGERVSPAPRIAAMAVLSDAGRPGRSARSPRGSDPPSIPNPQ

SEQ ID NO: 73 - protein, 545 aa, synthetic construct
MNRREQRIGFAIHLFAAFISGGCDGAGMDENTTTVVVRETLDPTADQRAILQRYADASRCSFNYALGLKHGTQQLWAHGRDRLIAQGQTPAEAARNAPKVDVPSQFAVQKIFLAQRDQPLPGPLLPGQEPRLLFPWWKGVNAIVCQQAFRDADTAFNNWKSSGRRKGAPVGYPRFKRRGRCRDSFRMFAVRLVEQDLRHVRIGGGGGQPAFSVRLHRPARRLARLLARGGVAKSVTISREGHRWVAAFNVRVPVGPVPRPSRRQREAGTVGVDLGVKVFAATSDPVIINDHKIQLFENPRHLENTRRQLRKWQRRMARRHVRGLRSHEQSQGWKEARDQVARLHALVAARRASSQHLVTKRLVTQYAHVALEDLRVKNMTASARGTAESPGRNVRAKAGLNRAILDVGFGEIRRQIEYKALLYGAQVTVVDPAYTSQTCNRCGHVDAKSRRTRDQFTCTRCGHATHADIGAAINIKARAELTSESAAPGLANHDQGVHCGAPANQTRPKARRYAPPAKHGMPYSGEVSGKVPKGRASHSPVSQPG

SEQ ID NO: 74 - protein, 433 aa, synthetic construct
MPADKEPKDILIFRTRLKPNKTQEEALWRNCAGYRWVYNYMLALQKERYEKWREAKEAWEKENPDGGKFKAPDDLKPHSAYDLKKLLPVLKSDEPTAWLGELDSQVLQDAVLNFGKTWQRFLGRSKTGSGFPKFRNRDKNNYISRSNGGKQQWVNENHINLPKIGNVKMYERPHIKNRPDAHLLDLTRPSGYIISRKANHWWISLRYQAPHIEPKKRKGEEVGIDLGVARWATLSDGRHIGRDDRIEAKLKRLLERKDFYYRQLARRPKQKSEEEGRTYSGSNREKTKKKLAKTWARIAEIKRNYSHCASKELSQQFAKIALEELKIQNMTRSAKGTVEEPGRNVRQKSGLNRSINQQNWYQFRSMLEYKMERNGGEVVTVNPKNTSITCSKCGHADKANRPSQSEFKCQKCGFEENADLNAAINICHIAFGG

SEQ ID NO: 75 - protein, 681 aa, synthetic construct
MPHETRLVQRAYKFALDPTPEQAAQFASHAGGARFAFNWGIATYAAALNARQAQKDAGQRITIDLPDHFTLCKLWTAYKDTYRDTPDPDGRTTHWVENNFVGTYQAALRDAHGAWQKMWDSRAGRRKGRAVGRPRFKKKGRSQDSFQMHGDTLRIDTGSAVRPVGAPRVKRRPAEVGEPWGHALRRLTDSARKFYHERRDRKGFGCATPVGVPNKRGWVVDHPCPGAVTHVLTYRAKAVRRSDPTVVDRTVAHKRNLCDEHAAGVAQERGIDLPAEAKKAGVTGYGPAASTSGSRYMSLPKVGQVKIPGKLRIGQRRRVTPTPGETQWVDRSARVARKLARLLRRSETAGPVVCPTCNGTGEVQVTTKAGEPKTSKCGVYGPHVAPDDKRPGCRGSGKVEQARIVRATLSRGASGTWWCSVTAEVVMQVRTAPSKRQTRNGVVGLDLGVRHLAVASTGDTYTNSRFLDANLADLRRLQKALSRAEKDSKRREKAKRRVGALHEQVALMRKDACDRITSEMANTYAKVGVEGWDAQRLAEKGSEGVPVRLRKARNRALADAAPGMFRWQLTYKTSWCGSQYNQGEPHWETGRICSVCGRVRTKPVPLTEEQFRCDGGHVVDRRVNSARVMEKVTAGLIAPPGVVDEPRGGDVRPVTPRRDGRSPAKRAARTRKRGKAGTPDP

SEQ ID NO: 76 - protein, 528 aa, synthetic construct
MPHITIKRAYRVALSPTVAQQCRLARHEGANRAAYNFHLAAKQQAHQQWKAAVETVWQDQYAHLAPDEGYRVAKKAVNQAKAVRFPTYMDSMKALRADKKYAWHAEVNGYALSSGMQAVDRAWKNWVSSYTGERAGQAVGYPRFRKKGRTRRSFTLFHDVKTPTLRPDGYRRLVLPEKISGRRGGSVRLHGNIRLLARRINNQTAWIRSVTISYTGKYWWASILVDERIDQPAHPTPRQRAGGSVGMDLGVHCLAALSTGEVIANPRHLKTAANRLAKAQRQLARTGWWILNSSGHPTQLSRRRPSQGVAYKPTTGRLKARARVARLHAELADRRATTQHALTKHLVANYNRIAIEDLNVAGMTRSAKGSQEAPGSNVAAKAGLNRSILDLGFGEIRRQLEYKTGWYGSQLVVADRYAPTSKMCSVCRAVKPKLSLAERTYTCNWCGTNIDRDLNAACNILNVATNANNSDACGTQESRNARPATSRASAQPVATTLDGQAITSQVTPAKQLAGHPTQTEAKRYKPDT

SEQ ID NO: 77 - protein, 741 aa, synthetic construct
MPIISPGNQESNADGAIELRIAADIDETTGCTFSATGLPDGLEFERKKFEDDEEHTWQTGRIIGTPKRAGIYQVTVTAIDKAGTKTTASFVWTVCAMRAYRFALDLSDPQITAMQQHAGTARWAYNKALEAKVNAHRAYTERLKALLASGLTPQQAKAQMKKESAALKAQTAIWEHHRQCLTAMNLGRALPAKTPRGPQELIDDLAAIRAMVPDGVDPALLTLVGNWKGQPPTALCWARDRHEARQKWIKTHLVMARQTVTHLKQQLFDLGDTIPNMIENLANWRNTRDLPKEEGGSPWWQEVSSYVFSGGMGRADAAWSNWLKSLSGQRAGKAVGYPRFKKRGQCADSFPLFHDVTNPSIRIEGYRHLRLPNIGEVRVHNSGHRSGTRNRVTATNAKGVKRTVSGQSKGRLGSTKRLVRMIERGDAIVQSVTVVRGGHRWYANVLVKLTPEAMRQREMVARAHQKVSKKRAQGRGNVGVEWGVRTLATLSNGESFANPKPGKKNQRRLRVASQKVSRKPHKRGQPISANRAAAIRQLGRVHHEIAETRKGNHHQISAAISLGYRGVAVRGLDVKSMTKSAKGTVEKPGKHVKVKSTFNRAALDAAPGMLQNQISYKTTQYGAKFGVAPKDLPSSQTCSACGWRDPSIPLTQMTFRCGNVECGKKIDREVNAARNIRNSVFPVASDSGDTLNACVDGIGPPGSRGQPSPKQEDPEPHPPPEDGPAEGHSGEAIPRRSHTPG

SEQ ID NO: 78 - protein, 611 aa, synthetic construct
MPQQQPDKPATVTKVIKFMVDMKAMPDTQRELLERHAGTARAAWNWGLAEVNAQQRLVQAHVKRQALAESSDDWDAAKKLLADKKWRTAAYHMAEEQLGKVPNAVALSARFTEMGRDPQSRFGWWSTEKHGVNRFAASTALRDLDTARXRFLSGAAKRGKGRKKRADGFPGGWPRFKKKGRSQDAFALFNIAVSDSWKPLQRRGASKKAPLNHSGEPMLESHRINLPSLGSVRVTQNTTKLRRMVRRGGHPKSARFVRNGDRWEIAINVSFQADNPYVAPPTKPNRIQIAGGVTGIDLGLGALIAFPDGRLIENPQVGKKEQAKLARLRRKYSRQHVTESPECFEGSGVHVKGSCAWRGGKGVPAKMTSSSRETLRGIRKTERLVAQQRATVIHQQTKMLTTQFATVCIEDLRVANMSARPKAKDNGDGSFAQNGRSRKKGLNKSILRSSFYEFRRQLEYKSKLYGSKVVVIDRWTPTSKTCSSCGSVKPKLKLSERIYRCQNCGLVMDRDVNAARNILSAGLAEMERRGAERVVQTRVPGDAVSGSHLAHGPHTGTEPCGTTVGKTPKPSETAKHSRRGPGLANDATGSSNGAVTPTQCRSGTTRNRRAA

SEQ ID NO: 79 - protein, 594 aa, synthetic construct
MPQTEVLRAYRFALDPSDAERAELARYAGACRWAFNYALAKKTQSYRAWAERRTAYLAAGLSEAEAKARIKADGAELTDRIKVWDHHRKCLMNTATGKQPLPATQPPAGQEALACRLAAARADAAATGCERRLLAEARTTVNALKAEAFSAGYRTPNATDTSALWRMDRDRPKEEGGSPWWTEVNVYCFTSGFDRAQVAWKNWQDSLAGRRAGCRNRYPRFKKKSRAAESFTLFHDVKRPIIRLDGYRRLVMPGLGSIRIHDGGKRLARLVDRGQAVIQSVTVTRGGHRWYASVLAKVQQDVPVLWEHVDDAGTRVRYLTRTQAENAAENGGRIEQIGRPSARQRAGGLVGVDLGSRYLAALSSPLDPADPTSILLPHPRLLADSTAKLAKAQRTLSRTQRGSRRRVKAAARVARVHHQIKVRRASFLHGLSKKLATRFTHVAIEDLNLTALTASAKGSPDKPGKNVKVTARFNRHLLDAALGSLRSRLAYKTAWYGSQLVILDKAEPVASTCAKCKERNPNSAPSHSKFHCPSCGAVVHRHENSTANIVRAARRQLTTVASDRGETQNARRAAVSPGARKGPGQGALKREDTG

SEQ ID NO: 80 - protein, 593 aa, synthetic construct
MPRTEVLRAYRFALDASDAQRAALSRYAGACRWAYNYALAKKTRAHQAWAERRTAYLEAGLSEAEAKERIKADGAELTDRIKVWDHHRKSLALTVAGKPPLPAMQSPAGQGVLIRRLAAVRADAAGSGSERELLAAARATVNALKVEAFSAGFRTPTSTDTSALWRIERDRPRKEGGSPWWSEVNVYCFTSGFDRAQVAWRYWQDSLAGRRAGQRTGYPRFKKKGHAESFALFHDVKRPIIRLDGYRRLVMPGLGSIRIHDSGKRLARLVDRGQAVIQSVTVTRGGHRWYASVLAKVQQDVPVLWEHVDDDGTRTPYLSRTQAETAAENGGRVEQIGRPTARQRAGDLVGVDLGSPYLAALSSPLHPADPATALVPHPRLLADSLPKLAKAQRAMSRCQQGSERWRKATAQVSRLHQQITVRRASFLHGLSKTLATGFTHVAIEDLRLTALLTSAKGNPDKPGKAAKRKSHSNRHLLETGQGSLRKKLEYKTAWHGSQLVVLDHREPVAGTCSKCKERNPSSDSSHSKFHCLSCGAVVHRHENNTANIVHTALRQLMTVASDRGETQNARRATVSPLARKGPGREALKREDTG

SEQ ID NO: 81 - protein, 493 aa, synthetic construct
MPTEIRTIQQAYRFALDPTPAQERMLRSHAGASRFAYNWGNARIIKALDARKAEEAAGGEAKTKVPGHFDLCKQWTSWKDEHADDPEPAEGERRTSTAWVSENFVGTYQAALRDAAKAWGDFFKSAKGERKGRRLGRPRFKKRGKARDSFQVHGGTLRIESAGAGFRPKGADKGATRDMVVLPKIGPVFLHESARKLRRRVDAGTARIVRGTIARESDGRWHIAITAEVRQEVRTGPSARQRAGGIAGADFGVRDIATLSDGTAIANPRHLEGALGKLAKAQRALSRCEKDSAGRRKAVARVGRLHARVRHLRLDGLHKATSGLVHSRAVLAVEGFDVQETARYRRRGKADPGKYRENVPARVRADRNRALADTGIGIARWQLQSKGAWYGCQVLVMDKHAPTGRTCSACGTAKAKPVPPADELFTCEACGSMMPRRVNTARALALRARVAVTVAPSTGETLNARGGDVRPGAARGNRQPPLKREASTSPRAG

SEQ ID NO: 82 - protein, 612 aa, synthetic construct
MPTEIRTIQQAYRFALDPTPRQERMLRSHAGAARFAYNWGIARTVNALDAREAEKAAVQSAAAEAAARVAELEQLVADAAADAAAEYTPPMTAVGDATIRLRNLQAQLAGAKADAATASGGKPETKVPGHFDLCKQWTAWKDEHASDPEPEPGGRRTNTAWVAENFVGTYQAALRDAAKAWADFFKSAKGERKGRRLGRPKFKKRGKAKARDSFQVHGQTLRVVSAGAGFRPKGADRGATRDMVVLPKIGPVFLHESGRKLRRRTDKGTARIVRGTIARESDGRWYIALTAEVQREVRTGPSARQREGGVVGADFGVRELATLSSGNVIPNPRHLEADLGRLAQAQRALSRCEPGSKRRAKAVRRVGRLHARVRAERLDSLHKATSALVHSHERIVVEGFDVQETARYRKRGKVDPKKKEKSKSVPGKVRADRNRALADTGIGIARWQLESKSAWYGCQVVKTDKHAPTGRACSACGTVKAKPVPPADELFTCEACGTRMPRRLNTARVLLSVTVAASTRETLRRRVGAAVTGTATPAGEAVKETINAPGGSVSPSAARGGGQFPVKGEASTRKGTTLAENAASRVPGENAMSYSGHRAAGIEHRAAEPRPG

SEQ ID NO: 83 - protein, 506 aa, synthetic construct
MPTEMRLAQRAFRFALDPTPRQARMFASHAGGARFAYNWGNAQIIAALDARQAEKDAGAEPTVKTPSHFDLCKAWTAWKNEHAADPEPADGERRTNTAWVAENFVGTYQAALRDAAKAWSDFFASRSGKRKGRRLGRPRFKKKGKSRDSFQVHGGTLRMEDAVHVTLPKIGTITVMSDDSLHPAMRRSRARATHLAPRHMGNRRRARTLWRALRRGGGARLIRGTVTRGADGLWWLSLTAEIPLQVRASPSRAQQEGGMIGADFGVREVATFSNGVTIRNSRHLEAALAELRAAQKALSRCQKDSMRREKAKARIGVIHADVARLRETALHRATTVLVRQHDVIAMEGWDVQQVMRGGSKDVPRRIRRDRNRALADTGVGMARQMLSYKGPQMGAIVMVTDPQAKTGRTCSVCRTPRTTALPPHHEMFTSDQCGHVLDRRLNTAQALAGWAAQELSKRGPAPAGPSRPRGGNVRPAADRKVGGGRSPVKRAASTRLGRGEPGTPGG

SEQ ID NO: 84 - protein, 607 aa, synthetic construct
MPTEPRLIQKAYKFALDPTPTQARAFASHAGGARFAYNWGISTYAAALDARKAQTDAGQDPTVDVPNHFALCKAWTQYKDTYRLTGDPDGRPVHWVEDNFVGTYQAALRDAHGAWQKMWDSRNGQRKGRAVGRPRFKKKGRSPDSFQMHGDSLRLDSGRALRPADATARKPLNRAERAKLAPTPGMTPTERSAAQKRLRAGRKARAGHVHGPQVSQSGTIYVNLPKVGPVRVPGRVRIPQVTPSVAGWVDRNSRTARKLLRQLAKAATTGPVVCPTCAGTGTVTVTTKKGERRDTKCGKYHPTVRPEDKLPGCQGKGKVEPARIVRATISRGASGTWWCSITTEQVITVPVITTRRPAHPTRRQLADGSIGVDLGVKYLAVLSTGDTYMNSRFLDSALTDLKRMQKVLSRTAKDSHRRLKARRRVGTLHEQVALMRRDATNRVTTELARKYATISVEGWDAQRLAELGSKDLPKRLRRNRNRALADAAPGMLRWQLEYKTSWYGSTLFKGEPHWETGRICSVCGTARTKPVPLAEEQFRCPQGHVLPRRVNSARVMDRVARGLVAAPATPEPRGGDVRPATPRRGGPSPAKRVARSRKRGKTGTPDP

SEQ ID NO: 85 - protein, 572 aa, synthetic construct
MPVEIQTIQQAYKFALDPTPRQARMLASHAGAARFAFNWGNARVIAALDAREAEKAAGGEAKTPLPSHFDLCKAWTAWKDEHAADPEPPEGERRTNTAWVSENFVGSYQAALRDAAKAWSDFFKSRSGKRKGRPLGRPRFKKRGRARDSFQVHGQTLRPENCGAGFRPKGADKGATRDMIVLPKIGPVFLGESARKLRRWLRKPDVACPDCCGWGSPGKVPAAADSKAKAVADCTACPGAGRDCPVCDGSGKVRECPACGGSLRVPAARIVRGTVARESDGRWLVSLTVQRAREVRAVRVKTPLKNGGTAREYQPSPSARQRKGGIAGVDFGVRDLATLSDGTVVANPRHLEGDLGRLARAQRVLSRREPGSKGRREAVARVGRLHARVRHLRSDSLHKATSGLVHAYETIAVEGFDVQETARYRRRGKADPKKGKDVPARVRADRNRALADTGIGTSRWQLLSKGAWYGCQVLVMDKHAPTGRTCSACGTAKAKPVPPAEEMFTCQACGNVMPRRVNTARALELRARKAVHVAPSTGETVNARGGAVSPAAVTGSGQVPLKREASTRPRPG

SEQ ID NO: 86 - protein, 508 aa, synthetic construct
MPVENRLIQQAFVFALDATPRQQRAFASHAGGARFAYNWGIQKIAEALDAREAEKAAGQTPATKIPGHFDLCRMWTEWKNTAQWVDRETGEVTAGVPWVSRNFVGTYQAALRDAAAAWKRFFDSRSGKLAGRRVGRPRFKKKGRSRESFQVHGAQLKVVDAHHVQLPKIGVVKTHESTRKLLRRIRKGDTTCPTCQATGQVPGKDTPRKCPACKGHGRVPTARLVRGTVSRGSDGRWQIAFTVELVREVRTGPSRRQRAGGTIGVDLGVRFLATLSTGEQVKHPRHLEAALDRLAAAQRALARCEKGSKRRAKAVARVARLHARVANLRRDAAHKFTSHLVHSHERIAVEGWDVQQVMQHGSAGLPRRVRRARNRLLADAGLGEIRWQLKSKSAWYGATVVVADPHAPTGRTCSRCGQVRAKPVPPVEELFACPSCGWCGDRRLNTARVLAQVARGDIVSDASSGGESLNARGGDVRPGALRRGGRSPVKREARAWLKSRGETGTPGP

SEQ ID NO: 87 - protein, 542 aa, synthetic construct
MPVEVRTVQQAYRFPLDPTPAQARAFMSHAGGARYAFNWGLATKAAALDARQAQKDAGEELSVPVPNHFALCLLWTEFKDHGVVCRRCGMPVTAGGDGDHAASSRGEGETSDSCRDGEPHDPGVGLPWVSANFSGTYQAALRDAHQAWQNFFDSRSGKRKGRFAGRPKFKSKRNPKRSFQTHGTGLRIADHRHVVLPKIGSVRTHEPTKKLLRRLRKGETACATCRTSGVVKVETKAGTKERKCGTCRGTGQAPYARIVRATVSLHTNNRWYISITVEAQREIRTGPSQRQREGGRIGLDLGVRSLLVTSRGDRIANPRHLDKALRRLRHAQQDLSRTEIGSGRRERSRKRVAQMHARVGHLRADTCHKITTDLVHRYAGIAVEGWDIQQTAERGSRHLETRKRRERNRNLADAALGNLRWQLQSKGRWYGCEVDVTDPHAPTGRTCSACGAVRTKPLPPAEELFMCPSCGYAVDRRVNTARSVARLARESKNGAAGSGSEAKNARGGGVRPGASRRAGQSPSNREARAGPKGPGKTGTPAG

SEQ ID NO: 88 - protein, 564 aa, synthetic construct
MPVKDELITQAYRYALDPTPAQERAFTSHVGGARFAYNWGLATYAAALDAREAEKAAGEKPTTRLPGHFELCRLWTAHKDTTEWVDRDTGETTTGIPWVSRNFSGTYQAALRDVHGAWKKFWDSRNGSRAGRKMGRPRFKSKHRSRPAFQVHGSGLQVADSHHVKLPTVGTVKTCESTRKLLRLLQTGQKTCPDCSGQGRIRRGPKTSRSQRRLFHGRPAWTSDRFKTCQSCKGNGKLDPTPDARLQACPTCKATGQVPGKGAPKNCPDCKGHTQVPTARIVRGTISQHSDGRWYLALTVQRIRQVRTSPSRAQRNGGTIGIDLGVRSLVVTSDGQTVDHPKHLTKSLGKLAAAQKVASRREKGSARREKANRKVARLHARVGHLRSDATQKLTSHLIHHHQRIGVEGWDVQQTAQHGSKDVPKKVRAKRNLALADANLGQIRWQLQSKAVWYGTHVVVSGKHTATGRTCSVCSQERANPVPPHHDEFQCPECGWVGDRRVNTARVLAQLAQQQQNDASSAGESLNARGADVSPARPRPGGQLAVKREARSRSEGRGDPGSPGP

SEQ ID NO: 89 - protein, 498 aa, synthetic construct
MPYDAVPNVVLRRAQQSVHDAYLSYLRLRRNGATEAKPPGFRSSRRAMPCLGYQTQTRSRAGTVEDWLPQRGPKWALVRVPQPRSSVARISDARVRLRYHRPIPDGAEVQLATWSFDRAGGHWYVSLQCSLAVPASEPSSTPVVVGLDRGVRDLAACVGVDSATRQIVVDRAVQPSPGLTPARRRRLRLLERSVARSHRAVCPGYEPGQRHPSGMCMWRRRKPARARRAEAEIARLRAADARARHEVIEVLTHDLVDGSPQRSWQPADVVAVESLRVKDMMRSARGTADDPGANVTAKAGLNRSIQAASWSRLSIRLCAKAGRARLVGRTVEVVEVDARNTSRTCPECDDVDPANRRHGGKSFACGRCGHRDDADRVAARNIVTRALDLIEGRLAPADGAPSAGCGGLGVSELPPGDGGSGPALVPRGESAGEAPLRSRRTAHSAHRIHASAPAADDAGVSARSGQAPHHEEVRYGDRDGQLVEVALASGTVMAGGAP

SEQ ID NO: 90 - protein, 538 aa, synthetic construct
MQATESPAGFPSSQEAQSSICRAYRFALDLSPEQIQDMQRHAGAARWAFNFALEMKVAAHQRWRADVEALIAGGVPEADARKQVKAPFPKVKDIAAYWRTVRGDSRGGDAAAQTGRSPWWHEVSSYAISTGMRNAETAWSNWLKSFKKQRKGARVGYPRFKARHRSRDSFTIYHDVRKPTIPIADYRHLQIPRLGLVRVHNAGRRIGAGKGQQRLGSTKRLVRMIERGEATLKSVTVSRGGTRWYASVLLEITEAGMRQRESVTRKHQGAPKQLQRTRPEIGVEWGVRTLATLSDGTTFANPRYGKRNERRLRRASQNLSRKPYARGTPSSANRQKAVDRLRKVHHQTAEARTSGLHQLSVRIAVNYPWVAMRELNVKSMTKSARGSQEEPGRLVKVKARFNRAILDAAPYELRRQIEYKCDAFGASFGLAPGDLRSSQDCSECGWRDPSIPLEQVIFRCGNDECGLVLDRELNSARNIRNHAVVAPDGGETLNACGEDIRRPGDRSQSSMKQEDWPPPDGQPSRGSDSPALLASPDL

SEQ ID NO: 91 - protein, 659 aa, synthetic construct
MSAQAPAFLELEAHARVRVLFGCPVNMTVWRVTGSLCPVAICGPAQRLGSGGTPRVAAKSHPAGRGHGPAAVTMPRAEVLRAYRFALDPSGAERAALSRYAGACRWAYNYALARKMRAHQAWADRRSAYLAGGLSEAEAKERIRADGAELTDRIKVWDHHRKTLTLTVAGKPPLPAMQCPAGQEALVRRLAAARADAAGTGSERELLAEGRAMVNALKAQAFTAGFRTPTAIDTSALWRMDRDLPQQEGGSPWWREVNVYCFTSGFDRAQAAWKNWQESLAGRRAGRHHGYPRFKKKGHTESFTLFHDVKRPIIRLESYRRLVMPGLGSIRIHDSGKRLARLVERGQAVIQSVTVTRGGHRWYASVLAKVQQDVPVLWEHVHDDGTRTSYLSRTQAEEAAGSGGHVEQIGRPTARQRAGGLVGVGLGSHYLAALSSPLDPADPATALVQHPRLLADSLAKLSKAQRAMSRCQQGSRRWSKATAGVSRIHQQITVRRASFLHGLSKKLATGFTHVAIEDLDITALTTSAKGTRDEPGKNVKAQARFNRHLLDAGLGSLRKKLAYKTAWYGSQLVVLDQGEPVTATCAKCKERNPSSDPSCSTFHCPSCGAAVHRHENSTANIVDAAHRKLTTVASDRGETQNARRATASPGARKAPGKGH

SEQ ID NO: 92 - protein, 526 aa, synthetic construct
MSAQHDDDGQPLAATPSPAPAPTLAPTAVPLPVPTPGPGPVVRAYRLALDPTPTQATAFARHAGASRWAFNYALAAKKAAHAACREQVDALTAAGVPEAEARKAVKVEVPGAFTVQKTWQHERTEVCPWWGEVSSKAFVQAFRDADKAWTNWLASLKGQRAGHRVGYPRFKKRGRCRDSFRLEGAIRPEGYRHLLLPRIGPVRTHQTCKPLARALERQGGRITSVTVSRGAHRWYASVVVTFPSGTLPTPQRAAPTRAQQRAGVVGVDLGVKHLAALSALGADGTLAESLVANPRHGARGARRLAKAQRALSRTQRGSHRRAKAAAIVARRHADLAAQRATSIHVLTKHLATTYAGVAIEDLHVSGMTRSAKGSLAKPGRNVRAKAGLNRSLADVSFGEIRRQLAYKTRWYGSTLRVVGRFEPTSKTCSACGRQDPHLSLAERIYECPCGLRLDRDLNAARNIRVAGFEPAAWAAAVARGSRETSNARRGPASPHTRPGVGLGPLTREDHPDTAAAVAVGVVTSGR

SEQ ID NO: 93 - protein, 549 aa, synthetic construct
MSDQQPQPDATDSPTTIVVQRAWRCTLAPTPAQQQMLCQHAGAARWAFNLALSAKIVSRGVWEQRVQALVDEEGVPEDQARKQVKVKTPGSNVLDKARVRVRGTDRWGERCTADWVDARRVLTDNKIDEEVADEILTRWASRVDDPSEGIAPWLAEVPNSLVQRGEKNADKAWQTWMDSVTGRRKGRRVGFPRFKKRGVRDSFYLTNTESGPCLGSNRHVRLGGKLGTVRVCDADGKRALRRLHRRLRQGTCRIMSVTVSRGGHRWYASVMTEETLPAPRPSRRAVEAGTIGVHLGVHDRAVLSTGEIIENPRIKARHARAIAKAQRALARTGWTVNDDGRKRPTRRREKARQRVARLAHLEAQRRNTHTHHLSKRLAAEYAEIVMLDLDIQGMTRTARRCRPPLHGWDAQAKRTANTAFLDVAPFELRRQVAYKTTWRGARLTVAPKGTAVVGICPECGAVRAKRPVRGDRITCPCGAVYGRGHAAALILARHGAVACNTRETLNARGEDVRPTAPRDSGRSPVKREGPRHLRGSPLGSDAEAFPLRT

SEQ ID NO: 94 - protein, 533 aa, synthetic construct
MSDSVITRAYKFRLCPSFEQRVRLWGCAEMARMAWNWTVALCEREYEEALIAAGVLEQRELDGCERRKQRVAVVARARARARENKVVVQSPSINRGRLYKEWCVMRDSTANSIRNYHSHTYSYPIARVVQAYKDWWRKKGGRAGAPRYHRDSHPSSFTIQLSRTVWDDDGIRIPGVGYVRTTWRNRGRWCGESPSAIPPGKPCSITVTRKANAWYASIAMKDVGFDETAGTGVVGLDLGVSSVLTTSDGQSWAPPRPLEKALRRVAILQRRRQRKPKRSRRRTLLDIQIASLHARVAAIRYDHLHNVSTHLAKTFGVVVVEGFDVVGLVSNEVQWRAIRRAMMDIAWGELRRQLEYKLQWRGGTLMTMGVFDPTNQQCASCWKTGTVTMNACPPSQAIYRCSTCDAKVSRQMNTAKLLELFGRFGPPPQQGTGAQPGPRPPRRRGKGHARGGAESTACSAAPVKREQTLHAPPQGASPGARALLARTVSDGCTQDGGSATPNPSCNKPQRKPLVRAREQGNSEPVAAEVQEGV

SEQ ID NO: 95 - protein, 436 aa, synthetic construct
MSEQTRFHAFRYTLAPTPSQEAAFFRYAGAALWAYNHAIGVKKAAHQEWRTQVDALVASGIPEEQARKQVKVKIPNSFEIGKNFNRIKGDSREGIDGICPWWHEVNRYCFKSAFADADQAWKNWLASLKGTRKGRKVGYPRFKSKRHSRRSFRLYEGIRPVGYRRLRLPSLGEIRIHGTTKPLVKLLNSGQATIKAVTVSQGGHRWYASVLCEVTTNLPDGPTRRQRSRGTIGVDMGVKNLATLSKPLNPDDPTTAIVPNPRHLEATDRRLRRAQRALARKQKGSKRREKAARRVARLHHQVAVRRATAIHELTKQLATSFEAVAIEDLNVQGMTRTAKGTIDRPGRNVKAKAGLNRAILDAGFGELRRQLEYKTTWYGSRLLTVDRWMPSSKTCSGCGWKAPELLLQTRVFRCGGCGLVLDRDVNAARNIERHAA

SEQ ID NO: 96 - protein, 483 aa, synthetic construct
MSGVGATVLRVVDPGSTVVDENERRRQRAYRFALDPTPAQEAVLTAHADAARWAFNFALAQKKAANETWRLQVAELTGLGFTEAEARKTAVKTPNAPEVARRWTAWRDNPAADPWRGGICPWWRGINRFAFSSGFRDADQAWSNWMSSLAGKRAGRRVGEPRFKRKGRVTPSFRLHHDVKKPTIRTDGYRRLRMPNIGTVRLHDTAKRMVRALERGGRVQSVTCSRRGHRWYASVLVDEPDVTPGRETQVGPSHRQKNAGRIGVDLGTKALAALSEPVPGLSDEHGLIENPRHLKKARRRLVRAARQMSRRVGPDKRTGQKPSNRWKRARARLSKIQREVTVQRASHLHWITKTLSTSYAEVAIEDLNVAGMTRSAKGDVAEPGRNVRAKTGLNRSILDAAPGEFRRQLDYKTPWYGSTVAVCDRWAPTSKTCSACGAAKTKLPLSERVYTCNHCGFVCDRDVNAARNIAAMAVPVDPGGGRR

SEQ ID NO: 97 - protein, 578 aa, synthetic construct
MSKQVIPIARGRGGKAMAEKTSTDDGALYRAYKFRLDPNQAQKAELMRCVGAARCTFNLLNEYNLQILRNEQEYRRTRAAEGIDYGTINGELKKLGKKDPEYKFLGQAEYEKRYLTPEKQRHEAIAQAIADGADPAIVWPETERFTEPWLHTIARRVLVSGIKNADKAWDNYNKSRMKQRAGARMGVPRRKRKGISHDSFTVDRDPRKDEVGAYGTPYKQGEPEYVRRKAQLKRRSIKTTPTIGDYRHVRLSHLGVIRTHNTTKPLVKAVRAGANVKSYTVSRAANRWYVSILVELTRPSATPTRAQRAAGAVGVDLGVRYLAALSDEQAPQRFARYPSLEFTGDGVPTLANPRWARTAERRLVRLQRALARAQKGSNRRARIVKQIARHHHLVALRRESGLHQVSKRLTTGYTLIGLEDLAVAGMTVSAAGTIEAPGKNVRQKAGLNRSILDAAFSTLRRQLEYKASWYGSRVQIIDRFFASSQTCSACGARAKTKLDLRVRVFECAACGVRIDRDVNAARNICAEAVRMHEAQLAPGTGESLNGRGVADSDTTGSVVLEDGALDASRPAATGGGSP

SEQ ID NO: 98 - protein, 519 aa, synthetic construct
MSQDRTRGFVVKLAPTWEQHRLMLSVARARRRVKNFLVLEARRRLSVSIWQSCVAYAATKGLEAAEVRRQWADKKEGRPALRAAGFKITPPAALDYRATTKWAGVRSRRWMLSVSSEARKFACNSFRTAQQNYVSSIMGRRKGAPLGPPAVESRFAKPTWTYQVPPSRWRAWVTSTHIWIPGVGAVRVSEDPLKGAHGGEVALVSVKRDGSRWYAVIHYRKMRDVERPFGRNSGSVGVDMNVGDNGIVLSTGKRYPVPRSLEVLDAKIRKHQRINRHKAGPRPGKSPSVRWRKQNRRLRDLHREVVRVRTDWLHKVTSEIVKEFRVVVVEGFSVKILTASARGTVEAPGVNVRQKAGLNRKILQAGFGSFREMLKYKTGAIGGVFVMIDRFFPSSKLCSRCGWKDVDQTLRDRVFRCRECGLTIDRDHNAARNIRRAYEDSVVDASTTESTGGEHRPWTGQPLIEGHVLTIKSPGKTPAREQKRKRTKDVRGRSADLGQAGGAHGPKTSSDARGDDAPV

SEQ ID NO: 99 - protein, 440 aa, synthetic construct
MSRQIILRAYRYALDPTPAQSGDLNRHAGAARWAYNHALAVKVAAHEEWRRRVAGLVEAGTPEVEARKQVKVPVPAKPAIQKALNQVKGDSRTGVDGVCPWWHEVNTYAFQSAFLDADTAWKNWMDSLKGRRKGRPVGYPRFKKRGAVASFRLHHDVKRPSIRLAGYRRLRLPRIGEVRIHGSGKDLARAVARGDAVVQSVTVSRRGHRWYASVLCKVTVEIPDGPTRAQRARGAVGVDAGVKVLAALSKPLDAADPGTVIVPNGRPLAVASRRLVKAQRALARKQKGSNRRVKAVRRVARLHHEVALRRGTAIHTLTKRLAAGFDTVAVEDLNVAGMVRSAKGTVEQPGRNVRAKAGLNRSVLDAALGEMRRQLEYKTGWYGSRLAVVDRWFPSSKTCSVCGAVKESLALSERVYVCSVCGARLDRDVNAARNIEAAGI

SEQ ID NO: 100 - protein, 495 aa, synthetic construct
MSTGDVELRAYRFALDLTPAQEQQIRQHAGAARWAYNHALAAKFAALDQRQATIAALVEQGVDPKAAAAQAPKIPTKPAIQKALNEAKGDDRTGADGHCPWWHTVSTYAFQSAFADADTAWGNWLSSITGNRKGQRVRKPRFKSKHRSRDSFRIHHDVHNPRIRPDAGYRRIIVPRLGSLRLHGSTKRLCRALDRGAVIQSVTISRGGHRWYASILTKAPTATATPSGRQRAAGTVGVDAGVHHLAALSTGDLIDNPRHLNHAHTRLTKAQRALSRTKKGSTRRRRAASRVGRIHHHIAEQRATTLHTLTKRLATGWATVAVEDLSVAGMTRSARGTVEQPGTNVRAKSGLNRSILDTSPGELRRQLTYKTRWYGSTLAICDRWYPSSQTCSTCGARSKLRLSQRVFHCAACGLRLDRDVNAAINIATHAVVAVASDTGETQNARRDPTPTPAPAEQQRQVTDAGRPHHTGAATSAEQSADHLKTARQPPLALVS

SEQ ID NO: 101 - protein, 494 aa, synthetic construct
MTAPEPQLRAYRFALDLTAEQETRCRQHAGAARWAYNHALAAKFAALDARRAVVADRTAAGDDPKTAGAHAPKIPTKPTIQKNLNQVKGDSRAGIDGLCPWFHEVSTYAFQSAFADADTAWKNWTDSITGRRGGRPVKRPRYKTKHRSRDSFRIHHDVTHPTIRLDTGYRRIIVPRFGSLRVYNSTKRLRRAVAAGAVIQSVTISRGGHRWYASILTKHPSQPAATASRRQRAAGTVGVDVGVHHLAALSTGELIDNPRHLAAARTRLTKTQRALARTEKGSQRRRRAAARVGRRHHEVAERRATTLHHLSKTLATQWAVVAIEDLNVAGMTRSARGTIENPGTNVAAKSGLNRAVIDAAPGELRRQLTYKTRWYGSTLAMCRRWIPTSQLCSACGARAKLTLAERTYHCAACGLILDRDLNAARNIAAHAVAVAPGTGETLNARRASTDTPPPVAVSVDVMTREDHTTGVATSVGQPADHPQSTCPPEYPLVS

SEQ ID NO: 102 - protein, 548 aa, synthetic construct
MTDTSPRPPVVHRGYKLRLDPNLAQLEVLRQQVGTARVAYNMMCAYTHDIQAARDGRWKELVSTGVNFSVAWDQVKKEAKANFALQYPGYQQFSKILTQQVARHRHAAAAIEAGADPAAVWGEEERYATPWLHTAHRRVLVSGLQMCGNSLSNWLTSQSGKRKGPAMGPPQFKRKHHSRESFTIPAPEAMGPKGFATYKRGEARSGEITDYRHVRLSHMGTFRTVDSTKRLVRALRQGGKIKSYTVSRAADRWYVSFLVERPAPQNPPHPTRRQQAAGAVGLDFGVSRPVTLSTGESIPNPRHLARAEKKIKRTQRKLARTQKGSNRRRKLAQRLARHHHTVALRRHGFLHEVTTALAGGFAAIGVEDLNVAGMTSSARGTVDNPGKNVKQKAGLNRAILDVSPGEFRRQLDYKCTERGVALIAVDQFFPSSQICSACGSKTKMPLAKRVYDCQQCGILIDRDVNAAINVLREAARLAQFSLGDSSAPEGAEGKWPWTPTAHRTRPGVGDGAGVEAARPAWSQQSSNRLLVPYNVRIQSEQKHPLQVR

SEQ ID NO: 103 - protein, 462 aa, synthetic construct
MTEIKRAFRFALDPTPAQTEFLQRYANASRCAFNFAHAFMLAHHHNWHRGRNTLIAAGMDKAEATKKAPRVKMPGRDRAQAFWRDTRGQGFVGPLREGAERAGAYVWWEGVNNRAYYTAFEDAATAWKNYLDSAAGRRAGERVGLPRFKAKGRCRESFRLVHNTKKPEIRFIEPRRLRIPGGGGQPAFTVRLHQRASRLIALIEAGKAVITSVTVARAGHRWYASVLCTVDQAIPDQPTCRQRQAGRIGVDLGVKSLLALTDPLHLTPGTPAATLVGNPRHYDNIARKLARAQRQMARRHVKGARQQSKGFQEARDRVARLQAQLAARRVTGLHLISKRLVQQYSEIALETLNTKGMTRSAKGTVDRPGRNVRAKAGLNRAILDASFRELNRQIEYKARWHGVQVARVPTFFPSSRTCSTCGWTNTTQTLKDRTFHCESCTMILDRDTNAARNIKKHAVPVQ

SEQ ID NO: 104 - protein, 492 aa, synthetic construct
MTQVETLRAYKFALDPTAAQLADLARHAGAARWAFNHALGSKVAAHRQWRAAVDALVAGGMPEPQARKAVKVPVPGNQAIKKTLNGLKGDSRSDPALPDGFHGPPRPCPWWHEVSTYAFQSAFIDADRAWGNWLDSLTGRRAGGPVGYPRFKRKGRARDSFRLHHDVKKPTIRLDGYRRLQLPRLGSIRVHDSGKRLARLIAKGHAVIQSVTVFRGGNRWYASVLAKVQQDIPDKPTRAQTGRGTVGVDWGIKHLATLSQPLDPADPATLHVANPRHLDAWNRQLATAQRALSRTERGSKRRAKAARRVGAIQHRIAQRRATTVHLLTKRLATGFATVAVEDLNVRGMSASARGTVEQPGSRVRQKAGLNRGILDAAPGELRRQLTYKTSWYGSTLAVLDRWHPSSKTCSSCGTAKPKLTLSERVFTCTTCGLTIDRDHNAAVNIARHAVVPLVEGDANARRSPRPADAGRDGHAERQKREGPPPGGSPRRE

SEQ ID NO: 105 - protein, 495 aa, synthetic construct
MTSEPTHELRAYRFALDLTKPQEELCRKHAGAARWAFNHALAAKFAALDARRTAIADLVAGGMDPKTAAAQAPKVPGKPAIQKALNEVKGDDRRGLDGLCPWWHELSTYAFQSAFADVDTAWSNWLGSVTGKRAGKRLGAPKFKSKHKSRDSFRIHHNVAKPSIRPDTGYRRIIVPRFGSLRVHDSTKRLSRALDRGAVIQSVTISRGGHRWYASILTKQPAVPVVASQRQLRAGTVGVDIGVHHLAALSTGEIIDNPGHLRSGQKRLTKAQRALSRTEKGSQRRRRAAAKVGRRHHEIAERRASTLHQLTKRLATEFAVVAVEDLNVAGMTRSAAGTIDNPGKNVVQKSGLNRALLDVAPGELRRQVAYKTRWYGSTLAVCGRWVPTSQLCSACGVRAKLTLADRIFRCAACGLTLDRDTNAAVNIAALAVAVAPGTEETRNARRAAADPPPLVGTESVAALKREGHASGVVTPAEQSAGHPKHADPAEYPLVS

SEQ ID NO: 106 - protein, 524 aa, synthetic construct
MTSQEVLRAYRFALDPSDSQAALLTRYAGAARWAFNHALAAKQAEHQRWRAEVQALVESGETEAEARKRIKLVVPSKPAIQKAWVTGRGDSRSAVDGSCPWWWEVNNHCFQSGFIDADAAWRNWLSSLRGQRGGHRVGYPRYKKKGRSRDSFRLHHDAKRPSIRLVGYRRINLPKFGEVRIHNSGKPLARMVGRGQAVIQSVTVSRAGSRWYASVLCRVQQEIPQRLTARQRAGGVVGVDLGSTHLAVLSGRLRQADHDSNVVEHPRHLQRCMTRLTKAQRALSKTVKGSVRRGRAARKVARIHHVVAERRATHLHALTRQLAENFSHIAVEGFDVQGLMKRPPVPGEGRRASSITARFNRYLLDAAPGEVRRQLAYKALWYGSTMVVLTPGEPVNQVCSRCGSQNSRVSVSDSRFSCRDCGFSIGRRHNAAQNIRHAAQRMIGNVTSGSGETEKARGVAVRPSAGSAKGAQRRSEKTSGHRGLMPPRESDLAAPCVPHQGDMQGDQSTGSTPERDGFCDPGCG

SEQ ID NO: 107 - protein, 513 aa, synthetic construct
MTTARANEIPTCQTQHLRSTHMTDVELSAYRFALDTTPAQLTMLRQHAGAARWAYNHALGVKFAALDERKTVIAGLVEQGLDPKTSAAQAPKIPTKPAIQKALNTTKGDDRISAAGDCPWWHTVSTYAFQSAFADADTAWKNWLASLTGKRSGPIGAPRFKSKHRSRDSFRIHHDVNNPTIRPDDGYRRIIVPRLGSLRVHDSTKRLKRAIDRGAVIQSVTISRGGHRWYASILVKAPAAHAAPTRRQRQAGTVGVDLGVHHLAALSTGDIIDNPRHLAAGQKRLTKAQRALSRTEKGSNRRRRAAARVGRRHHEITERRATTLHTLTKHLATNWATVAIEDLNVAGMTRSARGTIDNPGTNVRAKAGLSRAILDTSPGELRRQLTYKTGWYGSTLAICDRWFPSSQQCCECKVRTKLRLSQRVFTCPACGYGPIDRDVHAARNIAAYAAVASDTGETLTARRDTAEAPTRVGRRRGAVDAGRPHRETGAATPAEQPAGHPKHADQRTLPLVS

SEQ ID NO: 108 - protein, 632 aa, synthetic construct
MTTETVMQQLAFKVALDPTPRQARAMGSHAGGARFAYNWGIARIAEALKQREAERQAGGEPTTPVPDHFALCKLWTQWKDTAEWVDRATGEVTRGVPWVAENFVGTYQAALRDAARAWANYFDSRTGQRAGRAIGKPRFKSKRTARKSFQVHGSSLRLVSAVKVNLPKIGTVTVMSDDSRHPAMARSRRRVPGQRHMGNRRRSRQLWQRLRHGQALAERAAEILSAAYADGNPDRVLEHLTALADERARARAVAAAEERLQKAKAAAAKAKPEKREKAQQRVAQAEEALRRAQAITANRKDGWSARKLAEVCRTGLITPVQAADLAEVFGLGEQQRAALAEAALQPRLVKATVTLGADGLWWLSLSAEVPVRVRTSPSRRQRERGATGLDLGVRNVVTSSKRLGGDQNLPNPRYLEQALVELRAAQKHLSRCTPGSARHAKAKARVGLIHADVARLREQHHHRLSTRLVRTFAGIAVEGYDLQELARRGSEGLPGEVRRRRNRALADTGAGMLRQQLQYKTARYGSHLVVAEPDAPTGRTCATCGQAKAKPVPPYHEVFACEACGRTRPRRLNTALALEAVAASSGSPHGGSDQPRGEDVRPAASRRGGQSSMKRAARSRPPGRGQTGTPGP

SEQ ID NO: 109 - protein, 495 aa, synthetic construct
MTTGDVEMRAYRFALDLTPTQEQQCRQHAGAARWAYNHALAAKFAALDARQATITTLVEQGVDPKVAATQAPKIPTKPAIQKALNATKGDNRTDLDGDCPWWHTVSTYAFQSAMIDVDTAWKNWLDSITGKRRGQRVSRPRFKTKHRSRDSFRIHHDVKNPSIRPDTGYRRIIVPRLGSLRVHDSTKKLCRALDRGAIIQSVTISRGGHRWYASILTKTPAAITAAPTRRQRKAGTVGVDVGVHHLAALSTGDIIDNPRHLDRARARLNKAQRKLSRTQRGSTRRRRAAAVVGRRHHEVAEQRATTLHTLTKRLATGWATVAIEDLNVLGMTRSARGTIDQPGTNVRAKAGLNRAILDAAPGELRHQLNYKARWYASTIAVCDRWYPSSQTCSTCGARTKLRLSQRAYRCAECGLDLDRDVNAAINIATYAVAVTPDTEETQNARRGRAPAPTSVGRRRQVTDAGRPHHHGAATSAEQSTDHPKTADQRPLTLVS

SEQ ID NO: 110 - protein, 499 aa, synthetic construct
MTTVEHDLRAYRLALDLTAEQTSAVRQHAGAARWAFNHALAAKLAALDARMSTIAAATAAGADPAAARASAPRIPTKPTIQKALNQIKGDDRTGVDGLCPWWNSVSTYTFQSAFADADQAWSNWMNSLTGKRAGRRVGRPRFKSKRRSRDSFRIHHDVKNPTIRPDTGYRRIIVPRLGSVRVHNSTKRLRRALDRGAVIQSVTISRAGHRWYAAVLVKAPRTAAAPTTRQRAAGRIGVDLGVHHLAALSDGTIIDNPRHHRHARARLTKAQRALARTQKGSNRRRRAAATVGRRHHELAERRATTTHTLTKQLTTRWATVAIEDLNVAGMTRSARGTIEAPGTNVAAKAGLNRAILDASFGELRRQLNYKTDWYGSTLAVCDRWAPTSQLCAECGERANLRLSQRTFRCPACTYGHETIVDRDVNAARNIAALAVAVAPGTEETQTARRAEPDPRPRGGNRSGPAVKREDRTLPGAATPVEQSTGHPKPADQRSLPLVS

SEQ ID NO: 111 - protein, 449 aa, synthetic construct
MVAVQRAFKFALDPTPTQLERLSRYAGASRMAYNFALGLKGQTHQQWRSLVDELIAAGLEEKEAHRRVQIKTPTKPTVQKIFNQLRGGPGEGPGGLAPWHHEVATWCFQSAWMDADQAWKNWLDSLTGKRAGHKVGYPRFKKKNRSRDSFRLHHDVREPTLRLESYRRLNLGKFGVVRLHESGKRMHRLVSSGAAVVKSVTVSRSGSRWYASVQCEIQTERPAPTRRQRVNGRVGMDVGVHYLAALSQPIQDYVLIDNPRHLSRASKRLARAQRALSRTQKGSMRRRKAAARVGKLHQEVAQQRATTLHWLSKRLATTFACVAIEDLNVAGMTRSARGTVEEPGSNVAAKAGLNSSILDAAPAELRRQLEYKTSWYGSQLAVLDRWFPSSKTCSACGWQNPNQTLADRVFSCAECGLRLDRDLNAARNIAAHAEVVSASGTGTPGRGGP

SEQ ID NO: 112 - protein, 726 aa, synthetic construct
MVRSRLRWMVTRHRRRTALVHGCCLLPWRWRSTLRCSSGRSEGAEGEAGTTPESPICDLDYEKNRGFLHYFSRHSHIQGGNLRRPNTPEQSSFLDATPQQKSHVSVLWLWANLFSKYSWLPQNTPLSCQGYPLWSLQEISKQVIPISRRRGGKAMAEKTSTDDGVLYRAYKFRLDPNQAQKTELMRCVGAARHTYNLLTTYNLQILHNKQEYRRTRAAEGADHETINGELKKLREKDPAYQILYKAGYKTGNEYVPGYRQLYLTPEIKRHRAASKAIAAGADPAVVWPETERYSEPWLHSINSRVLDSGLLNAGKAWKNYKESLMHLRAGARMGVPRRKRKGVSRDSFTVDRDPNNDEVGAYGTPYKKGTPEFARRTAQLKRRGIKTAPTIEDYRHVRLSHLGVIRTHNTTKPLVKAVRAGANVKSYTVSRAANRWYVSILVKLSRTPATPTRAQRSAGAVGVDLGVRYLAALSDEQAPQRFAQYPSLEFTDNGAPTLANPRWARTAEKRLVRLQRALARAQKGSNRRARLVRQIARHHHLVALRRESGLHQVSKRLATGYTLIGLEDLAVAGMTASAAGTIKAPGKNVRQKAGLNRSILDAAFGTLRRQLEYKASWYGSQVQIIDRFFASSQTCSACGARAKTKLGLHVRVFECAACGARIDRDVNAARNIRAEAVRMYEAQLAPGTGESLNGRGATDSDAAGSVVLGDVALDVSRPAASGGGSP

SEQ ID NO: 113 - protein, 494 aa, synthetic construct
MVRSVGEDLRAYRFALDLTPAQARAVAEHAGAARWAYNHALAVKFAALKQRQTVIAELVAAGVDAQVAARQAPRIPSKPQIQKDLNTAKGDSRTGVDGLCPWWWTVSTYAFQSAMADADRAWHNWISSVTGQRAGKRVGRPRFKSKHRCRDSFRIHHDVKQPTIRPDTSGYRRLIVPRLGSLRTHDSTKRLRRALDRGAVIQSVTITRGGHRWYASVLVKTLDAPAVGPTRAQRKAGIVGVDIGVHTLAALSTGELIANPRHLNSSRDRLIAAQRALARTVKGSNRRRRAARVLSRRHHELAERRATTLHQLTKRLATGWSVVAVEDLQVAGMTRSARGTVDNPGRNVRAKAGLNRAILDVAPSELRRQLTYKTGWYGSSLVVCDRFYPSTQTCSACGAKAKLTLADRVFRCAACGFGIDRDLNAARNIAAHAAVASGTRETINARRVDQRHPPQVGARRRPAMKREGHHACQTVVVTSAGQPADHPKTSVRST

SEQ ID NO: 114 - protein, 522 aa, synthetic construct
PPMTATDAATPPAGVLRAVRVILDPTPRQAAALASHAGAARAAFNYHLAEKMAAHRAYAAEVAYRTYIDFAGLDPNAAYAAAKKAVTAAKTHRIPGMPDSIKKMYADPDYGWLPDINRYAISSGMRAADTAWSNWLASLSGERSGPRVGYPRFKKKGRARSAFTLYHDVKAPSLRPDGPRRWRFPAKVGGSIRLKGNVRRLARRIARGTACVKNVTVAQSGGQWVASILVEDFAQLPAGPTRRQRAAGTVGVDVGVTHLAALSTGEHVPNPRHLRRAQARLVKAQRALSRTQWRVEGTGELVAVPVRGRRHVETSGRRKARARLAKAHAEVAQARATTLHALTKTLATSYAVVVVEDLAVKGMTAAPAARPDPASPGAFLPNGAAAKGGLNRAVLDAAFGEIRRQLTYKTSWYRSTLQVAPRFYPSSKTCSACGAVKAKLRLAERVFSCPACGHAEDRDINAAKNLAARSWTPAESGSLKTPAEPAHASRRRADNDAGRPWPPQAPVTVGEESPTRPPPSPA

SEQ ID NO: 115 - protein, 653 aa, synthetic construct
QAAHRDADVAWQRFLHGKSRRPRFKKKGKCTESFQVHGDDLGIPETTEAERIRFPEAVAALRPHGRRPVQQQTAQHITLPKIGPARVMSDDSLHPAMRRSRRRGSGVTPAHRPGRKLKAARARLEAAGRAYEHAAETMPEVPASTLHEVSAARDAAAKAEQAVAYARQRDAGHGRHMGNRRRFRQLHRHMRKSGENAARLGPLLRQVREDAGWTLDQAVTLLGTEADARAVAAVRARLAAAEDAADIAAAAAAEAVAAGDAEGAAAAEKDQRNARNRVKGALKRLGDLAAAKPGEKASRTDRWSAAKLKKMEATGVTLGLDQASVICSAYRLGGQLREQVTDLAAQARIVRATITLGADGLWWCSVGAEIPYAVRTAPSKRQEAHGTAGIDFGTARIMTVTGRRPVGAPSYYEKELAALGAAQRHAGRTVPGSGRHRKAKARAGLIHADVARLRADTLHRATTSLSRNFSVLSFEGFNVQQLMRDGSQGMPRQARGRRNRSLADAGIGMAREMLRQKGPRCGATVVTLGPDVITITGPRLEDARETDLPPDAKPNGTCSGCGQARTKPARPHEALYRCDACGRVRLRTLNSAENIRRWADEALTADPGCAISGPDQSRGGDEPATARAGRSPVKRAATTSSRPRRGEAGTPGG

SEQ ID NO: 116 - protein, 427 aa, synthetic construct
RHAHAARIAFNYALAAKIAAHEEWKRQVAALVESGVPEKDAREQTNANVRIPAKPDNQKAFNQVRGDSRKGIDGICPWFHEVSTYAFQSAFEDADAAWRNWLASQKGERKGQKVGYPKLKRRYRRRESFRLYGTIRLASYRRLYIPKIKEIRIHGTGKHLARLVERGDAVIQSVTISREGHRWYASILAKVTMDIPDQPTRSQRERGAVGVDLGVKTLAALSKPLDPANPASQLIPNSKPLEAAQRRLLKAQRALSRKQKGSRRWVKTKRRIAKLNHQIAVRRAAAIHQVTKQLATRFATVAIEDLNIRGMTSSARGTIDNPGRNVRAKAGLNRAILDAAPGEFRRQLEYKTAWYGSRLVVVDRWLPSSKTCSACGTVKEHLRLSDRVFECETCGARLDRDLNAARNIEAAATRVCSLPSPLMEGRR

SEQ ID NO: 117 - protein, 474 aa, synthetic construct
YNWGLQRIAEALDARQAEKTAGLKPTTRVPGHFDLCKAWTQWKDTTEWTDRDTGEVTVGVPWVARNFVGTYQAALRDAAAAWKRFFDSRAGRLAGRRVGRPRFKKKGRSRASFQVHGAQLQVVDAHHVKLPKVGVVKTHESTRKLLRRIRKGDTTCPTCKATGQVPGKDTPKKCPACKGSGRVPVARLVRGTVSQGSDGRWSIALTVEVVREIRTGPSDRQRAGGTIGVDLGVRSLVVTSAGEQFEHPRHLEAALDRLAAAQRALARCEKGSKRRAKAAARVARLHARVANLRRDATHKLTSRLVHSHERIGVEGWDVQQTAQRGSADVPKRVRRDRNRVLADANLGELRWQLQSKAAWYGCQVQVADRHAATGRTCSACGQVRAKPVPPFEEQFTCPACGWCGDRRWNTARVLAAVARGEHQQYDDASSGGESLNARGGDVRPAALRRGGRSSLKREARARPPGRGETGIPGP

SEQ ID NO: 118 - RNA, 29 nt, synthetic construct
  source 1..29: mol_type = other RNA
gtcggccccacgcgtgtagggagcgatcg

SEQ ID NO: 119 - RNA, 250 nt, synthetic construct
  source 1..250: mol_type = other RNA
gaacgcggcccggaacatcgaacgccacgcagtgctgatcgatcgaaacgtcgcctgcgataggcgggagacgctaaacgcccgtggagcatccataagaccaaccacctctcggggcggtaggcacgacgcatcgaagcgggaaggctccggcgctcggcctgagtcacctcagcagagtgatctgctgacgctcccaaccttgaataacgaaacggcaacgcctccatagcggtgcaggtcaataagg

SEQ ID NO: 120 - RNA, 279 nt, synthetic construct
  source 1..279: mol_type = other RNA
gaacgcggcccggaacatcgaacgccacgcagtgctgatcgatcgaaacgtcgcctgcgataggcgggagacgctaaacgcccgtggagcatccataagaccaaccacctctcggggcggtaggcacgacgcatcgaagcgggaaggctccggcgctcggcctgagtcacctcagcagagtgatctgctgacgctcccaaccttgaataacgaaacggcaacgcctccatagcggtgcaggtcaataagggtcggccccacgcgtgtagggagcgatcg

SEQ ID NO: 121 - DNA, 1518 bp, synthetic construct
  source 1..1518: mol_type = other DNA
atggtgcagacggagatcctgaaggcgtttcggtttgcgttggatccgacgtctgtgcaggttgctgccctttcccggcatgctggtgcggccaggtgggcgttcaaccatgctctcgcggccaaggtcggcgcgcatgagcggtggcgggcggaggtagccaagcttgtcggggacggtgttcctgaggagcaggctcgtaggcaggtgcgcgtcccggttccgatgaagccggcgatccagaaggcgttgaacgcggtcaagggtgactctcgcaagggcttggatggtgcgtgcccgtggtggcatgaggtcaacacttacgcgttccagtccgctttcatcgacgcggaccaggcgtggaagaactggttggactcgttgtcggggaagcgggtcggccgccgggtggggtacccgcggttcaagaagaaggggcgggcccgcgactcgtttcgcttgcaccacgacgtgaagaagccaagcatccggctggccgggtaccggcggttgcggctgccgaggatcggggaagtccggcttcatgactcggggaagcgtctggcacggctgatcgaccgaggtgacgcggtggtgcagtcggtgacggtgtcgcggggtggccatcgctggtatgcgtctgtgctgtgcaaggtcaccgtgcaggtaccggatcggccgtcacggcgccagcgggaacgaggcgctgttggggtggaccttggcgttaaggtcctcgcggctttgtccaagccactggtggtcgacgacccgtcgagtgccctggtgcggaatccgcagcatctgcggcaggccgagcggcgtctactgaaggctcagcgggcgttggcgcgtacacaaaaaggttcagcccgacgcgagaaggccaagcggcgagttggtcgcgcgcatcacgaggttgctgtgcgccggcatgctgcgctccatcagatcaccaagcgcctgaccaccggcttcgcggtcgtcgcgcttgaggatctgaacgtggccggtatgacaaggtcagcgcggggaacagtggcagcgccgggaaagaacgtgcggcagaaggcaggcctgaaccgcgtcatcctggactccgctccagccgagttgcgtcgccaggtgaactacaaggccacctggtatggatctgagctggcggtcgcagaccgctggttcccctcgagtaagacctgttcgggttgcggatggcaaaacccacacctgaagctgtccgacagggtgtttcgttgcacagactgcgggctggtgatggaccgggacatgaacgcggcccggaacatcgaacgccacgcagtgctgatcgatcgaaacgtcgcctgcgataggcgggagacgctaaacgcccgtggagcatccataagaccaaccacctctcggggcggtaggcacgacgcatcgaagcgggaaggctccggcgctcggcctgagtcacctcagcagagtgatctgctgacgctcccaaccttgaataacgaaacggcaacgcctcca

SEQ ID NO: 122 - DNA, 1518 bp, synthetic construct
  source 1..1518: mol_type = other DNA
atggtgcagacagagatcctgaaggcctttcggttcgccctcgatcctacttccgtccaggtggccgccctgagccggcacgccggggccgccaggtgggccttcaaccacgccctcgccgccaaggtgggggcccacgagcggtggcgggccgaggtggccaagctcgtgggcgatggcgtgcccgaggagcaggcccggcggcaggtccgggtccccgtgcctatgaagccagccatccagaaggccctgaacgccgtgaagggggattcccggaagggcctggatggggcctgcccatggtggcacgaggtgaacacctacgccttccagagcgcctttattgacgccgaccaggcatggaagaactggctcgacagcctgagcggcaagagagtggggaggagggtgggctacccccggtttaagaagaagggccgggctcgggatagctttagattgcaccacgatgtgaagaagcccagcatcaggctggctggctacagaaggctgaggctgcctaggattggcgaggtgaggctgcacgacagcggcaagcggctcgccaggctcattgacagaggcgacgccgtggtgcagtccgtgactgtgagtaggggcggacacaggtggtacgcctccgtgctctgcaaggtgacagtgcaggtgcccgatcggcccagcaggcggcagcgggagaggggcgccgtgggagtggacctgggggtgaaggtgctggccgccctgtccaagcccctggtcgtcgacgacccaagcagcgccctggtgagaaacccccagcacctgaggcaggctgagaggcggctgctcaaggcccagcgggccctggccaggacacagaagggcagcgccaggagagagaaggccaagcggcgggtggggagggcccatcacgaggtggccgtccggcggcacgccgccctgcaccagatcaccaagcggctgaccacagggttcgccgtggtggccctggaggatctgaacgtcgccggcatgaccaggtccgccagggggacagtggccgccccagggaagaacgtccggcagaaggccgggctgaaccgggtcatcctggacagcgcccctgccgagctgcggaggcaggtgaactacaaggccacctggtacgggagcgagctggccgtggccgacaggtggttcccctccagcaagacctgcagcgggtgcggctggcagaacccccacttgaagctctccgatagggtgtttaggtgcaccgactgcggcctggtcatggatagagatatgaacgccgctaggaacatcgagaggcacgctgtgttgattgataggaacgtggcctgcgaccggcgggagactttgaacgccaggggggccagcatccggcccaccacaagccggggggggcggcacgacgccagcaagagggaggggagcggggcccggccagagtccccccagcagtctgatctgctcacactccccacactgaacaacgaaaccgccacacccccc

SEQ ID NO: 123 - RNA, 279 nt, synthetic construct; identical to SEQ ID NO: 120
  source 1..279: mol_type = other RNA

SEQ ID NO: 124 - DNA, 8198 bp, synthetic construct
  source 1..8198: mol_type = other DNA
tttccataggctccgcccccctgacaagcatcacgaaatctgacgctcaaatcagtggtggcgaaacccgacaggactataaagataccaggcgtttccccctggcggctccctcgtgcgctctcctgttcctgcctttcggtttaccggtgtcattccgctgttatggccgcgtttgtctcattccacgcctgacactcagttccgggtaggcagttcgctccaagctggactgtatgcacgaaccccccgttcagtccgaccgctgcgccttatccggtaactatcgtcttgagtccaacccggaaagacatgcaaaagcaccactggcagcagccactggtaattgatttagaggagttagtcttgaagtcatgcgccggttaaggctaaactgaaaggacaagttttggtgactgcgctcctccaagccagttacctcggttcaaagagttggtagctcagagaaccttcgaaaaaccgccctgcaaggcggttttttcgttttcagagcaagagattacgcgcagaccaaaacgatctcaagaagatcatcttattaatcagataaaatatttctagatttcagtgcaatttatctcttcaaatgtagcacctgaagtcagccccatacgatataagttgtgacgtaaaatgagacgttgatcggcacgtaagaggttccaactttcaccataatgaaataagatcactaccgggcgtattttttgagttatcgagattttcaggagctaaggaagctaaaatggagaaaaaaatcactggatataccaccgttgatatatcccaatggcatcgtaaagaacattttgaggcatttcagtcagttgctcaatgtacctataaccagaccgttcagctgggtcatccaccggatcaattcccctgctcgcgcaggctgggtgccaagctctcgggtaacatcaaggcccgatccttggagcccttgccctcccgcacgatgatcgtgccgtgatcgaaatccagatccttgacccgcagttgcaaaccctcactgatccggctcacggtaactgatgccgtatttgcagtaccagcgtacggcccacagaatgatgtcacgctgaaaatgccggcctttgaatgggttcatgtgcagctccatcagcaaaaggggatgataagtttatcaccaccgactatttgcaacagtgccgttgatcgtgctatgatcgactgatgtcatcagcggtggagtgcaatgtcgtgcaatacgaatggcgaaaagccgagctcatcggtcagcttctcaaccttggggttacccccggcggtgtgctgctggtccacagctccttccgtagcgtccggcccctcgaagatgggccacttggactgatcgaggccctgcgtgctgcgctgggtccgggagggacgctcgtcatgccctcgtggtcaggtctggacgacgagccgttcgatcctgccacgtcgcccgttacaccggaccttggagttgtctctgacacattctggcgcctgccaaatgtaaagcgcagcgcccatccatttgcctttgcggcagcggggccacaggcagagcagatcatctctgatccattgcccctgccacctcactcgcctgcaagcccggtcgcccgtgtccatgaactcgatgggcaggtacttctcctcggcgtgggacacgatgccaacacgacgctgcatcttgccgagttgatggcaaaggttccctatggggtgccgagacactgcaccattcttcaggatggcaagttggtacgcgtcgattatctcgagaatgaccactgctgtgagcgctttgccttggcggacaggtggctcaaggagaagagccttcagaaggaaggtccagtcggtcatgcctttgctcggttgatccgctcccgcgacattgtggcgacagccctgggtcaactgggccgagatccgttgatcttcctgcatccgccagaggcgggatgcgaagaatgcgatgccgctcgccagtcgattggctgagctcatgagcggagaacgagatgacgttggaggggcaaggtcgcgctgattgctggggcaacacgtgaaaggcgagatcaccaaggtagtcggcaaataatgtctaacggtacccggggatcctctagagtcgacctgcataatgtgcctgtcaaatggacgaagcagggattctgcaaaccctatgctactccgtcaagccgtcaattgtctgattcgttaccaattatgacaacttgacggctacatcattcactttttcttcacaaccggcacggaactcgctcgggctggccccggtgcattttttaaatacccgcgagaaatagagttgatcgtcaaaaccaacattgcgaccgacggtggcgataggcatccgggtggtgctcaaaagcagcttcgcctggctgatacgttggtcctcgcgccagcttaagacgctaatccctaactgctggcggaaaagatgtgacagacgcgacggcgacaagcaaacatgctgtgcgacgctggcgatatcaaaattgctgtctgccaggtgatcgctgatgtactgacaagcctcgcgtacccgattatccatcggtggatggagcgactcgttaatcgcttccatgcgccgcagtaacaattgctcaagcagatttatcgccagcagctccgaatagcgcccttccccttgcccggcgttaatgatttgcccaaacaggtcgctgaaatgcggctggtgcgcttcatccgggcgaaagaaccccgtattggcaaatattgacggccagttaagccattcatgccagtaggcgcgcggacgaaagtaaacccactggtgataccattcgcgagcctccggatgacgaccgtagtgatgaatctctcctggcgggaacagcaaaatatcacccggtcggcaaacaaattctcgtccctgatttttcaccaccccctgaccgcgaatggtgagattgagaatataacctttcattcccagcggtcggtcgataaaaaaatcgagataaccgttggcctcaatcggcgttaaacccgccaccagatgggcattaaacgagtatcccggcagcaggggatcattttgcgcttcagccatacttttcatactcccgccattcagagaagaaaccaattgtccatattgcatcagacattgccgtcactgcgtcttttactggctcttctcgctaaccaaaccggtaaccccgcttattaaaagcattctgtaacaaagcgggaccaaagccatgacaaaaacgcgtaacaaaagtgtctataatcacggcagaaaagtccacattgattatttgcacggcgtcacactttgctatgccatagcatttttatccataagattagcggatcctacctgacgctttttatcgcaactctctactgtttctccatacccgtttttttgggctagcgaaaagatgtttcgtgaagccgtcgacgcttataaaaaatggatattaatactgaaactgagatcaagcaaaagcattcactaaccccctttcctgttttcctaatcagcccggcatttcgcgggcgatattttcacagctatttcaggagttcagccatgaacgcttattacattcaggatcgtcttgaggctcagagctgggcgcgtcactaccagcagctcgcccgtgaagagaaagaggcagaactggcagacgacatggaaaaaggcctgccccagcacctgtttgaatcgctatgcatcgatcatttgcaacgccacggggccagcaaaaaatccattacccgtgcgtttgatgacgatgttgagtttcaggagcgcatggcagaacacatccggtacatggttgaaaccattgctcaccaccaggttgatattgattcagaggtataaaacgaatgagtactgcactcgcaacgctggctgggaagctggctgaacgtgtcggcatggattctgtcgacccacaggaactgatcaccactcttcgccagacggcatttaaaggtgatgccagcgatgcgcagttcatcgcattactgatcgttgccaaccagtacggccttaatccgtggacgaaagaaatttacgcctttcctgataagcagaatggcatcgttccggtggtgggcgttgatggctggtcccgcatcatcaatgaaaaccagcagtttgatggcatggactttgagcaggacaatgaatcctgtacatgccggatttaccgcaaggaccgtaatcatccgatctgcgttaccgaatggatggatgaatgccgccgcgaaccattcaaaactcgcgaaggcagagaaatcacggggccgtggcagtcgcatcccaaacggatgttacgtcataaagccatgattcagtgtgcccgtctggccttcggatttgctggtatctatgacaaggatgaagccgagcgcattgtcgaaaatactgcatacactgcagaacgtcagccggaacgcgacatcactccggttaacgatgaaaccatgcaggagattaacactctgctgatcgccctggataaaacatgggatgacgacttattgccgctctgttcccagatatttcgccgcgacattcgtgcatcgtcagaactgacacaggccgaagcagtaaaagctcttggattcctgaaacagaaagccgcagagcagaaggtggcagcatgacaccggacattatcctgcagcgtaccgggatcgatgtgagagctgtcgaacagggggatgatgcgtggcacaaattacggctcggcgtcatcaccgcttcagaagttcacaacgtgatagcaaaaccccgctccggaaagaagtggcctgacatgaaaatgtcctacttccacaccctgcttgctgaggtttgcaccggtgtggctccggaagttaacgctaaagcactggcctggggaaaacagtacgagaacgacgccagaaccctgtttgaattcacttccggcgtgaatgttactgaatccccgatcatctatcgcgacgaaagtatgcgtaccgcctgctctcccgatggtttatgcagtgacggcaacggccttgaactgaaatgcccgtttacctcccgggatttcatgaagttccggctcggtggtttcgaggccataaagtcagcttacatggcccaggtgcagtacagcatgtgggtgacgcgaaaaaatgcctggtactttgccaactatgacccgcgtatgaagcgtgaaggcctgcattatgtcgtgattgagcgggatgaaaagtacatggcgagttttgacgagatcgtgccggagttcatcgaaaaaatggacgaggcactggctgaaattggttttgtatttggggagcaatggcgatgacgcatcctcacgataataagcttcctgctgaacatcaaaggcaagaaaacatctgttgtcaaagacagcatccttgaacaaggacaattaacagttaacaaataaaaacgcaaaagaaaatgccgatattgactaccggaagcagtgtgaccgtgtgcttctcaaatgcctgattcaggctgtctatgtgtgactgttgagctgtaacaagttgtctcaggtgttcaatttcatgttctagttgctttgttttactggtttcacctgttctattaggtgttacatgctgttcatctgttacattgtcgatctgttcatggtgaacagctttaaatgcaccaaaaactcgtaaaagctctgatgtatctatcttttttacaccgttttcatctgtgcatatagctatactgatttcgtcagactcacagtcaaacatgccggtcagttggcctggtgatggcgggatcgttgtatatttcttgacaccttttcggcaccgccctaaaattctgcgtcctcataatatatgaggcgatttattacgtgtttacgaagcaaaagctaaaaccaggagctatttaatggtgcagacggagatcctgaaggcgtttcggtttgcgttggatccgacgtctgtgcaggttgctgccctttcccggcatgctggtgcggccaggtgggcgttcaaccatgctctcgcggccaaggtcggcgcgcatgagcggtggcgggcggaggtagccaagcttgtcggggacggtgttcctgaggagcaggctcgtaggcaggtgcgcgtcccggttccgatgaagccggcgatccagaaggcgttgaacgcggtcaagggtgactctcgcaagggcttggatggtgcgtgcccgtggtggcatgaggtcaacacttacgcgttccagtccgctttcatcgacgcggaccaggcgtggaagaactggttggactcgttgtcggggaagcgggtcggccgccgggtggggtacccgcggttcaagaagaaggggcgggcccgcgactcgtttcgcttgcaccacgacgtgaagaagccaagcatccggctggccgggtaccggcggttgcggctgccgaggatcggggaagtccggcttcatgactcggggaagcgtctggcacggctgatcgaccgaggtgacgcggtggtgcagtcggtgacggtgtcgcggggtggccatcgctggtatgcgtctgtgctgtgcaaggtcaccgtgcaggtaccggatcggccgtcacggcgccagcgggaacgaggcgctgttggggtggaccttggcgttaaggtcctcgcggctttgtccaagccactggtggtcgacgacccgtcgagtgccctggtgcggaatccgcagcatctgcggcaggccgagcggcgtctactgaaggctcagcgggcgttggcgcgtacacaaaaaggttcagcccgacgcgagaaggccaagcggcgagttggtcgcgcgcatcacgaggttgctgtgcgccggcatgctgcgctccatcagatcaccaagcgcctgaccaccggcttcgcggtcgtcgcgcttgaggatctgaacgtggccggtatgacaaggtcagcgcggggaacagtggcagcgccgggaaagaacgtgcggcagaaggcaggcctgaaccgcgtcatcctggactccgctccagccgagttgcgtcgccaggtgaactacaaggccacctggtatggatctgagctggcggtcgcagaccgctggttcccctcgagtaagacctgttcgggttgcggatggcaaaacccacacctgaagctgtccgacagggtgtttcgttgcacagactgcgggctggtgatggaccgggacatgaacgcggcccggaacatcgaacgccacgcagtgctgatcgatcgaaacgtcgcctgcgataggcgggagacgctaaacgcccgtggagcatccataagaccaaccacctctcggggcggtaggcacgacgcatcgaagcgggaaggctccggcgctcggcctgagtcacctcagcagagtgatctgctgacgctcccaaccttgaataacgaaacggcaacgcctccatagcggtgcaggtcaataagggtcggccccacgcgtgtagggagcgatcgcgagaccattggtctcaggccggcatggtcccagcctcctcgctggcgccggctgggcaacatgcttcggcatggcgaatgggacccaattattgaacaccctaacgggtgtttttttgtttctggtctacctggctggttggcgtactgttgtggtaaatacccatatggacagttttccctttgatatgtaacggtgaacagttgttctacttttgtttgttagtcttgatgcttcactgatagatacaagagcgtcgggtgatgctgccaacttactgatttagtgtatgatggtgtttttgaggtgctccagtggcttctgtttctatcagctgtccctcctgttcagctactgacggggtggtgcgtaacggcaaaagcaccgccggacatcagcgctagcggagtgtatactggcttactatgttggcactgatgagggtgtcagtgaagtgcttcatgtggcaggagaaaaaaggctgcaccggtgcgtcagcagaatatgtgatacaggatatattccgcttcctcgctcactgactcgctacgctcggtcgttcgactgcggcgagcggaaatggcttacgaacggggcggagatttcctggaagatgccaggaagatacttaacagggaagtgagagggccgcggcaaagccgtt

SEQ ID NO: 125 - DNA, 1952 bp, synthetic construct
  source 1..1952: mol_type = other DNA
tttacaccgttttcatctgtgcatatagctatactgatttcgtcagactcacagtcaaacatgccggtcagttggcctggtgatggcgggatcgttgtatatttcttgacaccttttcggcaccgccctaaaattctgcgtcctcataatatatgaggcgatttattacgtgtttacgaagcaaaagctaaaaccaggagctatttaatggtgcagacggagatcctgaaggcgtttcggtttgcgttggatccgacgtctgtgcaggttgctgccctttcccggcatgctggtgcggccaggtgggcgttcaaccatgctctcgcggccaaggtcggcgcgcatgagcggtggcgggcggaggtagccaagcttgtcggggacggtgttcctgaggagcaggctcgtaggcaggtgcgcgtcccggttccgatgaagccggcgatccagaaggcgttgaacgcggtcaagggtgactctcgcaagggcttggatggtgcgtgcccgtggtggcatgaggtcaacacttacgcgttccagtccgctttcatcgacgcggaccaggcgtggaagaactggttggactcgttgtcggggaagcgggtcggccgccgggtggggtacccgcggttcaagaagaaggggcgggcccgcgactcgtttcgcttgcaccacgacgtgaagaagccaagcatccggctggccgggtaccggcggttgcggctgccgaggatcggggaagtccggcttcatgactcggggaagcgtctggcacggctgatcgaccgaggtgacgcggtggtgcagtcggtgacggtgtcgcggggtggccatcgctggtatgcgtctgtgctgtgcaaggtcaccgtgcaggtaccggatcggccgtcacggcgccagcgggaacgaggcgctgttggggtggaccttggcgttaaggtcctcgcggctttgtccaagccactggtggtcgacgacccgtcgagtgccctggtgcggaatccgcagcatctgcggcaggccgagcggcgtctactgaaggctcagcgggcgttggcgcgtacacaaaaaggttcagcccgacgcgagaaggccaagcggcgagttggtcgcgcgcatcacgaggttgctgtgcgccggcatgctgcgctccatcagatcaccaagcgcctgaccaccggcttcgcggtcgtcgcgcttgaggatctgaacgtggccggtatgacaaggtcagcgcggggaacagtggcagcgccgggaaagaacgtgcggcagaaggcaggcctgaaccgcgtcatcctggactccgctccagccgagttgcgtcgccaggtgaactacaaggccacctggtatggatctgagctggcggtcgcagaccgctggttcccctcgagtaagacctgttcgggttgcggatggcaaaacccacacctgaagctgtccgacagggtgtttcgttgcacagactgcgggctggtgatggaccgggacatgaacgcggcccggaacatcgaacgccacgcagtgctgatcgatcgaaacgtcgcctgcgataggcgggagacgctaaacgcccgtggagcatccataagaccaaccacctctcggggcggtaggcacgacgcatcgaagcgggaaggctccggcgctcggcctgagtcacctcagcagagtgatctgctgacgctcccaaccttgaataacgaaacggcaacgcctccatagcggtgcaggtcaataagggtcggccccacgcgtgtagggagcgatcgcgagaccattggtctcaggccggcatggtcccagcctcctcgctggcgccggctgggcaacatgcttcggcatggcgaatgggacccaattattgaacaccctaacgggtgtttttttgtttctggtctacctggctggttggcgtactgttgtggtaaatacccatatggacagtt

SEQ ID NO: 126 - DNA, 6296 bp, synthetic construct
  source 1..6296: mol_type = other DNA
gtggtaaatacccatatggacagttttccctttgatatgtaacggtgaacagttgttctacttttgtttgttagtcttgatgcttcactgatagatacaagagcgtcgggtgatgctgccaacttactgatttagtgtatgatggtgtttttgaggtgctccagtggcttctgtttctatcagctgtccctcctgttcagctactgacggggtggtgcgtaacggcaaaagcaccgccggacatcagcgctagcggagtgtatactggcttactatgttggcactgatgagggtgtcagtgaagtgcttcatgtggcaggagaaaaaaggctgcaccggtgcgtcagcagaatatgtgatacaggatatattccgcttcctcgctcactgactcgctacgctcggtcgttcgactgcggcgagcggaaatggcttacgaacggggcggagatttcctggaagatgccaggaagatacttaacagggaagtgagagggccgcggcaaagccgtttttccataggctccgcccccctgacaagcatcacgaaatctgacgctcaaatcagtggtggcgaaacccgacaggactataaagataccaggcgtttccccctggcggctccctcgtgcgctctcctgttcctgcctttcggtttaccggtgtcattccgctgttatggccgcgtttgtctcattccacgcctgacactcagttccgggtaggcagttcgctccaagctggactgtatgcacgaaccccccgttcagtccgaccgctgcgccttatccggtaactatcgtcttgagtccaacccggaaagacatgcaaaagcaccactggcagcagccactggtaattgatttagaggagttagtcttgaagtcatgcgccggttaaggctaaactgaaaggacaagttttggtgactgcgctcctccaagccagttacctcggttcaaagagttggtagctcagagaaccttcgaaaaaccgccctgcaaggcggttttttcgttttcagagcaagagattacgcgcagaccaaaacgatctcaagaagatcatcttattaatcagataaaatatttctagatttcagtgcaatttatctcttcaaatgtagcacctgaagtcagccccatacgatataagttgtgacgtaaaatgagacgttgatcggcacgtaagaggttccaactttcaccataatgaaataagatcactaccgggcgtattttttgagttatcgagattttcaggagctaaggaagctaaaatggagaaaaaaatcactggatataccaccgttgatatatcccaatggcatcgtaaagaacattttgaggcatttcagtcagttgctcaatgtacctataaccagaccgttcagctgggtcatccaccggatcaattcccctgctcgcgcaggctgggtgccaagctctcgggtaacatcaaggcccgatccttggagcccttgccctcccgcacgatgatcgtgccgtgatcgaaatccagatccttgacccgcagttgcaaaccctcactgatccggctcacggtaactgatgccgtatttgcagtaccagcgtacggcccacagaatgatgtcacgctgaaaatgccggcctttgaatgggttcatgtgcagctccatcagcaaaaggggatgataagtttatcaccaccgactatttgcaacagtgccgttgatcgtgctatgatcgactgatgtcatcagcggtggagtgcaatgtcgtgcaatacgaatggcgaaaagccgagctcatcggtcagcttctcaaccttggggttacccccggcggtgtgctgctggtccacagctccttccgtagcgtccggcccctcgaagatgggccacttggactgatcgaggccctgcgtgctgcgctgggtccgggagggacgctcgtcatgccctcgtggtcaggtctggacgacgagccgttcgatcctgccacgtcgcccgttacaccggaccttggagttgtctctgacacattctggcgcctgccaaatgtaaagcgcagcgcccatccatttgcctttgcggcagcggggccacaggcagagcagatcatctctgatccattgcccctgccacctcactcgcctgcaagcccggtcgcccgtgtccatgaactcgatgggcaggtacttctcctcggcgtgggacacgatgccaacacgacgctgcatcttgccgagttgatggcaaaggttccctatggggtgccgagacactgcaccattcttcaggatggcaagttggtacgcgtcgattatctcgagaatgaccactgctgtgagcgctttgccttggcggacaggtggctcaaggagaagagccttcagaaggaaggtccagtcggtcatgcctttgctcggttgatccgctcccgcgacattgtggcgacagccctgggtcaactgggccgagatccgttgatcttcctgcatccgccagaggcgggatgcgaagaatgcgatgccgctcgccagtcgattggctgagctcatgagcggagaacgagatgacgttggaggggcaaggtcgcgctgattgctggggcaacacgtgaaaggcgagatcaccaaggtagtcggcaaataatgtctaacggtacccggggatcctctagagtcgacctgcataatgtgcctgtcaaatggacgaagcagggattctgcaaaccctatgctactccgtcaagccgtcaattgtctgattcgttaccaattatgacaacttgacggctacatcattcactttttcttcacaaccggcacggaactcgctcgggctggccccggtgcattttttaaatacccgcgagaaatagagttgatcgtcaaaaccaacattgcgaccgacggtggcgataggcatccgggtggtgctcaaaagcagcttcgcctggctgatacgttggtcctcgcgccagcttaagacgctaatccctaactgctggcggaaaagatgtgacagacgcgacggcgacaagcaaacatgctgtgcgacgctggcgatatcaaaattgctgtctgccaggtgatcgctgatgtactgacaagcctcgcgtacccgattatccatcggtggatggagcgactcgttaatcgcttccatgcgccgcagtaacaattgctcaagcagatttatcgccagcagctccgaatagcgcccttccccttgcccggcgttaatgatttgcccaaacaggtcgctgaaatgcggctggtgcgcttcatccgggcgaaagaaccccgtattggcaaatattgacggccagttaagccattcatgccagtaggcgcgcggacgaaagtaaacccactggtgataccattcgcgagcctccggatgacgaccgtagtgatgaatctctcctggcgggaacagcaaaatatcacccggtcggcaaacaaattctcgtccctgatttttcaccaccccctgaccgcgaatggtgagattgagaatataacctttcattcccagcggtcggtcgataaaaaaatcgagataaccgttggcctcaatcggcgttaaacccgccaccagatgggcattaaacgagtatcccggcagcaggggatcattttgcgcttcagccatacttttcatactcccgccattcagagaagaaaccaattgtccatattgcatcagacattgccgtcactgcgtcttttactggctcttctcgctaaccaaaccggtaaccccgcttattaaaagcattctgtaacaaagcgggaccaaagccatgacaaaaacgcgtaacaaaagtgtctataatcacggcagaaaagtccacattgattatttgcacggcgtcacactttgctatgccatagcatttttatccataagattagcggatcctacctgacgctttttatcgcaactctctactgtttctccatacccgtttttttgggctagcgaaaagatgtttcgtgaagccgtcgacgcttataaaaaatggatattaatactgaaactgagatcaagcaaaagcattcactaaccccctttcctgttttcctaatcagcccggcatttcgcgggcgatattttcacagctatttcaggagttcagccatgaacgcttattacattcaggatcgtcttgaggctcagagctgggcgcgtcactaccagcagctcgcccgtgaagagaaagaggcagaactggcagacgacatggaaaaaggcctgccccagcacctgtttgaatcgctatgcatcgatcatttgcaacgccacggggccagcaaaaaatccattacccgtgcgtttgatgacgatgttgagtttcaggagcgcatggcagaacacatccggtacatggttgaaaccattgctcaccaccaggttgatattgattcagaggtataaaacgaatgagtactgcactcgcaacgctggctgggaagctggctgaacgtgtcggcatggattctgtcgacccacaggaactgatcaccactcttcgccagacggcatttaaaggtgatgccagcgatgcgcagttcatcgcattactgatcgttgccaaccagtacggccttaatccgtggacgaaagaaatttacgcctttcctgataagcagaatggcatcgttccggtggtgggcgttgatggctggtcccgcatcatcaatgaaaaccagcagtttgatggcatggactttgagcaggacaatgaatcctgtacatgccggatttaccgcaaggaccgtaatcatccgatctgcgttaccgaatggatggatgaatgccgccgcgaaccattcaaaactcgcgaaggcagagaaatcacggggccgtggcagtcgcatcccaaacggatgttacgtcataaagccatgattcagtgtgcccgtctggccttcggatttgctggtatctatgacaaggatgaagccgagcgcattgtcgaaaatactgcatacactgcagaacgtcagccggaacgcgacatcactccggttaacgatgaaaccatgcaggagattaacactctgctgatcgccctggataaaacatgggatgacgacttattgccgctctgttcccagatatttcgccgcgacattcgtgcatcgtcagaactgacacaggccgaagcagtaaaagctcttggattcctgaaacagaaagccgcagagcagaaggtggcagcatgacaccggacattatcctgcagcgtaccgggatcgatgtgagagctgtcgaacagggggatgatgcgtggcacaaattacggctcggcgtcatcaccgcttcagaagttcacaacgtgatagcaaaaccccgctccggaaagaagtggcctgacatgaaaatgtcctacttccacaccctgcttgctgaggtttgcaccggtgtggctccggaagttaacgctaaagcactggcctggggaaaacagtacgagaacgacgccagaaccctgtttgaattcacttccggcgtgaatgttactgaatccccgatcatctatcgcgacgaaagtatgcgtaccgcctgctctcccgatggtttatgcagtgacggcaacggccttgaactgaaatgcccgtttacctcccgggatttcatgaagttccggctcggtggtttcgaggccataaagtcagcttacatggcccaggtgcagtacagcatgtgggtgacgcgaaaaaatgcctggtactttgccaactatgacccgcgtatgaagcgtgaaggcctgcattatgtcgtgattgagcgggatgaaaagtacatggcgagttttgacgagatcgtgccggagttcatcgaaaaaatggacgaggcactggctgaaattggttttgtatttggggagcaatggcgatgacgcatcctcacgataataagcttcctgctgaacatcaaaggcaagaaaacatctgttgtcaaagacagcatccttgaacaaggacaattaacagttaacaaataaaaacgcaaaagaaaatgccgatattgactaccggaagcagtgtgaccgtgtgcttctcaaatgcctgattcaggctgtctatgtgtgactgttgagctgtaacaagttgtctcaggtgttcaatttcatgttctagttgctttgttttactggtttcacctgttctattaggtgttacatgctgttcatctgttacattgtcgatctgttcatggtgaacagctttaaatgcaccaaaaactcgtaaaagctctgatgtatctatcttttttacaccgttttcatctgtgcata

SEQ ID NO: 127 - DNA, 8201 bp, synthetic construct
  source 1..8201: mol_type = other DNA
tttccataggctccgcccccctgacaagcatcacgaaatctgacgctcaaatcagtggtggcgaaacccgacaggactataaagataccaggcgtttccccctggcggctccctcgtgcgctctcctgttcctgcctttcggtttaccggtgtcattccgctgttatggccgcgtttgtctcattccacgcctgacactcagttccgggtaggcagttcgctccaagctggactgtatgcacgaaccccccgttcagtccgaccgctgcgccttatccggtaactatcgtcttgagtccaacccggaaagacatgcaaaagcaccactggcagcagccactggtaattgatttagaggagttagtcttgaagtcatgcgccggttaaggctaaactgaaaggacaagttttggtgactgcgctcctccaagccagttacctcggttcaaagagttggtagctcagagaaccttcgaaaaaccgccctgcaaggcggttttttcgttttcagagcaagagattacgcgcagaccaaaacgatctcaagaagatcatcttattaatcagataaaatatttctagatttcagtgcaatttatctcttcaaatgtagcacctgaagtcagccccatacgatataagttgtgacgtaaaatgagacgttgatcggcacgtaagaggttccaactttcaccataatgaaataagatcactaccgggcgtattttttgagttatcgagattttcaggagctaaggaagctaaaatggagaaaaaaatcactggatataccaccgttgatatatcccaatggcatcgtaaagaacattttgaggcatttcagtcagttgctcaatgtacctataaccagaccgttcagctgggtcatccaccggatcaattcccctgctcgcgcaggctgggtgccaagctctcgggtaacatcaaggcccgatccttggagcccttgccctcccgcacgatgatcgtgccgtgatcgaaatccagatccttgacccgcagttgcaaaccctcactgatccggctcacggtaactgatgccgtatttgcagtaccagcgtacggcccacagaatgatgtcacgctgaaaatgccggcctttgaatgggttcatgtgcagctccatcagcaaaaggggatgataagtttatcaccaccgactatttgcaacagtgccgttgatcgtgctatgatcgactgatgtcatcagcggtggagtgcaatgtcgtgcaatacgaatggcgaaaagccgagctcatcggtcagcttctcaaccttggggttacccccggcggtgtgctgctggtccacagctccttccgtagcgtccggcccctcgaagatgggccacttggactgatcgaggccctgcgtgctgcgctgggtccgggagggacgctcgtcatgccctcgtggtcaggtctggacgacgagccgttcgatcctgccacgtcgcccgttacaccggaccttggagttgtctctgacacattctggcgcctgccaaatgtaaagcgcagcgcccatccatttgcctttgcggcagcggggccacaggcagagcagatcatctctgatccattgcccctgccacctcactcgcctgcaagcccggtcgcccgtgtccatgaactcgatgggcaggtacttctcctcggcgtgggacacgatgccaacacgacgctgcatcttgccgagttgatggcaaaggttccctatggggtgccgagacactgcaccattcttcaggatggcaagttggtacgcgtcgattatctcgagaatgaccactgctgtgagcgctttgccttggcggacaggtggctcaaggagaagagccttcagaaggaaggtccagtcggtcatgcctttgctcggttgatccgctcccgcgacattgtggcgacagccctgggtcaactgggccgagatccgttgatcttcctgcatccgccagaggcgggatgcgaagaatgcgatgccgctcgccagtcgattggctgagctcatgagcggagaacgagatgacgttggaggggcaaggtcgcgctgattgctggggcaacacgtgaaaggcgagatcaccaaggtagtcggcaaataatgtctaacggtacccggggatcctctagagtcgacctgcataatgtgcctgtcaaatggacgaagcagggattctgcaaaccctatgctactccgtcaagccgtcaattgtctgattcgttaccaattatgacaacttgacggctacatcattcactttttcttcacaaccggcacggaactcgctcgggctggccccggtgcattttttaaatacccgcgagaaatagagttgatcgtcaaaaccaacattgcgaccgacggtggcgataggcatccgggtggtgctcaaaagcagcttcgcctggctgatacgttggtcctcgcgccagcttaagacgctaatccctaactgctggcggaaaagatgtgacagacgcgacggcgacaagcaaacatgctgtgcgacgctggcgatatcaaaattgctgtctgccaggtgatcgctgatgtactgacaagcctcgcgtacccgattatccatcggtggatggagcgactcgttaatcgcttccatgcgccgcagtaacaattgctcaagcagatttatcgccagcagctccgaatagcgcccttccccttgcccggcgttaatgatttgcccaaacaggtcgctgaaatgcggctggtgcgcttcatccgggcgaaagaaccccgtattggcaaatattgacggccagttaagccattcatgccagtaggcgcgcggacgaaagtaaacccactggtgataccattcgcgagcctccggatgacgaccgtagtgatgaatctctcctggcgggaacagcaaaatatcacccggtcggcaaacaaattctcgtccctgatttttcaccaccccctgaccgcgaatggtgagattgagaatataacctttcattcccagcggtcggtcgataaaaaaatcgagataaccgttggcctcaatcggcgttaaacccgccaccagatgggcattaaacgagtatcccggcagcaggggatcattttgcgcttcagccatacttttcatactcccgccattcagagaagaaaccaattgtccatattgcatcagacattgccgtcactgcgtcttttactggctcttctcgctaaccaaaccggtaaccccgcttattaaaagcattctgtaacaaagcgggaccaaagccatgacaaaaacgcgtaacaaaagtgtctataatcacggcagaaaagtccacattgattatttgcacggcgtcacactttgctatgccatagcatttttatccataagattagcggatcctacctgacgctttttatcgcaactctctactgtttctccatacccgtttttttgggctagcgaaaagatgtttcgtgaagccgtcgacgcttataaaaaatggatattaatactgaaactgagatcaagcaaaagcattcactaaccccctttcctgttttcctaatcagcccggcatttcgcgggcgatattttcacagctatttcaggagttcagccatgaacgcttattacattcaggatcgtcttgaggctcagagctgggcgcgtcactaccagcagctcgcccgtgaagagaaagaggcagaactggcagacgacatggaaaaaggcctgccccagcacctgtttgaatcgctatgcatcgatcatttgcaacgccacggggccagcaaaaaatccattacccgtgcgtttgatgacgatgttgagtttcaggagcgcatggcagaacacatccggtacatggttgaaaccattgctcaccaccaggttgatattgattcagaggtataaaacgaatgagtactgcactcgcaacgctggctgggaagctggctgaacgtgtcggcatggattctgtcgacccacaggaactgatcaccactcttcgccagacggcatttaaaggtgatgccagcgatgcgcagttcatcgcattactgatcgttgccaaccagtacggccttaatccgtggacgaaagaaatttacgcctttcctgataagcagaatggcatcgttccggtggtgggcgttgatggctggtcccgcatcatcaatgaaaaccagcagtttgatggcatggactttgagcaggacaatgaatcctgtacatgccggatttaccgcaaggaccgtaatcatccgatctgcgttaccgaatggatggatgaatgccgccgcgaaccattcaaaactcgcgaaggcagagaaatcacggggccgtggcagtcgcatcccaaacggatgttacgtcataaagccatgattcagtgtgcccgtctggccttcggatttgctggtatctatgacaaggatgaagccgagcgcattgtcgaaaatactgcatacactgcagaacgtcagccggaacgcgacatcactccggttaacgatgaaaccatgcaggagattaacactctgctgatcgccctggataaaacatgggatgacgacttattgccgctctgttcccagatatttcgccgcgacattcgtgcatcgtcagaactgacacaggccgaagcagtaaaagctcttggattcctgaaacagaaagccgcagagcagaaggtggcagcatgacaccggacattatcctgcagcgtaccgggatcgatgtgagagctgtcgaacagggggatgatgcgtggcacaaattacggctcggcgtcatcaccgcttcagaagttcacaacgtgatagcaaaaccccgctccggaaagaagtggcctgacatgaaaatgtcctacttccacaccctgcttgctgaggtttgcaccggtgtggctccggaagttaacgctaaagcactggcctggggaaaacagtacgagaacgacgccagaaccctgtttgaattcacttccggcgtgaatgttactgaatccccgatcatctatcgcgacgaaagtatgcgtaccgcctgctctcccgatggtttatgcagtgacggcaacggccttgaactgaaatgcccgtttacctcccgggatttcatgaagttccggctcggtggtttcgaggccataaagtcagcttacatggcccaggtgcagtacagcatgtgggtgacgcgaaaaaatgcctggtactttgccaactatgacccgcgtatgaagcgtgaaggcctgcattatgtcgtgattgagcgggatgaaaagtacatggcgagttttgacgagatcgtgccggagttcatcgaaaaaatggacgaggcactggctgaaattggttttgtatttggggagcaatggcgatgacgcatcctcacgataataagcttcctgctgaacatcaaaggcaagaaaacatctgttgtcaaagacagcatccttgaacaaggacaattaacagttaacaaataaaaacgcaaaagaaaatgccgatattgactaccggaagcagtgtgaccgtgtgcttctcaaatgcctgattcaggctgtctatgtgtgactgttgagctgtaacaagttgtctcaggtgttcaatttcatgttctagttgctttgttttactggtttcacctgttctattaggtgttacatgctgttcatctgttacattgtcgatctgttcatggtgaacagctttaaatgcaccaaaaactcgtaaaagctctgatgtatctatcttttttacaccgttttcatctgtgcatatagctatactgatttcgtcagactcacagtcaaacatgccggtcagttggcctggtgatggcgggatcgttgtatatttcttgacaccttttcggcaccgccctaaaattctgcgtcctcataatatatgaggcgatttattacgtgtttacgaagcaaaagctaaaaccaggagctatttaatggtgcagacggagatcctgaaggcgtttcggtttgcgttggatccgacgtctgtgcaggttgctgccctttcccggcatgctggtgcggccaggtgggcgttcaaccatgctctcgcggccaaggtcggcgcgcatgagcggtggcgggcggaggtagccaagcttgtcggggacggtgttcctgaggagcaggctcgtaggcaggtgcgcgtcccggttccgatgaagccggcgatccagaaggcgttgaacgcggtcaagggtgactctcgcaagggcttggatggtgcgtgcccgtggtggcatgaggtcaacacttacgcgttccagtccgctttcatcgacgcggaccaggcgtggaagaactggttggactcgttgtcggggaagcgggtcggccgccgggtggggtacccgcggttcaagaagaaggggcgggcccgcgactcgtttcgcttgcaccacgacgtgaagaagccaagcatccggctggccgggtaccggcggttgcggctgccgaggatcggggaagtccggcttcatgactcggggaagcgtctggcacggctgatcgaccgaggtgacgcggtggtgcagtcggtgacggtgtcgcggggtggccatcgctggtatgcgtctgtgctgtgcaaggtcaccgtgcaggtaccggatcggccgtcacggcgccagcgggaacgaggcgctgttggggtggaccttggcgttaaggtcctcgcggctttgtccaagccactggtggtcgacgacccgtcgagtgccctggtgcggaatccgcagcatctgcggcaggccgagcggcgtctactgaaggctcagcgggcgttggcgcgtacacaaaaaggttcagcccgacgcgagaaggccaagcggcgagttggtcgcgcgcatcacgaggttgctgtgcgccggcatgctgcgctccatcagatcaccaagcgcctgaccaccggcttcgcggtcgtcgcgcttgaggatctgaacgtggccggtatgacaaggtcagcgcggggaacagtggcagcgccgggaaagaacgtgcggcagaaggcaggcctgaaccgcgtcatcctggactccgctccagccgagttgcgtcgccaggtgaactacaaggccacctggtatggatctgagctggcggtcgcagaccgctggttcccctcgagtaagacctgttcgggttgcggatggcaaaacccacacctgaagctgtccgacagggtgtttcgttgcacagactgcgggctggtgatggaccgggacatgaacgcggcccggaacatcgaacgccacgcagtgctgatcgatcgaaacgtcgcctgcgataggcgggagacgctaaacgcccgtggagcatccataagaccaaccacctctcggggcggtaggcacgacgcatcgaagcgggaaggctccggcgctcggcctgagtcacctcagcagagtgatctgctgacgctcccaaccttgaataacgaaacggcaacgcctccatagcggtgcaggtcaataagggtcggccccacgcgtgtagggagcgatcgtgtcctcttcctctttagcgggccggcatggtcccagcctcctcgctggcgccggctgggcaacatgcttcggcatggcgaatgggacccaattattgaacaccctaacgggtgtttttttgtttctggtctacctggctggttggcgtactgttgtggtaaatacccatatggacagttttccctttgatatgtaacggtgaacagttgttctacttttgtttgttagtcttgatgcttcactgatagatacaagagcgtcgggtgatgctgccaacttactgatttagtgtatgatggtgtttttgaggtgctccagtggcttctgtttctatcagctgtccctcctgttcagctactgacggggtggtgcgtaacggcaaaagcaccgccggacatcagcgctagcggagtgtatactggcttactatgttggcactgatgagggtgtcagtgaagtgcttcatgtggcaggagaaaaaaggctgcaccggtgcgtcagcagaatatgtgatacaggatatattccgcttcctcgctcactgactcgctacgctcggtcgttcgactgcggcgagcggaaatggcttacgaacggggcggagatttcctggaagatgccaggaagatacttaacagggaagtgagagggccgcggcaaagccgtt

SEQ ID NO: 128 - DNA, 24 bp, synthetic construct
  source 1..24: mol_type = other DNA
atcgtgtcctcttcctctttagcg

SEQ ID NO: 129 - DNA, 24 bp, synthetic construct
  source 1..24: mol_type = other DNA
ggcccgctaaagaggaagaggaca

SEQ ID NO: 130 - DNA, 2707 bp, synthetic construct
  source 1..2707: mol_type = other DNA
gaatcggccaacgcgcggggagaggcggtttgcgtattgggcgctcttccgcttcctcgctcactgactcgctgcgctcggtcgttcggctgcggcgagcggtatcagctcactcaaaggcggtaatacggttatccacagaatcaggggataacgcaggaaagaacatgtgagcaaaaggccagcaaaaggccaggaaccgtaaaaaggccgcgttgctggcgtttttccataggctccgcccccctgacgagcatcacaaaaatcgacgctcaagtcagaggtggcgaaacccgacaggactataaagataccaggcgtttccccctggaagctccctcgtgcgctctcctgttccgaccctgccgcttaccggatacctgtccgcctttctcccttcgggaagcgtggcgctttctcatagctcacgctgtaggtatctcagttcggtgtaggtcgttcgctccaagctgggctgtgtgcacgaaccccccgttcagcccgaccgctgcgccttatccggtaactatcgtcttgagtccaacccggtaagacacgacttatcgccactggcagcagccactggtaacaggattagcagagcgaggtatgtaggcggtgctacagagttcttgaagtggtggcctaactacggctacactagaagaacagtatttggtatctgcgctctgctgaagccagttaccttcggaaaaagagttggtagctcttgatccggcaaacaaaccaccgctggtagcggtggtttttttgtttgcaagcagcagattacgcgcagaaaaaaaggatctcaagaagatcctttgatcttttctacggggtctgacgctcagtggaacgaaaactcacgttaagggattttggtcatgagattatcaaaaaggatcttcacctagatccttttaaattaaaaatgaagttttaaatcaatctaaagtatatatgagtaaacttggtctgacagttaccaatgcttaatcagtgaggcacctatctcagcgatctgtctatttcgttcatccatagttgcctgactccccgtcgtgtagataactacgatacgggagggcttaccatctggccccagtgctgcaatgataccgcgagacccacgctcaccggctccagatttatcagcaataaaccagccagccggaagggccgagcgcagaagtggtcctgcaactttatccgcctccatccagtctattaattgttgccgggaagctagagtaagtagttcgccagttaatagtttgcgcaacgttgttgccattgctacaggcatcgtggtgtcacgctcgtcgtttggtatggcttcattcagctccggttcccaacgatcaaggcgagttacatgatcccccatgttgtgcaaaaaagcggttagctccttcggtcctccgatcgttgtcagaagtaagttggccgcagtgttatcactcatggttatggcagcactgcataattctcttactgtcatgccatccgtaagatgcttttctgtgactggtgagtactcaaccaagtcattctgagaatagtgtatgcggcgaccgagttgctcttgcccggcgtcaatacgggataataccgcgccacatagcagaactttaaaagtgctcatcattggaaaacgttcttcggggcgaaaactctcaaggatcttaccgctgttgagatccagttcgatgtaacccactcgtgcacccaactgatcttcagcatcttttactttcaccagcgtttctgggtgagcaaaaacaggaaggcaaaatgccgcaaaaaagggaataagggcgacacggaaatgttgaatactcatactcttcctttttcaatattattgaagcatttatcagggttattgtctcatgagcggatacatatttgaatgtatttagaaaaataaacaaataggggttccgcgcacatttccccgaaaagtgccacctgacgtctaagaaaccattattatcatgacattaacctataaaaataggcgtatcacgaggccctttcgtctcgcgcgtttcggtgatgacggtgaaaacctctgacacatgcagctcccggagacggtcacagcttgtctgtaagcggatgccgggagcagacaagcccgtcagggcgcgtcagcgggtgttggcgggtgtcggggctggcttaactatgcggcatcagagcagattgtactgagagtgcaccatatgcggtgtgaaataccgcacagatgcgtaaggagaaaataccgcatcaggcgccattcgccattcaggctgcgcaactgttgggaagggcgatcggtgcgggcctcttcgctattacgccagctggcgaaagggggatgtgctgcaaggcgattaagttgggtaacgccagggttttcccagtcacgacgttgtaaaacgacggccagtgaattcgacaaattctaaacgctaaagaggaagaggacannnnnnagttgacccaacgtcgccggcgtgcacaagcttggcgtaatcatggtcatagctgtttcctgtgtgaaattgttatccgctcacaattccacacaacatacgagccggaagcataaagtgtaaagcctggggtgcctaatgagtgagctaactcacattaattgcgttgcgctcactgcccgctttccagtcgggaaacctgtcgtgccagctgcattaat

SEQ ID NO: 131 - DNA, 46 bp, synthetic construct
  source 1..46: mol_type = other DNA
ccggcgacgttgggtcaactnnnnnntgtcctcttcctctttagcg

SEQ ID NO: 132 - DNA, 30 bp, synthetic construct
  source 1..30: mol_type = other DNA
agttgacccaacgtcgccggcgtgcacaag

SEQ ID NO: 133 - DNA, 51 bp, synthetic construct
  source 1..51: mol_type = other DNA
gtgactggagttcagacgtgtgctcttccgatctcaggaaacagctatgac

SEQ ID NO: 134 - DNA, 43 bp, synthetic construct
  source 1..43: mol_type = other DNA
gttcagagttctacagtccgacgatcgtaaaacgacggccagt

SEQ ID NO: 135 - DNA, 66 bp, synthetic construct
  source 1..66: mol_type = other DNA
caagcagaagacggcatacgagatcggttcaagtgactggagttcagacgtgtgctcttccgatct

SEQ ID NO: 136 - DNA, 63 bp, synthetic construct
  source 1..63: mol_type = other DNA
aatgatacggcgaccaccgagatctacacgctggattgttcagagttctacagtccgacgatc

SEQ ID NO: 137 - DNA, 2053 bp, synthetic construct
  source 1..2053: mol_type = other DNA
tagctatactgatttcgtcagactcacagtcaaacatgccggtcagttggcctggtgatggcgggatcgttgtatatttcttgacaccttttcggcaccgccctaaaattctgcgtcctcataatatatgaggcgatttattacgtgtttacgaagcaaaagctaaaaccaggagctatttaatgacaagcaccacgctcgcaccagaagaacccctcatggtgttccgcggcgcgcggtttcgtctcgatccaaccggggaacaacaaggcatattaagccagcaagcaggtgcagcgcgcgttgcatataacatgatgtgcaccctcaacaaagacatcctcgaagcccgaagtcagctgtattcaacgctgatcaaagatggaaaaactaaagataaggccaaaaaagaacttaaagctgccgcaaaggaagatccttcactagctattgtctgggcgcgtgatttcgataaaaactacatcaccccagaacgcaatcgccataagcacgccgcccaacgaattgctgcaggtgaaaacccagtcgatgtatggaacccagacgaagaacgtttcaacgaaccctggctccacaccgcaaaccgccgagtgcttagatcagggcaaaaacaatacgagcaagcactcgataacttctttaagtctcagaacggatccagggctgggcaaaaaatgggcaagcctcgttttaaaactaaaattcgctccacagactcattcaccatcgacgccgttgatgtctcctcatcgaccacactcatcagagatataggccccaaagaccatgcccgatacaaaaccggtgaagcctcaacaggaatcattgcagactaccgccacgtcagactctcccacctaggcacatttcgcgtctttggatccactaaagccctggtccgacaactcgatagaggcgggcggattaaatcctgcacagtgtctcgatccgctgatcgctggtacgtctcattccttgtcgaactccccatcgagatagcacgctctacacctacgaaaaagcaatataaagcaggtgcagtcgggattgatctgggagtaaaaagcctcgctgccctatctaccggcgagattatccccaacccacgtttcttacgcaccgcagataaaaagatcaagaagcttcaacgcaaaatcgctcggtgccaaaaaggatcaaaaaattccatccggttaaagcgacgtcttgcacgctgccaccatgaactcgcgctgcaacgtgcagggtatctgaacgaactcactagcatgctggcatcgagtttttccgcgatcgcactagaagatctcaacgtggcggggatgacatcatccgcgcgcggaaccgtggaaaatccgggtaaaaatgtgaaacaaaaagcagggttaaacaggtcaattctcgacatctcaccagggcgtatccgcacgttgttggagtataaatgcactgatcgcggtgttgagctgcaggttattgatcgttttttcccctcatcgcagttatgttcgtcctgtggatcaaaaaccacgatccccttggcgcagcgtatctatcactgtgatgtgtgtggtggtgtcattgatcgtgatgtcaatgccgctatcaatattgtctatgaagccaagcgattggtggaacaaaaatgtagtgaacactcggctccggagggggcagaggataaacggccgtggagtgtacatctcccatcaacgcagtatgttgatggactgtatacgaggaagcggcaaggccccagcggtcatagcagttgagtaattggctgctctttatcgtgttgtgttgaaggaaaatcgtggtaagtggtgatggattcgctggtcaggaagtgttcttcccacgcacacgaggaagatccccgagaccattggtctcaggccggcatggtcccagcctcctcgctggcgccggctgggcaacatgcttcggcatggcgaatgggacccaattattgaacaccctaacgggtgtttttttgtttctggtctacctggctggttggcgtactgtt

SEQ ID NO: 138 - DNA, 2074 bp, synthetic construct
  source 1..2074: mol_type = other DNA
tagctatactgatttcgtcagactcacagtcaaacatgccggtcagttggcctggtgatggcgggatcgttgtatatttcttgacaccttttcggcaccgccctaaaattctgcgtcctcataatatatgaggcgatttattacgtgtttacgaagcaaaagctaaaaccaggagctatttaatggctactactgataagaaggatgaagaaaaccttcgagcgtataagttccgtcttgacccaaatcaagctcagactaccgctctctatcaggcagtcggtgcggctcggtatacatacaatatgctcaccgcatataacttggaagttaatagacttcgtgatgattattggaagagacgccatgatgaggatatctccgacgcagatattaaaaaagaacttaatgcgcttgccaaagaagataaacgctataagcagttaaattacggagcatttggaacccaatatttgactcctgagaaaaaacgtcatgaacaagccgaacaccgtattgaaaatggcgaagatccgtcagttgtgtggaaccaagagacggagcggtcggctaatccgtggcttcataccgcaaatcagcgagtgctggtgagtggtctgcaaaatgcgagtgatgcttgggacaatttctgggcttcccgtacgggtaaacgtgctgggcgtctggtgggtacaccgcgtttcaagaagaaaggtgtttcgcgggattcttttacggttccggcaccggaaaagatgggcgcttacggcaccgcgtatctgcgaggggaacctgcctacaagcaggggcgacgtaagattacagactatcgtcatgtgcggttatcttatctaggtactatacgcacctttaactcgaccaagccactagtgaaagcggttgtagctggcgccaagattcgtagctatacggtctctcggaatgctgaccgctggtatgtatctttcttagtgaagttttcggagcctatacgtcgttctgcaacaaagcgtgctcgtgctgctggttctgtaggtgttgatttaggagttaagtacctggcgtcactttcagattccgaggctccacaacgcttcccgaatctaaaatttgtcgaagggctgcctagccttgagaacccgcgctggagtgaggcaagctcgcgacggctgcataagttacagcgtgctctagcacgttctcagaaagggtcgaatcgacgttctcgtttagtgaagcagatagctcggttgcaccatatgacggcgttgcgtcgtgagtcgaatctgcatcagctgacgaaaaaacttgctaccgagtataccctggtaggatttgaagatttgaatgtttccggtatgaccgcctctgcgaaggggacggttgagaatccggggaagaatgttgcccaaaagtctgggttgaaccgggtagttttggatgcggcattcggcgtgttccgtaaccagctggagtataaggctgtctggtatggttctgcgtttgagaaggttgaccgttattttgcttcgtcgcagacgtgttcggagtgtgggaggaaagcgaaaaccaagctgactctgcgcgaccgtgtcttcgactgtgcgtactgtgggaatatgatggatcgtgatcttaacgcggccgtcaatatttgccgtgaggcgcagaggctttttgacgaaaaactcgcctcagaagatagggagagtctaaacggacgtggaagtcgaggcgctcttcggggtgctgagactgtggaagcgtcaagaccacctgcgagtcatcgtagagggtcaccgtagatgagtaatcatctgcccatctattgcattatgcacgcaactgaatagagttttgcagacatgcgggcgttatacctagtcagcaagtgtctgccccgcgtgtgcatgggtggttcccgagaccattggtctcaggccggcatggtcccagcctcctcgctggcgccggctgggcaacatgcttcggcatggcgaatgggacccaattattgaacaccctaacgggtgtttttttgtttctggtctacctggctggttggcgtactgtt

SEQ ID NO: 139 - DNA, 2074 bp, synthetic construct
  source 1..2074: mol_type = other DNA
tagctatactgatttcgtcagactcacagtcaaacatgccggtcagttggcctggtgatggcgggatcgttgtatatttcttgacaccttttcggcaccgccctaaaattctgcgtcctcataatatatgaggcgatttattacgtgtttacgaagcaaaagctaaaaccaggagctatttaatgcccctgaacggatggacgatgctggcgcaggaggaggtgcgagcgatgacgactaccacgggtaccgacctggccccgaggctgcgcgcgttcaagcaccgcctggaccccaaccccgcccaggccaccctgctggcccagtacgccggcgccgcgcgcgtggcctacaacatgctcatcgcccacaaccgggccgccctggccgccggtgccgcccgtcgcaccgagctggccgagagcgggctggccggccccgagctggccgcgcgcatgaaggccgagcgcgccgccgaccccaccctccgcgtggccagctaccagtcgtactccacggcccacctgactccgctgatccgccgccaccgtgaggctgccgccgcgatcgccgccggtgccgacccggccgaggcatggaccgacgagcgatacgccgagccctggatgcacaccgtgccccgccgcgtcctggtctccggcctccagaacgccgcgaaggccaccgagaactggatggcctccgcctccggcacgcgcgccggcgcgcgcgtcggcctgccgcggttcaagaagaagggccggtcccgggacagcttcaccatccccgcccccgaggtcatcggcgccgcgggcaccccctacaagcgcggcgagcaccgccgcggggtgatcaccgaccaccggcacctgcgcctggcctccctggggaccatccgcacctacgacaagaccagccgcctggtccgcgcctgccgccgcggcgcccagatccggtccatgaccatctcccaggctggcggacggtggtacgcctcgatcctcgttgccgaccccacccccatccggaccgggcccagccgtcgccagcgcgccaacggcgccgtcggcgtggacctgggcgtcaagcacctggccgccctctccaccggcgaggtcatcgacaacggccgccccggtgcccgccaggccgcccgcctgacccgtctccagcgcgcctacgcccgcacccagcccggctcgaaccgccgcgagcgcgtgcgccggcagatcgcggcactccatcacgggatcgcactacgtcgggcggggctgctgcatcaggtgtccacgagactggcgatggacttcgcggtggtcgccctggaggacctgaacgtggcggggatgacccgttcggcccgcgggacgctcgaggcgccgggtaggaacgtggccgccaagtccgggttgaaccgggcgatcctggatgccgggctggggatgctgcgccggcagctggactacaagacctcctgggcagggtcccaggtgaagatgatcgaccgattcgcgccctcctcgaaggcgtgctcgcgctgcgggacagtcaaatccacgctgtccctggccgagcggaccttcgagtgcgaggcctgccacctggtgatcgaccgcgacgtgaacgccgcgatcaacatccgggcgtgggctgtgcaggaggagcgtagagcaggggtcgagctcgcccgaggccgtcgggagagtcgaaacggacgtggagctgctgtctcgggcccgccatctggcggggccgcggggcaggggcgtggaagcgtcaagcccgcaccccagggtgtgggcatgtccagccgggcaactggctggtcatcccaacccccctcaaccgaaggggaaagcgcagagcgcggagcatccgccctggccaggtagtggaagccccgcgcacgcagggatgagcctcgagaccattggtctcaggccggcatggtcccagcctcctcgctggcgccggctgggcaacatgcttcggcatggcgaatgggacccaattattgaacaccctaacgggtgtttttttgtttctggtctacctggctggttggcgtactgtt

SEQ ID NO: 140 - DNA, 8349 bp, synthetic construct
  source 1..8349: mol_type = other DNA
tggctggttggcgtactgttgtggtaaatacccatatggacagttttccctttgatatgtaacggtgaacagttgttctacttttgtttgttagtcttgatgcttcactgatagatacaagagcgtcgggtgatgctgccaacttactgatttagtgtatgatggtgtttttgaggtgctccagtggcttctgtttctatcagctgtccctcctgttcagctactgacggggtggtgcgtaacggcaaaagcaccgccggacatcagcgctagcggagtgtatactggcttactatgttggcactgatgagggtgtcagtgaagtgcttcatgtggcaggagaaaaaaggctgcaccggtgcgtcagcagaatatgtgatacaggatatattccgcttcctcgctcactgactcgctacgctcggtcgttcgactgcggcgagcggaaatggcttacgaacggggcggagatttcctggaagatgccaggaagatacttaacagggaagtgagagggccgcggcaaagccgtttttccataggctccgcccccctgacaagcatcacgaaatctgacgctcaaatcagtggtggcgaaacccgacaggactataaagataccaggcgtttccccctggcggctccctcgtgcgctctcctgttcctgcctttcggtttaccggtgtcattccgctgttatggccgcgtttgtctcattccacgcctgacactcagttccgggtaggcagttcgctccaagctggactgtatgcacgaaccccccgttcagtccgaccgctgcgccttatccggtaactatcgtcttgagtccaacccggaaagacatgcaaaagcaccactggcagcagccactggtaattgatttagaggagttagtcttgaagtcatgcgccggttaaggctaaactgaaaggacaagttttggtgactgcgctcctccaagccagttacctcggttcaaagagttggtagctcagagaaccttcgaaaaaccgccctgcaaggcggttttttcgttttcagagcaagagattacgcgcagaccaaaacgatctcaagaagatcatcttattaatcagataaaatatttctagatttcagtgcaatttatctcttcaaatgtagcacctgaagtcagccccatacgatataagttgtgacgtaaaatgagacgttgatcggcacgtaagaggttccaactttcaccataatgaaataagatcactaccgggcgtattttttgagttatcgagattttcaggagctaaggaagctaaaatggagaaaaaaatcactggatataccaccgttgatatatcccaatggcatcgtaaagaacattttgaggcatttcagtcagttgctcaatgtacctataaccagaccgttcagctgggtcatccaccggatcaattcccctgctcgcgcaggctgggtgccaagctctcgggtaacatcaaggcccgatccttggagcccttgccctcccgcacgatgatcgtgccgtgatcgaaatccagatccttgacccgcagttgcaaaccctcactgatccggctcacggtaactgatgccgtatttgcagtaccagcgtacggcccacagaatgatgtcacgctgaaaatgccggcctttgaatgggttcatgtgcagctccatcagcaaaaggggatgataagtttatcaccaccgactatttgcaacagtgccgttgatcgtgctatgatcgactgatgtcatcagcggtggagtgcaatgtcgtgcaatacgaatggcgaaaagccgagctcatcggtcagcttctcaaccttggggttacccccggcggtgtgctgctggtccacagctccttccgtagcgtccggcccctcgaagatgggccacttggactgatcgaggccctgcgtgctgcgctgggtccgggagggacgctcgtcatgccctcgtggtcaggtctggacgacgagccgttcgatcctgccacgtcgcccgttacaccggaccttggagttgtctctgacacattctggcgcctgccaaatgtaaagcgcagcgcccatccatttgcctttgcggcagcggggccacaggcagagcagatcatctctgatccattgcccctgccacctcactcgcctgcaagcccggtcgcccgtgtccatgaactcgatgggcaggtacttctcctcggcgtgggacacgatgccaacacgacgctgcatcttgccgagttgatggcaaaggttccctatggggtgccgagacactgcaccattcttcaggatggcaagttggtacgcgtcgattatctcgagaatgaccactgctgtgagcgctttgccttggcggacaggtggctcaaggagaagagccttcagaaggaaggtccagtcggtcatgcctttgctcggttgatccgctcccgcgacattgtggcgacagccctgggtcaactgggccgagatccgttgatcttcctgcatccgccagaggcgggatgcgaagaatgcgatgccgctcgccagtcgattggctgagctcatgagcggagaacgagatgacgttggaggggcaaggtcgcgctgattgctggggcaacacgtgaaaggcgagatcaccaaggtagtcggcaaataatgtctaacggtacccggggatcctctagagtcgacctgcataatgtgcctgtcaaatggacgaagcagggattctgcaaaccctatgctactccgtcaagccgtcaattgtctgattcgttaccaattatgacaacttgacggctacatcattcactttttcttcacaaccggcacggaactcgctcgggctggccccggtgcattttttaaatacccgcgagaaatagagttgatcgtcaaaaccaacattgcgaccgacggtggcgataggcatccgggtggtgctcaaaagcagcttcgcctggctgatacgttggtcctcgcgccagcttaagacgctaatccctaactgctggcggaaaagatgtgacagacgcgacggcgacaagcaaacatgctgtgcgacgctggcgatatcaaaattgctgtctgccaggtgatcgctgatgtactgacaagcctcgcgtacccgattatccatcggtggatggagcgactcgttaatcgcttccatgcgccgcagtaacaattgctcaagcagatttatcgccagcagctccgaatagcgcccttccccttgcccggcgttaatgatttgcccaaacaggtcgctgaaatgcggctggtgcgcttcatccgggcgaaagaaccccgtattggcaaatattgacggccagttaagccattcatgccagtaggcgcgcggacgaaagtaaacccactggtgataccattcgcgagcctccggatgacgaccgtagtgatgaatctctcctggcgggaacagcaaaatatcacccggtcggcaaacaaattctcgtccctgatttttcaccaccccctgaccgcgaatggtgagattgagaatataacctttcattcccagcggtcggtcgataaaaaaatcgagataaccgttggcctcaatcggcgttaaacccgccaccagatgggcattaaacgagtatcccggcagcaggggatcattttgcgcttcagccatacttttcatactcccgccattcagagaagaaaccaattgtccatattgcatcagacattgccgtcactgcgtcttttactggctcttctcgctaaccaaaccggtaaccccgcttattaaaagcattctgtaacaaagcgggaccaaagccatgacaaaaacgcgtaacaaaagtgtctataatcacggcagaaaagtccacattgattatttgcacggcgtcacactttgctatgccatagcatttttatccataagattagcggatcctacctgacgctttttatcgcaactctctactgtttctccatacccgtttttttgggctagcgaaaagatgtttcgtgaagccgtcgacgcttataaaaaatggatattaatactgaaactgagatcaagcaaaagcattcactaaccccctttcctgttttcctaatcagcccggcatttcgcgggcgatattttcacagctatttcaggagttcagccatgaacgcttattacattcaggatcgtcttgaggctcagagctgggcgcgtcactaccagcagctcgcccgtgaagagaaagaggcagaactggcagacgacatggaaaaaggcctgccccagcacctgtttgaatcgctatgcatcgatcatttgcaacgccacggggccagcaaaaaatccattacccgtgcgtttgatgacgatgttgagtttcaggagcgcatggcagaacacatccggtacatggttgaaaccattgctcaccaccaggttgatattgattcagaggtataaaacgaatgagtactgcactcgcaacgctggctgggaagctggctgaacgtgtcggcatggattctgtcgacccacaggaactgatcaccactcttcgccagacggcatttaaaggtgatgccagcgatgcgcagttcatcgcattactgatcgttgccaaccagtacggccttaatccgtggacgaaagaaatttacgcctttcctgataagcagaatggcatcgttccggtggtgggcgttgatggctggtcccgcatcatcaatgaaaaccagcagtttgatggcatggactttgagcaggacaatgaatcctgtacatgccggatttaccgcaaggaccgtaatcatccgatctgcgttaccgaatggatggatgaatgccgccgcgaaccattcaaaactcgcgaaggcagagaaatcacggggccgtggcagtcgcatcccaaacggatgttacgtcataaagccatgattcagtgtgcccgtctggccttcggatttgctggtatctatgacaaggatgaagccgagcgcattgtcgaaaatactgcatacactgcagaacgtcagccggaacgcgacatcactccggttaacgatgaaaccatgcaggagattaacactctgctgatcgccctggataaaacatgggatgacgacttattgccgctctgttcccagatatttcgccgcgacattcgtgcatcgtcagaactgacacaggccgaagcagtaaaagctcttggattcctgaaacagaaagccgcagagcagaaggtggcagcatgacaccggacattatcctgcagcgtaccgggatcgatgtgagagctgtcgaacagggggatgatgcgtggcacaaattacggctcggcgtcatcaccgcttcagaagttcacaacgtgatagcaaaaccccgctccggaaagaagtggcctgacatgaaaatgtcctacttccacaccctgcttgctgaggtttgcaccggtgtggctccggaagttaacgctaaagcactggcctggggaaaacagtacgagaacgacgccagaaccctgtttgaattcacttccggcgtgaatgttactgaatccccgatcatctatcgcgacgaaagtatgcgtaccgcctgctctcccgatggtttatgcagtgacggcaacggccttgaactgaaatgcccgtttacctcccgggatttcatgaagttccggctcggtggtttcgaggccataaagtcagcttacatggcccaggtgcagtacagcatgtgggtgacgcgaaaaaatgcctggtactttgccaactatgacccgcgtatgaagcgtgaaggcctgcattatgtcgtgattgagcgggatgaaaagtacatggcgagttttgacgagatcgtgccggagttcatcgaaaaaatggacgaggcactggctgaaattggttttgtatttggggagcaatggcgatgacgcatcctcacgataataagcttcctgctgaacatcaaaggcaagaaaacatctgttgtcaaagacagcatccttgaacaaggacaattaacagttaacaaataaaaacgcaaaagaaaatgccgatattgactaccggaagcagtgtgaccgtgtgcttctcaaatgcctgattcaggctgtctatgtgtgactgttgagctgtaacaagttgtctcaggtgttcaatttcatgttctagttgctttgttttactggtttcacctgttctattaggtgttacatgctgttcatctgttacattgtcgatctgttcatggtgaacagctttaaatgcaccaaaaactcgtaaaagctctgatgtatctatcttttttacaccgttttcatctgtgcatatagctatactgatttcgtcagactcacagtcaaacatgccggtcagttggcctggtgatggcgggatcgttgtatatttcttgacaccttttcggcaccgccctaaaattctgcgtcctcataatatatgaggcgatttattacgtgtttacgaagcaaaagctaaaaccaggagctatttaatgacaagcaccacgctcgcaccagaagaacccctcatggtgttccgcggcgcgcggtttcgtctcgatccaaccggggaacaacaaggcatattaagccagcaagcaggtgcagcgcgcgttgcatataacatgatgtgcaccctcaacaaagacatcctcgaagcccgaagtcagctgtattcaacgctgatcaaagatggaaaaactaaagataaggccaaaaaagaacttaaagctgccgcaaaggaagatccttcactagctattgtctgggcgcgtgatttcgataaaaactacatcaccccagaacgcaatcgccataagcacgccgcccaacgaattgctgcaggtgaaaacccagtcgatgtatggaacccagacgaagaacgtttcaacgaaccctggctccacaccgcaaaccgccgagtgcttagatcagggcaaaaacaatacgagcaagcactcgataacttctttaagtctcagaacggatccagggctgggcaaaaaatgggcaagcctcgttttaaaactaaaattcgctccacagactcattcaccatcgacgccgttgatgtctcctcatcgaccacactcatcagagatataggccccaaagaccatgcccgatacaaaaccggtgaagcctcaacaggaatcattgcagactaccgccacgtcagactctcccacctaggcacatttcgcgtctttggatccactaaagccctggtccgacaactcgatagaggcgggcggattaaatcctgcacagtgtctcgatccgctgatcgctggtacgtctcattccttgtcgaactccccatcgagatagcacgctctacacctacgaaaaagcaatataaagcaggtgcagtcgggattgatctgggagtaaaaagcctcgctgccctatctaccggcgagattatccccaacccacgtttcttacgcaccgcagataaaaagatcaagaagcttcaacgcaaaatcgctcggtgccaaaaaggatcaaaaaattccatccggttaaagcgacgtcttgcacgctgccaccatgaactcgcgctgcaacgtgcagggtatctgaacgaactcactagcatgctggcatcgagtttttccgcgatcgcactagaagatctcaacgtggcggggatgacatcatccgcgcgcggaaccgtggaaaatccgggtaaaaatgtgaaacaaaaagcagggttaaacaggtcaattctcgacatctcaccagggcgtatccgcacgttgttggagtataaatgcactgatcgcggtgttgagctgcaggttattgatcgttttttcccctcatcgcagttatgttcgtcctgtggatcaaaaaccacgatccccttggcgcagcgtatctatcactgtgatgtgtgtggtggtgtcattgatcgtgatgtcaatgccgctatcaatattgtctatgaagccaagcgattggtggaacaaaaatgtagtgaacactcggctccggagggggcagaggataaacggccgtggagtgtacatctcccatcaacgcagtatgttgatggactgtatacgaggaagcggcaaggccccagcggtcatagcagttgagtaattggctgctctttatcgtgttgtgttgaaggaaaatcgtggtaagtggtgatggattcgctggtcaggaagtgttcttcccacgcacacgaggaagatccccgagaccattggtctcaggccggcatggtcccagcctcctcgctggcgccggctgggcaacatgcttcggcatggcgaatgggacccaattattgaacaccctaacgggtgtttttttgtttctggtctacc

SEQ ID NO: 141 - DNA, 8370 bp, synthetic construct
  source 1..8370: mol_type = other DNA
tttccataggctccgcccccctgacaagcatcacgaaatctgacgctcaaatcagtggtggcgaaacccgacaggactataaagataccaggcgtttccccctggcggctccctcgtgcgctctcctgttcctgcctttcggtttaccggtgtcattccgctgttatggccgcgtttgtctcattccacgcctgacactcagttccgggtaggcagttcgctccaagctggactgtatgcacgaaccccccgttcagtccgaccgctgcgccttatccggtaactatcgtcttgagtccaacccggaaagacatgcaaaagcaccactggcagcagccactggtaattgatttagaggagttagtcttgaagtcatgcgccggttaaggctaaactgaaaggacaagttttggtgactgcgctcctccaagccagttacctcggttcaaagagttggtagctcagagaaccttcgaaaaaccgccctgcaaggcggttttttcgttttcagagcaagagattacgcgcagaccaaaacgatctcaagaagatcatcttattaatcagataaaatatttctagatttcagtgcaatttatctcttcaaatgtagcacctgaagtcagccccatacgatataagttgtgacgtaaaatgagacgttgatcggcacgtaagaggttccaactttcaccataatgaaataagatcactaccgggcgtattttttgagttatcgagattttcaggagctaaggaagctaaaatggagaaaaaaatcactggatataccaccgttgatatatcccaatggcatcgtaaagaacattttgaggcatttcagtcagttgctcaatgtacctataaccagaccgttcagctgggtcatccaccggatcaattcccctgctcgcgcaggctgggtgccaagctctcgggtaacatcaaggcccgatccttggagcccttgccctcccgcacgatgatcgtgccgtgatcgaaatccagatccttgacccgcagttgcaaaccctcactgatccggctcacggtaactgatgccgtatttgcagtaccagcgtacggcccacagaatgatgtcacgctgaaaatgccggcctttgaatgggttcatgtgcagctccatcagcaaaaggggatgataagtttatcaccaccgactatttgcaacagtgccgttgatcgtgctatgatcgactgatgtcatcagcggtggagtgcaatgtcgtgcaatacgaatggcgaaaagccgagctcatcggtcagcttctcaaccttggggttacccccggcggtgtgctgctggtccacagctccttccgtagcgtccggcccctcgaagatgggccacttggactgatcgaggccctgcgtgctgcgctgggtccgggagggacgctcgtcatgccctcgtggtcaggtctggacgacgagccgttcgatcctgccacgtcgcccgttacaccggaccttggagttgtctctgacacattctggcgcctgccaaatgtaaagcgcagcgcccatccatttgcctttgcggcagcggggccacaggcagagcagatcatctctgatccattgcccctgccacctcactcgcctgcaagcccggtcgcccgtgtccatgaactcgatgggcaggtacttctcctcggcgtgggacacgatgccaacacgacgctgcatcttgccgagttgatggcaaaggttccctatggggtgccgagacactgcaccattcttcaggatggcaagttggtacgcgtcgattatctcgagaatgaccactgctgtgagcgctttgccttggcggacaggtggctcaaggagaagagccttcagaaggaaggtccagtcggtcatgcctttgctcggttgatccgctcccgcgacattgtggcgacagccctgggtcaactgggccgagatccgttgatcttcctgcatccgccagaggcgggatgcgaagaatgcgatgccgctcgccagtcgattggctgagctcatgagcggagaacgagatgacgttggaggggcaaggtcgcgctgattgctggggcaacacgtgaaaggcgagatcaccaaggtagtcggcaaataatgtctaacggtacccggggatcctctagagtcgacctgcataatgtgcctgtcaaatggacgaagcagggattctgcaaaccctatgctactccgtcaagccgtcaattgtctgattcgttaccaattatgacaacttgacggctacatcattcactttttcttcacaaccggcacggaactcgctcgggctggccccggtgcattttttaaatacccgcgagaaatagagttgatcgtcaaaaccaacattgcgaccgacggtggcgataggcatccgggtggtgctcaaaagcagcttcgcctggctgatacgttggtcctcgcgccagcttaagacgctaatccctaactgctggcggaaaagatgtgacagacgcgacggcgacaagcaaacatgctgtgcgacgctggcgatatcaaaattgctgtctgccaggtgatcgctgatgtactgacaagcctcgcgtacccgattatccatcggtggatggagcgactcgttaatcgcttccatgcgccgcagtaacaattgctcaagcagatttatcgccagcagctccgaatagcgcccttccccttgcccggcgttaatgatttgcccaaacaggtcgctgaaatgcggctggtgcgcttcatccgggcgaaagaaccccgtattggcaaatattgacggccagttaagccattcatgccagtaggcgcgcggacgaaagtaaacccactggtgataccattcgcgagcctccggatgacgaccgtagtgatgaatctctcctggcgggaacagcaaaatatcacccggtcggcaaacaaattctcgtccctgatttttcaccaccccctgaccgcgaatggtgagattgagaatataacctttcattcccagcggtcggtcgataaaaaaatcgagataaccgttggcctcaatcggcgttaaacccgccaccagatgggcattaaacgagtatcccggcagcaggggatcattttgcgcttcagccatacttttcatactcccgccattcagagaagaaaccaattgtccatattgcatcagacattgccgtcactgcgtcttttactggctcttctcgctaaccaaaccggtaaccccgcttattaaaagcattctgtaacaaagcgggaccaaagccatgacaaaaacgcgtaacaaaagtgtctataatcacggcagaaaagtccacattgattatttgcacggcgtcacactttgctatgccatagcatttttatccataagattagcggatcctacctgacgctttttatcgcaactctctactgtttctccatacccgtttttttgggctagcgaaaagatgtttcgtgaagccgtcgacgcttataaaaaatggatattaatactgaaactgagatcaagcaaaagcattcactaaccccctttcctgttttcctaatcagcccggcatttcgcgggcgatattttcacagctatttcaggagttcagccatgaacgcttattacattcaggatcgtcttgaggctcagagctgggcgcgtcactaccagcagctcgcccgtgaagagaaagaggcagaactggcagacgacatggaaaaaggcctgccccagcacctgtttgaatcgctatgcatcgatcatttgcaacgccacggggccagcaaaaaatccattacccgtgcgtttgatgacgatgttgagtttcaggagcgcatggcagaacacatccggtacatggttgaaaccattgctcaccaccaggttgatattgattcagaggtataaaacgaatgagtactgcactcgcaacgctggctgggaagctggctgaacgtgtcggcatggattctgtcgacccacaggaactgatcaccactcttcgccagacggcatttaaaggtgatgccagcgatgcgcagttcatcgcattactgatcgttgccaaccagtacggccttaatccgtggacgaaagaaatttacgcctttcctgataagcagaatggcatcgttccggtggtgggcgttgatggctggtcccgcatcatcaatgaaaaccagcagtttgatggcatggactttgagcaggacaatgaatcctgtacatgccggatttaccgcaaggaccgtaatcatccgatctgcgttaccgaatggatggatgaatgccgccgcgaaccattcaaaactcgcgaaggcagagaaatcacggggccgtggcagtcgcatcccaaacggatgttacgtcataaagccatgattcagtgtgcccgtctggccttcggatttgctggtatctatgacaaggatgaagccgagcgcattgtcgaaaatactgcatacactgcagaacgtcagccggaacgcgacatcactccggttaacgatgaaaccatgcaggagattaacactctgctgatcgccctggataaaacatgggatgacgacttattgccgctctgttcccagatatttcgccgcgacattcgtgcatcgtcagaactgacacaggccgaagcagtaaaagctcttggattcctgaaacagaaagccgcagagcagaaggtggcagcatgacaccggacattatcctgcagcgtaccgggatcgatgtgagagctgtcgaacagggggatgatgcgtggcacaaattacggctcggcgtcatcaccgcttcagaagttcacaacgtgatagcaaaaccccgctccggaaagaagtggcctgacatgaaaatgtcctacttccacaccctgcttgctgaggtttgcaccggtgtggctccggaagttaacgctaaagcactggcctggggaaaacagtacgagaacgacgccagaaccctgtttgaattcacttccggcgtgaatgttactgaatccccgatcatctatcgcgacgaaagtatgcgtaccgcctgctctcccgatggtttatgcagtgacggcaacggccttgaactgaaatgcccgtttacctcccgggatttcatgaagttccggctcggtggtttcgaggccataaagtcagcttacatggcccaggtgcagtacagcatgtgggtgacgcgaaaaaatgcctggtactttgccaactatgacccgcgtatgaagcgtgaaggcctgcattatgtcgtgattgagcgggatgaaaagtacatggcgagttttgacgagatcgtgccggagttcatcgaaaaaatggacgaggcactggctgaaattggttttgtatttggggagcaatggcgatgacgcatcctcacgataataagcttcctgctgaacatcaaaggcaagaaaacatctgttgtcaaagacagcatccttgaacaaggacaattaacagttaacaaataaaaacgcaaaagaaaatgccgatattgactaccggaagcagtgtgaccgtgtgcttctcaaatgcctgattcaggctgtctatgtgtgactgttgagctgtaacaagttgtctcaggtgttcaatttcatgttctagttgctttgttttactggtttcacctgttctattaggtgttacatgctgttcatctgttacattgtcgatctgttcatggtgaacagctttaaatgcaccaaaaactcgtaaaagctctgatgtatctatcttttttacaccgttttcatctgtgcatatagctatactgatttcgtcagactcacagtcaaacatgccggtcagttggcctggtgatggcgggatcgttgtatatttcttgacaccttttcggcaccgccctaaaattctgcgtcctcataatatatgaggcgatttattacgtgtttacgaagcaaaagctaaaaccaggagctatttaatggctactactgataagaaggatgaagaaaaccttcgagcgtataagttccgtcttgacccaaatcaagctcagactaccgctctctatcaggcagtcggtgcggctcggtatacatacaatatgctcaccgcatataacttggaagttaatagacttcgtgatgattattggaagagacgccatgatgaggatatctccgacgcagatattaaaaaagaacttaatgcgcttgccaaagaagataaacgctataagcagttaaattacggagcatttggaacccaatatttgactcctgagaaaaaacgtcatgaacaagccgaacaccgtattgaaaatggcgaagatccgtcagttgtgtggaaccaagagacggagcggtcggctaatccgtggcttcataccgcaaatcagcgagtgctggtgagtggtctgcaaaatgcgagtgatgcttgggacaatttctgggcttcccgtacgggtaaacgtgctgggcgtctggtgggtacaccgcgtttcaagaagaaaggtgtttcgcgggattcttttacggttccggcaccggaaaagatgggcgcttacggcaccgcgtatctgcgaggggaacctgcctacaagcaggggcgacgtaagattacagactatcgtcatgtgcggttatcttatctaggtactatacgcacctttaactcgaccaagccactagtgaaagcggttgtagctggcgccaagattcgtagctatacggtctctcggaatgctgaccgctggtatgtatctttcttagtgaagttttcggagcctatacgtcgttctgcaacaaagcgtgctcgtgctgctggttctgtaggtgttgatttaggagttaagtacctggcgtcactttcagattccgaggctccacaacgcttcccgaatctaaaatttgtcgaagggctgcctagccttgagaacccgcgctggagtgaggcaagctcgcgacggctgcataagttacagcgtgctctagcacgttctcagaaagggtcgaatcgacgttctcgtttagtgaagcagatagctcggttgcaccatatgacggcgttgcgtcgtgagtcgaatctgcatcagctgacgaaaaaacttgctaccgagtataccctggtaggatttgaagatttgaatgtttccggtatgaccgcctctgcgaaggggacggttgagaatccggggaagaatgttgcccaaaagtctgggttgaaccgggtagttttggatgcggcattcggcgtgttccgtaaccagctggagtataaggctgtctggtatggttctgcgtttgagaaggttgaccgttattttgcttcgtcgcagacgtgttcggagtgtgggaggaaagcgaaaaccaagctgactctgcgcgaccgtgtcttcgactgtgcgtactgtgggaatatgatggatcgtgatcttaacgcggccgtcaatatttgccgtgaggcgcagaggctttttgacgaaaaactcgcctcagaagatagggagagtctaaacggacgtggaagtcgaggcgctcttcggggtgctgagactgtggaagcgtcaagaccacctgcgagtcatcgtagagggtcaccgtagatgagtaatcatctgcccatctattgcattatgcacgcaactgaatagagttttgcagacatgcgggcgttatacctagtcagcaagtgtctgccccgcgtgtgcatgggtggttcccgagaccattggtctcaggccggcatggtcccagcctcctcgctggcgccggctgggcaacatgcttcggcatggcgaatgggacccaattattgaacaccctaacgggtgtttttttgtttctggtctacctggctggttggcgtactgttgtggtaaatacccatatggacagttttccctttgatatgtaacggtgaacagttgttctacttttgtttgttagtcttgatgcttcactgatagatacaagagcgtcgggtgatgctgccaacttactgatttagtgtatgatggtgtttttgaggtgctccagtggcttctgtttctatcagctgtccctcctgttcagctactgacggggtggtgcgtaacggcaaaagcaccgccggacatcagcgctagcggagtgtatactggcttactatgttggcactgatgagggtgtcagtgaagtgcttcatgtggcaggagaaaaaaggctgcaccggtgcgtcagcagaatatgtgatacaggatatattccgcttcctcgctcactgactcgctacgctcggtcgttcgactgcggcgagcggaaatggcttacgaacggggcggagatttcctggaagatgccaggaagatacttaacagggaagtgagagggccgcggcaaagccgtt

SEQ ID NO: 142 - DNA, 8370 bp, synthetic construct
  source 1..8370: mol_type = other DNA
tggctggttggcgtactgttgtggtaaatacccatatggacagttttccctttgatatgtaacggtgaacagttgttctacttttgtttgttagtcttgatgcttcactgatagatacaagagcgtcgggtgatgctgccaacttactgatttagtgtatgatggtgtttttgaggtgctccagtggcttctgtttctatcagctgtccctcctgttcagctactgacggggtggtgcgtaacggcaaaagcaccgccggacatcagcgctagcggagtgtatactggcttactatgttggcactgatgagggtgtcagtgaagtgcttcatgtggcaggagaaaaaaggctgcaccggtgcgtcagcagaatatgtgatacaggatatattccgcttcctcgctcactgactcgctacgctcggtcgttcgactgcggcgagcggaaatggcttacgaacggggcggagatttcctggaagatgccaggaagatacttaacagggaagtgagagggccgcggcaaagccgtttttccataggctccgcccccctgacaagcatcacgaaatctgacgctcaaatcagtggtggcgaaacccgacaggactataaagataccaggcgtttccccctggcggctccctcgtgcgctctcctgttcctgcctttcggtttaccggtgtcattccgctgttatggccgcgtttgtctcattccacgcctgacactcagttccgggtaggcagttcgctccaagctggactgtatgcacgaaccccccgttcagtccgaccgctgcgccttatccggtaactatcgtcttgagtccaacccggaaagacatgcaaaagcaccactggcagcagccactggtaattgatttagaggagttagtcttgaagtcatgcgccggttaaggctaaactgaaaggacaagttttggtgactgcgctcctccaagccagttacctcggttcaaagagttggtagctcagagaaccttcgaaaaaccgccctgcaaggcggttttttcgttttcagagcaagagattacgcgcagaccaaaacgatctcaagaagatcatcttattaatcagataaaatatttctagatttcagtgcaatttatctcttcaaatgtagcacctgaagtcagccccatacgatataagttgtgacgtaaaatgagacgttgatcggcacgtaagaggttccaactttcaccataatgaaataagatcactaccgggcgtattttttgagttatcgagattttcaggagctaaggaagctaaaatggagaaaaaaatcactggatataccaccgttgatatatcccaatggcatcgtaaagaacattttgaggcatttcagtcagttgctcaatgtacctataaccagaccgttcagctgggtcatccaccggatcaattcccctgctcgcgcaggctgggtgccaagctctcgggtaacatcaaggcccgatccttggagcccttgccctcccgcacgatgatcgtgccgtgatcgaaatccagatccttgacccgcagttgcaaaccctcactgatccggctcacggtaactgatgccgtatttgcagtaccagcgtacggcccacagaatgatgtcacgctgaaaatgccggcctttgaatgggttcatgtgcagctccatcagcaaaaggggatgataagtttatcaccaccgactatttgcaacagtgccgttgatcgtgctatgatcgactgatgtcatcagcggtggagtgcaatgtcgtgcaatacgaatggcgaaaagccgagctcatcggtcagcttctcaaccttggggttacccccggcggtgtgctgctggtccacagctccttccgtagcgtccggcccctcgaagatgggccacttggactgatcgaggccctgcgtgctgcgctgggtccgggagggacgctcgtcatgccctcgtggtcaggtctggacgacgagccgttcgatcctgccacgtcgcccgttacaccggaccttggagttgtctctgacacattctggcgcctgccaaatgtaaagcgcagcgcccatccatttgcctttgcggcagcggggccacaggcagagcagatcatctctgatccattgcccctgccacctcactcgcctgcaagcccggtcgcccgtgtccatgaactcgatgggcaggtacttctcctcggcgtgggacacgatgccaacacgacgctgcatcttgccgagttgatggcaaaggttccctatggggtgccgagacactgcaccattcttcaggatggcaagttggtacgcgtcgattatctcgagaatgaccactgctgtgagcgctttgccttggcggacaggtggctcaaggagaagagccttcagaaggaaggtccagtcggtcatgcctttgctcggttgatccgctcccgcgacattgtggcgacagccctgggtcaactgggccgagatccgttgatcttcctgcatccgccagaggcgggatgcgaagaatgcgatgccgctcgccagtcgattggctgagctcatgagcggagaacgagatgacgttggaggggcaaggtcgcgctgattgctggggcaacacgtgaaaggcgagatcaccaaggtagtcggcaaataatgtctaacggtacccggggatcctctagagtcgacctgcataatgtgcctgtcaaatggacgaagcagggattctgcaaaccctatgctactccgtcaagccgtcaattgtctgattcgttaccaattatgacaacttgacggctacatcattcactttttcttcacaaccggcacggaactcgctcgggctggccccggtgcattttttaaatacccgcgagaaatagagttgatcgtcaaaaccaacattgcgaccgacggtggcgataggcatccgggtggtgctcaaaagcagcttcgcctggctgatacgttggtcctcgcgccagcttaagacgctaatccctaactgctggcggaaaagatgtgacagacgcgacggcgacaagcaaacatgctgtgcgacgctggcgatatcaaaattgctgtctgccaggtgatcgctgatgtactgacaagcctcgcgtacccgattatccatcggtggatggagcgactcgttaatcgcttccatgcgccgcagtaacaattgctcaagcagatttatcgccagcagctccgaatagcgcccttccccttgcccggcgttaatgatttgcccaaacaggtcgctgaaatgcggctggtgcgcttcatccgggcgaaagaaccccgtattggcaaatattgacggccagttaagccattcatgccagtaggcgcgcggacgaaagtaaacccactggtgataccattcgcgagcctccggatgacgaccgtagtgatgaatctctcctggcgggaacagcaaaatatcacccggtcggcaaacaaattctcgtccctgatttttcaccaccccctgaccgcgaatggtgagattgagaatataacctttcattcccagcggtcggtcgataaaaaaatcgagataaccgttggcctcaatcggcgttaaacccgccaccagatgggcattaaacgagtatcccggcagcaggggatcattttgcgcttcagccatacttttcatactcccgccattcagagaagaaaccaattgtccatattgcatcagacattgccgtcactgcgtcttttactggctcttctcgctaaccaaaccggtaaccccgcttattaaaagcattctgtaacaaagcgggaccaaagccatgacaaaaacgcgtaacaaaagtgtctataatcacggcagaaaagtccacattgattatttgcacggcgtcacactttgctatgccatagcatttttatccataagattagcggatcctacctgacgctttttatcgcaactctctactgtttctccatacccgtttttttgggctagcgaaaagatgtttcgtgaagccgtcgacgcttataaaaaatggatattaatactgaaactgagatcaagcaaaagcattcactaaccccctttcctgttttcctaatcagcccggcatttcgcgggcgatattttcacagctatttcaggagttcagccatgaacgcttattacattcaggatcgtcttgaggctcagagctgggcgcgtcactaccagcagctcgcccgtgaagagaaagaggcagaactggcagacgacatggaaaaaggcctgccccagcacctgtttgaatcgctatgcatcgatcatttgcaacgccacggggccagcaaaaaatccattacccgtgcgtttgatgacgatgttgagtttcaggagcgcatggcagaacacatccggtacatggttgaaaccattgctcaccaccaggttgatattgattcagaggtataaaacgaatgagtactgcactcgcaacgctggctgggaagctggctgaacgtgtcggcatggattctgtcgacccacaggaactgatcaccactcttcgccagacggcatttaaaggtgatgccagcgatgcgcagttcatcgcattactgatcgttgccaaccagtacggccttaatccgtggacgaaagaaatttacgcctttcctgataagcagaatggcatcgttccggtggtgggcgttgatggctggtcccgcatcatcaatgaaaaccagcagtttgatggcatggactttgagcaggacaatgaatcctgtacatgccggatttaccgcaaggaccgtaatcatccgatctgcgttaccgaatggatggatgaatgccgccgcgaaccattcaaaactcgcgaaggcagagaaatcacggggccgtggcagtcgcatcccaaacggatgttacgtcataaagccatgattcagtgtgcccgtctggccttcggatttgctggtatctatgacaaggatgaagccgagcgcattgtcgaaaatactgcatacactgcagaacgtcagccggaacgcgacatcactccggttaacgatgaaaccatgcaggagattaacactctgctgatcgccctggataaaacatgggatgacgacttattgccgctctgttcccagatatttcgccgcgacattcgtgcatcgtcagaactgacacaggccgaagcagtaaaagctcttggattcctgaaacagaaagccgcagagcagaaggtggcagcatgacaccggacattatcctgcagcgtaccgggatcgatgtgagagctgtcgaacagggggatgatgcgtggcacaaattacggctcggcgtcatcaccgcttcagaagttcacaacgtgatagcaaaaccccgctccggaaagaagtggcctgacatgaaaatgtcctacttccacaccctgcttgctgaggtttgcaccggtgtggctccggaagttaacgctaaagcactggcctggggaaaacagtacgagaacgacgccagaaccctgtttgaattcacttccggcgtgaatgttactgaatccccgatcatctatcgcgacgaaagtatgcgtaccgcctgctctcccgatggtttatgcagtgacggcaacggccttgaactgaaatgcccgtttacctcccgggatttcatgaagttccggctcggtggtttcgaggccataaagtcagcttacatggcccaggtgcagtacagcatgtgggtgacgcgaaaaaatgcctggtactttgccaactatgacccgcgtatgaagcgtgaaggcctgcattatgtcgtgattgagcgggatgaaaagtacatggcgagttttgacgagatcgtgccggagttcatcgaaaaaatggacgaggcactggctgaaattggttttgtatttggggagcaatggcgatgacgcatcctcacgataataagcttcctgctgaacatcaaaggcaagaaaacatctgttgtcaaagacagcatccttgaacaaggacaattaacagttaacaaataaaaacgcaaaagaaaatgccgatattgactaccggaagcagtgtgaccgtgtgcttctcaaatgcctgattcaggctgtctatgtgtgactgttgagctgtaacaagttgtctcaggtgttcaatttcatgttctagttgctttgttttactggtttcacctgttctattaggtgttacatgctgttcatctgttacattgtcgatctgttcatggtgaacagctttaaatgcaccaaaaactcgtaaaagctctgatgtatctatcttttttacaccgttttcatctgtgcatatagctatactgatttcgtcagactcacagtcaaacatgccggtcagttggcctggtgatggcgggatcgttgtatatttcttgacaccttttcggcaccgccctaaaattctgcgtcctcataatatatgaggcgatttattacgtgtttacgaagcaaaagctaaaaccaggagctatttaatgcccctgaacggatggacgatgctggcgcaggaggaggtgcgagcgatgacgactaccacgggtaccgacctggccccgaggctgcgcgcgttcaagcaccgcctggaccccaaccccgcccaggccaccctgctggcccagtacgccggcgccgcgcgcgtggcctacaacatgctcatcgcccacaaccgggccgccctggccgccggtgccgcccgtcgcaccgagctggccgagagcgggctggccggccccgagctggccgcgcgcatgaaggccgagcgcgccgccgaccccaccctccgcgtggccagctaccagtcgtactccacggcccacctgactccgctgatccgccgccaccgtgaggctgccgccgcgatcgccgccggtgccgacccggccgaggcatggaccgacgagcgatacgccgagccctggatgcacaccgtgccccgccgcgtcctggtctccggcctccagaacgccgcgaaggccaccgagaactggatggcctccgcctccggcacgcgcgccggcgcgcgcgtcggcctgccgcggttcaagaagaagggccggtcccgggacagcttcaccatccccgcccccgaggtcatcggcgccgcgggcaccccctacaagcgcggcgagcaccgccgcggggtgatcaccgaccaccggcacctgcgcctggcctccctggggaccatccgcacctacgacaagaccagccgcctggtccgcgcctgccgccgcggcgcccagatccggtccatgaccatctcccaggctggcggacggtggtacgcctcgatcctcgttgccgaccccacccccatccggaccgggcccagccgtcgccagcgcgccaacggcgccgtcggcgtggacctgggcgtcaagcacctggccgccctctccaccggcgaggtcatcgacaacggccgccccggtgcccgccaggccgcccgcctgacccgtctccagcgcgcctacgcccgcacccagcccggctcgaaccgccgcgagcgcgtgcgccggcagatcgcggcactccatcacgggatcgcactacgtcgggcggggctgctgcatcaggtgtccacgagactggcgatggacttcgcggtggtcgccctggaggacctgaacgtggcggggatgacccgttcggcccgcgggacgctcgaggcgccgggtaggaacgtggccgccaagtccgggttgaaccgggcgatcctggatgccgggctggggatgctgcgccggcagctggactacaagacctcctgggcagggtcccaggtgaagatgatcgaccgattcgcgccctcctcgaaggcgtgctcgcgctgcgggacagtcaaatccacgctgtccctggccgagcggaccttcgagtgcgaggcctgccacctggtgatcgaccgcgacgtgaacgccgcgatcaacatccgggcgtgggctgtgcaggaggagcgtagagcaggggtcgagctcgcccgaggccgtcgggagagtcgaaacggacgtggagctgctgtctcgggcccgccatctggcggggccgcggggcaggggcgtggaagcgtcaagcccgcaccccagggtgtgggcatgtccagccgggcaactggctggtcatcccaacccccctcaaccgaaggggaaagcgcagagcgcggagcatccgccctggccaggtagtggaagccccgcgcacgcagggatgagcctcgagaccattggtctcaggccggcatggtcccagcctcctcgctggcgccggctgggcaacatgcttcggcatggcgaatgggacccaattattgaacaccctaacgggtgtttttttgtttctggtctacc

SEQ ID NO: 143 - DNA, 24 bp, synthetic construct
  source 1..24: mol_type = other DNA
tccctgtcctcttcctctttagcg

SEQ ID NO: 144 - DNA, 24 bp, synthetic construct
  source 1..24: mol_type = other DNA
ttcctgtcctcttcctctttagcg

SEQ ID NO: 145 - DNA, 24 bp, synthetic construct
  source 1..24: mol_type = other DNA
gccttgtcctcttcctctttagcg

SEQ ID NO: 146 - DNA, 8352 bp, synthetic construct
  source 1..8352: mol_type = other DNA
tggctggttggcgtactgttgtggtaaatacccatatggacagttttccctttgatatgtaacggtgaacagttgttctacttttgtttgttagtcttgatgcttcactgatagatacaagagcgtcgggtgatgctgccaacttactgatttagtgtatgatggtgtttttgaggtgctccagtggcttctgtttctatcagctgtccctcctgttcagctactgacggggtggtgcgtaacggcaaaagcaccgccggacatcagcgctagcggagtgtatactggcttactatgttggcactgatgagggtgtcagtgaagtgcttcatgtggcaggagaaaaaaggctgcaccggtgcgtcagcagaatatgtgatacaggatatattccgcttcctcgctcactgactcgctacgctcggtcgttcgactgcggcgagcggaaatggcttacgaacggggcggagatttcctggaagatgccaggaagatacttaacagggaagtgagagggccgcggcaaagccgtttttccataggctccgcccccctgacaagcatcacgaaatctgacgctcaaatcagtggtggcgaaacccgacaggactataaagataccaggcgtttccccctggcggctccctcgtgcgctctcctgttcctgcctttcggtttaccggtgtcattccgctgttatggccgcgtttgtctcattccacgcctgacactcagttccgggtaggcagttcgctccaagctggactgtatgcacgaaccccccgttcagtccgaccgctgcgccttatccggtaactatcgtcttgagtccaacccggaaagacatgcaaaagcaccactggcagcagccactggtaattgatttagaggagttagtcttgaagtcatgcgccggttaaggctaaactgaaaggacaagttttggtgactgcgctcctccaagccagttacctcggttcaaagagttggtagctcagagaaccttcgaaaaaccgccctgcaaggcggttttttcgttttcagagcaagagattacgcgcagaccaaaacgatctcaagaagatcatcttattaatcagataaaatatttctagatttcagtgcaatttatctcttcaaatgtagcacctgaagtcagccccatacgatataagttgtgacgtaaaatgagacgttgatcggcacgtaagaggttccaactttcaccataatgaaataagatcactaccgggcgtattttttgagttatcgagattttcaggagctaaggaagctaaaatggagaaaaaaatcactggatataccaccgttgatatatcccaatggcatcgtaaagaacattttgaggcatttcagtcagttgctcaatgtacctataaccagaccgttcagctgggtcatccaccggatcaattcccctgctcgcgcaggctgggtgccaagctctcgggtaacatcaaggcccgatccttggagcccttgccctcccgcacgatgatcgtgccgtgatcgaaatccagatccttgacccgcagttgcaaaccctcactgatccggctcacggtaactgatgccgtatttgcagtaccagcgtacggcccacagaatgatgtcacgctgaaaatgccggcctttgaatgggttcatgtgcagctccatcagcaaaaggggatgataagtttatcaccaccgactatttgcaacagtgccgttgatcgtgctatgatcgactgatgtcatcagcggtggagtgcaatgtcgtgcaatacgaatggcgaaaagccgagctcatcggtcagcttctcaaccttggggttacccccggcggtgtgctgctggtccacagctccttccgtagcgtccggcccctcgaagatgggccacttggactgatcgaggccctgcgtgctgcgctgggtccgggagggacgctcgtcatgccctcgtggtcaggtctggacgacgagccgttcgatcctgccacgtcgcccgttacaccggaccttggagttgtctctgacacattctggcgcctgccaaatgtaaagcgcagcgcccatccatttgcctttgcggcagcggggccacaggcagagcagatcatctctgatccattgcccctgccacctcactcgcctgcaagcccggtcgcccgtgtccatgaactcgatgggcaggtacttctcctcggcgtgggacacgatgccaacacgacgctgcatcttgccgagttgatggcaaaggttccctatggggtgccgagacactgcaccattcttcaggatggcaagttggtacgcgtcgattatctcgagaatgaccactgctgtgagcgctttgccttggcggacaggtggctcaaggagaagagccttcagaaggaaggtccagtcggtcatgcctttgctcggttgatccgctcccgcgacattgtggcgacagccctgggtcaactgggccgagatccgttgatcttcctgcatccgccagaggcgggatgcgaagaatgcgatgccgctcgccagtcgattggctgagctcatgagcggagaacgagatgacgttggaggggcaaggtcgcgctgattgctggggcaacacgtgaaaggcgagatcaccaaggtagtcggcaaataatgtctaacggtacccggggatcctctagagtcgacctgcataatgtgcctgtcaaatggacgaagcagggattctgcaaaccctatgctactccgtcaagccgtcaattgtctgattcgttaccaattatgacaacttgacggctacatcattcactttttcttcacaaccggcacggaactcgctcgggctggccccggtgcattttttaaatacccgcgagaaatagagttgatcgtcaaaaccaacattgcgaccgacggtggcgataggcatccgggtggtgctcaaaagcagcttcgcctggctgatacgttggtcctcgcgccagcttaagacgctaatccctaactgctggcggaaaagatgtgacagacgcgacggcgacaagcaaacatgctgtgcgacgctggcgatatcaaaattgctgtctgccaggtgatcgctgatgtactgacaagcctcgcgtacccgattatccatcggtggatggagcgactcgttaatcgcttccatgcgccgcagtaacaattgctcaagcagatttatcgccagcagctccgaatagcgcccttccccttgcccggcgttaatgatttgcccaaacaggtcgctgaaatgcggctggtgcgcttcatccgggcgaaagaaccccgtattggcaaatattgacggccagttaagccattcatgccagtaggcgcgcggacgaaagtaaacccactggtgataccattcgcgagcctccggatgacgaccgtagtgatgaatctctcctggcgggaacagcaaaatatcacccggtcggcaaacaaattctcgtccctgatttttcaccaccccctgaccgcgaatggtgagattgagaatataacctttcattcccagcggtcggtcgataaaaaaatcgagataaccgttggcctcaatcggcgttaaacccgccaccagatgggcattaaacgagtatcccggcagcaggggatcattttgcgcttcagccatacttttcatactcccgccattcagagaagaaaccaattgtccatattgcatcagacattgccgtcactgcgtcttttactggctcttctcgctaaccaaaccggtaaccccgcttattaaaagcattctgtaacaaagcgggaccaaagccatgacaaaaacgcgtaacaaaagtgtctataatcacggcagaaaagtccacattgattatttgcacggcgtcacactttgctatgccatagcatttttatccataagattagcggatcctacctgacgctttttatcgcaactctctactgtttctccatacccgtttttttgggctagcgaaaagatgtttcgtgaagccgtcgacgcttataaaaaatggatattaatactgaaactgagatcaagcaaaagcattcactaaccccctttcctgttttcctaatcagcccggcatttcgcgggcgatattttcacagctatttcaggagttcagccatgaacgcttattacattcaggatcgtcttgaggctcagagctgggcgcgtcactaccagcagctcgcccgtgaagagaaagaggcagaactggcagacgacatggaaaaaggcctgccccagcacctgtttgaatcgctatgcatcgatcatttgcaacgccacggggccagcaaaaaatccattacccgtgcgtttgatgacgatgttgagtttcaggagcgcatggcagaacacatccggtacatggttgaaaccattgctcaccaccaggttgatattgattcagaggtataaaacgaatgagtactgcactcgcaacgctggctgggaagctggctgaacgtgtcggcatggattctgtcgacccacaggaactgatcaccactcttcgccagacggcatttaaaggtgatgccagcgatgcgcagttcatcgcattactgatcgttgccaaccagtacggccttaatccgtggacgaaagaaatttacgcctttcctgataagcagaatggcatcgttccggtggtgggcgttgatggctggtcccgcatcatcaatgaaaaccagcagtttgatggcatggactttgagcaggacaatgaatcctgtacatgccggatttaccgcaaggaccgtaatcatccgatctgcgttaccgaatggatggatgaatgccgccgcgaaccattcaaaactcgcgaaggcagagaaatcacggggccgtggcagtcgcatcccaaacggatgttacgtcataaagccatgattcagtgtgcccgtctggccttcggatttgctggtatctatgacaaggatgaagccgagcgcattgtcgaaaatactgcatacactgcagaacgtcagccggaacgcgacatcactccggttaacgatgaaaccatgcaggagattaacactctgctgatcgccctggataaaacatgggatgacgacttattgccgctctgttcccagatatttcgccgcgacattcgtgcatcgtcagaactgacacaggccgaagcagtaaaagctcttggattcctgaaacagaaagccgcagagcagaaggtggcagcatgacaccggacattatcctgcagcgtaccgggatcgatgtgagagctgtcgaacagggggatgatgcgtggcacaaattacggctcggcgtcatcaccgcttcagaagttcacaacgtgatagcaaaaccccgctccggaaagaagtggcctgacatgaaaatgtcctacttccacaccctgcttgctgaggtttgcaccggtgtggctccggaagttaacgctaaagcactggcctggggaaaacagtacgagaacgacgccagaaccctgtttgaattcacttccggcgtgaatgttactgaatccccgatcatctatcgcgacgaaagtatgcgtaccgcctgctctcccgatggtttatgcagtgacggcaacggccttgaactgaaatgcccgtttacctcccgggatttcatgaagttccggctcggtggtttcgaggccataaagtcagcttacatggcccaggtgcagtacagcatgtgggtgacgcgaaaaaatgcctggtactttgccaactatgacccgcgtatgaagcgtgaaggcctgcattatgtcgtgattgagcgggatgaaaagtacatggcgagttttgacgagatcgtgccggagttcatcgaaaaaatggacgaggcactggctgaaattggttttgtatttggggagcaatggcgatgacgcatcctcacgataataagcttcctgctgaacatcaaaggcaagaaaacatctgttgtcaaagacagcatccttgaacaaggacaattaacagttaacaaataaaaacgcaaaagaaaatgccgatattgactaccggaagcagtgtgaccgtgtgcttctcaaatgcctgattcaggctgtctatgtgtgactgttgagctgtaacaagttgtctcaggtgttcaatttcatgttctagttgctttgttttactggtttcacctgttctattaggtgttacatgctgttcatctgttacattgtcgatctgttcatggtgaacagctttaaatgcaccaaaaactcgtaaaagctctgatgtatctatcttttttacaccgttttcatctgtgcatatagctatactgatttcgtcagactcacagtcaaacatgccggtcagttggcctggtgatggcgggatcgttgtatatttcttgacaccttttcggcaccgccctaaaattctgcgtcctcataatatatgaggcgatttattacgtgtttacgaagcaaaagctaaaaccaggagctatttaatgacaagcaccacgctcgcaccagaagaacccctcatggtgttccgcggcgcgcggtttcgtctcgatccaaccggggaacaacaaggcatattaagccagcaagcaggtgcagcgcgcgttgcatataacatgatgtgcaccctcaacaaagacatcctcgaagcccgaagtcagctgtattcaacgctgatcaaagatggaaaaactaaagataaggccaaaaaagaacttaaagctgccgcaaaggaagatccttcactagctattgtctgggcgcgtgatttcgataaaaactacatcaccccagaacgcaatcgccataagcacgccgcccaacgaattgctgcaggtgaaaacccagtcgatgtatggaacccagacgaagaacgtttcaacgaaccctggctccacaccgcaaaccgccgagtgcttagatcagggcaaaaacaatacgagcaagcactcgataacttctttaagtctcagaacggatccagggctgggcaaaaaatgggcaagcctcgttttaaaactaaaattcgctccacagactcattcaccatcgacgccgttgatgtctcctcatcgaccacactcatcagagatataggccccaaagaccatgcccgatacaaaaccggtgaagcctcaacaggaatcattgcagactaccgccacgtcagactctcccacctaggcacatttcgcgtctttggatccactaaagccctggtccgacaactcgatagaggcgggcggattaaatcctgcacagtgtctcgatccgctgatcgctggtacgtctcattccttgtcgaactccccatcgagatagcacgctctacacctacgaaaaagcaatataaagcaggtgcagtcgggattgatctgggagtaaaaagcctcgctgccctatctaccggcgagattatccccaacccacgtttcttacgcaccgcagataaaaagatcaagaagcttcaacgcaaaatcgctcggtgccaaaaaggatcaaaaaattccatccggttaaagcgacgtcttgcacgctgccaccatgaactcgcgctgcaacgtgcagggtatctgaacgaactcactagcatgctggcatcgagtttttccgcgatcgcactagaagatctcaacgtggcggggatgacatcatccgcgcgcggaaccgtggaaaatccgggtaaaaatgtgaaacaaaaagcagggttaaacaggtcaattctcgacatctcaccagggcgtatccgcacgttgttggagtataaatgcactgatcgcggtgttgagctgcaggttattgatcgttttttcccctcatcgcagttatgttcgtcctgtggatcaaaaaccacgatccccttggcgcagcgtatctatcactgtgatgtgtgtggtggtgtcattgatcgtgatgtcaatgccgctatcaatattgtctatgaagccaagcgattggtggaacaaaaatgtagtgaacactcggctccggagggggcagaggataaacggccgtggagtgtacatctcccatcaacgcagtatgttgatggactgtatacgaggaagcggcaaggccccagcggtcatagcagttgagtaattggctgctctttatcgtgttgtgttgaaggaaaatcgtggtaagtggtgatggattcgctggtcaggaagtgttcttcccacgcacacgaggaagatccctgtcctcttcctctttagcgggccggcatggtcccagcctcctcgctggcgccggctgggcaacatgcttcggcatggcgaatgggacccaattattgaacaccctaacgggtgtttttttgtttctggtctacc

SEQ ID NO: 147 - DNA, 8373 bp, synthetic construct
  source 1..8373: mol_type = other DNA
tttccataggctccgcccccctgacaagcatcacgaaatctgacgctcaaatcagtggtggcgaaacccgacaggactataaagataccaggcgtttccccctggcggctccctcgtgcgctctcctgttcctgcctttcggtttaccggtgtcattccgctgttatggccgcgtttgtctcattccacgcctgacactcagttccgggtaggcagttcgctccaagctggactgtatgcacgaaccccccgttcagtccgaccgctgcgccttatccggtaactatcgtcttgagtccaacccggaaagacatgcaaaagcaccactggcagcagccactggtaattgatttagaggagttagtcttgaagtcatgcgccggttaaggctaaactgaaaggacaagttttggtgactgcgctcctccaagccagttacctcggttcaaagagttggtagctcagagaaccttcgaaaaaccgccctgcaaggcggttttttcgttttcagagcaagagattacgcgcagaccaaaacgatctcaagaagatcatcttattaatcagataaaatatttctagatttcagtgcaatttatctcttcaaatgtagcacctgaagtcagccccatacgatataagttgtgacgtaaaatgagacgttgatcggcacgtaagaggttccaactttcaccataatgaaataagatcactaccgggcgtattttttgagttatcgagattttcaggagctaaggaagctaaaatggagaaaaaaatcactggatataccaccgttgatatatcccaatggcatcgtaaagaacattttgaggcatttcagtcagttgctcaatgtacctataaccagaccgttcagctgggtcatccaccggatcaattcccctgctcgcgcaggctgggtgccaagctctcgggtaacatcaaggcccgatccttggagcccttgccctcccgcacgatgatcgtgccgtgatcgaaatccagatccttgacccgcagttgcaaaccctcactgatccggctcacggtaactgatgccgtatttgcagtaccagcgtacggcccacagaatgatgtcacgctgaaaatgccggcctttgaatgggttcatgtgcagctccatcagcaaaaggggatgataagtttatcaccaccgactatttgcaacagtgccgttgatcgtgctatgatcgactgatgtcatcagcggtggagtgcaatgtcgtgcaatacgaatggcgaaaagccgagctcatcggtcagcttctcaaccttggggttacccccggcggtgtgctgctggtccacagctccttccgtagcgtccggcccctcgaagatgggccacttggactgatcgaggccctgcgtgctgcgctgggtccgggagggacgctcgtcatgccctcgtggtcaggtctggacgacgagccgttcgatcctgccacgtcgcccgttacaccggaccttggagttgtctctgacacattctggcgcctgccaaatgtaaagcgcagcgcccatccatttgcctttgcggcagcggggccacaggcagagcagatcatctctgatccattgcccctgccacctcactcgcctgcaagcccggtcgcccgtgtccatgaactcgatgggcaggtacttctcctcggcgtgggacacgatgccaacacgacgctgcatcttgccgagttgatggcaaaggttccctatggggtgccgagacactgcaccattcttcaggatggcaagttggtacgcgtcgattatctcgagaatgaccactgctgtgagcgctttgccttggcggacaggtggctcaaggagaagagccttcagaaggaaggtccagtcggtcatgcctttgctcggttgatccgctcccgcgacattgtggcgacagccctgggtcaactgggccgagatccgttgatcttcctgcatccgccagaggcgggatgcgaagaatgcgatgccgctcgccagtcgattggctgagctcatgagcggagaacgagatgacgttggaggggcaaggtcgcgctgattgctggggcaacacgtgaaaggcgagatcaccaaggtagtcggcaaataatgtctaacggtacccggggatcctctagagtcgacctgcataatgtgcctgtcaaatggacgaagcagggattctgcaaaccctatgctactccgtcaagccgtcaattgtctgattcgttaccaattatgacaacttgacggctacatcattcactttttcttcacaaccggcacggaactcgctcgggctggccccggtgcattttttaaatacccgcgagaaatagagttgatcgtcaaaaccaacattgcgaccgacggtggcgataggcatccgggtggtgctcaaaagcagcttcgcctggctgatacgttggtcctcgcgccagcttaagacgctaatccctaactgctggcggaaaagatgtgacagacgcgacggcgacaagcaaacatgctgtgcgacgctggcgatatcaaaattgctgtctgccaggtgatcgctgatgtactgacaagcctcgcgtacccgattatccatcggtggatggagcgactcgttaatcgcttccatgcgccgcagtaacaattgctcaagcagatttatcgccagcagctccgaatagcgcccttccccttgcccggcgttaatgatttgcccaaacaggtcgctgaaatgcggctggtgcgcttcatccgggcgaaagaaccccgtattggcaaatattgacggccagttaagccattcatgccagtaggcgcgcggacgaaagtaaacccactggtgataccattcgcgagcctccggatgacgaccgtagtgatgaatctctcctggcgggaacagcaaaatatcacccggtcggcaaacaaattctcgtccctgatttttcaccaccccctgaccgcgaatggtgagattgagaatataacctttcattcccagcggtcggtcgataaaaaaatcgagataaccgttggcctcaatcggcgttaaacccgccaccagatgggcattaaacgagtatcccggcagcaggggatcattttgcgcttcagccatacttttcatactcccgccattcagagaagaaaccaattgtccatattgcatcagacattgccgtcactgcgtcttttactggctcttctcgctaaccaaaccggtaaccccgcttattaaaagcattctgtaacaaagcgggaccaaagccatgacaaaaacgcgtaacaaaagtgtctataatcacggcagaaaagtccacattgattatttgcacggcgtcacactttgctatgccatagcatttttatccataagattagcggatcctacctgacgctttttatcgcaactctctactgtttctccatacccgtttttttgggctagcgaaaagatgtttcgtgaagccgtcgacgcttataaaaaatggatattaatactgaaactgagatcaagcaaaagcattcactaaccccctttcctgttttcctaatcagcccggcatttcgcgggcgatattttcacagctatttcaggagttcagccatgaacgcttattacattcaggatcgtcttgaggctcagagctgggcgcgtcactaccagcagctcgcccgtgaagagaaagaggcagaactggcagacgacatggaaaaaggcctgccccagcacctgtttgaatcgctatgcatcgatcatttgcaacgccacggggccagcaaaaaatccattacccgtgcgtttgatgacgatgttgagtttcaggagcgcatggcagaacacatccggtacatggttgaaaccattgctcaccaccaggttgatattgattcagaggtataaaacgaatgagtactgcactcgcaacgctggctgggaagctggctgaacgtgtcggcatggattctgtcgacccacaggaactgatcaccactcttcgccagacggcatttaaaggtgatgccagcgatgcgcagttcatcgcattactgatcgttgccaaccagtacggccttaatccgtggacgaaagaaatttacgcctttcctgataagcagaatggcatcgttccggtggtgggcgttgatggctggtcccgcatcatcaatgaaaaccagcagtttgatggcatggactttgagcaggacaatgaatcctgtacatgccggatttaccgcaaggaccgtaatcatccgatctgcgttaccgaatggatggatgaatgccgccgcgaaccattcaaaactcgcgaaggcagagaaatcacggggccgtggcagtcgcatcccaaacggatgttacgtcataaagccatgattcagtgtgcccgtctggccttcggatttgctggtatctatgacaaggatgaagccgagcgcattgtcgaaaatactgcatacactgcagaacgtcagccggaacgcgacatcactccggttaacgatgaaaccatgcaggagattaacactctgctgatcgccctggataaaacatgggatgacgacttattgccgctctgttcccagatatttcgccgcgacattcgtgcatcgtcagaactgacacaggccgaagcagtaaaagctcttggattcctgaaacagaaagccgcagagcagaaggtggcagcatgacaccggacattatcctgcagcgtaccgggatcgatgtgagagctgtcgaacagggggatgatgcgtggcacaaattacggctcggcgtcatcaccgcttcagaagttcacaacgtgatagcaaaaccccgctccggaaagaagtggcctgacatgaaaatgtcctacttccacaccctgcttgctgaggtttgcaccggtgtggctccggaagttaacgctaaagcactggcctggggaaaacagtacgagaacgacgccagaaccctgtttgaattcacttccggcgtgaatgttactgaatccccgatcatctatcgcgacgaaagtatgcgtaccgcctgctctcccgatggtttatgcagtgacggcaacggccttgaactgaaatgcccgtttacctcccgggatttcatgaagttccggctcggtggtttcgaggccataaagtcagcttacatggcccaggtgcagtacagcatgtgggtgacgcgaaaaaatgcctggtactttgccaactatgacccgcgtatgaagcgtgaaggcctgcattatgtcgtgattgagcgggatgaaaagtacatggcgagttttgacgagatcgtgccggagttcatcgaaaaaatggacgaggcactggctgaaattggttttgtatttggggagcaatggcgatgacgcatcctcacgataataagcttcctgctgaacatcaaaggcaagaaaacatctgttgtcaaagacagcatccttgaacaaggacaattaacagttaacaaataaaaacgcaaaagaaaatgccgatattgactaccggaagcagtgtgaccgtgtgcttctcaaatgcctgattcaggctgtctatgtgtgactgttgagctgtaacaagttgtctcaggtgttcaatttcatgttctagttgctttgttttactggtttcacctgttctattaggtgttacatgctgttcatctgttacattgtcgatctgttcatggtgaacagctttaaatgcaccaaaaactcgtaaaagctctgatgtatctatcttttttacaccgttttcatctgtgcatatagctatactgatttcgtcagactcacagtcaaacatgccggtcagttggcctggtgatggcgggatcgttgtatatttcttgacaccttttcggcaccgccctaaaattctgcgtcctcataatatatgaggcgatttattacgtgtttacgaagcaaaagctaaaaccaggagctatttaatggctactactgataagaaggatgaagaaaaccttcgagcgtataagttccgtcttgacccaaatcaagctcagactaccgctctctatcaggcagtcggtgcggctcggtatacatacaatatgctcaccgcatataacttggaagttaatagacttcgtgatgattattggaagagacgccatgatgaggatatctccgacgcagatattaaaaaagaacttaatgcgcttgccaaagaagataaacgctataagcagttaaattacggagcatttggaacccaatatttgactcctgagaaaaaacgtcatgaacaagccgaacaccgtattgaaaatggcgaagatccgtcagttgtgtggaaccaagagacggagcggtcggctaatccgtggcttcataccgcaaatcagcgagtgctggtgagtggtctgcaaaatgcgagtgatgcttgggacaatttctgggcttcccgtacgggtaaacgtgctgggcgtctggtgggtacaccgcgtttcaagaagaaaggtgtttcgcgggattcttttacggttccggcaccggaaaagatgggcgcttacggcaccgcgtatctgcgaggggaacctgcctacaagcaggggcgacgtaagattacagactatcgtcatgtgcggttatcttatctaggtactatacgcacctttaactcgaccaagccactagtgaaagcggttgtagctggcgccaagattcgtagctatacggtctctcggaatgctgaccgctggtatgtatctttcttagtgaagttttcggagcctatacgtcgttctgcaacaaagcgtgctcgtgctgctggttctgtaggtgttgatttaggagttaagtacctggcgtcactttcagattccgaggctccacaacgcttcccgaatctaaaatttgtcgaagggctgcctagccttgagaacccgcgctggagtgaggcaagctcgcgacggctgcataagttacagcgtgctctagcacgttctcagaaagggtcgaatcgacgttctcgtttagtgaagcagatagctcggttgcaccatatgacggcgttgcgtcgtgagtcgaatctgcatcagctgacgaaaaaacttgctaccgagtataccctggtaggatttgaagatttgaatgtttccggtatgaccgcctctgcgaaggggacggttgagaatccggggaagaatgttgcccaaaagtctgggttgaaccgggtagttttggatgcggcattcggcgtgttccgtaaccagctggagtataaggctgtctggtatggttctgcgtttgagaaggttgaccgttattttgcttcgtcgcagacgtgttcggagtgtgggaggaaagcgaaaaccaagctgactctgcgcgaccgtgtcttcgactgtgcgtactgtgggaatatgatggatcgtgatcttaacgcggccgtcaatatttgccgtgaggcgcagaggctttttgacgaaaaactcgcctcagaagatagggagagtctaaacggacgtggaagtcgaggcgctcttcggggtgctgagactgtggaagcgtcaagaccacctgcgagtcatcgtagagggtcaccgtagatgagtaatcatctgcccatctattgcattatgcacgcaactgaatagagttttgcagacatgcgggcgttatacctagtcagcaagtgtctgccccgcgtgtgcatgggtggttcctgtcctcttcctctttagcgggccggcatggtcccagcctcctcgctggcgccggctgggcaacatgcttcggcatggcgaatgggacccaattattgaacaccctaacgggtgtttttttgtttctggtctacctggctggttggcgtactgttgtggtaaatacccatatggacagttttccctttgatatgtaacggtgaacagttgttctacttttgtttgttagtcttgatgcttcactgatagatacaagagcgtcgggtgatgctgccaacttactgatttagtgtatgatggtgtttttgaggtgctccagtggcttctgtttctatcagctgtccctcctgttcagctactgacggggtggtgcgtaacggcaaaagcaccgccggacatcagcgctagcggagtgtatactggcttactatgttggcactgatgagggtgtcagtgaagtgcttcatgtggcaggagaaaaaaggctgcaccggtgcgtcagcagaatatgtgatacaggatatattccgcttcctcgctcactgactcgctacgctcggtcgttcgactgcggcgagcggaaatggcttacgaacggggcggagatttcctggaagatgccaggaagatacttaacagggaagtgagagggccgcggcaaagccgtt

SEQ ID NO: 148 - DNA, 8373 bp, synthetic construct
  source 1..8373: mol_type = other DNA
tggctggttggcgtactgttgtggtaaatacccatatggacagttttccctttgatatgtaacggtgaacagttgttctacttttgtttgttagtcttgatgcttcactgatagatacaagagcgtcgggtgatgctgccaacttactgatttagtgtatgatggtgtttttgaggtgctccagtggcttctgtttctatcagctgtccctcctgttcagctactgacggggtggtgcgtaacggcaaaagcaccgccggacatcagcgctagcggagtgtatactggcttactatgttggcactgatgagggtgtcagtgaagtgcttcatgtggcaggagaaaaaaggctgcaccggtgcgtcagcagaatatgtgatacaggatatattccgcttcctcgctcactgactcgctacgctcggtcgttcgactgcggcgagcggaaatggcttacgaacggggcggagatttcctggaagatgccaggaagatacttaacagggaagtgagagggccgcggcaaagccgtttttccataggctccgcccccctgacaagcatcacgaaatctgacgctcaaatcagtggtggcgaaacccgacaggactataaagataccaggcgtttccccctggcggctccctcgtgcgctctcctgttcctgcctttcggtttaccggtgtcattccgctgttatggccgcgtttgtctcattccacgcctgacactcagttccgggtaggcagttcgctccaagctggactgtatgcacgaaccccccgttcagtccgaccgctgcgccttatccggtaactatcgtcttgagtccaacccggaaagacatgcaaaagcaccactggcagcagccactggtaattgatttagaggagttagtcttgaagtcatgcgccggttaaggctaaactgaaaggacaagttttggtgactgcgctcctccaagccagttacctcggttcaaagagttggtagctcagagaaccttcgaaaaaccgccctgcaaggcggttttttcgttttcagagcaagagattacgcgcagaccaaaacgatctcaagaagatcatcttattaatcagataaaatatttctagatttcagtgcaatttatctcttcaaatgtagcacctgaagtcagccccatacgatataagttgtgacgtaaaatgagacgttgatcggcacgtaagaggttccaactttcaccataatgaaataagatcactaccgggcgtattttttgagttatcgagattttcaggagctaaggaagctaaaatggagaaaaaaatcactggatataccaccgttgatatatcccaatggcatcgtaaagaacattttgaggcatttcagtcagttgctcaatgtacctataaccagaccgttcagctgggtcatccaccggatcaattcccctgctcgcgcaggctgggtgccaagctctcgggtaacatcaaggcccgatccttggagcccttgccctcccgcacgatgatcgtgccgtgatcgaaatccagatccttgacccgcagttgcaaaccctcactgatccggctcacggtaactgatgccgtatttgcagtaccagcgtacggcccacagaatgatgtcacgctgaaaatgccggcctttgaatgggttcatgtgcagctccatcagcaaaaggggatgataagtttatcaccaccgactatttgcaacagtgccgttgatcgtgctatgatcgactgatgtcatcagcggtggagtgcaatgtcgtgcaatacgaatggcgaaaagccgagctcatcggtcagcttctcaaccttggggttacccccggcggtgtgctgctggtccacagctccttccgtagcgtccggcccctcgaagatgggccacttggactgatcgaggccctgcgtgctgcgctgggtccgggagggacgctcgtcatgccctcgtggtcaggtctggacgacgagccgttcgatcctgccacgtcgcccgttacaccggaccttggagttgtctctgacacattctggcgcctgccaaatgtaaagcgcagcgcccatccatttgcctttgcggcagcggggccacaggcagagcagatcatctctgatccattgcccctgccacctcactcgcctgcaagcccggtcgcccgtgtccatgaactcgatgggcaggtacttctcctcggcgtgggacacgatgccaacacgacgctgcatcttgccgagttgatggcaaaggttccctatggggtgccgagacactgcaccattcttcaggatggcaagttggtacgcgtcgattatctcgagaatgaccactgctgtgagcgctttgccttggcggacaggtggctcaaggagaagagccttcagaaggaaggtccagtcggtcatgcctttgctcggttgatccgctcccgcgacattgtggcgacagccctgggtcaactgggccgagatccgttgatcttcctgcatccgccagaggcgggatgcgaagaatgcgatgccgctcgccagtcgattggctgagctcatgagcggagaacgagatgacgttggaggggcaaggtcgcgctgattgctggggcaacacgtgaaaggcgagatcaccaaggtagtcggcaaataatgtctaacggtacccggggatcctctagagtcgacctgcataatgtgcctgtcaaatggacgaagcagggattctgcaaaccctatgctactccgtcaagccgtcaattgtctgattcgttaccaattatgacaacttgacggctacatcattcactttttcttcacaaccggcacggaactcgctcgggctggccccggtgcattttttaaatacccgcgagaaatagagttgatcgtcaaaaccaacattgcgaccgacggtggcgataggcatccgggtggtgctcaaaagcagcttcgcctggctgatacgttggtcctcgcgccagcttaagacgctaatccctaactgctggcggaaaagatgtgacagacgcgacggcgacaagcaaacatgctgtgcgacgctggcgatatcaaaattgctgtctgccaggtgatcgctgatgtactgacaagcctcgcgtacccgattatccatcggtggatggagcgactcgttaatcgcttccatgcgccgcagtaacaattgctcaagcagatttatcgccagcagctccgaatagcgcccttccccttgcccggcgttaatgatttgcccaaacaggtcgctgaaatgcggctggtgcgcttcatccgggcgaaagaaccccgtattggcaaatattgacggccagttaagccattcatgccagtaggcgcgcggacgaaagtaaacccactggtgataccattcgcgagcctccggatgacgaccgtagtgatgaatctctcctggcgggaacagcaaaatatcacccggtcggcaaacaaattctcgtccctgatttttcaccaccccctgaccgcgaatggtgagattgagaatataacctttcattcccagcggtcggtcgataaaaaaatcgagataaccgttggcctcaatcggcgttaaacccgccaccagatgggcattaaacgagtatcccggcagcaggggatcattttgcgcttcagccatacttttcatactcccgccattcagagaagaaaccaattgtccatattgcatcagacattgccgtcactgcgtcttttactggctcttctcgctaaccaaaccggtaaccccgcttattaaaagcattctgtaacaaagcgggaccaaagccatgacaaaaacgcgtaacaaaagtgtctataatcacggcagaaaagtccacattgattatttgcacggcgtcacactttgctatgccatagcatttttatccataagattagcggatcctacctgacgctttttatcgcaactctctactgtttctccatacccgtttttttgggctagcgaaaagatgtttcgtgaagccgtcgacgcttataaaaaatggatattaatactgaaactgagatcaagcaaaagcattcactaaccccctttcctgttttcctaatcagcccggcatttcgcgggcgatattttcacagctatttcaggagttcagccatgaacgcttattacattcaggatcgtcttgaggctcagagctgggcgcgtcactaccagcagctcgcccgtgaagagaaagaggcagaactggcagacgacatggaaaaaggcctgccccagcacctgtttgaatcgctatgcatcgatcatttgcaacgccacggggccagcaaaaaatccattacccgtgcgtttgatgacgatgttgagtttcaggagcgcatggcagaacacatccggtacatggttgaaaccattgctcaccaccaggttgatattgattcagaggtataaaacgaatgagtactgcactcgcaacgctggctgggaagctggctgaacgtgtcggcatggattctgtcgacccacaggaactgatcaccactcttcgccagacggcatttaaaggtgatgccagcgatgcgcagttcatcgcattactgatcgttgccaaccagtacggccttaatccgtggacgaaagaaatttacgcctttcctgataagcagaatggcatcgttccggtggtgggcgttgatggctggtcccgcatcatcaatgaaaaccagcagtttgatggcatggactttgagcaggacaatgaatcctgtacatgccggatttaccgcaaggaccgtaatcatccgatctgcgttaccgaatggatggatgaatgccgccgcgaaccattcaaaactcgcgaaggcagagaaatcacggggccgtggcagtcgcatcccaaacggatgttacgtcataaagccatgattcagtgtgcccgtctggccttcggatttgctggtatctatgacaaggatgaagccgagcgcattgtcgaaaatactgcatacactgcagaacgtcagccggaacgcgacatcactccggttaacgatgaaaccatgcaggagattaacactctgctgatcgccctggataaaacatgggatgacgacttattgccgctctgttcccagatatttcgccgcgacattcgtgcatcgtcagaactgacacaggccgaagcagtaaaagctcttggattcctgaaacagaaagccgcagagcagaaggtggcagcatgacaccggacattatcctgcagcgtaccgggatcgatgtgagagctgtcgaacagggggatgatgcgtggcacaaattacggctcggcgtcatcaccgcttcagaagttcacaacgtgatagcaaaaccccgctccggaaagaagtggcctgacatgaaaatgtcctacttccacaccctgcttgctgaggtttgcaccggtgtggctccggaagttaacgctaaagcactggcctggggaaaacagtacgagaacgacgccagaaccctgtttgaattcacttccggcgtgaatgttactgaatccccgatcatctatcgcgacgaaagtatgcgtaccgcctgctctcccgatggtttatgcagtgacggcaacggccttgaactgaaatgcccgtttacctcccgggatttcatgaagttccggctcggtggtttcgaggccataaagtcagcttacatggcccaggtgcagtacagcatgtgggtgacgcgaaaaaatgcctggtactttgccaactatgacccgcgtatgaagcgtgaaggcctgcattatgtcgtgattgagcgggatgaaaagtacatggcgagttttgacgagatcgtgccggagttcatcgaaaaaatggacgaggcactggctgaaattggttttgtatttggggagcaatggcgatgacgcatcctcacgataataagcttcctgctgaacatcaaaggcaagaaaacatctgttgtcaaagacagcatccttgaacaaggacaattaacagttaacaaataaaaacgcaaaagaaaatgccgatattgactaccggaagcagtgtgaccgtgtgcttctcaaatgcctgattcaggctgtctatgtgtgactgttgagctgtaacaagttgtctcaggtgttcaatttcatgttctagttgctttgttttactggtttcacctgttctattaggtgttacatgctgttcatctgttacattgtcgatctgttcatggtgaacagctttaaatgcaccaaaaactcgtaaaagctctgatgtatctatcttttttacaccgttttcatctgtgcatatagctatactgatttcgtcagactcacagtcaaacatgccggtcagttggcctggtgatggcgggatcgttgtatatttcttgacaccttttcggcaccgccctaaaattctgcgtcctcataatatatgaggcgatttattacgtgtttacgaagcaaaagctaaaaccaggagctatttaatgcccctgaacggatggacgatgctggcgcaggaggaggtgcgagcgatgacgactaccacgggtaccgacctggccccgaggctgcgcgcgttcaagcaccgcctggaccccaaccccgcccaggccaccctgctggcccagtacgccggcgccgcgcgcgtggcctacaacatgctcatcgcccacaaccgggccgccctggccgccggtgccgcccgtcgcaccgagctggccgagagcgggctggccggccccgagctggccgcgcgcatgaaggccgagcgcgccgccgaccccaccctccgcgtggccagctaccagtcgtactccacggcccacctgactccgctgatccgccgccaccgtgaggctgccgccgcgatcgccgccggtgccgacccggccgaggcatggaccgacgagcgatacgccgagccctggatgcacaccgtgccccgccgcgtcctggtctccggcctccagaacgccgcgaaggccaccgagaactggatggcctccgcctccggcacgcgcgccggcgcgcgcgtcggcctgccgcggttcaagaagaagggccggtcccgggacagcttcaccatccccgcccccgaggtcatcggcgccgcgggcaccccctacaagcgcggcgagcaccgccgcggggtgatcaccgaccaccggcacctgcgcctggcctccctggggaccatccgcacctacgacaagaccagccgcctggtccgcgcctgccgccgcggcgcccagatccggtccatgaccatctcccaggctggcggacggtggtacgcctcgatcctcgttgccgaccccacccccatccggaccgggcccagccgtcgccagcgcgccaacggcgccgtcggcgtggacctgggcgtcaagcacctggccgccctctccaccggcgaggtcatcgacaacggccgccccggtgcccgccaggccgcccgcctgacccgtctccagcgcgcctacgcccgcacccagcccggctcgaaccgccgcgagcgcgtgcgccggcagatcgcggcactccatcacgggatcgcactacgtcgggcggggctgctgcatcaggtgtccacgagactggcgatggacttcgcggtggtcgccctggaggacctgaacgtggcggggatgacccgttcggcccgcgggacgctcgaggcgccgggtaggaacgtggccgccaagtccgggttgaaccgggcgatcctggatgccgggctggggatgctgcgccggcagctggactacaagacctcctgggcagggtcccaggtgaagatgatcgaccgattcgcgccctcctcgaaggcgtgctcgcgctgcgggacagtcaaatccacgctgtccctggccgagcggaccttcgagtgcgaggcctgccacctggtgatcgaccgcgacgtgaacgccgcgatcaacatccgggcgtgggctgtgcaggaggagcgtagagcaggggtcgagctcgcccgaggccgtcgggagagtcgaaacggacgtggagctgctgtctcgggcccgccatctggcggggccgcggggcaggggcgtggaagcgtcaagcccgcaccccagggtgtgggcatgtccagccgggcaactggctggtcatcccaacccccctcaaccgaaggggaaagcgcagagcgcggagcatccgccctggccaggtagtggaagccccgcgcacgcagggatgagccttgtcctcttcctctttagcgggccggcatggtcccagcctcctcgctggcgccggctgggcaacatgcttcggcatggcgaatgggacccaattattgaacaccctaacgggtgtttttttgtttctggtctacc

SEQ ID NO: 149 - DNA, 8037 bp, synthetic construct
  source 1..8037: mol_type = other DNA
tttccataggctccgcccccctgacaagcatcacgaaatctgacgctcaaatcagtggtggcgaaacccgacaggactataaagataccaggcgtttccccctggcggctccctcgtgcgctctcctgttcctgcctttcggtttaccggtgtcattccgctgttatggccgcgtttgtctcattccacgcctgacactcagttccgggtaggcagttcgctccaagctggactgtatgcacgaaccccccgttcagtccgaccgctgcgccttatccggtaactatcgtcttgagtccaacccggaaagacatgcaaaagcaccactggcagcagccactggtaattgatttagaggagttagtcttgaagtcatgcgccggttaaggctaaactgaaaggacaagttttggtgactgcgctcctccaagccagttacctcggttcaaagagttggtagctcagagaaccttcgaaaaaccgccctgcaaggcggttttttcgttttcagagcaagagattacgcgcagaccaaaacgatctcaagaagatcatcttattaatcagataaaatatttctagatttcagtgcaatttatctcttcaaatgtagcacctgaagtcagccccatacgatataagttgtgacgtaaaatgagacgttgatcggcacgtaagaggttccaactttcaccataatgaaataagatcactaccgggcgtattttttgagttatcgagattttcaggagctaaggaagctaaaatggagaaaaaaatcactggatataccaccgttgatatatcccaatggcatcgtaaagaacattttgaggcatttcagtcagttgctcaatgtacctataaccagaccgttcagctgggtcatccaccggatcaattcccctgctcgcgcaggctgggtgccaagctctcgggtaacatcaaggcccgatccttggagcccttgccctcccgcacgatgatcgtgccgtgatcgaaatccagatccttgacccgcagttgcaaaccctcactgatccggctcacggtaactgatgccgtatttgcagtaccagcgtacggcccacagaatgatgtcacgctgaaaatgccggcctttgaatgggttcatgtgcagctccatcagcaaaaggggatgataagtttatcaccaccgactatttgcaacagtgccgttgatcgtgctatgatcgactgatgtcatcagcggtggagtgcaatgtcgtgcaatacgaatggcgaaaagccgagctcatcggtcagcttctcaaccttggggttacccccggcggtgtgctgctggtccacagctccttccgtagcgtccggcccctcgaagatgggccacttggactgatcgaggccctgcgtgctgcgctgggtccgggagggacgctcgtcatgccctcgtggtcaggtctggacgacgagccgttcgatcctgccacgtcgcccgttacaccggaccttggagttgtctctgacacattctggcgcctgccaaatgtaaagcgcagcgcccatccatttgcctttgcggcagcggggccacaggcagagcagatcatctctgatccattgcccctgccacctcactcgcctgcaagcccggtcgcccgtgtccatgaactcgatgggcaggtacttctcctcggcgtgggacacgatgccaacacgacgctgcatcttgccgagttgatggcaaaggttccctatggggtgccgagacactgcaccattcttcaggatggcaagttggtacgcgtcgattatctcgagaatgaccactgctgtgagcgctttgccttggcggacaggtggctcaaggagaagagccttcagaaggaaggtccagtcggtcatgcctttgctcggttgatccgctcccgcgacattgtggcgacagccctgggtcaactgggccgagatccgttgatcttcctgcatccgccagaggcgggatgcgaagaatgcgatgccgctcgccagtcgattggctgagctcatgagcggagaacgagatgacgttggaggggcaaggtcgcgctgattgctggggcaacacgtgaaaggcgagatcaccaaggtagtcggcaaataatgtctaacggtacccggggatcctctagagtcgacctgcataatgtgcctgtcaaatggacgaagcagggattctgcaaaccctatgctactccgtcaagccgtcaattgtctgattcgttaccaattatgacaacttgacggctacatcattcactttttcttcacaaccggcacggaactcgctcgggctggccccggtgcattttttaaatacccgcgagaaatagagttgatcgtcaaaaccaacattgcgaccgacggtggcgataggcatccgggtggtgctcaaaagcagcttcgcctggctgatacgttggtcctcgcgccagcttaagacgctaatccctaactgctggcggaaaagatgtgacagacgcgacggcgacaagcaaacatgctgtgcgacgctggcgatatcaaaattgctgtctgccaggtgatcgctgatgtactgacaagcctcgcgtacccgattatccatcggtggatggagcgactcgttaatcgcttccatgcgccgcagtaacaattgctcaagcagatttatcgccagcagctccgaatagcgcccttccccttgcccggcgttaatgatttgcccaaacaggtcgctgaaatgcggctggtgcgcttcatccgggcgaaagaaccccgtattggcaaatattgacggccagttaagccattcatgccagtaggcgcgcggacgaaagtaaacccactggtgataccattcgcgagcctccggatgacgaccgtagtgatgaatctctcctggcgggaacagcaaaatatcacccggtcggcaaacaaattctcgtccctgatttttcaccaccccctgaccgcgaatggtgagattgagaatataacctttcattcccagcggtcggtcgataaaaaaatcgagataaccgttggcctcaatcggcgttaaacccgccaccagatgggcattaaacgagtatcccggcagcaggggatcattttgcgcttcagccatacttttcatactcccgccattcagagaagaaaccaattgtccatattgcatcagacattgccgtcactgcgtcttttactggctcttctcgctaaccaaaccggtaaccccgcttattaaaagcattctgtaacaaagcgggaccaaagccatgacaaaaacgcgtaacaaaagtgtctataatcacggcagaaaagtccacattgattatttgcacggcgtcacactttgctatgccatagcatttttatccataagattagcggatcctacctgacgctttttatcgcaactctctactgtttctccatacccgtttttttgggctagcgaaaagatgtttcgtgaagccgtcgacgcttataaaaaatggatattaatactgaaactgagatcaagcaaaagcattcactaaccccctttcctgttttcctaatcagcccggcatttcgcgggcgatattttcacagctatttcaggagttcagccatgaacgcttattacattcaggatcgtcttgaggctcagagctgggcgcgtcactaccagcagctcgcccgtgaagagaaagaggcagaactggcagacgacatggaaaaaggcctgccccagcacctgtttgaatcgctatgcatcgatcatttgcaacgccacggggccagcaaaaaatccattacccgtgcgtttgatgacgatgttgagtttcaggagcgcatggcagaacacatccggtacatggttgaaaccattgctcaccaccaggttgatattgattcagaggtataaaacgaatgagtactgcactcgcaacgctggctgggaagctggctgaacgtgtcggcatggattctgtcgacccacaggaactgatcaccactcttcgccagacggcatttaaaggtgatgccagcgatgcgcagttcatcgcattactgatcgttgccaaccagtacggccttaatccgtggacgaaagaaatttacgcctttcctgataagcagaatggcatcgttccggtggtgggcgttgatggctggtcccgcatcatcaatgaaaaccagcagtttgatggcatggactttgagcaggacaatgaatcctgtacatgccggatttaccgcaaggaccgtaatcatccgatctgcgttaccgaatggatggatgaatgccgccgcgaaccattcaaaactcgcgaaggcagagaaatcacggggccgtggcagtcgcatcccaaacggatgttacgtcataaagccatgattcagtgtgcccgtctggccttcggatttgctggtatctatgacaaggatgaagccgagcgcattgtcgaaaatactgcatacactgcagaacgtcagccggaacgcgacatcactccggttaacgatgaaaccatgcaggagattaacactctgctgatcgccctggataaaacatgggatgacgacttattgccgctctgttcccagatatttcgccgcgacattcgtgcatcgtcagaactgacacaggccgaagcagtaaaagctcttggattcctgaaacagaaagccgcagagcagaaggtggcagcatgacaccggacattatcctgcagcgtaccgggatcgatgtgagagctgtcgaacagggggatgatgcgtggcacaaattacggctcggcgtcatcaccgcttcagaagttcacaacgtgatagcaaaaccccgctccggaaagaagtggcctgacatgaaaatgtcctacttccacaccctgcttgctgaggtttgcaccggtgtggctccggaagttaacgctaaagcactggcctggggaaaacagtacgagaacgacgccagaaccctgtttgaattcacttccggcgtgaatgttactgaatccccgatcatctatcgcgacgaaagtatgcgtaccgcctgctctcccgatggtttatgcagtgacggcaacggccttgaactgaaatgcccgtttacctcccgggatttcatgaagttccggctcggtggtttcgaggccataaagtcagcttacatggcccaggtgcagtacagcatgtgggtgacgcgaaaaaatgcctggtactttgccaactatgacccgcgtatgaagcgtgaaggcctgcattatgtcgtgattgagcgggatgaaaagtacatggcgagttttgacgagatcgtgccggagttcatcgaaaaaatggacgaggcactggctgaaattggttttgtatttggggagcaatggcgatgacgcatcctcacgataataagcttcctgctgaacatcaaaggcaagaaaacatctgttgtcaaagacagcatccttgaacaaggacaattaacagttaacaaataaaaacgcaaaagaaaatgccgatattgactaccggaagcagtgtgaccgtgtgcttctcaaatgcctgattcaggctgtctatgtgtgactgttgagctgtaacaagttgtctcaggtgttcaatttcatgttctagttgctttgttttactggtttcacctgttctattaggtgttacatgctgttcatctgttacattgtcgatctgttcatggtgaacagctttaaatgcaccaaaaactcgtaaaagctctgatgtatctatcttttttacaccgttttcatctgtgcatatagctatactgatttcgtcagactcacagtcaaacatgccggtcagttggcctggtgatggcgggatcgttgtatatttcttgacaccttttcggcaccgccctaaaattctgcgtcctcataatatatgaggcgatttattacgtgtttacgaagcaaaagctaaaaccaggagctatttaatggtgcagacggagatcctgaaggcgtttcggtttgcgttggatccgacgtctgtgcaggttgctgccctttcccggcatgctggtgcggccaggtgggcgttcaaccatgctctcgcggccaaggtcggcgcgcatgagcggtggcgggcggaggtagccaagcttgtcggggacggtgttcctgaggagcaggctcgtaggcaggtgcgcgtcccggttccgatgaagccggcgatccagaaggcgttgaacgcggtcaagggtgactctcgcaagggcttggatggtgcgtgcccgtggtggcatgaggtcaacacttacgcgttccagtccgctttcatcgacgcggaccaggcgtggaagaactggttggactcgttgtcggggaagcgggtcggccgccgggtggggtacccgcggttcaagaagaaggggcgggcccgcgactcgtttcgcttgcaccacgacgtgaagaagccaagcatccggctggccgggtaccggcggttgcggctgccgaggatcggggaagtccggcttcatgactcggggaagcgtctggcacggctgatcgaccgaggtgacgcggtggtgcagtcggtgacggtgtcgcggggtggccatcgctggtatgcgtctgtgctgtgcaaggtcaccgtgcaggtaccggatcggccgtcacggcgccagcgggaacgaggcgctgttggggtggaccttggcgttaaggtcctcgcggctttgtccaagccactggtggtcgacgacccgtcgagtgccctggtgcggaatccgcagcatctgcggcaggccgagcggcgtctactgaaggctcagcgggcgttggcgcgtacacaaaaaggttcagcccgacgcgagaaggccaagcggcgagttggtcgcgcgcatcacgaggttgctgtgcgccggcatgctgcgctccatcagatcaccaagcgcctgaccaccggcttcgcggtcgtcgcgcttgaggatctgaacgtggccggtatgacaaggtcagcgcggggaacagtggcagcgccgggaaagaacgtgcggcagaaggcaggcctgaaccgcgtcatcctggactccgctccagccgagttgcgtcgccaggtgaactacaaggccacctggtatggatctgagctggcggtcgcagaccgctggttcccctcgagtaagacctgttcgggttgcggatggcaaaacccacacctgaagctgtccgacagggtgtttcgttgcacagactgcgggctggtgatggaccgggacatgaacgcggcccggaacatcgaacgccacgcagtgctgatcgatcgaaacgtcgcctgcgataggcgggagacgctaaacgcccgtggagcatccataagaccaaccacctctcggggcggtaggcacgacgcatcgaagcgggaaggctccggcgctcggcctgagtcacctcagcagagtgatctgctgacgctcccaaccttgaataacgaaacggcaacgcctccatagcggtgcaggtcaataaggtggctggttggcgtactgttgtggtaaatacccatatggacagttttccctttgatatgtaacggtgaacagttgttctacttttgtttgttagtcttgatgcttcactgatagatacaagagcgtcgggtgatgctgccaacttactgatttagtgtatgatggtgtttttgaggtgctccagtggcttctgtttctatcagctgtccctcctgttcagctactgacggggtggtgcgtaacggcaaaagcaccgccggacatcagcgctagcggagtgtatactggcttactatgttggcactgatgagggtgtcagtgaagtgcttcatgtggcaggagaaaaaaggctgcaccggtgcgtcagcagaatatgtgatacaggatatattccgcttcctcgctcactgactcgctacgctcggtcgttcgactgcggcgagcggaaatggcttacgaacggggcggagatttcctggaagatgccaggaagatacttaacagggaagtgagagggccgcggcaaagccgtt

SEQ ID NO: 150 - DNA, 41 bp, synthetic construct
  source 1..41: mol_type = other DNA
tcatctgtgcatatagctatactgatttcgtcagactcaca

SEQ ID NO: 151 - DNA, 36 bp, synthetic construct
  source 1..36: mol_type = other DNA
cgccaaccagccaccttattgacctgcaccgctatg

SEQ ID NO: 152 - DNA, 33 bp, synthetic construct
  source 1..33: mol_type = other DNA
caggtcaataaggtggctggttggcgtactgtt

SEQ ID NO: 153 - DNA, 43 bp, synthetic construct
  source 1..43: mol_type = other DNA
atcagtatagctatatgcacagatgaaaacggtgtaaaaaaga

SEQ ID NO: 154 - DNA, 5040 bp, synthetic construct
  source 1..5040: mol_type = other DNA
tcgcgcgtttcggtgatgacggtgaaaacctctgacacatgcagctcccggagacggtcacagcttgtctgtaagcggatgccgggagcagacaagcccgtcagggcgcgtcagcgggtgttggcgggtgtcggggctggcttaactatgcggcatcagagcagattgtactgagagtgcaccatatgcggtgtgaaataccgcacagatgcgtaaggagaaaataccgcatcaggcgccattcgccattcaggctgcgcaactgttgggaagggcgatcggtgcgggcctcttcgctattacgccagctggcgaaagggggatgtgctgcaaggcgattaagttgggtaacgccagggttttcccagtcacgacgttgtaaaacgacggccagtgaattgacgcgtattgggatggtaccgggccccccctcgaggtcgacggtatcgatacggcatcagagcagattgtactgagagtgcaccataatcggcattttcttttgcgtttttatttgttaactgttaattgtccttgttcaaggatgctgtctttgacaacagatgttttcttgcctttgatgttcagcaggaagctaggcgcaaacgttgattgtttgtctgcgtagaatcctctgtttgtcatatagcttgtaatcacgacattgtttcctttcgcttgaggtacagcgaagtgtgagtaagtaaaggttacatcgttaggatcaagatccatttttaacacaaggccagttttgttcagcggcttgtatgggccagttaaagaattagaaacataaccaagcatgtaaatatcgttagacgtaatgccgtcaatcgtcatttttgatccgcgggagtcagtgaacagataccatttgccgttcattttaaagacgttcgcgcgttcaatttcatctgttactgtgttagatgcaatcagcggtttcatcacttttttcagtgtgtaatcatcgtttagctcaatcataccgagagcgccgtttgctaactcagccgtgcgttttttatcgctttgcagaagtttttgactttcttgacggaagaatgatgtgcttttgccatagtatgctttgttaaataaagattcttcgccttggtagccatcttcagttccagtgtttgcttcaaatactaagtatttgtggcctttatcttctacgtagtgaggatctctcagcgtatggttgtcgcctgagctgtagttgccttcatcgatgaactgctgtacattttgatacgtttttccgtcaccgtcaaagattgatttataatcctctacaccgttgatgttcaaagagctgtctgatgctgatacgttaacttgtgcagttgtcagtgtttgtttgccgtaatgtttaccggagaaatcagtgtagaataaacggatttttccgtcagatgtaaatgtggctgaacctgaccattcttgtgtttggtcttttaggatagaatcatttgcatcgaatttgtcgctgtctttaaagacgcggccagcgtttttccagctgtcaatagaagtttcgccgactttttgatagaacatgtaaatcgatgtgtcatccgcatttttaggatctccggctaatgcaaagacgatgtggtagccgtgatagtttgcgacagtgccgtcagcgttttgtaatggccagctgtcccaaacgtccaggccttttgcagaagagatatttttaattgtggacgaatcgaactcaggaacttgatatttttcatttttttgctgttcagggatttgcagcatatcatggcgtgtaatatgggaaatgccgtatgtttccttatatggcttttggttcgtttctttcgcaaacgcttgagttgcgcctcctgccagcagtgcggtagtaaaggttaatactgttgcttgttttgcaaactttttgatgttcatcgttcatgtctccttttttatgtactgtgttagcggtctgcttcttccagccctcctgtttgaagatggcaagttagttacgcacaataaaaaaagacctaaaatatgtaaggggtgacgccaaagtatacactttgccctttacacattttaggtcttgcctgctttatcagtaacaaacccgcgcgatttacttttcgacctcattctattagactctcgtttggattgcaactggtctattttcctcttttgtttgatagaaaatcataaaaggatttgcagactacgggcctaaagaactaaaaaatctatctgtttcttttcattctctgtattttttatagtttctgttgcatgggcataaagttgcaagcttgatatcttgacagctagctcagtcctaggtataatactagtgaacgcggcccggaacatcgaacgccacgcagtgctgatcgatcgaaacgtcgcctgcgataggcgggagacgctaaacgcccgtggagcatccataagaccaaccacctctcggggcggtaggcacgacgcatcgaagcgggaaggctccggcgctcggcctgagtcacctcagcagagtgatctgctgacgctcccaaccttgaataacgaaacggcaacgcctccatagcggtgcaggtcaataagggtcggccccacgcgtgtagggagcgatcgcgagaccattggtctcaggccggcatggtcccagcctcctcgctggcgccggctgggcaacatgcttcggcatggcgaatgggacccaattattgaacaccctaacgggtgtttttttgtttctggtctaccgatatcgaattcctgcagcccgggggatccactagttctagagcggccgccaccgcggtggagctcatcccaatggcgcgccgagcttggctcgagcatggtcatagctgtttcctgtgtgaaattgttatccgctcacaattccacacaacatacgagccggaagcataaagtgtaaagcctggggtgcctaatgagtgagctaactcacattaattgcgttgcgctcactgcccgctttccagtcgggaaacctgtcgtgccagctgcattaatgaatcggccaacgcgcggggagaggcggtttgcgtattgggcgctcttccgcttcctcgctcactgactcgctgcgctcggtcgttcggctgcggcgagcggtatcagctcactcaaaggcggtaatacggttatccacagaatcaggggataacgcaggaaagaacatgtgagcaaaaggccagcaaaaggccaggaaccgtaaaaaggccgcgttgctggcgtttttccataggctccgcccccctgacgagcatcacaaaaatcgacgctcaagtcagaggtggcgaaacccgacaggactataaagataccaggcgtttccccctggaagctccctcgtgcgctctcctgttccgaccctgccgcttaccggatacctgtccgcctttctcccttcgggaagcgtggcgctttctcatagctcacgctgtaggtatctcagttcggtgtaggtcgttcgctccaagctgggctgtgtgcacgaaccccccgttcagcccgaccgctgcgccttatccggtaactatcgtcttgagtccaacccggtaagacacgacttatcgccactggcagcagccactggtaacaggattagcagagcgaggtatgtaggcggtgctacagagttcttgaagtggtggcctaactacggctacactagaagaacagtatttggtatctgcgctctgctgaagccagttaccttcggaaaaagagttggtagctcttgatccggcaaacaaaccaccgctggtagcggtggtttttttgtttgcaagcagcagattacgcgcagaaaaaaaggatctcaagaagatcctttgatcttttctacggggtctgacgctcagtggaacgaaaactcacgttaagggattttggtcatgagattatcaaaaaggatcttcacctagatccttttaaattaaaaatgaagttttaaatcaatctaaagtatatatgagtaaacttggtctgacagttagaaaaactcatcgagcatcaaatgaaactgcaatttattcatatcaggattatcaataccatatttttgaaaaagccgtttctgtaatgaaggagaaaactcaccgaggcagttccataggatggcaagatcctggtatcggtctgcgattccgactcgtccaacatcaatacaacctattaatttcccctcgtcaaaaataaggttatcaagtgagaaatcaccatgagtgacgactgaatccggtgagaatggcaaaagtttatgcatttctttccagacttgttcaacaggccagccattacgctcgtcatcaaaatcactcgcatcaaccaaaccgttattcattcgtgattgcgcctgagcgagacgaaatacgcgatcgctgttaaaaggacaattacaaacaggaatcgaatgcaaccggcgcaggaacactgccagcgcatcaacaatattttcacctgaatcaggatattcttctaatacctggaatgctgttttcccagggatcgcagtggtgagtaaccatgcatcatcaggagtacggataaaatgcttgatggtcggaagaggcataaattccgtcagccagtttagtctgaccatctcatctgtaacatcattggcaacgctacctttgccatgtttcagaaacaactctggcgcatcgggcttcccatacaatcgatagattgtcgcacctgattgcccgacattatcgcgagcccatttatacccatataaatcagcatccatgttggaatttaatcgcggcctagagcaagacgtttcccgttgaatatggctcatactcttcctttttcaatattattgaagcatttatcagggttattgtctcatgagcggatacatatttgaatgtatttagaaaaataaacaaataggggttccgcgcacatttccccgaaaagtgccacctgacgtctaagaaaccattattatcatgacattaacctataaaaataggcgtatcacgaggccctttcgtc

SEQ ID NO: 155 - DNA, 496 bp, synthetic construct
  source 1..496: mol_type = other DNA
ggcataaagttgcaagcttgatatcttgacagctagctcagtcctaggtataatactagtgaacgcggcccggaacatcgaacgccacgcagtgctgatcgatcgaaacgtcgcctgcgataggcgggagacgctaaacgcccgtggagcatccataagaccaaccacctctcggggcggtaggcacgacgcatcgaagcgggaaggctccggcgctcggcctgagtcacctcagcagagtgatctgctgacgctcccaaccttgaataacgaaacggcaacgcctccatagcggtgcaggtcaataagggtcggccccacgcgtgtagggagcgatcgcgagaccattggtctcaggccggcatggtcccagcctcctcgctggcgccggctgggcaacatgcttcggcatggcgaatgggacccaattattgaacaccctaacgggtgtttttttgtttctggtctaccgatatcgaattcctgcagcccgggg

SEQ ID NO: 156 - DNA, 4594 bp, synthetic construct
  source 1..4594: mol_type = other DNA
gatatcgaattcctgcagcccgggggatccactagttctagagcggccgccaccgcggtggagctcatcccaatggcgcgccgagcttggctcgagcatggtcatagctgtttcctgtgtgaaattgttatccgctcacaattccacacaacatacgagccggaagcataaagtgtaaagcctggggtgcctaatgagtgagctaactcacattaattgcgttgcgctcactgcccgctttccagtcgggaaacctgtcgtgccagctgcattaatgaatcggccaacgcgcggggagaggcggtttgcgtattgggcgctcttccgcttcctcgctcactgactcgctgcgctcggtcgttcggctgcggcgagcggtatcagctcactcaaaggcggtaatacggttatccacagaatcaggggataacgcaggaaagaacatgtgagcaaaaggccagcaaaaggccaggaaccgtaaaaaggccgcgttgctggcgtttttccataggctccgcccccctgacgagcatcacaaaaatcgacgctcaagtcagaggtggcgaaacccgacaggactataaagataccaggcgtttccccctggaagctccctcgtgcgctctcctgttccgaccctgccgcttaccggatacctgtccgcctttctcccttcgggaagcgtggcgctttctcatagctcacgctgtaggtatctcagttcggtgtaggtcgttcgctccaagctgggctgtgtgcacgaaccccccgttcagcccgaccgctgcgccttatccggtaactatcgtcttgagtccaacccggtaagacacgacttatcgccactggcagcagccactggtaacaggattagcagagcgaggtatgtaggcggtgctacagagttcttgaagtggtggcctaactacggctacactagaagaacagtatttggtatctgcgctctgctgaagccagttaccttcggaaaaagagttggtagctcttgatccggcaaacaaaccaccgctggtagcggtggtttttttgtttgcaagcagcagattacgcgcagaaaaaaaggatctcaagaagatcctttgatcttttctacggggtctgacgctcagtggaacgaaaactcacgttaagggattttggtcatgagattatcaaaaaggatcttcacctagatccttttaaattaaaaatgaagttttaaatcaatctaaagtatatatgagtaaacttggtctgacagttagaaaaactcatcgagcatcaaatgaaactgcaatttattcatatcaggattatcaataccatatttttgaaaaagccgtttctgtaatgaaggagaaaactcaccgaggcagttccataggatggcaagatcctggtatcggtctgcgattccgactcgtccaacatcaatacaacctattaatttcccctcgtcaaaaataaggttatcaagtgagaaatcaccatgagtgacgactgaatccggtgagaatggcaaaagtttatgcatttctttccagacttgttcaacaggccagccattacgctcgtcatcaaaatcactcgcatcaaccaaaccgttattcattcgtgattgcgcctgagcgagacgaaatacgcgatcgctgttaaaaggacaattacaaacaggaatcgaatgcaaccggcgcaggaacactgccagcgcatcaacaatattttcacctgaatcaggatattcttctaatacctggaatgctgttttcccagggatcgcagtggtgagtaaccatgcatcatcaggagtacggataaaatgcttgatggtcggaagaggcataaattccgtcagccagtttagtctgaccatctcatctgtaacatcattggcaacgctacctttgccatgtttcagaaacaactctggcgcatcgggcttcccatacaatcgatagattgtcgcacctgattgcccgacattatcgcgagcccatttatacccatataaatcagcatccatgttggaatttaatcgcggcctagagcaagacgtttcccgttgaatatggctcatactcttcctttttcaatattattgaagcatttatcagggttattgtctcatgagcggatacatatttgaatgtatttagaaaaataaacaaataggggttccgcgcacatttccccgaaaagtgccacctgacgtctaagaaaccattattatcatgacattaacctataaaaataggcgtatcacgaggccctttcgtctcgcgcgtttcggtgatgacggtgaaaacctctgacacatgcagctcccggagacggtcacagcttgtctgtaagcggatgccgggagcagacaagcccgtcagggcgcgtcagcgggtgttggcgggtgtcggggctggcttaactatgcggcatcagagcagattgtactgagagtgcaccatatgcggtgtgaaataccgcacagatgcgtaaggagaaaataccgcatcaggcgccattcgccattcaggctgcgcaactgttgggaagggcgatcggtgcgggcctcttcgctattacgccagctggcgaaagggggatgtgctgcaaggcgattaagttgggtaacgccagggttttcccagtcacgacgttgtaaaacgacggccagtgaattgacgcgtattgggatggtaccgggccccccctcgaggtcgacggtatcgatacggcatcagagcagattgtactgagagtgcaccataatcggcattttcttttgcgtttttatttgttaactgttaattgtccttgttcaaggatgctgtctttgacaacagatgttttcttgcctttgatgttcagcaggaagctaggcgcaaacgttgattgtttgtctgcgtagaatcctctgtttgtcatatagcttgtaatcacgacattgtttcctttcgcttgaggtacagcgaagtgtgagtaagtaaaggttacatcgttaggatcaagatccatttttaacacaaggccagttttgttcagcggcttgtatgggccagttaaagaattagaaacataaccaagcatgtaaatatcgttagacgtaatgccgtcaatcgtcatttttgatccgcgggagtcagtgaacagataccatttgccgttcattttaaagacgttcgcgcgttcaatttcatctgttactgtgttagatgcaatcagcggtttcatcacttttttcagtgtgtaatcatcgtttagctcaatcataccgagagcgccgtttgctaactcagccgtgcgttttttatcgctttgcagaagtttttgactttcttgacggaagaatgatgtgcttttgccatagtatgctttgttaaataaagattcttcgccttggtagccatcttcagttccagtgtttgcttcaaatactaagtatttgtggcctttatcttctacgtagtgaggatctctcagcgtatggttgtcgcctgagctgtagttgccttcatcgatgaactgctgtacattttgatacgtttttccgtcaccgtcaaagattgatttataatcctctacaccgttgatgttcaaagagctgtctgatgctgatacgttaacttgtgcagttgtcagtgtttgtttgccgtaatgtttaccggagaaatcagtgtagaataaacggatttttccgtcagatgtaaatgtggctgaacctgaccattcttgtgtttggtcttttaggatagaatcatttgcatcgaatttgtcgctgtctttaaagacgcggccagcgtttttccagctgtcaatagaagtttcgccgactttttgatagaacatgtaaatcgatgtgtcatccgcatttttaggatctccggctaatgcaaagacgatgtggtagccgtgatagtttgcgacagtgccgtcagcgttttgtaatggccagctgtcccaaacgtccaggccttttgcagaagagatatttttaattgtggacgaatcgaactcaggaacttgatatttttcatttttttgctgttcagggatttgcagcatatcatggcgtgtaatatgggaaatgccgtatgtttccttatatggcttttggttcgtttctttcgcaaacgcttgagttgcgcctcctgccagcagtgcggtagtaaaggttaatactgttgcttgttttgcaaactttttgatgttcatcgttcatgtctccttttttatgtactgtgttagcggtctgcttcttccagccctcctgtttgaagatggcaagttagttacgcacaataaaaaaagacctaaaatatgtaaggggtgacgccaaagtatacactttgccctttacacattttaggtcttgcctgctttatcagtaacaaacccgcgcgatttacttttcgacctcattctattagactctcgtttggattgcaactggtctattttcctcttttgtttgatagaaaatcataaaaggatttgcagactacgggcctaaagaactaaaaaatctatctgtttcttttcattctctgtattttttatagtttctgttgcatgggcataaagttgcaagcttgatatc

SEQ ID NO: 157 - DNA, 5043 bp, synthetic construct
  source 1..5043: mol_type = other DNA
tcgcgcgtttcggtgatgacggtgaaaacctctgacacatgcagctcccggagacggtcacagcttgtctgtaagcggatgccgggagcagacaagcccgtcagggcgcgtcagcgggtgttggcgggtgtcggggctggcttaactatgcggcatcagagcagattgtactgagagtgcaccatatgcggtgtgaaataccgcacagatgcgtaaggagaaaataccgcatcaggcgccattcgccattcaggctgcgcaactgttgggaagggcgatcggtgcgggcctcttcgctattacgccagctggcgaaagggggatgtgctgcaaggcgattaagttgggtaacgccagggttttcccagtcacgacgttgtaaaacgacggccagtgaattgacgcgtattgggatggtaccgggccccccctcgaggtcgacggtatcgatacggcatcagagcagattgtactgagagtgcaccataatcggcattttcttttgcgtttttatttgttaactgttaattgtccttgttcaaggatgctgtctttgacaacagatgttttcttgcctttgatgttcagcaggaagctaggcgcaaacgttgattgtttgtctgcgtagaatcctctgtttgtcatatagcttgtaatcacgacattgtttcctttcgcttgaggtacagcgaagtgtgagtaagtaaaggttacatcgttaggatcaagatccatttttaacacaaggccagttttgttcagcggcttgtatgggccagttaaagaattagaaacataaccaagcatgtaaatatcgttagacgtaatgccgtcaatcgtcatttttgatccgcgggagtcagtgaacagataccatttgccgttcattttaaagacgttcgcgcgttcaatttcatctgttactgtgttagatgcaatcagcggtttcatcacttttttcagtgtgtaatcatcgtttagctcaatcataccgagagcgccgtttgctaactcagccgtgcgttttttatcgctttgcagaagtttttgactttcttgacggaagaatgatgtgcttttgccatagtatgctttgttaaataaagattcttcgccttggtagccatcttcagttccagtgtttgcttcaaatactaagtatttgtggcctttatcttctacgtagtgaggatctctcagcgtatggttgtcgcctgagctgtagttgccttcatcgatgaactgctgtacattttgatacgtttttccgtcaccgtcaaagattgatttataatcctctacaccgttgatgttcaaagagctgtctgatgctgatacgttaacttgtgcagttgtcagtgtttgtttgccgtaatgtttaccggagaaatcagtgtagaataaacggatttttccgtcagatgtaaatgtggctgaacctgaccattcttgtgtttggtcttttaggatagaatcatttgcatcgaatttgtcgctgtctttaaagacgcggccagcgtttttccagctgtcaatagaagtttcgccgactttttgatagaacatgtaaatcgatgtgtcatccgcatttttaggatctccggctaatgcaaagacgatgtggtagccgtgatagtttgcgacagtgccgtcagcgttttgtaatggccagctgtcccaaacgtccaggccttttgcagaagagatatttttaattgtggacgaatcgaactcaggaacttgatatttttcatttttttgctgttcagggatttgcagcatatcatggcgtgtaatatgggaaatgccgtatgtttccttatatggcttttggttcgtttctttcgcaaacgcttgagttgcgcctcctgccagcagtgcggtagtaaaggttaatactgttgcttgttttgcaaactttttgatgttcatcgttcatgtctccttttttatgtactgtgttagcggtctgcttcttccagccctcctgtttgaagatggcaagttagttacgcacaataaaaaaagacctaaaatatgtaaggggtgacgccaaagtatacactttgccctttacacattttaggtcttgcctgctttatcagtaacaaacccgcgcgatttacttttcgacctcattctattagactctcgtttggattgcaactggtctattttcctcttttgtttgatagaaaatcataaaaggatttgcagactacgggcctaaagaactaaaaaatctatctgtttcttttcattctctgtattttttatagtttctgttgcatgggcataaagttgcaagcttgatatcttgacagctagctcagtcctaggtataatactagtgaacgcggcccggaacatcgaacgccacgcagtgctgatcgatcgaaacgtcgcctgcgataggcgggagacgctaaacgcccgtggagcatccataagaccaaccacctctcggggcggtaggcacgacgcatcgaagcgggaaggctccggcgctcggcctgagtcacctcagcagagtgatctgctgacgctcccaaccttgaataacgaaacggcaacgcctccatagcggtgcaggtcaataagggtcggccccacgcgtgtagggagcgatcgtgtttgttaccaactgcctgggccggcatggtcccagcctcctcgctggcgccggctgggcaacatgcttcggcatggcgaatgggacccaattattgaacaccctaacgggtgtttttttgtttctggtctaccgatatcgaattcctgcagcccgggggatccactagttctagagcggccgccaccgcggtggagctcatcccaatggcgcgccgagcttggctcgagcatggtcatagctgtttcctgtgtgaaattgttatccgctcacaattccacacaacatacgagccggaagcataaagtgtaaagcctggggtgcctaatgagtgagctaactcacattaattgcgttgcgctcactgcccgctttccagtcgggaaacctgtcgtgccagctgcattaatgaatcggccaacgcgcggggagaggcggtttgcgtattgggcgctcttccgcttcctcgctcactgactcgctgcgctcggtcgttcggctgcggcgagcggtatcagctcactcaaaggcggtaatacggttatccacagaatcaggggataacgcaggaaagaacatgtgagcaaaaggccagcaaaaggccaggaaccgtaaaaaggccgcgttgctggcgtttttccataggctccgcccccctgacgagcatcacaaaaatcgacgctcaagtcagaggtggcgaaacccgacaggactataaagataccaggcgtttccccctggaagctccctcgtgcgctctcctgttccgaccctgccgcttaccggatacctgtccgcctttctcccttcgggaagcgtggcgctttctcatagctcacgctgtaggtatctcagttcggtgtaggtcgttcgctccaagctgggctgtgtgcacgaaccccccgttcagcccgaccgctgcgccttatccggtaactatcgtcttgagtccaacccggtaagacacgacttatcgccactggcagcagccactggtaacaggattagcagagcgaggtatgtaggcggtgctacagagttcttgaagtggtggcctaactacggctacactagaagaacagtatttggtatctgcgctctgctgaagccagttaccttcggaaaaagagttggtagctcttgatccggcaaacaaaccaccgctggtagcggtggtttttttgtttgcaagcagcagattacgcgcagaaaaaaaggatctcaagaagatcctttgatcttttctacggggtctgacgctcagtggaacgaaaactcacgttaagggattttggtcatgagattatcaaaaaggatcttcacctagatccttttaaattaaaaatgaagttttaaatcaatctaaagtatatatgagtaaacttggtctgacagttagaaaaactcatcgagcatcaaatgaaactgcaatttattcatatcaggattatcaataccatatttttgaaaaagccgtttctgtaatgaaggagaaaactcaccgaggcagttccataggatggcaagatcctggtatcggtctgcgattccgactcgtccaacatcaatacaacctattaatttcccctcgtcaaaaataaggttatcaagtgagaaatcaccatgagtgacgactgaatccggtgagaatggcaaaagtttatgcatttctttccagacttgttcaacaggccagccattacgctcgtcatcaaaatcactcgcatcaaccaaaccgttattcattcgtgattgcgcctgagcgagacgaaatacgcgatcgctgttaaaaggacaattacaaacaggaatcgaatgcaaccggcgcaggaacactgccagcgcatcaacaatattttcacctgaatcaggatattcttctaatacctggaatgctgttttcccagggatcgcagtggtgagtaaccatgcatcatcaggagtacggataaaatgcttgatggtcggaagaggcataaattccgtcagccagtttagtctgaccatctcatctgtaacatcattggcaacgctacctttgccatgtttcagaaacaactctggcgcatcgggcttcccatacaatcgatagattgtcgcacctgattgcccgacattatcgcgagcccatttatacccatataaatcagcatccatgttggaatttaatcgcggcctagagcaagacgtttcccgttgaatatggctcatactcttcctttttcaatattattgaagcatttatcagggttattgtctcatgagcggatacatatttgaatgtatttagaaaaataaacaaataggggttccgcgcacatttccccgaaaagtgccacctgacgtctaagaaaccattattatcatgacattaacctataaaaataggcgtatcacgaggccctttcgtc

SEQ ID NO: 158 - DNA, 20 bp, synthetic construct
  source 1..20: mol_type = other DNA
tgtttgttaccaactgcctg

SEQ ID NO: 159 - DNA, 24 bp, synthetic construct
  source 1..24: mol_type = other DNA
atcgtgtttgttaccaactgcctg

SEQ ID NO: 160 - DNA, 24 bp, synthetic construct
  source 1..24: mol_type = other DNA
ggcccaggcagttggtaacaaaca

SEQ ID NO: 161 - DNA, 90 bp, synthetic construct
  source 1..90: mol_type = other DNA
tgcgggatctcaaaatccagcgatgagccgcccaccagcaccacagcgttatcgatcggcaccagttcgccctccttgatgtacaccact

SEQ ID NO: 162 - DNA, 20 bp, synthetic construct
  source 1..20: mol_type = other DNA
tcatcattggcatcctgaaa

SEQ ID NO: 163 - DNA, 20 bp, synthetic construct
  source 1..20: mol_type = other DNA
tggtcagcctgctgattaaa

SEQ ID NO: 164 - DNA, 7178 bp, synthetic construct
  source 1..7178: mol_type = other DNA
tggcgaatgggacgcgccctgtagcggcgcattaagcgcggcgggtgtggtggttacgcgcagcgtgaccgctacacttgccagcgccctagcgcccgctcctttcgctttcttcccttcctttctcgccacgttcgccggctttccccgtcaagctctaaatcgggggctccctttagggttccgatttagtgctttacggcacctcgaccccaaaaaacttgattagggtgatggttcacgtagtgggccatcgccctgatagacggtttttcgccctttgacgttggagtccacgttctttaatagtggactcttgttccaaactggaacaacactcaaccctatctcggtctattcttttgatttataagggattttgccgatttcggcctattggttaaaaaatgagctgatttaacaaaaatttaacgcgaattttaacaaaatattaacgtttacaatttcaggtggcacttttcggggaaatgtgcgcggaacccctatttgtttatttttctaaatacattcaaatatgtatccgctcatgaattaattcttagaaaaactcatcgagcatcaaatgaaactgcaatttattcatatcaggattatcaataccatatttttgaaaaagccgtttctgtaatgaaggagaaaactcaccgaggcagttccataggatggcaagatcctggtatcggtctgcgattccgactcgtccaacatcaatacaacctattaatttcccctcgtcaaaaataaggttatcaagtgagaaatcaccatgagtgacgactgaatccggtgagaatggcaaaagtttatgcatttctttccagacttgttcaacaggccagccattacgctcgtcatcaaaatcactcgcatcaaccaaaccgttattcattcgtgattgcgcctgagcgagacgaaatacgcgatcgctgttaaaaggacaattacaaacaggaatcgaatgcaaccggcgcaggaacactgccagcgcatcaacaatattttcacctgaatcaggatattcttctaatacctggaatgctgttttcccggggatcgcagtggtgagtaaccatgcatcatcaggagtacggataaaatgcttgatggtcggaagaggcataaattccgtcagccagtttagtctgaccatctcatctgtaacatcattggcaacgctacctttgccatgtttcagaaacaactctggcgcatcgggcttcccatacaatcgatagattgtcgcacctgattgcccgacattatcgcgagcccatttatacccatataaatcagcatccatgttggaatttaatcgcggcctagagcaagacgtttcccgttgaatatggctcataacaccccttgtattactgtttatgtaagcagacagttttattgttcatgaccaaaatcccttaacgtgagttttcgttccactgagcgtcagaccccgtagaaaagatcaaaggatcttcttgagatcctttttttctgcgcgtaatctgctgcttgcaaacaaaaaaaccaccgctaccagcggtggtttgtttgccggatcaagagctaccaactctttttccgaaggtaactggcttcagcagagcgcagataccaaatactgtccttctagtgtagccgtagttaggccaccacttcaagaactctgtagcaccgcctacatacctcgctctgctaatcctgttaccagtggctgctgccagtggcgataagtcgtgtcttaccgggttggactcaagacgatagttaccggataaggcgcagcggtcgggctgaacggggggttcgtgcacacagcccagcttggagcgaacgacctacaccgaactgagatacctacagcgtgagctatgagaaagcgccacgcttcccgaagggagaaaggcggacaggtatccggtaagcggcagggtcggaacaggagagcgcacgagggagcttccagggggaaacgcctggtatctttatagtcctgtcgggtttcgccacctctgacttgagcgtcgatttttgtgatgctcgtcaggggggcggagcctatggaaaaacgccagcaacgcggcctttttacggttcctggccttttgctggccttttgctcacatgttctttcctgcgttatcccctgattctgtggataaccgtattaccgcctttgagtgagctgataccgctcgccgcagccgaacgaccgagcgcagcgagtcagtgagcgaggaagcggaagagcgcctgatgcggtattttctccttacgcatctgtgcggtatttcacaccgcatatatggtgcactctcagtacaatctgctctgatgccgcatagttaagccagtatacactccgctatcgctacgtgactgggtcatggctgcgccccgacacccgccaacacccgctgacgcgccctgacgggcttgtctgctcccggcatccgcttacagacaagctgtgaccgtctccgggagctgcatgtgtcagaggttttcaccgtcatcaccgaaacgcgcgaggcagctgcggtaaagctcatcagcgtggtcgtgaagcgattcacagatgtctgcctgttcatccgcgtccagctcgttgagtttctccagaagcgttaatgtctggcttctgataaagcgggccatgttaagggcggttttttcctgtttggtcactgatgcctccgtgtaagggggatttctgttcatgggggtaatgataccgatgaaacgagagaggatgctcacgatacgggttactgatgatgaacatgcccggttactggaacgttgtgagggtaaacaactggcggtatggatgcggcgggaccagagaaaaatcactcagggtcaatgccagcgcttcgttaatacagatgtaggtgttccacagggtagccagcagcatcctgcgatgcagatccggaacataatggtgcagggcgctgacttccgcgtttccagactttacgaaacacggaaaccgaagaccattcatgttgttgctcaggtcgcagacgttttgcagcagcagtcgcttcacgttcgctcgcgtatcggtgattcattctgctaaccagtaaggcaaccccgccagcctagccgggtcctcaacgacaggagcacgatcatgcgcacccgtggggccgccatgccggcgataatggcctgcttctcgccgaaacgtttggtggcgggaccagtgacgaaggcttgagcgagggcgtgcaagattccgaataccgcaagcgacaggccgatcatcgtcgcgctccagcgaaagcggtcctcgccgaaaatgacccagagcgctgccggcacctgtcctacgagttgcatgataaagaagacagtcataagtgcggcgacgatagtcatgccccgcgcccaccggaaggagctgactgggttgaaggctctcaagggcatcggtcgagatcccggtgcctaatgagtgagctaacttacattaattgcgttgcgctcactgcccgctttccagtcgggaaacctgtcgtgccagctgcattaatgaatcggccaacgcgcggggagaggcggtttgcgtattgggcgccagggtggtttttcttttcaccagtgagacgggcaacagctgattgcccttcaccgcctggccctgagagagttgcagcaagcggtccacgctggtttgccccagcaggcgaaaatcctgtttgatggtggttaacggcgggatataacatgagctgtcttcggtatcgtcgtatcccactaccgagatatccgcaccaacgcgcagcccggactcggtaatggcgcgcattgcgcccagcgccatctgatcgttggcaaccagcatcgcagtgggaacgatgccctcattcagcatttgcatggtttgttgaaaaccggacatggcactccagtcgccttcccgttccgctatcggctgaatttgattgcgagtgagatatttatgccagccagccagacgcagacgcgccgagacagaacttaatgggcccgctaacagcgcgatttgctggtgacccaatgcgaccagatgctccacgcccagtcgcgtaccgtcttcatgggagaaaataatactgttgatgggtgtctggtcagagacatcaagaaataacgccggaacattagtgcaggcagcttccacagcaatggcatcctggtcatccagcggatagttaatgatcagcccactgacgcgttgcgcgagaagattgtgcaccgccgctttacaggcttcgacgccgcttcgttctaccatcgacaccaccacgctggcacccagttgatcggcgcgagatttaatcgccgcgacaatttgcgacggcgcgtgcagggccagactggaggtggcaacgccaatcagcaacgactgtttgcccgccagttgttgtgccacgcggttgggaatgtaattcagctccgccatcgccgcttccactttttcccgcgttttcgcagaaacgtggctggcctggttcaccacgcgggaaacggtctgataagagacaccggcatactctgcgacatcgtataacgttactggtttcacattcaccaccctgaattgactctcttccgggcgctatcatgccataccgcgaaaggttttgcgccattcgatggtgtccgggatctcgacgctctcccttatgcgactcctgcattaggaagcagcccagtagtaggttgaggccgttgagcaccgccgccgcaaggaatggtgcatgcaaggagatggcgcccaacagtcccccggccacggggcctgccaccatacccacgccgaaacaagcgctcatgagcccgaagtggcgagcccgatcttccccatcggtgatgtcggcgatataggcgccagcaaccgcacctgtggcgccggtgatgccggccacgatgcgtccggcgtagaggatcgagatctcgatcccgcgaaattaatacgactcactataggggaattgtgagcggataacaattcccctctagaaataattttgtttaactttaagaaggagatataccatgggcagcagccatcatcatcatcatcacagcagcggcctggtgccgcgcggcagcatgtcggactcagaagtcaatcaagaagctaagccagaggtcaagccagaagtcaagcctgagactcacatcaatttaaaggtgtccgatggatcttcagagatcttcttcaagatcaaaaagaccactcctttaagaaggctgatggaagcgttcgctaaaagacagggtaaggaaatggactccttaagattcttgtacgacggtattagaattcaagctgatcagacccctgaagatttggacatggaggataacgatattattgaggctcacagagaacagattggtggtcatagtagtcttgaagtcctctttcagggacccatggtgcagacggagatcctgaaggcgtttcggtttgcgttggatccgacgtctgtgcaggttgctgccctttcccggcatgctggtgcggccaggtgggcgttcaaccatgctctcgcggccaaggtcggcgcgcatgagcggtggcgggcggaggtagccaagcttgtcggggacggtgttcctgaggagcaggctcgtaggcaggtgcgcgtcccggttccgatgaagccggcgatccagaaggcgttgaacgcggtcaagggtgactctcgcaagggcttggatggtgcgtgcccgtggtggcatgaggtcaacacttacgcgttccagtccgctttcatcgacgcggaccaggcgtggaagaactggttggactcgttgtcggggaagcgggtcggccgccgggtggggtacccgcggttcaagaagaaggggcgggcccgcgactcgtttcgcttgcaccacgacgtgaagaagccaagcatccggctggccgggtaccggcggttgcggctgccgaggatcggggaagtccggcttcatgactcggggaagcgtctggcacggctgatcgaccgaggtgacgcggtggtgcagtcggtgacggtgtcgcggggtggccatcgctggtatgcgtctgtgctgtgcaaggtcaccgtgcaggtaccggatcggccgtcacggcgccagcgggaacgaggcgctgttggggtggaccttggcgttaaggtcctcgcggctttgtccaagccactggtggtcgacgacccgtcgagtgccctggtgcggaatccgcagcatctgcggcaggccgagcggcgtctactgaaggctcagcgggcgttggcgcgtacacaaaaaggttcagcccgacgcgagaaggccaagcggcgagttggtcgcgcgcatcacgaggttgctgtgcgccggcatgctgcgctccatcagatcaccaagcgcctgaccaccggcttcgcggtcgtcgcgcttgaggatctgaacgtggccggtatgacaaggtcagcgcggggaacagtggcagcgccgggaaagaacgtgcggcagaaggcaggcctgaaccgcgtcatcctggactccgctccagccgagttgcgtcgccaggtgaactacaaggccacctggtatggatctgagctggcggtcgcagaccgctggttcccctcgagtaagacctgttcgggttgcggatggcaaaacccacacctgaagctgtccgacagggtgtttcgttgcacagactgcgggctggtgatggaccgggacatgaacgcggcccggaacatcgaacgccacgcagtgctgatcgatcgaaacgtcgcctgcgataggcgggagacgctaaacgcccgtggagcatccataagaccaaccacctctcggggcggtaggcacgacgcatcgaagcgggaaggctccggcgctcggcctgagtcacctcagcagagtgatctgctgacgctcccaaccttgaataacgaaacggcaacgcctccataagcttaagaattcgagctccgtcgacaagcttgcggccgcactcgagcaccaccaccaccaccactgagatccggctgctaacaaagcccgaaaggaagctgagttggctgctgccaccgctgagcaataactagcataaccccttggggcctctaaacgggtcttgaggggttttttgctgaaaggaggaactatatccggat

SEQ ID NO: 165 - DNA, 46 bp, synthetic construct
  source 1..46: mol_type = other DNA
tcttgaagtcctctttcagggacccatggtgcagacggagatcctg

SEQ ID NO: 166 - DNA, 47 bp, synthetic construct
  source 1..47: mol_type = other DNA
gtcgacggagctcgaattcttaagcttatggaggcgttgccgtttcg

SEQ ID NO: 167 - DNA, 5657 bp, synthetic construct
  source 1..5657: mol_type = other DNA
gcttaagaattcgagctccgtcgacaagcttgcggccgcactcgagcaccaccaccaccaccactgagatccggctgctaacaaagcccgaaaggaagctgagttggctgctgccaccgctgagcaataactagcataaccccttggggcctctaaacgggtcttgaggggttttttgctgaaaggaggaactatatccggattggcgaatgggacgcgccctgtagcggcgcattaagcgcggcgggtgtggtggttacgcgcagcgtgaccgctacacttgccagcgccctagcgcccgctcctttcgctttcttcccttcctttctcgccacgttcgccggctttccccgtcaagctctaaatcgggggctccctttagggttccgatttagtgctttacggcacctcgaccccaaaaaacttgattagggtgatggttcacgtagtgggccatcgccctgatagacggtttttcgccctttgacgttggagtccacgttctttaatagtggactcttgttccaaactggaacaacactcaaccctatctcggtctattcttttgatttataagggattttgccgatttcggcctattggttaaaaaatgagctgatttaacaaaaatttaacgcgaattttaacaaaatattaacgtttacaatttcaggtggcacttttcggggaaatgtgcgcggaacccctatttgtttatttttctaaatacattcaaatatgtatccgctcatgaattaattcttagaaaaactcatcgagcatcaaatgaaactgcaatttattcatatcaggattatcaataccatatttttgaaaaagccgtttctgtaatgaaggagaaaactcaccgaggcagttccataggatggcaagatcctggtatcggtctgcgattccgactcgtccaacatcaatacaacctattaatttcccctcgtcaaaaataaggttatcaagtgagaaatcaccatgagtgacgactgaatccggtgagaatggcaaaagtttatgcatttctttccagacttgttcaacaggccagccattacgctcgtcatcaaaatcactcgcatcaaccaaaccgttattcattcgtgattgcgcctgagcgagacgaaatacgcgatcgctgttaaaaggacaattacaaacaggaatcgaatgcaaccggcgcaggaacactgccagcgcatcaacaatattttcacctgaatcaggatattcttctaatacctggaatgctgttttcccggggatcgcagtggtgagtaaccatgcatcatcaggagtacggataaaatgcttgatggtcggaagaggcataaattccgtcagccagtttagtctgaccatctcatctgtaacatcattggcaacgctacctttgccatgtttcagaaacaactctggcgcatcgggcttcccatacaatcgatagattgtcgcacctgattgcccgacattatcgcgagcccatttatacccatataaatcagcatccatgttggaatttaatcgcggcctagagcaagacgtttcccgttgaatatggctcataacaccccttgtattactgtttatgtaagcagacagttttattgttcatgaccaaaatcccttaacgtgagttttcgttccactgagcgtcagaccccgtagaaaagatcaaaggatcttcttgagatcctttttttctgcgcgtaatctgctgcttgcaaacaaaaaaaccaccgctaccagcggtggtttgtttgccggatcaagagctaccaactctttttccgaaggtaactggcttcagcagagcgcagataccaaatactgtccttctagtgtagccgtagttaggccaccacttcaagaactctgtagcaccgcctacatacctcgctctgctaatcctgttaccagtggctgctgccagtggcgataagtcgtgtcttaccgggttggactcaagacgatagttaccggataaggcgcagcggtcgggctgaacggggggttcgtgcacacagcccagcttggagcgaacgacctacaccgaactgagatacctacagcgtgagctatgagaaagcgccacgcttcccgaagggagaaaggcggacaggtatccggtaagcggcagggtcggaacaggagagcgcacgagggagcttccagggggaaacgcctggtatctttatagtcctgtcgggtttcgccacctctgacttgagcgtcgatttttgtgatgctcgtcaggggggcggagcctatggaaaaacgccagcaacgcggcctttttacggttcctggccttttgctggccttttgctcacatgttctttcctgcgttatcccctgattctgtggataaccgtattaccgcctttgagtgagctgataccgctcgccgcagccgaacgaccgagcgcagcgagtcagtgagcgaggaagcggaagagcgcctgatgcggtattttctccttacgcatctgtgcggtatttcacaccgcatatatggtgcactctcagtacaatctgctctgatgccgcatagttaagccagtatacactccgctatcgctacgtgactgggtcatggctgcgccccgacacccgccaacacccgctgacgcgccctgacgggcttgtctgctcccggcatccgcttacagacaagctgtgaccgtctccgggagctgcatgtgtcagaggttttcaccgtcatcaccgaaacgcgcgaggcagctgcggtaaagctcatcagcgtggtcgtgaagcgattcacagatgtctgcctgttcatccgcgtccagctcgttgagtttctccagaagcgttaatgtctggcttctgataaagcgggccatgttaagggcggttttttcctgtttggtcactgatgcctccgtgtaagggggatttctgttcatgggggtaatgataccgatgaaacgagagaggatgctcacgatacgggttactgatgatgaacatgcccggttactggaacgttgtgagggtaaacaactggcggtatggatgcggcgggaccagagaaaaatcactcagggtcaatgccagcgcttcgttaatacagatgtaggtgttccacagggtagccagcagcatcctgcgatgcagatccggaacataatggtgcagggcgctgacttccgcgtttccagactttacgaaacacggaaaccgaagaccattcatgttgttgctcaggtcgcagacgttttgcagcagcagtcgcttcacgttcgctcgcgtatcggtgattcattctgctaaccagtaaggcaaccccgccagcctagccgggtcctcaacgacaggagcacgatcatgcgcacccgtggggccgccatgccggcgataatggcctgcttctcgccgaaacgtttggtggcgggaccagtgacgaaggcttgagcgagggcgtgcaagattccgaataccgcaagcgacaggccgatcatcgtcgcgctccagcgaaagcggtcctcgccgaaaatgacccagagcgctgccggcacctgtcctacgagttgcatgataaagaagacagtcataagtgcggcgacgatagtcatgccccgcgcccaccggaaggagctgactgggttgaaggctctcaagggcatcggtcgagatcccggtgcctaatgagtgagctaacttacattaattgcgttgcgctcactgcccgctttccagtcgggaaacctgtcgtgccagctgcattaatgaatcggccaacgcgcggggagaggcggtttgcgtattgggcgccagggtggtttttcttttcaccagtgagacgggcaacagctgattgcccttcaccgcctggccctgagagagttgcagcaagcggtccacgctggtttgccccagcaggcgaaaatcctgtttgatggtggttaacggcgggatataacatgagctgtcttcggtatcgtcgtatcccactaccgagatatccgcaccaacgcgcagcccggactcggtaatggcgcgcattgcgcccagcgccatctgatcgttggcaaccagcatcgcagtgggaacgatgccctcattcagcatttgcatggtttgttgaaaaccggacatggcactccagtcgccttcccgttccgctatcggctgaatttgattgcgagtgagatatttatgccagccagccagacgcagacgcgccgagacagaacttaatgggcccgctaacagcgcgatttgctggtgacccaatgcgaccagatgctccacgcccagtcgcgtaccgtcttcatgggagaaaataatactgttgatgggtgtctggtcagagacatcaagaaataacgccggaacattagtgcaggcagcttccacagcaatggcatcctggtcatccagcggatagttaatgatcagcccactgacgcgttgcgcgagaagattgtgcaccgccgctttacaggcttcgacgccgcttcgttctaccatcgacaccaccacgctggcacccagttgatcggcgcgagatttaatcgccgcgacaatttgcgacggcgcgtgcagggccagactggaggtggcaacgccaatcagcaacgactgtttgcccgccagttgttgtgccacgcggttgggaatgtaattcagctccgccatcgccgcttccactttttcccgcgttttcgcagaaacgtggctggcctggttcaccacgcgggaaacggtctgataagagacaccggcatactctgcgacatcgtataacgttactggtttcacattcaccaccctgaattgactctcttccgggcgctatcatgccataccgcgaaaggttttgcgccattcgatggtgtccgggatctcgacgctctcccttatgcgactcctgcattaggaagcagcccagtagtaggttgaggccgttgagcaccgccgccgcaaggaatggtgcatgcaaggagatggcgcccaacagtcccccggccacggggcctgccaccatacccacgccgaaacaagcgctcatgagcccgaagtggcgagcccgatcttccccatcggtgatgtcggcgatataggcgccagcaaccgcacctgtggcgccggtgatgccggccacgatgcgtccggcgtagaggatcgagatctcgatcccgcgaaattaatacgactcactataggggaattgtgagcggataacaattcccctctagaaataattttgtttaactttaagaaggagatataccatgggcagcagccatcatcatcatcatcacagcagcggcctggtgccgcgcggcagcatgtcggactcagaagtcaatcaagaagctaagccagaggtcaagccagaagtcaagcctgagactcacatcaatttaaaggtgtccgatggatcttcagagatcttcttcaagatcaaaaagaccactcctttaagaaggctgatggaagcgttcgctaaaagacagggtaaggaaatggactccttaagattcttgtacgacggtattagaattcaagctgatcagacccctgaagatttggacatggaggataacgatattattgaggctcacagagaacagattggtggtcatagtagtcttgaagtcctctttcagggaccc

SEQ ID NO: 168 - DNA, 20 bp, synthetic construct
  source 1..20: mol_type = other DNA
ccgcatatatcgcaaaacaa

SEQ ID NO: 169 - DNA, 20 bp, synthetic construct
  source 1..20: mol_type = other DNA
ctggctgtgaacaaagtgga

SEQ ID NO: 170 - RNA, 254 nt, synthetic construct
  source 1..254: mol_type = other RNA
aaacgtcgcctgcgataggcgggagacgctaaacgcccgtggagcatccataagaccaaccacctctcggggcggtaggcacgacgcatcgaagcgggaaggctccggcgctcggcctgagtcacctcagcagagtgatctgctgacgctcccaaccttgaataacgaaacggcaacgcctccatagcggtgcaggtcaataagggtcggccccacgcgtgtagggagcgatcgcggttcaggtgaaagtgaaa

SEQ ID NO: 171 - DNA, 274 bp, synthetic construct
  source 1..274: mol_type = other DNA
taatacgactcactatagggaaacgtcgcctgcgataggcgggagacgctaaacgcccgtggagcatccataagaccaaccacctctcggggcggtaggcacgacgcatcgaagcgggaaggctccggcgctcggcctgagtcacctcagcagagtgatctgctgacgctcccaaccttgaataacgaaacggcaacgcctccatagcggtgcaggtcaataagggtcggccccacgcgtgtagggagcgatcgcggttcaggtgaaagtgaaa

SEQ ID NO: 172 - RNA, 205 nt, synthetic construct
  source 1..205: mol_type = other RNA
aaacgtcgcctgcgataggcgggagacgctaaacgcccgtggagcatccataagaccaaccacctctcggggcggtaggcacgacgcatcgaagcgggaaggctccggcgctcggcctgagtcacctcagcagagtgatctgctgacgctcccaaccttgaataacgaaacggcaacgcctccatagcggtgcaggtcaataagg

SEQ ID NO: 173 - DNA, 225 bp, synthetic construct
  source 1..225: mol_type = other DNA
taatacgactcactatagggaaacgtcgcctgcgataggcgggagacgctaaacgcccgtggagcatccataagaccaaccacctctcggggcggtaggcacgacgcatcgaagcgggaaggctccggcgctcggcctgagtcacctcagcagagtgatctgctgacgctcccaaccttgaataacgaaacggcaacgcctccatagcggtgcaggtcaataagg

SEQ ID NO: 174 - RNA, 49 nt, synthetic construct
  source 1..49: mol_type = other RNA
gtcggccccacgcgtgtagggagcgatcgcggttcaggtgaaagtgaaa

SEQ ID NO: 175 - DNA, 69 bp, synthetic construct
  source 1..69: mol_type = other DNA
taatacgactcactataggggtcggccccacgcgtgtagggagcgatcgcggttcaggtgaaagtgaaa

SEQ ID NO: 176 - DNA, 58 bp, synthetic construct
  source 1..58: mol_type = other DNA
ggctgtgagaaagcggttcaggtgaaagtgaaaacactgcccgacgcccagttcgaag

SEQ ID NO: 177 - DNA, 58 bp, synthetic construct
  source 1..58: mol_type = other DNA
cttcgaactgggcgtcgggcagtgttttcactttcacctgaaccgctttctcacagcc

SEQ ID NO: 178 - DNA, 7204 bp, synthetic construct
  source 1..7204: mol_type = other DNA
ggtaccgattagtgaacggatctcgacggtatcgatcacgagactagcctcgagcggccgcccccttcaccgagggcctatttcccatgattccttcatatttgcatatacgatacaaggctgttagagagataattggaattaatttgactgtaaacacaaagatattagtacaaaatacgtgacgtagaaagtaataatttcttgggtagtttgcagttttaaaattatgttttaaaatggactatcatatgcttaccgtaacttgaaagtatttcgatttcttggctttatatatcttgtggaaaggacgaaacaccgaacgcggcccggaacatcgaacgccacgcagtgctgatcgatcgaaacgtcgcctgcgataggcgggagacgctaaacgcccgtggagcatccataagaccaaccacctctcggggcggtaggcacgacgcatcgaagcgggaaggctccggcgctcggcctgagtcacctcagcagagtgatctgctgacgctcccaaccttgaataacgaaacggcaacgcctccatagcggtgcaggtcaataagggtcggccccacgcgtgtagggagcgatcgcgagacccgagagagggtcggtctcctttttttgaattctcgacctcgagacaaatggcagtattcatccacaattttaaaagaaaaggggggattggggggtacagtgcaggggaaagaatagtagacataatagcaacagacatacaaactaaagaattacaaaaacaaattacaaaaattcaaaattttcgggtttattacagggacagcagagatccactttggccgcggctcgagggggttggggttgcgccttttccaaggcagccctgggtttgcgcagggacgcggctgctctgggcgtggttccgggaaacgcagcggcgccgaccctgggactcgcacattcttcacgtccgttcgcagcgtcacccggatcttcgccgctacccttgtgggccccccggcgacgcttcctgctccgcccctaagtcgggaaggttccttgcggttcgcggcgtgccggacgtgacaaacggaagccgcacgtctcactagtaccctcgcagacggacagcgccagggagcaatggcagcgcgccgaccgcgatgggctgtggccaatagcggctgctcagcagggcgcgccgagagcagcggccgggaaggggcggtgcgggaggcggggtgtggggcggtagtgtgggccctgttcctgcccgcgcggtgttccgcattctgcaagcctccggagcgcacgtcggcagtcggctccctcgttgaccgaatcaccgacctctctccccagggggatccaccggagcttaccatgaccgagtacaagcccacggtgcgcctcgccacccgcgacgacgtccccagggccgtacgcaccctcgccgccgcgttcgccgactaccccgccacgcgccacaccgtcgatccggaccgccacatcgagcgggtcaccgagctgcaagaactcttcctcacgcgcgtcgggctcgacatcggcaaggtgtgggtcgcggacgacggcgccgcggtggcggtctggaccacgccggagagcgtcgaagcgggggcggtgttcgccgagatcggcccgcgcatggccgagttgagcggttcccggctggccgcgcagcaacagatggaaggcctcctggcgccgcaccggcccaaggagcccgcgtggttcctggccaccgtcggcgtctcgcccgaccaccagggcaagggtctgggcagcgccgtcgtgctccccggagtggaggcggccgagcgcgccggggtgcccgccttcctggaaacctccgcgccccgcaacctccccttctacgagcggctcggcttcaccgtcaccgccgacgtcgaggtgcccgaaggaccgcgcacctggtgcatgacccgcaagcccggtgcctgacgcccgccccacgacccgcagcgcccgaccgaaaggagcgcacgaccccatgcatcggtacctttaagaccaatgacttacaaggcagctgtagatcttagccactttctagagtcggggcggccggccgcttcgagcagacatgataagatacattgatgagtttggacaaaccacaactagaatgcagtgaaaaaaatgctttatttgtgaaatttgtgatgctattgctttatttgtaaccattataagctgcaataaacaagttaacaacaacaattgcattcattttatgtttcaggttcagggggaggtgtgggaggttttttaaagcaagtaaaacctctacaaatgtggtaaaatcgataaggatccgtcgaccgatgcccttgagagccttcaacccagtcagctccttccggtgggcgcggggcatgactatcgtcgccgcacttatgactgtcttctttatcatgcaactcgtaggacaggtgccggcagcgctcttccgcttcctcgctcactgactcgctgcgctcggtcgttcggctgcggcgagcggtatcagctcactcaaaggcggtaatacggttatccacagaatcaggggataacgcaggaaagaacatgtgagcaaaaggccagcaaaaggccaggaaccgtaaaaaggccgcgttgctggcgtttttccataggctccgcccccctgacgagcatcacaaaaatcgacgctcaagtcagaggtggcgaaacccgacaggactataaagataccaggcgtttccccctggaagctccctcgtgcgctctcctgttccgaccctgccgcttaccggatacctgtccgcctttctcccttcgggaagcgtggcgctttctcaatgctcacgctgtaggtatctcagttcggtgtaggtcgttcgctccaagctgggctgtgtgcacgaaccccccgttcagcccgaccgctgcgccttatccggtaactatcgtcttgagtccaacccggtaagacacgacttatcgccactggcagcagccactggtaacaggattagcagagcgaggtatgtaggcggtgctacagagttcttgaagtggtggcctaactacggctacactagaaggacagtatttggtatctgcgctctgctgaagccagttaccttcggaaaaagagttggtagctcttgatccggcaaacaaaccaccgctggtagcggtggtttttttgtttgcaagcagcagattacgcgcagaaaaaaaggatctcaagaagatcctttgatcttttctacggggtctgacgctcagtggaacgaaaactcacgttaagggattttggtcatgagattatcaaaaaggatcttcacctagatccttttaaattaaaaatgaagttttaaatcaatctaaagtatatatgagtaaacttggtctgacagttaccaatgcttaatcagtgaggcacctatctcagcgatctgtctatttcgttcatccatagttgcctgactccccgtcgtgtagataactacgatacgggagggcttaccatctggccccagtgctgcaatgataccgcgggacccacgctcaccggctccagatttatcagcaataaaccagccagccggaagggccgagcgcagaagtggtcctgcaactttatccgcctccatccagtctattaattgttgccgggaagctagagtaagtagttcgccagttaatagtttgcgcaacgttgttgccattgctacaggcatcgtggtgtcacgctcgtcgtttggtatggcttcattcagctccggttcccaacgatcaaggcgagttacatgatcccccatgttgtgcaaaaaagcggttagctccttcggtcctccgatcgttgtcagaagtaagttggccgcagtgttatcactcatggttatggcagcactgcataattctcttactgtcatgccatccgtaagatgcttttctgtgactggtgagtactcaaccaagtcattctgagaatagtgtatgcggcgaccgagttgctcttgcccggcgtcaatacgggataataccgcgccacatagcagaactttaaaagtgctcatcattggaaaacgttcttcggggcgaaaactctcaaggatcttaccgctgttgagatccagttcgatgtaacccactcgtgcacccaactgatcttcagcatcttttactttcaccagcgtttctgggtgagcaaaaacaggaaggcaaaatgccgcaaaaaagggaataagggcgacacggaaatgttgaatactcatactcttcctttttcaatattattgaagcatttatcagggttattgtctcatgagcggatacatatttgaatgtatttagaaaaataaacaaataggggttccgcgcacatttccccgaaaagtgccacctgcaggaaacagctatgaccatgattacgccaagctctagctagaggtcgacggtatcgagccccagctggttctttccgcctcagaagccatagagcccaccgcatccccagcatgcctgctattgtcttcccaatcctcccccttgctgtcctgccccaccccaccccccagaatagaatgacacctactcagacaatgcgatgcaatttcctcattttattaggaaaggacagtgggagtggcaccttccagggtcaaggaaggcacgggggaggggcaaacaacagatggctggcaactagaaggcacagtcgaggctgatcagcgggtttaaactcaatggtgatggtgatgatgaccggttagactttcctcttcttcttgggagaaccaccagaggggggtgtggcggtttcgttgttcagtgtggggagtgtgagcagatcagactgctggggggactctggccgggccccgctcccctccctcttgctggcgtcgtgccgccccccccggcttgtggtgggccggatgctggcccccctggcgttcaaagtctcccgccggtcgcaggccacgttcctatcaatcaacacagcgtgcctctcgatgttcctagcggcgttcatatctctatccatgaccaggccgcagtcggtgcacctaaacaccctatcggagagcttcaagtgggggttctgccagccgcacccgctgcaggtcttgctggaggggaaccacctgtcggccacggccagctcgctcccgtaccaggtggccttgtagttcacctgcctccgcagctcggcaggggcgctgtccaggatgacccggttcagcccggccttctgccggacgttcttccctggggcggccactgtccccctggcggacctggtcatgccggcgacgttcagatcctccagggccaccacggcgaaccctgtggtcagccgcttggtgatctggtgcagggcggcgtgccgccggacggccacctcgtgatgggccctccccacccgccgcttggccttctctctcctggcgctgcccttctgtgtcctggccagggcccgctgggccttgagcagccgcctctcagcctgcctcaggtgctgggggtttctcaccagggcgctgcttgggtcgtcgacgaccaggggcttggacagggcggccagcaccttcacccccaggtccactcccacggcgcccctctcccgctgccgcctgctgggccgatcgggcacctgcactgtcaccttgcagagcacggaggcgtaccacctgtgtccgcccctactcacagtcacggactgcaccacggcgtcgcctctgtcaatgagcctggcgagccgcttgccgctgtcgtgcagcctcacctcgccaatcctaggcagcctcagccttctgtagccagccagcctgatgctgggcttcttcacatcgtggtgcaatctaaagctatcccgagcccggcccttcttcttaaaccgggggtagcccaccctcctccccactctcttgccgctcaggctgtcgagccagttcttccatgcctggtcggcgtcaataaaggcgctctggaaggcgtaggtgttcacctcgtgccaccatgggcaggccccatccaggcccttccgggaatcccccttcacggcgttcagggccttctggatggctggcttcataggcacggggacccggacctgccgccgggcctgctcctcgggcacgccatcgcccacgagcttggccacctcggcccgccaccgctcgtgggcccccaccttggcggcgagggcgtggttgaaggcccacctggcggccccggcgtgccggctcagggcggccacctggacggaagtaggatcgagggcgaaccgaaaggccttcaggatctctgtctgcaccatgaccttcctcttcttcttaggggccatggtggcggctctccctatagtgagtcgtattagcggccgcggatctctagcggatctgacggttcactaaaccagctctgcttatatagacctcccaccgtacacgcctaccgcccatttgcgtcaatggggcggagttgttacgacattttggaaagtcccgttgattttggtgccaaaacaaactcccattgacgtcaatggggtggagacttggaaatccccgtgagtcaaaccgctatccacgcccattgatgtactgccaaaaccgcatcaccatggtaatagcgatgactaatacgtagatgtactgccaagtaggaaagtcccataaggtcatgtactgggcataatgccaggcgggccatttaccgtcattgacgtcaatagggggcgtacttggcatatgatacacttgatgtactgccaagtgggcagtttaccgtaaatactccacccattgacgtcaatggaaagtccctattggcgttactatgggaacatacgtcattattgacgtcaatgggcgggggtcgttgggcggtcagccaggcgggccatttaccgtaagttatgtaacgcggaactccatatatgggctatgaactaatgaccccgtaattgattactattaataactagtcaataatcaatgtcaacgcgtatatctggcccgtacatcgcgaagcagcgcaaaacgcctaaccctaagcagattcttcatgcaattgtcggtcaagaatcgatagtactaacatacgctctccatcaaaacaaaacgaaacaaaacaaactagcaaaataggctgtccccagtgcaagtgcaggtgccagaacatttctctatcgata

SEQ ID NO: 179 - DNA, 2491 bp, synthetic construct
  source 1..2491: mol_type = other DNA
aacaacaacaattgcattcattttatgtttcaggttcagggggaggtgtgggaggttttttaaagcaagtaaaacctctacaaatgtggtaaaatcgataaggatccgtcgaccgatgcccttgagagccttcaacccagtcagctccttccggtgggcgcggggcatgactatcgtcgccgcacttatgactgtcttctttatcatgcaactcgtaggacaggtgccggcagcgctcttccgcttcctcgctcactgactcgctgcgctcggtcgttcggctgcggcgagcggtatcagctcactcaaaggcggtaatacggttatccacagaatcaggggataacgcaggaaagaacatgtgagcaaaaggccagcaaaaggccaggaaccgtaaaaaggccgcgttgctggcgtttttccataggctccgcccccctgacgagcatcacaaaaatcgacgctcaagtcagaggtggcgaaacccgacaggactataaagataccaggcgtttccccctggaagctccctcgtgcgctctcctgttccgaccctgccgcttaccggatacctgtccgcctttctcccttcgggaagcgtggcgctttctcaatgctcacgctgtaggtatctcagttcggtgtaggtcgttcgctccaagctgggctgtgtgcacgaaccccccgttcagcccgaccgctgcgccttatccggtaactatcgtcttgagtccaacccggtaagacacgacttatcgccactggcagcagccactggtaacaggattagcagagcgaggtatgtaggcggtgctacagagttcttgaagtggtggcctaactacggctacactagaaggacagtatttggtatctgcgctctgctgaagccagttaccttcggaaaaagagttggtagctcttgatccggcaaacaaaccaccgctggtagcggtggtttttttgtttgcaagcagcagattacgcgcagaaaaaaaggatctcaagaagatcctttgatcttttctacggggtctgacgctcagtggaacgaaaactcacgttaagggattttggtcatgagattatcaaaaaggatcttcacctagatccttttaaattaaaaatgaagttttaaatcaatctaaagtatatatgagtaaacttggtctgacagttaccaatgcttaatcagtgaggcacctatctcagcgatctgtctatttcgttcatccatagttgcctgactccccgtcgtgtagataactacgatacgggagggcttaccatctggccccagtgctgcaatgataccgcgggacccacgctcaccggctccagatttatcagcaataaaccagccagccggaagggccgagcgcagaagtggtcctgcaactttatccgcctccatccagtctattaattgttgccgggaagctagagtaagtagttcgccagttaatagtttgcgcaacgttgttgccattgctacaggcatcgtggtgtcacgctcgtcgtttggtatggcttcattcagctccggttcccaacgatcaaggcgagttacatgatcccccatgttgtgcaaaaaagcggttagctccttcggtcctccgatcgttgtcagaagtaagttggccgcagtgttatcactcatggttatggcagcactgcataattctcttactgtcatgccatccgtaagatgcttttctgtgactggtgagtactcaaccaagtcattctgagaatagtgtatgcggcgaccgagttgctcttgcccggcgtcaatacgggataataccgcgccacatagcagaactttaaaagtgctcatcattggaaaacgttcttcggggcgaaaactctcaaggatcttaccgctgttgagatccagttcgatgtaacccactcgtgcacccaactgatcttcagcatcttttactttcaccagcgtttctgggtgagcaaaaacaggaaggcaaaatgccgcaaaaaagggaataagggcgacacggaaatgttgaatactcatactcttcctttttcaatattattgaagcatttatcagggttattgtctcatgagcggatacatatttgaatgtatttagaaaaataaacaaataggggttccgcgcacatttccccgaaaagtgccacctgcaggaaacagctatgaccatgattacgccaagctctagctagaggtcgacggtatcgagccccagctggttctttccgcctcagaagccatagagcccaccgcatccccagcatgcctgctattgtcttcccaatcctcccccttgctgtcctgccccaccccaccccccagaatagaatgacacctactcagacaatgcgatgcaatttcctcattttattaggaaaggacagtgggagtggcaccttccagggtcaaggaaggcacgggggaggggcaaacaacagatggctggcaactagaaggcacagtcgaggctga

SEQ ID NO: 180 - DNA, 1566 bp, synthetic construct
  source 1..1566: mol_type = other DNA
ttttaaaagaaaaggggggattggggggtacagtgcaggggaaagaatagtagacataatagcaacagacatacaaactaaagaattacaaaaacaaattacaaaaattcaaaattttcgggtttattacagggacagcagagatccactttggccgcggctcgagggggttggggttgcgccttttccaaggcagccctgggtttgcgcagggacgcggctgctctgggcgtggttccgggaaacgcagcggcgccgaccctgggactcgcacattcttcacgtccgttcgcagcgtcacccggatcttcgccgctacccttgtgggccccccggcgacgcttcctgctccgcccctaagtcgggaaggttccttgcggttcgcggcgtgccggacgtgacaaacggaagccgcacgtctcactagtaccctcgcagacggacagcgccagggagcaatggcagcgcgccgaccgcgatgggctgtggccaatagcggctgctcagcagggcgcgccgagagcagcggccgggaaggggcggtgcgggaggcggggtgtggggcggtagtgtgggccctgttcctgcccgcgcggtgttccgcattctgcaagcctccggagcgcacgtcggcagtcggctccctcgttgaccgaatcaccgacctctctccccagggggatccaccggagcttaccatgaccgagtacaagcccacggtgcgcctcgccacccgcgacgacgtccccagggccgtacgcaccctcgccgccgcgttcgccgactaccccgccacgcgccacaccgtcgatccggaccgccacatcgagcgggtcaccgagctgcaagaactcttcctcacgcgcgtcgggctcgacatcggcaaggtgtgggtcgcggacgacggcgccgcggtggcggtctggaccacgccggagagcgtcgaagcgggggcggtgttcgccgagatcggcccgcgcatggccgagttgagcggttcccggctggccgcgcagcaacagatggaaggcctcctggcgccgcaccggcccaaggagcccgcgtggttcctggccaccgtcggcgtctcgcccgaccaccagggcaagggtctgggcagcgccgtcgtgctccccggagtggaggcggccgagcgcgccggggtgcccgccttcctggaaacctccgcgccccgcaacctccccttctacgagcggctcggcttcaccgtcaccgccgacgtcgaggtgcccgaaggaccgcgcacctggtgcatgacccgcaagcccggtgcctgacgcccgccccacgacccgcagcgcccgaccgaaaggagcgcacgaccccatgcatcggtacctttaagaccaatgacttacaaggcagctgtagatcttagccactttctagagtcggggcggccggccgcttcgagcagacatgataagatacattgatgagtttggacaaaccacaactagaatgcagtgaaaaaaatgctttatttgtgaaatttgtgatgctattgctttatttgtaaccattataagctgcaataaacaagtt

SEQ ID NO: 181 - DNA, 2474 bp, synthetic construct
  source 1..2474: mol_type = other DNA
tcagcgggtttaaactcaatggtgatggtgatgatgaccggttagactttcctcttcttcttgggagaaccaccagaggggggtgtggcggtttcgttgttcagtgtggggagtgtgagcagatcagactgctggggggactctggccgggccccgctcccctccctcttgctggcgtcgtgccgccccccccggcttgtggtgggccggatgctggcccccctggcgttcaaagtctcccgccggtcgcaggccacgttcctatcaatcaacacagcgtgcctctcgatgttcctagcggcgttcatatctctatccatgaccaggccgcagtcggtgcacctaaacaccctatcggagagcttcaagtgggggttctgccagccgcacccgctgcaggtcttgctggaggggaaccacctgtcggccacggccagctcgctcccgtaccaggtggccttgtagttcacctgcctccgcagctcggcaggggcgctgtccaggatgacccggttcagcccggccttctgccggacgttcttccctggggcggccactgtccccctggcggacctggtcatgccggcgacgttcagatcctccagggccaccacggcgaaccctgtggtcagccgcttggtgatctggtgcagggcggcgtgccgccggacggccacctcgtgatgggccctccccacccgccgcttggccttctctctcctggcgctgcccttctgtgtcctggccagggcccgctgggccttgagcagccgcctctcagcctgcctcaggtgctgggggtttctcaccagggcgctgcttgggtcgtcgacgaccaggggcttggacagggcggccagcaccttcacccccaggtccactcccacggcgcccctctcccgctgccgcctgctgggccgatcgggcacctgcactgtcaccttgcagagcacggaggcgtaccacctgtgtccgcccctactcacagtcacggactgcaccacggcgtcgcctctgtcaatgagcctggcgagccgcttgccgctgtcgtgcagcctcacctcgccaatcctaggcagcctcagccttctgtagccagccagcctgatgctgggcttcttcacatcgtggtgcaatctaaagctatcccgagcccggcccttcttcttaaaccgggggtagcccaccctcctccccactctcttgccgctcaggctgtcgagccagttcttccatgcctggtcggcgtcaataaaggcgctctggaaggcgtaggtgttcacctcgtgccaccatgggcaggccccatccaggcccttccgggaatcccccttcacggcgttcagggccttctggatggctggcttcataggcacggggacccggacctgccgccgggcctgctcctcgggcacgccatcgcccacgagcttggccacctcggcccgccaccgctcgtgggcccccaccttggcggcgagggcgtggttgaaggcccacctggcggccccggcgtgccggctcagggcggccacctggacggaagtaggatcgagggcgaaccgaaaggccttcaggatctctgtctgcaccatgaccttcctcttcttcttaggggccatggtggcggctctccctatagtgagtcgtattagcggccgcggatctctagcggatctgacggttcactaaaccagctctgcttatatagacctcccaccgtacacgcctaccgcccatttgcgtcaatggggcggagttgttacgacattttggaaagtcccgttgattttggtgccaaaacaaactcccattgacgtcaatggggtggagacttggaaatccccgtgagtcaaaccgctatccacgcccattgatgtactgccaaaaccgcatcaccatggtaatagcgatgactaatacgtagatgtactgccaagtaggaaagtcccataaggtcatgtactgggcataatgccaggcgggccatttaccgtcattgacgtcaatagggggcgtacttggcatatgatacacttgatgtactgccaagtgggcagtttaccgtaaatactccacccattgacgtcaatggaaagtccctattggcgttactatgggaacatacgtcattattgacgtcaatgggcgggggtcgttgggcggtcagccaggcgggccatttaccgtaagttatgtaacgcggaactccatatatgggctatgaactaatgaccccgtaattgattactattaataactagtcaataatcaatgtcaacgcgtatatctggcccgtacatcgcgaagcagcgcaaaacgcctaaccctaagcagattcttcatgcaattgtcggtcaagaatcgatagtactaacatacgctctccatcaaaacaaaacgaaacaaaacaaactagcaaaataggctgtccccagtgcaagtgcaggtgccagaacatttctctatcgata

SEQ ID NO: 182 - DNA, 673 bp, synthetic construct
  source 1..673: mol_type = other DNA
ggtaccgattagtgaacggatctcgacggtatcgatcacgagactagcctcgagcggccgcccccttcaccgagggcctatttcccatgattccttcatatttgcatatacgatacaaggctgttagagagataattggaattaatttgactgtaaacacaaagatattagtacaaaatacgtgacgtagaaagtaataatttcttgggtagtttgcagttttaaaattatgttttaaaatggactatcatatgcttaccgtaacttgaaagtatttcgatttcttggctttatatatcttgtggaaaggacgaaacaccgaacgcggcccggaacatcgaacgccacgcagtgctgatcgatcgaaacgtcgcctgcgataggcgggagacgctaaacgcccgtggagcatccataagaccaaccacctctcggggcggtaggcacgacgcatcgaagcgggaaggctccggcgctcggcctgagtcacctcagcagagtgatctgctgacgctcccaaccttgaataacgaaacggcaacgcctccatagcggtgcaggtcaataagggtcggccccacgcgtgtagggagcgatcgcgagacccgagagagggtcggtctcctttttttgaattctcgacctcgagacaaatggcagtattcatccacaa

SEQ ID NO: 183 - DNA, 24 bp, synthetic construct
  source 1..24: mol_type = other DNA
atcgagtgacagtatcctctgtat

SEQ ID NO: 184 - DNA, 24 bp, synthetic construct
  source 1..24: mol_type = other DNA
aaaaatacagaggatactgtcact

SEQ ID NO: 185 - DNA, 24 bp, synthetic construct
  source 1..24: mol_type = other DNA
atcgcagctcatttacagacggga

SEQ ID NO: 186 - DNA, 24 bp, synthetic construct
  source 1..24: mol_type = other DNA
aaaatcccgtctgtaaatgagctg

SEQ ID NO: 187 - DNA, 24 bp, synthetic construct
  source 1..24: mol_type = other DNA
atcggagctctacaccacacccaa

SEQ ID NO: 188 - DNA, 24 bp, synthetic construct
  source 1..24: mol_type = other DNA
aaaattgggtgtggtgtagagctc

SEQ ID NO: 189 - DNA, 24 bp, synthetic construct
  source 1..24: mol_type = other DNA
atcgttagcctggcatggtggtgc

SEQ ID NO: 190 - DNA, 24 bp, synthetic construct
  source 1..24: mol_type = other DNA
aaaagcaccaccatgccaggctaa

SEQ ID NO: 191 - DNA, 24 bp, synthetic construct
  source 1..24: mol_type = other DNA
atcgttaatttctaattccggaat

SEQ ID NO: 192 - DNA, 24 bp, synthetic construct
  source 1..24: mol_type = other DNA
aaaaattccggaattagaaattaa

SEQ ID NO: 193 - DNA, 7198 bp, synthetic construct
  source 1..7198: mol_type = other DNA
ggtaccgattagtgaacggatctcgacggtatcgatcacgagactagcctcgagcggccgcccccttcaccgagggcctatttcccatgattccttcatatttgcatatacgatacaaggctgttagagagataattggaattaatttgactgtaaacacaaagatattagtacaaaatacgtgacgtagaaagtaataatttcttgggtagtttgcagttttaaaattatgttttaaaatggactatcatatgcttaccgtaacttgaaagtatttcgatttcttggctttatatatcttgtggaaaggacgaaacaccgaacgcggcccggaacatcgaacgccacgcagtgctgatcgatcgaaacgtcgcctgcgataggcgggagacgctaaacgcccgtggagcatccataagaccaaccacctctcggggcggtaggcacgacgcatcgaagcgggaaggctccggcgctcggcctgagtcacctcagcagagtgatctgctgacgctcccaaccttgaataacgaaacggcaacgcctccatagcggtgcaggtcaataagggtcggccccacgcgtgtagggagcgatcgagtgacagtatcctctgtattttttttgaattctcgacctcgagacaaatggcagtattcatccacaattttaaaagaaaaggggggattggggggtacagtgcaggggaaagaatagtagacataatagcaacagacatacaaactaaagaattacaaaaacaaattacaaaaattcaaaattttcgggtttattacagggacagcagagatccactttggccgcggctcgagggggttggggttgcgccttttccaaggcagccctgggtttgcgcagggacgcggctgctctgggcgtggttccgggaaacgcagcggcgccgaccctgggactcgcacattcttcacgtccgttcgcagcgtcacccggatcttcgccgctacccttgtgggccccccggcgacgcttcctgctccgcccctaagtcgggaaggttccttgcggttcgcggcgtgccggacgtgacaaacggaagccgcacgtctcactagtaccctcgcagacggacagcgccagggagcaatggcagcgcgccgaccgcgatgggctgtggccaatagcggctgctcagcagggcgcgccgagagcagcggccgggaaggggcggtgcgggaggcggggtgtggggcggtagtgtgggccctgttcctgcccgcgcggtgttccgcattctgcaagcctccggagcgcacgtcggcagtcggctccctcgttgaccgaatcaccgacctctctccccagggggatccaccggagcttaccatgaccgagtacaagcccacggtgcgcctcgccacccgcgacgacgtccccagggccgtacgcaccctcgccgccgcgttcgccgactaccccgccacgcgccacaccgtcgatccggaccgccacatcgagcgggtcaccgagctgcaagaactcttcctcacgcgcgtcgggctcgacatcggcaaggtgtgggtcgcggacgacggcgccgcggtggcggtctggaccacgccggagagcgtcgaagcgggggcggtgttcgccgagatcggcccgcgcatggccgagttgagcggttcccggctggccgcgcagcaacagatggaaggcctcctggcgccgcaccggcccaaggagcccgcgtggttcctggccaccgtcggcgtctcgcccgaccaccagggcaagggtctgggcagcgccgtcgtgctccccggagtggaggcggccgagcgcgccggggtgcccgccttcctggaaacctccgcgccccgcaacctccccttctacgagcggctcggcttcaccgtcaccgccgacgtcgaggtgcccgaaggaccgcgcacctggtgcatgacccgcaagcccggtgcctgacgcccgccccacgacccgcagcgcccgaccgaaaggagcgcacgaccccatgcatcggtacctttaagaccaatgacttacaaggcagctgtagatcttagccactttctagagtcggggcggccggccgcttcgagcagacatgataagatacattgatgagtttggacaaaccacaactagaatgcagtgaaaaaaatgctttatttgtgaaatttgtgatgctattgctttatttgtaaccattataagctgcaataaacaagttaacaacaacaattgcattcattttatgtttcaggttcagggggaggtgtgggaggttttttaaagcaagtaaaacctctacaaatgtggtaaaatcgataaggatccgtcgaccgatgcccttgagagccttcaacccagtcagctccttccggtgggcgcggggcatgactatcgtcgccgcacttatgactgtcttctttatcatgcaactcgtaggacaggtgccggcagcgctcttccgcttcctcgctcactgactcgctgcgctcggtcgttcggctgcggcgagcggtatcagctcactcaaaggcggtaatacggttatccacagaatcaggggataacgcaggaaagaacatgtgagcaaaaggccagcaaaaggccaggaaccgtaaaaaggccgcgttgctggcgtttttccataggctccgcccccctgacgagcatcacaaaaatcgacgctcaagtcagaggtggcgaaacccgacaggactataaagataccaggcgtttccccctggaagctccctcgtgcgctctcctgttccgaccctgccgcttaccggatacctgtccgcctttctcccttcgggaagcgtggcgctttctcaatgctcacgctgtaggtatctcagttcggtgtaggtcgttcgctccaagctgggctgtgtgcacgaaccccccgttcagcccgaccgctgcgccttatccggtaactatcgtcttgagtccaacccggtaagacacgacttatcgccactggcagcagccactggtaacaggattagcagagcgaggtatgtaggcggtgctacagagttcttgaagtggtggcctaactacggctacactagaaggacagtatttggtatctgcgctctgctgaagccagttaccttcggaaaaagagttggtagctcttgatccggcaaacaaaccaccgctggtagcggtggtttttttgtttgcaagcagcagattacgcgcagaaaaaaaggatctcaagaagatcctttgatcttttctacggggtctgacgctcagtggaacgaaaactcacgttaagggattttggtcatgagattatcaaaaaggatcttcacctagatccttttaaattaaaaatgaagttttaaatcaatctaaagtatatatgagtaaacttggtctgacagttaccaatgcttaatcagtgaggcacctatctcagcgatctgtctatttcgttcatccatagttgcctgactccccgtcgtgtagataactacgatacgggagggcttaccatctggccccagtgctgcaatgataccgcgggacccacgctcaccggctccagatttatcagcaataaaccagccagccggaagggccgagcgcagaagtggtcctgcaactttatccgcctccatccagtctattaattgttgccgggaagctagagtaagtagttcgccagttaatagtttgcgcaacgttgttgccattgctacaggcatcgtggtgtcacgctcgtcgtttggtatggcttcattcagctccggttcccaacgatcaaggcgagttacatgatcccccatgttgtgcaaaaaagcggttagctccttcggtcctccgatcgttgtcagaagtaagttggccgcagtgttatcactcatggttatggcagcactgcataattctcttactgtcatgccatccgtaagatgcttttctgtgactggtgagtactcaaccaagtcattctgagaatagtgtatgcggcgaccgagttgctcttgcccggcgtcaatacgggataataccgcgccacatagcagaactttaaaagtgctcatcattggaaaacgttcttcggggcgaaaactctcaaggatcttaccgctgttgagatccagttcgatgtaacccactcgtgcacccaactgatcttcagcatcttttactttcaccagcgtttctgggtgagcaaaaacaggaaggcaaaatgccgcaaaaaagggaataagggcgacacggaaatgttgaatactcatactcttcctttttcaatattattgaagcatttatcagggttattgtctcatgagcggatacatatttgaatgtatttagaaaaataaacaaataggggttccgcgcacatttccccgaaaagtgccacctgcaggaaacagctatgaccatgattacgccaagctctagctagaggtcgacggtatcgagccccagctggttctttccgcctcagaagccatagagcccaccgcatccccagcatgcctgctattgtcttcccaatcctcccccttgctgtcctgccccaccccaccccccagaatagaatgacacctactcagacaatgcgatgcaatttcctcattttattaggaaaggacagtgggagtggcaccttccagggtcaaggaaggcacgggggaggggcaaacaacagatggctggcaactagaaggcacagtcgaggctgatcagcgggtttaaactcaatggtgatggtgatgatgaccggttagactttcctcttcttcttgggagaaccaccagaggggggtgtggcggtttcgttgttcagtgtggggagtgtgagcagatcagactgctggggggactctggccgggccccgctcccctccctcttgctggcgtcgtgccgccccccccggcttgtggtgggccggatgctggcccccctggcgttcaaagtctcccgccggtcgcaggccacgttcctatcaatcaacacagcgtgcctctcgatgttcctagcggcgttcatatctctatccatgaccaggccgcagtcggtgcacctaaacaccctatcggagagcttcaagtgggggttctgccagccgcacccgctgcaggtcttgctggaggggaaccacctgtcggccacggccagctcgctcccgtaccaggtggccttgtagttcacctgcctccgcagctcggcaggggcgctgtccaggatgacccggttcagcccggccttctgccggacgttcttccctggggcggccactgtccccctggcggacctggtcatgccggcgacgttcagatcctccagggccaccacggcgaaccctgtggtcagccgcttggtgatctggtgcagggcggcgtgccgccggacggccacctcgtgatgggccctccccacccgccgcttggccttctctctcctggcgctgcccttctgtgtcctggccagggcccgctgggccttgagcagccgcctctcagcctgcctcaggtgctgggggtttctcaccagggcgctgcttgggtcgtcgacgaccaggggcttggacagggcggccagcaccttcacccccaggtccactcccacggcgcccctctcccgctgccgcctgctgggccgatcgggcacctgcactgtcaccttgcagagcacggaggcgtaccacctgtgtccgcccctactcacagtcacggactgcaccacggcgtcgcctctgtcaatgagcctggcgagccgcttgccgctgtcgtgcagcctcacctcgccaatcctaggcagcctcagccttctgtagccagccagcctgatgctgggcttcttcacatcgtggtgcaatctaaagctatcccgagcccggcccttcttcttaaaccgggggtagcccaccctcctccccactctcttgccgctcaggctgtcgagccagttcttccatgcctggtcggcgtcaataaaggcgctctggaaggcgtaggtgttcacctcgtgccaccatgggcaggccccatccaggcccttccgggaatcccccttcacggcgttcagggccttctggatggctggcttcataggcacggggacccggacctgccgccgggcctgctcctcgggcacgccatcgcccacgagcttggccacctcggcccgccaccgctcgtgggcccccaccttggcggcgagggcgtggttgaaggcccacctggcggccccggcgtgccggctcagggcggccacctggacggaagtaggatcgagggcgaaccgaaaggccttcaggatctctgtctgcaccatgaccttcctcttcttcttaggggccatggtggcggctctccctatagtgagtcgtattagcggccgcggatctctagcggatctgacggttcactaaaccagctctgcttatatagacctcccaccgtacacgcctaccgcccatttgcgtcaatggggcggagttgttacgacattttggaaagtcccgttgattttggtgccaaaacaaactcccattgacgtcaatggggtggagacttggaaatccccgtgagtcaaaccgctatccacgcccattgatgtactgccaaaaccgcatcaccatggtaatagcgatgactaatacgtagatgtactgccaagtaggaaagtcccataaggtcatgtactgggcataatgccaggcgggccatttaccgtcattgacgtcaatagggggcgtacttggcatatgatacacttgatgtactgccaagtgggcagtttaccgtaaatactccacccattgacgtcaatggaaagtccctattggcgttactatgggaacatacgtcattattgacgtcaatgggcgggggtcgttgggcggtcagccaggcgggccatttaccgtaagttatgtaacgcggaactccatatatgggctatgaactaatgaccccgtaattgattactattaataactagtcaataatcaatgtcaacgcgtatatctggcccgtacatcgcgaagcagcgcaaaacgcctaaccctaagcagattcttcatgcaattgtcggtcaagaatcgatagtactaacatacgctctccatcaaaacaaaacgaaacaaaacaaactagcaaaataggctgtccccagtgcaagtgcaggtgccagaacatttctctatcgata

SEQ ID NO: 194 - DNA, 7198 bp, synthetic construct
  source 1..7198: mol_type = other DNA
ggtaccgattagtgaacggatctcgacggtatcgatcacgagactagcctcgagcggccgcccccttcaccgagggcctatttcccatgattccttcatatttgcatatacgatacaaggctgttagagagataattggaattaatttgactgtaaacacaaagatattagtacaaaatacgtgacgtagaaagtaataatttcttgggtagtttgcagttttaaaattatgttttaaaatggactatcatatgcttaccgtaacttgaaagtatttcgatttcttggctttatatatcttgtggaaaggacgaaacaccgaacgcggcccggaacatcgaacgccacgcagtgctgatcgatcgaaacgtcgcctgcgataggcgggagacgctaaacgcccgtggagcatccataagaccaaccacctctcggggcggtaggcacgacgcatcgaagcgggaaggctccggcgctcggcctgagtcacctcagcagagtgatctgctgacgctcccaaccttgaataacgaaacggcaacgcctccatagcggtgcaggtcaataagggtcggccccacgcgtgtagggagcgatcgcagctcatttacagacgggatttttttgaattctcgacctcgagacaaatggcagtattcatccacaattttaaaagaaaaggggggattggggggtacagtgcaggggaaagaatagtagacataatagcaacagacatacaaactaaagaattacaaaaacaaattacaaaaattcaaaattttcgggtttattacagggacagcagagatccactttggccgcggctcgagggggttggggttgcgccttttccaaggcagccctgggtttgcgcagggacgcggctgctctgggcgtggttccgggaaacgcagcggcgccgaccctgggactcgcacattcttcacgtccgttcgcagcgtcacccggatcttcgccgctacccttgtgggccccccggcgacgcttcctgctccgcccctaagtcgggaaggttccttgcggttcgcggcgtgccggacgtgacaaacggaagccgcacgtctcactagtaccctcgcagacggacagcgccagggagcaatggcagcgcgccgaccgcgatgggctgtggccaatagcggctgctcagcagggcgcgccgagagcagcggccgggaaggggcggtgcgggaggcggggtgtggggcggtagtgtgggccctgttcctgcccgcgcggtgttccgcattctgcaagcctccggagcgcacgtcggcagtcggctccctcgttgaccgaatcaccgacctctctccccagggggatccaccggagcttaccatgaccgagtacaagcccacggtgcgcctcgccacccgcgacgacgtccccagggccgtacgcaccctcgccgccgcgttcgccgactaccccgccacgcgccacaccgtcgatccggaccgccacatcgagcgggtcaccgagctgcaagaactcttcctcacgcgcgtcgggctcgacatcggcaaggtgtgggtcgcggacgacggcgccgcggtggcggtctggaccacgccggagagcgtcgaagcgggggcggtgttcgccgagatcggcccgcgcatggccgagttgagcggttcccggctggccgcgcagcaacagatggaaggcctcctggcgccgcaccggcccaaggagcccgcgtggttcctggccaccgtcggcgtctcgcccgaccaccagggcaagggtctgggcagcgccgtcgtgctccccggagtggaggcggccgagcgcgccggggtgcccgccttcctggaaacctccgcgccccgcaacctccccttctacgagcggctcggcttcaccgtcaccgccgacgtcgaggtgcccgaaggaccgcgcacctggtgcatgacccgcaagcccggtgcctgacgcccgccccacgacccgcagcgcccgaccgaaaggagcgcacgaccccatgcatcggtacctttaagaccaatgacttacaaggcagctgtagatcttagccactttctagagtcggggcggccggccgcttcgagcagacatgataagatacattgatgagtttggacaaaccacaactagaatgcagtgaaaaaaatgctttatttgtgaaatttgtgatgctattgctttatttgtaaccattataagctgcaataaacaagttaacaacaacaattgcattcattttatgtttcaggttcagggggaggtgtgggaggttttttaaagcaagtaaaacctctacaaatgtggtaaaatcgataaggatccgtcgaccgatgcccttgagagccttcaacccagtcagctccttccggtgggcgcggggcatgactatcgtcgccgcacttatgactgtcttctttatcatgcaactcgtaggacaggtgccggcagcgctcttccgcttcctcgctcactgactcgctgcgctcggtcgttcggctgcggcgagcggtatcagctcactcaaaggcggtaatacggttatccacagaatcaggggataacgcaggaaagaacatgtgagcaaaaggccagcaaaaggccaggaaccgtaaaaaggccgcgttgctggcgtttttccataggctccgcccccctgacgagcatcacaaaaatcgacgctcaagtcagaggtggcgaaacccgacaggactataaagataccaggcgtttccccctggaagctccctcgtgcgctctcctgttccgaccctgccgcttaccggatacctgtccgcctttctcccttcgggaagcgtggcgctttctcaatgctcacgctgtaggtatctcagttcggtgtaggtcgttcgctccaagctgggctgtgtgcacgaaccccccgttcagcccgaccgctgcgccttatccggtaactatcgtcttgagtccaacccggtaagacacgacttatcgccactggcagcagccactggtaacaggattagcagagcgaggtatgtaggcggtgctacagagttcttgaagtggtggcctaactacggctacactagaaggacagtatttggtatctgcgctctgctgaagccagttaccttcggaaaaagagttggtagctcttgatccggcaaacaaaccaccgctggtagcggtggtttttttgtttgcaagcagcagattacgcgcagaaaaaaaggatctcaagaagatcctttgatcttttctacggggtctgacgctcagtggaacgaaaactcacgttaagggattttggtcatgagattatcaaaaaggatcttcacctagatccttttaaattaaaaatgaagttttaaatcaatctaaagtatatatgagtaaacttggtctgacagttaccaatgcttaatcagtgaggcacctatctcagcgatctgtctatttcgttcatccatagttgcctgactccccgtcgtgtagataactacgatacgggagggcttaccatctggccccagtgctgcaatgataccgcgggacccacgctcaccggctccagatttatcagcaataaaccagccagccggaagggccgagcgcagaagtggtcctgcaactttatccgcctccatccagtctattaattgttgccgggaagctagagtaagtagttcgccagttaatagtttgcgcaacgttgttgccattgctacaggcatcgtggtgtcacgctcgtcgtttggtatggcttcattcagctccggttcccaacgatcaaggcgagttacatgatcccccatgttgtgcaaaaaagcggttagctccttcggtcctccgatcgttgtcagaagtaagttggccgcagtgttatcactcatggttatggcagcactgcataattctcttactgtcatgccatccgtaagatgcttttctgtgactggtgagtactcaaccaagtcattctgagaatagtgtatgcggcgaccgagttgctcttgcccggcgtcaatacgggataataccgcgccacatagcagaactttaaaagtgctcatcattggaaaacgttcttcggggcgaaaactctcaaggatcttaccgctgttgagatccagttcgatgtaacccactcgtgcacccaactgatcttcagcatcttttactttcaccagcgtttctgggtgagcaaaaacaggaaggcaaaatgccgcaaaaaagggaataagggcgacacggaaatgttgaatactcatactcttcctttttcaatattattgaagcatttatcagggttattgtctcatgagcggatacatatttgaatgtatttagaaaaataaacaaataggggttccgcgcacatttccccgaaaagtgccacctgcaggaaacagctatgaccatgattacgccaagctctagctagaggtcgacggtatcgagccccagctggttctttccgcctcagaagccatagagcccaccgcatccccagcatgcctgctattgtcttcccaatcctcccccttgctgtcctgccccaccccaccccccagaatagaatgacacctactcagacaatgcgatgcaatttcctcattttattaggaaaggacagtgggagtggcaccttccagggtcaaggaaggcacgggggaggggcaaacaacagatggctggcaactagaaggcacagtcgaggctgatcagcgggtttaaactcaatggtgatggtgatgatgaccggttagactttcctcttcttcttgggagaaccaccagaggggggtgtggcggtttcgttgttcagtgtggggagtgtgagcagatcagactgctggggggactctggccgggccccgctcccctccctcttgctggcgtcgtgccgccccccccggcttgtggtgggccggatgctggcccccctggcgttcaaagtctcccgccggtcgcaggccacgttcctatcaatcaacacagcgtgcctctcgatgttcctagcggcgttcatatctctatccatgaccaggccgcagtcggtgcacctaaacaccctatcggagagcttcaagtgggggttctgccagccgcacccgctgcaggtcttgctggaggggaaccacctgtcggccacggccagctcgctcccgtaccaggtggccttgtagttcacctgcctccgcagctcggcaggggcgctgtccaggatgacccggttcagcccggccttctgccggacgttcttccctggggcggccactgtccccctggcggacctggtcatgccggcgacgttcagatcctccagggccaccacggcgaaccctgtggtcagccgcttggtgatctggtgcagggcggcgtgccgccggacggccacctcgtgatgggccctccccacccgccgcttggccttctctctcctggcgctgcccttctgtgtcctggccagggcccgctgggccttgagcagccgcctctcagcctgcctcaggtgctgggggtttctcaccagggcgctgcttgggtcgtcgacgaccaggggcttggacagggcggccagcaccttcacccccaggtccactcccacggcgcccctctcccgctgccgcctgctgggccgatcgggcacctgcactgtcaccttgcagagcacggaggcgtaccacctgtgtccgcccctactcacagtcacggactgcaccacggcgtcgcctctgtcaatgagcctggcgagccgcttgccgctgtcgtgcagcctcacctcgccaatcctaggcagcctcagccttctgtagccagccagcctgatgctgggcttcttcacatcgtggtgcaatctaaagctatcccgagcccggcccttcttcttaaaccgggggtagcccaccctcctccccactctcttgccgctcaggctgtcgagccagttcttccatgcctggtcggcgtcaataaaggcgctctggaaggcgtaggtgttcacctcgtgccaccatgggcaggccccatccaggcccttccgggaatcccccttcacggcgttcagggccttctggatggctggcttcataggcacggggacccggacctgccgccgggcctgctcctcgggcacgccatcgcccacgagcttggccacctcggcccgccaccgctcgtgggcccccaccttggcggcgagggcgtggttgaaggcccacctggcggccccggcgtgccggctcagggcggccacctggacggaagtaggatcgagggcgaaccgaaaggccttcaggatctctgtctgcaccatgaccttcctcttcttcttaggggccatggtggcggctctccctatagtgagtcgtattagcggccgcggatctctagcggatctgacggttcactaaaccagctctgcttatatagacctcccaccgtacacgcctaccgcccatttgcgtcaatggggcggagttgttacgacattttggaaagtcccgttgattttggtgccaaaacaaactcccattgacgtcaatggggtggagacttggaaatccccgtgagtcaaaccgctatccacgcccattgatgtactgccaaaaccgcatcaccatggtaatagcgatgactaatacgtagatgtactgccaagtaggaaagtcccataaggtcatgtactgggcataatgccaggcgggccatttaccgtcattgacgtcaatagggggcgtacttggcatatgatacacttgatgtactgccaagtgggcagtttaccgtaaatactccacccattgacgtcaatggaaagtccctattggcgttactatgggaacatacgtcattattgacgtcaatgggcgggggtcgttgggcggtcagccaggcgggccatttaccgtaagttatgtaacgcggaactccatatatgggctatgaactaatgaccccgtaattgattactattaataactagtcaataatcaatgtcaacgcgtatatctggcccgtacatcgcgaagcagcgcaaaacgcctaaccctaagcagattcttcatgcaattgtcggtcaagaatcgatagtactaacatacgctctccatcaaaacaaaacgaaacaaaacaaactagcaaaataggctgtccccagtgcaagtgcaggtgccagaacatttctctatcgata

SEQ ID NO: 195 - DNA, 7198 bp, synthetic construct
  source 1..7198: mol_type = other DNA
ggtaccgattagtgaacggatctcgacggtatcgatcacgagactagcctcgagcggccgcccccttcaccgagggcctatttcccatgattccttcatatttgcatatacgatacaaggctgttagagagataattggaattaatttgactgtaaacacaaagatattagtacaaaatacgtgacgtagaaagtaataatttcttgggtagtttgcagttttaaaattatgttttaaaatggactatcatatgcttaccgtaacttgaaagtatttcgatttcttggctttatatatcttgtggaaaggacgaaacaccgaacgcggcccggaacatcgaacgccacgcagtgctgatcgatcgaaacgtcgcctgcgataggcgggagacgctaaacgcccgtggagcatccataagaccaaccacctctcggggcggtaggcacgacgcatcgaagcgggaaggctccggcgctcggcctgagtcacctcagcagagtgatctgctgacgctcccaaccttgaataacgaaacggcaacgcctccatagcggtgcaggtcaataagggtcggccccacgcgtgtagggagcgatcggagctctacaccacacccaatttttttgaattctcgacctcgagacaaatggcagtattcatccacaattttaaaagaaaaggggggattggggggtacagtgcaggggaaagaatagtagacataatagcaacagacatacaaactaaagaattacaaaaacaaattacaaaaattcaaaattttcgggtttattacagggacagcagagatccactttggccgcggctcgagggggttggggttgcgccttttccaaggcagccctgggtttgcgcagggacgcggctgctctgggcgtggttccgggaaacgcagcggcgccgaccctgggactcgcacattcttcacgtccgttcgcagcgtcacccggatcttcgccgctacccttgtgggccccccggcgacgcttcctgctccgcccctaagtcgggaaggttccttgcggttcgcggcgtgccggacgtgacaaacggaagccgcacgtctcactagtaccctcgcagacggacagcgccagggagcaatggcagcgcgccgaccgcgatgggctgtggccaatagcggctgctcagcagggcgcgccgagagcagcggccgggaaggggcggtgcgggaggcggggtgtggggcggtagtgtgggccctgttcctgcccgcgcggtgttccgcattctgcaagcctccggagcgcacgtcggcagtcggctccctcgttgaccgaatcaccgacctctctccccagggggatccaccggagcttaccatgaccgagtacaagcccacggtgcgcctcgccacccgcgacgacgtccccagggccgtacgcaccctcgccgccgcgttcgccgactaccccgccacgcgccacaccgtcgatccggaccgccacatcgagcgggtcaccgagctgcaagaactcttcctcacgcgcgtcgggctcgacatcggcaaggtgtgggtcgcggacgacggcgccgcggtggcggtctggaccacgccggagagcgtcgaagcgggggcggtgttcgccgagatcggcccgcgcatggccgagttgagcggttcccggctggccgcgcagcaacagatggaaggcctcctggcgccgcaccggcccaaggagcccgcgtggttcctggccaccgtcggcgtctcgcccgaccaccagggcaagggtctgggcagcgccgtcgtgctccccggagtggaggcggccgagcgcgccggggtgcccgccttcctggaaacctccgcgccccgcaacctccccttctacgagcggctcggcttcaccgtcaccgccgacgtcgaggtgcccgaaggaccgcgcacctggtgcatgacccgcaagcccggtgcctgacgcccgccccacgacccgcagcgcccgaccgaaaggagcgcacgaccccatgcatcggtacctttaagaccaatgacttacaaggcagctgtagatcttagccactttctagagtcggggcggccggccgcttcgagcagacatgataagatacattgatgagtttggacaaaccacaactagaatgcagtgaaaaaaatgctttatttgtgaaatttgtgatgctattgctttatttgtaaccattataagctgcaataaacaagttaacaacaacaattgcattcattttatgtttcaggttcagggggaggtgtgggaggttttttaaagcaagtaaaacctctacaaatgtggtaaaatcgataaggatccgtcgaccgatgcccttgagagccttcaacccagtcagctccttccggtgggcgcggggcatgactatcgtcgccgcacttatgactgtcttctttatcatgcaactcgtaggacaggtgccggcagcgctcttccgcttcctcgctcactgactcgctgcgctcggtcgttcggctgcggcgagcggtatcagctcactcaaaggcggtaatacggttatccacagaatcaggggataacgcaggaaagaacatgtgagcaaaaggccagcaaaaggccaggaaccgtaaaaaggccgcgttgctggcgtttttccataggctccgcccccctgacgagcatcacaaaaatcgacgctcaagtcagaggtggcgaaacccgacaggactataaagataccaggcgtttccccctggaagctccctcgtgcgctctcctgttccgaccctgccgcttaccggatacctgtccgcctttctcccttcgggaagcgtggcgctttctcaatgctcacgctgtaggtatctcagttcggtgtaggtcgttcgctccaagctgggctgtgtgcacgaaccccccgttcagcccgaccgctgcgccttatccggtaactatcgtcttgagtccaacccggtaagacacgacttatcgccactggcagcagccactggtaacaggattagcagagcgaggtatgtaggcggtgctacagagttcttgaagtggtggcctaactacggctacactagaaggacagtatttggtatctgcgctctgctgaagccagttaccttcggaaaaagagttggtagctcttgatccggcaaacaaaccaccgctggtagcggtggtttttttgtttgcaagcagcagattacgcgcagaaaaaaaggatctcaagaagatcctttgatcttttctacggggtctgacgctcagtggaacgaaaactcacgttaagggattttggtcatgagattatcaaaaaggatcttcacctagatccttttaaattaaaaatgaagttttaaatcaatctaaagtatatatgagtaaacttggtctgacagttaccaatgcttaatcagtgaggcacctatctcagcgatctgtctatttcgttcatccatagttgcctgactccccgtcgtgtagataactacgatacgggagggcttaccatctggccccagtgctgcaatgataccgcgggacccacgctcaccggctccagatttatcagcaataaaccagccagccggaagggccgagcgcagaagtggtcctgcaactttatccgcctccatccagtctattaattgttgccgggaagctagagtaagtagttcgccagttaatagtttgcgcaacgttgttgccattgctacaggcatcgtggtgtcacgctcgtcgtttggtatggcttcattcagctccggttcccaacgatcaaggcgagttacatgatcccccatgttgtgcaaaaaagcggttagctccttcggtcctccgatcgttgtcagaagtaagttggccgcagtgttatcactcatggttatggcagcactgcataattctcttactgtcatgccatccgtaagatgcttttctgtgactggtgagtactcaaccaagtcattctgagaatagtgtatgcggcgaccgagttgctcttgcccggcgtcaatacgggataataccgcgccacatagcagaactttaaaagtgctcatcattggaaaacgttcttcggggcgaaaactctcaaggatcttaccgctgttgagatccagttcgatgtaacccactcgtgcacccaactgatcttcagcatcttttactttcaccagcgtttctgggtgagcaaaaacaggaaggcaaaatgccgcaaaaaagggaataagggcgacacggaaatgttgaatactcatactcttcctttttcaatattattgaagcatttatcagggttattgtctcatgagcggatacatatttgaatgtatttagaaaaataaacaaataggggttccgcgcacatttccccgaaaagtgccacctgcaggaaacagctatgaccatgattacgccaagctctagctagaggtcgacggtatcgagccccagctggttctttccgcctcagaagccatagagcccaccgcatccccagcatgcctgctattgtcttcccaatcctcccccttgctgtcctgccccaccccaccccccagaatagaatgacacctactcagacaatgcgatgcaatttcctcattttattaggaaaggacagtgggagtggcaccttccagggtcaaggaaggcacgggggaggggcaaacaacagatggctggcaactagaaggcacagtcgaggctgatcagcgggtttaaactcaatggtgatggtgatgatgaccggttagactttcctcttcttcttgggagaaccaccagaggggggtgtggcggtttcgttgttcagtgtggggagtgtgagcagatcagactgctggggggactctggccgggccccgctcccctccctcttgctggcgtcgtgccgccccccccggcttgtggtgggccggatgctggcccccctggcgttcaaagtctcccgccggtcgcaggccacgttcctatcaatcaacacagcgtgcctctcgatgttcctagcggcgttcatatctctatccatgaccaggccgcagtcggtgcacctaaacaccctatcggagagcttcaagtgggggttctgccagccgcacccgctgcaggtcttgctggaggggaaccacctgtcggccacggccagctcgctcccgtaccaggtggccttgtagttcacctgcctccgcagctcggcaggggcgctgtccaggatgacccggttcagcccggccttctgccggacgttcttccctggggcggccactgtccccctggcggacctggtcatgccggcgacgttcagatcctccagggccaccacggcgaaccctgtggtcagccgcttggtgatctggtgcagggcggcgtgccgccggacggccacctcgtgatgggccctccccacccgccgcttggccttctctctcctggcgctgcccttctgtgtcctggccagggcccgctgggccttgagcagccgcctctcagcctgcctcaggtgctgggggtttctcaccagggcgctgcttgggtcgtcgacgaccaggggcttggacagggcggccagcaccttcacccccaggtccactcccacggcgcccctctcccgctgccgcctgctgggccgatcgggcacctgcactgtcaccttgcagagcacggaggcgtaccacctgtgtccgcccctactcacagtcacggactgcaccacggcgtcgcctctgtcaatgagcctggcgagccgcttgccgctgtcgtgcagcctcacctcgccaatcctaggcagcctcagccttctgtagccagccagcctgatgctgggcttcttcacatcgtggtgcaatctaaagctatcccgagcccggcccttcttcttaaaccgggggtagcccaccctcctccccactctcttgccgctcaggctgtcgagccagttcttccatgcctggtcggcgtcaataaaggcgctctggaaggcgtaggtgttcacctcgtgccaccatgggcaggccccatccaggcccttccgggaatcccccttcacggcgttcagggccttctggatggctggcttcataggcacggggacccggacctgccgccgggcctgctcctcgggcacgccatcgcccacgagcttggccacctcggcccgccaccgctcgtgggcccccaccttggcggcgagggcgtggttgaaggcccacctggcggccccggcgtgccggctcagggcggccacctggacggaagtaggatcgagggcgaaccgaaaggccttcaggatctctgtctgcaccatgaccttcctcttcttcttaggggccatggtggcggctctccctatagtgagtcgtattagcggccgcggatctctagcggatctgacggttcactaaaccagctctgcttatatagacctcccaccgtacacgcctaccgcccatttgcgtcaatggggcggagttgttacgacattttggaaagtcccgttgattttggtgccaaaacaaactcccattgacgtcaatggggtggagacttggaaatccccgtgagtcaaaccgctatccacgcccattgatgtactgccaaaaccgcatcaccatggtaatagcgatgactaatacgtagatgtactgccaagtaggaaagtcccataaggtcatgtactgggcataatgccaggcgggccatttaccgtcattgacgtcaatagggggcgtacttggcatatgatacacttgatgtactgccaagtgggcagtttaccgtaaatactccacccattgacgtcaatggaaagtccctattggcgttactatgggaacatacgtcattattgacgtcaatgggcgggggtcgttgggcggtcagccaggcgggccatttaccgtaagttatgtaacgcggaactccatatatgggctatgaactaatgaccccgtaattgattactattaataactagtcaataatcaatgtcaacgcgtatatctggcccgtacatcgcgaagcagcgcaaaacgcctaaccctaagcagattcttcatgcaattgtcggtcaagaatcgatagtactaacatacgctctccatcaaaacaaaacgaaacaaaacaaactagcaaaataggctgtccccagtgcaagtgcaggtgccagaacatttctctatcgata

SEQ ID NO: 196 - DNA, 7198 bp, synthetic construct
  source 1..7198: mol_type = other DNA
ggtaccgattagtgaacggatctcgacggtatcgatcacgagactagcctcgagcggccgcccccttcaccgagggcctatttcccatgattccttcatatttgcatatacgatacaaggctgttagagagataattggaattaatttgactgtaaacacaaagatattagtacaaaatacgtgacgtagaaagtaataatttcttgggtagtttgcagttttaaaattatgttttaaaatggactatcatatgcttaccgtaacttgaaagtatttcgatttcttggctttatatatcttgtggaaaggacgaaacaccgaacgcggcccggaacatcgaacgccacgcagtgctgatcgatcgaaacgtcgcctgcgataggcgggagacgctaaacgcccgtggagcatccataagaccaaccacctctcggggcggtaggcacgacgcatcgaagcgggaaggctccggcgctcggcctgagtcacctcagcagagtgatctgctgacgctcccaaccttgaataacgaaacggcaacgcctccatagcggtgcaggtcaataagggtcggccccacgcgtgtagggagcgatcgttagcctggcatggtggtgctttttttgaattctcgacctcgagacaaatggcagtattcatccacaattttaaaagaaaaggggggattggggggtacagtgcaggggaaagaatagtagacataatagcaacagacatacaaactaaagaattacaaaaacaaattacaaaaattcaaaattttcgggtttattacagggacagcagagatccactttggccgcggctcgagggggttggggttgcgccttttccaaggcagccctgggtttgcgcagggacgcggctgctctgggcgtggttccgggaaacgcagcggcgccgaccctgggactcgcacattcttcacgtccgttcgcagcgtcacccggatcttcgccgctacccttgtgggccccccggcgacgcttcctgctccgcccctaagtcgggaaggttccttgcggttcgcggcgtgccggacgtgacaaacggaagccgcacgtctcactagtaccctcgcagacggacagcgccagggagcaatggcagcgcgccgaccgcgatgggctgtggccaatagcggctgctcagcagggcgcgccgagagcagcggccgggaaggggcggtgcgggaggcggggtgtggggcggtagtgtgggccctgttcctgcccgcgcggtgttccgcattctgcaagcctccggagcgcacgtcggcagtcggctccctcgttgaccgaatcaccgacctctctccccagggggatccaccggagcttaccatgaccgagtacaagcccacggtgcgcctcgccacccgcgacgacgtccccagggccgtacgcaccctcgccgccgcgttcgccgactaccccgccacgcgccacaccgtcgatccggaccgccacatcgagcgggtcaccgagctgcaagaactcttcctcacgcgcgtcgggctcgacatcggcaaggtgtgggtcgcggacgacggcgccgcggtggcggtctggaccacgccggagagcgtcgaagcgggggcggtgttcgccgagatcggcccgcgcatggccgagttgagcggttcccggctggccgcgcagcaacagatggaaggcctcctggcgccgcaccggcccaaggagcccgcgtggttcctggccaccgtcggcgtctcgcccgaccaccagggcaagggtctgggcagcgccgtcgtgctccccggagtggaggcggccgagcgcgccggggtgcccgccttcctggaaacctccgcgccccgcaacctccccttctacgagcggctcggcttcaccgtcaccgccgacgtcgaggtgcccgaaggaccgcgcacctggtgcatgacccgcaagcccggtgcctgacgcccgccccacgacccgcagcgcccgaccgaaaggagcgcacgaccccatgcatcggtacctttaagaccaatgacttacaaggcagctgtagatcttagccactttctagagtcggggcggccggccgcttcgagcagacatgataagatacattgatgagtttggacaaaccacaactagaatgcagtgaaaaaaatgctttatttgtgaaatttgtgatgctattgctttatttgtaaccattataagctgcaataaacaagttaacaacaacaattgcattcattttatgtttcaggttcagggggaggtgtgggaggttttttaaagcaagtaaaacctctacaaatgtggtaaaatcgataaggatccgtcgaccgatgcccttgagagccttcaacccagtcagctccttccggtgggcgcggggcatgactatcgtcgccgcacttatgactgtcttctttatcatgcaactcgtaggacaggtgccggcagcgctcttccgcttcctcgctcactgactcgctgcgctcggtcgttcggctgcggcgagcggtatcagctcactcaaaggcggtaatacggttatccacagaatcaggggataacgcaggaaagaacatgtgagcaaaaggccagcaaaaggccaggaaccgtaaaaaggccgcgttgctggcgtttttccataggctccgcccccctgacgagcatcacaaaaatcgacgctcaagtcagaggtggcgaaacccgacaggactataaagataccaggcgtttccccctggaagctccctcgtgcgctctcctgttccgaccctgccgcttaccggatacctgtccgcctttctcccttcgggaagcgtggcgctttctcaatgctcacgctgtaggtatctcagttcggtgtaggtcgttcgctccaagctgggctgtgtgcacgaaccccccgttcagcccgaccgctgcgccttatccggtaactatcgtcttgagtccaacccggtaagacacgacttatcgccactggcagcagccactggtaacaggattagcagagcgaggtatgtaggcggtgctacagagttcttgaagtggtggcctaactacggctacactagaaggacagtatttggtatctgcgctctgctgaagccagttaccttcggaaaaagagttggtagctcttgatccggcaaacaaaccaccgctggtagcggtggtttttttgtttgcaagcagcagattacgcgcagaaaaaaaggatctcaagaagatcctttgatcttttctacggggtctgacgctcagtggaacgaaaactcacgttaagggattttggtcatgagattatcaaaaaggatcttcacctagatccttttaaattaaaaatgaagttttaaatcaatctaaagtatatatgagtaaacttggtctgacagttaccaatgcttaatcagtgaggcacctatctcagcgatctgtctatttcgttcatccatagttgcctgactccccgtcgtgtagataactacgatacgggagggcttaccatctggccccagtgctgcaatgataccgcgggacccacgctcaccggctccagatttatcagcaataaaccagccagccggaagggccgagcgcagaagtggtcctgcaactttatccgcctccatccagtctattaattgttgccgggaagctagagtaagtagttcgccagttaatagtttgcgcaacgttgttgccattgctacaggcatcgtggtgtcacgctcgtcgtttggtatggcttcattcagctccggttcccaacgatcaaggcgagttacatgatcccccatgttgtgcaaaaaagcggttagctccttcggtcctccgatcgttgtcagaagtaagttggccgcagtgttatcactcatggttatggcagcactgcataattctcttactgtcatgccatccgtaagatgcttttctgtgactggtgagtactcaaccaagtcattctgagaatagtgtatgcggcgaccgagttgctcttgcccggcgtcaatacgggataataccgcgccacatagcagaactttaaaagtgctcatcattggaaaacgttcttcggggcgaaaactctcaaggatcttaccgctgttgagatccagttcgatgtaacccactcgtgcacccaactgatcttcagcatcttttactttcaccagcgtttctgggtgagcaaaaacaggaaggcaaaatgccgcaaaaaagggaataagggcgacacggaaatgttgaatactcatactcttcctttttcaatattattgaagcatttatcagggttattgtctcatgagcggatacatatttgaatgtatttagaaaaataaacaaataggggttccgcgcacatttccccgaaaagtgccacctgcaggaaacagctatgaccatgattacgccaagctctagctagaggtcgacggtatcgagccccagctggttctttccgcctcagaagccatagagcccaccgcatccccagcatgcctgctattgtcttcccaatcctcccccttgctgtcctgccccaccccaccccccagaatagaatgacacctactcagacaatgcgatgcaatttcctcattttattaggaaaggacagtgggagtggcaccttccagggtcaaggaaggcacgggggaggggcaaacaacagatggctggcaactagaaggcacagtcgaggctgatcagcgggtttaaactcaatggtgatggtgatgatgaccggttagactttcctcttcttcttgggagaaccaccagaggggggtgtggcggtttcgttgttcagtgtggggagtgtgagcagatcagactgctggggggactctggccgggccccgctcccctccctcttgctggcgtcgtgccgccccccccggcttgtggtgggccggatgctggcccccctggcgttcaaagtctcccgccggtcgcaggccacgttcctatcaatcaacacagcgtgcctctcgatgttcctagcggcgttcatatctctatccatgaccaggccgcagtcggtgcacctaaacaccctatcggagagcttcaagtgggggttctgccagccgcacccgctgcaggtcttgctggaggggaaccacctgtcggccacggccagctcgctcccgtaccaggtggccttgtagttcacctgcctccgcagctcggcaggggcgctgtccaggatgacccggttcagcccggccttctgccggacgttcttccctggggcggccactgtccccctggcggacctggtcatgccggcgacgttcagatcctccagggccaccacggcgaaccctgtggtcagccgcttggtgatctggtgcagggcggcgtgccgccggacggccacctcgtgatgggccctccccacccgccgcttggccttctctctcctggcgctgcccttctgtgtcctggccagggcccgctgggccttgagcagccgcctctcagcctgcctcaggtgctgggggtttctcaccagggcgctgcttgggtcgtcgacgaccaggggcttggacagggcggccagcaccttcacccccaggtccactcccacggcgcccctctcccgctgccgcctgctgggccgatcgggcacctgcactgtcaccttgcagagcacggaggcgtaccacctgtgtccgcccctactcacagtcacggactgcaccacggcgtcgcctctgtcaatgagcctggcgagccgcttgccgctgtcgtgcagcctcacctcgccaatcctaggcagcctcagccttctgtagccagccagcctgatgctgggcttcttcacatcgtggtgcaatctaaagctatcccgagcccggcccttcttcttaaaccgggggtagcccaccctcctccccactctcttgccgctcaggctgtcgagccagttcttccatgcctggtcggcgtcaataaaggcgctctggaaggcgtaggtgttcacctcgtgccaccatgggcaggccccatccaggcccttccgggaatcccccttcacggcgttcagggccttctggatggctggcttcataggcacggggacccggacctgccgccgggcctgctcctcgggcacgccatcgcccacgagcttggccacctcggcccgccaccgctcgtgggcccccaccttggcggcgagggcgtggttgaaggcccacctggcggccccggcgtgccggctcagggcggccacctggacggaagtaggatcgagggcgaaccgaaaggccttcaggatctctgtctgcaccatgaccttcctcttcttcttaggggccatggtggcggctctccctatagtgagtcgtattagcggccgcggatctctagcggatctgacggttcactaaaccagctctgcttatatagacctcccaccgtacacgcctaccgcccatttgcgtcaatggggcggagttgttacgacattttggaaagtcccgttgattttggtgccaaaacaaactcccattgacgtcaatggggtggagacttggaaatccccgtgagtcaaaccgctatccacgcccattgatgtactgccaaaaccgcatcaccatggtaatagcgatgactaatacgtagatgtactgccaagtaggaaagtcccataaggtcatgtactgggcataatgccaggcgggccatttaccgtcattgacgtcaatagggggcgtacttggcatatgatacacttgatgtactgccaagtgggcagtttaccgtaaatactccacccattgacgtcaatggaaagtccctattggcgttactatgggaacatacgtcattattgacgtcaatgggcgggggtcgttgggcggtcagccaggcgggccatttaccgtaagttatgtaacgcggaactccatatatgggctatgaactaatgaccccgtaattgattactattaataactagtcaataatcaatgtcaacgcgtatatctggcccgtacatcgcgaagcagcgcaaaacgcctaaccctaagcagattcttcatgcaattgtcggtcaagaatcgatagtactaacatacgctctccatcaaaacaaaacgaaacaaaacaaactagcaaaataggctgtccccagtgcaagtgcaggtgccagaacatttctctatcgata

SEQ ID NO: 197 - DNA, 7198 bp, synthetic construct
  source 1..7198: mol_type = other DNA
ggtaccgattagtgaacggatctcgacggtatcgatcacgagactagcctcgagcggccgcccccttcaccgagggcctatttcccatgattccttcatatttgcatatacgatacaaggctgttagagagataattggaattaatttgactgtaaacacaaagatattagtacaaaatacgtgacgtagaaagtaataatttcttgggtagtttgcagttttaaaattatgttttaaaatggactatcatatgcttaccgtaacttgaaagtatttcgatttcttggctttatatatcttgtggaaaggacgaaacaccgaacgcggcccggaacatcgaacgccacgcagtgctgatcgatcgaaacgtcgcctgcgataggcgggagacgctaaacgcccgtggagcatccataagaccaaccacctctcggggcggtaggcacgacgcatcgaagcgggaaggctccggcgctcggcctgagtcacctcagcagagtgatctgctgacgctcccaaccttgaataacgaaacggcaacgcctccatagcggtgcaggtcaataagggtcggccccacgcgtgtagggagcgatcgttaatttctaattccggaattttttttgaattctcgacctcgagacaaatggcagtattcatccacaattttaaaagaaaaggggggattggggggtacagtgcaggggaaagaatagtagacataatagcaacagacatacaaactaaagaattacaaaaacaaattacaaaaattcaaaattttcgggtttattacagggacagcagagatccactttggccgcggctcgagggggttggggttgcgccttttccaaggcagccctgggtttgcgcagggacgcggctgctctgggcgtggttccgggaaacgcagcggcgccgaccctgggactcgcacattcttcacgtccgttcgcagcgtcacccggatcttcgccgctacccttgtgggccccccggcgacgcttcctgctccgcccctaagtcgggaaggttccttgcggttcgcggcgtgccggacgtgacaaacggaagccgcacgtctcactagtaccctcgcagacggacagcgccagggagcaatggcagcgcgccgaccgcgatgggctgtggccaatagcggctgctcagcagggcgcgccgagagcagcggccgggaaggggcggtgcgggaggcggggtgtggggcggtagtgtgggccctgttcctgcccgcgcggtgttccgcattctgcaagcctccggagcgcacgtcggcagtcggctccctcgttgaccgaatcaccgacctctctccccagggggatccaccggagcttaccatgaccgagtacaagcccacggtgcgcctcgccacccgcgacgacgtccccagggccgtacgcaccctcgccgccgcgttcgccgactaccccgccacgcgccacaccgtcgatccggaccgccacatcgagcgggtcaccgagctgcaagaactcttcctcacgcgcgtcgggctcgacatcggcaaggtgtgggtcgcggacgacggcgccgcggtggcggtctggaccacgccggagagcgtcgaagcgggggcggtgttcgccgagatcggcccgcgcatggccgagttgagcggttcccggctggccgcgcagcaacagatggaaggcctcctggcgccgcaccggcccaaggagcccgcgtggttcctggccaccgtcggcgtctcgcccgaccaccagggcaagggtctgggcagcgccgtcgtgctccccggagtggaggcggccgagcgcgccggggtgcccgccttcctggaaacctccgcgccccgcaacctccccttctacgagcggctcggcttcaccgtcaccgccgacgtcgaggtgcccgaaggaccgcgcacctggtgcatgacccgcaagcccggtgcctgacgcccgccccacgacccgcagcgcccgaccgaaaggagcgcacgaccccatgcatcggtacctttaagaccaatgacttacaaggcagctgtagatcttagccactttctagagtcggggcggccggccgcttcgagcagacatgataagatacattgatgagtttggacaaaccacaactagaatgcagtgaaaaaaatgctttatttgtgaaatttgtgatgctattgctttatttgtaaccattataagctgcaataaacaagttaacaacaacaattgcattcattttatgtttcaggttcagggggaggtgtgggaggttttttaaagcaagtaaaacctctacaaatgtggtaaaatcgataaggatccgtcgaccgatgcccttgagagccttcaacccagtcagctccttccggtgggcgcggggcatgactatcgtcgccgcacttatgactgtcttctttatcatgcaactcgtaggacaggtgccggcagcgctcttccgcttcctcgctcactgactcgctgcgctcggtcgttcggctgcggcgagcggtatcagctcactcaaaggcggtaatacggttatccacagaatcaggggataacgcaggaaagaacatgtgagcaaaaggccagcaaaaggccaggaaccgtaaaaaggccgcgttgctggcgtttttccataggctccgcccccctgacgagcatcacaaaaatcgacgctcaagtcagaggtggcgaaacccgacaggactataaagataccaggcgtttccccctggaagctccctcgtgcgctctcctgttccgaccctgccgcttaccggatacctgtccgcctttctcccttcgggaagcgtggcgctttctcaatgctcacgctgtaggtatctcagttcggtgtaggtcgttcgctccaagctgggctgtgtgcacgaaccccccgttcagcccgaccgctgcgccttatccggtaactatcgtcttgagtccaacccggtaagacacgacttatcgccactggcagcagccactggtaacaggattagcagagcgaggtatgtaggcggtgctacagagttcttgaagtggtggcctaactacggctacactagaaggacagtatttggtatctgcgctctgctgaagccagttaccttcggaaaaagagttggtagctcttgatccggcaaacaaaccaccgctggtagcggtggtttttttgtttgcaagcagcagattacgcgcagaaaaaaaggatctcaagaagatcctttgatcttttctacggggtctgacgctcagtggaacgaaaactcacgttaagggattttggtcatgagattatcaaaaaggatcttcacctagatccttttaaattaaaaatgaagttttaaatcaatctaaagtatatatgagtaaacttggtctgacagttaccaatgcttaatcagtgaggcacctatctcagcgatctgtctatttcgttcatccatagttgcctgactccccgtcgtgtagataactacgatacgggagggcttaccatctggccccagtgctgcaatgataccgcgggacccacgctcaccggctccagatttatcagcaataaaccagccagccggaagggccgagcgcagaagtggtcctgcaactttatccgcctccatccagtctattaattgttgccgggaagctagagtaagtagttcgccagttaatagtttgcgcaacgttgttgccattgctacaggcatcgtggtgtcacgctcgtcgtttggtatggcttcattcagctccggttcccaacgatcaaggcgagttacatgatcccccatgttgtgcaaaaaagcggttagctccttcggtcctccgatcgttgtcagaagtaagttggccgcagtgttatcactcatggttatggcagcactgcataattctcttactgtcatgccatccgtaagatgcttttctgtgactggtgagtactcaaccaagtcattctgagaatagtgtatgcggcgaccgagttgctcttgcccggcgtcaatacgggataataccgcgccacatagcagaactttaaaagtgctcatcattggaaaacgttcttcggggcgaaaactctcaaggatcttaccgctgttgagatccagttcgatgtaacccactcgtgcacccaactgatcttcagcatcttttactttcaccagcgtttctgggtgagcaaaaacaggaaggcaaaatgccgcaaaaaagggaataagggcgacacggaaatgttgaatactcatactcttcctttttcaatattattgaagcatttatcagggttattgtctcatgagcggatacatatttgaatgtatttagaaaaataaacaaataggggttccgcgcacatttccccgaaaagtgccacctgcaggaaacagctatgaccatgattacgccaagctctagctagaggtcgacggtatcgagccccagctggttctttccgcctcagaagccatagagcccaccgcatccccagcatgcctgctattgtcttcccaatcctcccccttgctgtcctgccccaccccaccccccagaatagaatgacacctactcagacaatgcgatgcaatttcctcattttattaggaaaggacagtgggagtggcaccttccagggtcaaggaaggcacgggggaggggcaaacaacagatggctggcaactagaaggcacagtcgaggctgatcagcgggtttaaactcaatggtgatggtgatgatgaccggttagactttcctcttcttcttgggagaaccaccagaggggggtgtggcggtttcgttgttcagtgtggggagtgtgagcagatcagactgctggggggactctggccgggccccgctcccctccctcttgctggcgtcgtgccgccccccccggcttgtggtgggccggatgctggcccccctggcgttcaaagtctcccgccggtcgcaggccacgttcctatcaatcaacacagcgtgcctctcgatgttcctagcggcgttcatatctctatccatgaccaggccgcagtcggtgcacctaaacaccctatcggagagcttcaagtgggggttctgccagccgcacccgctgcaggtcttgctggaggggaaccacctgtcggccacggccagctcgctcccgtaccaggtggccttgtagttcacctgcctccgcagctcggcaggggcgctgtccaggatgacccggttcagcccggccttctgccggacgttcttccctggggcggccactgtccccctggcggacctggtcatgccggcgacgttcagatcctccagggccaccacggcgaaccctgtggtcagccgcttggtgatctggtgcagggcggcgtgccgccggacggccacctcgtgatgggccctccccacccgccgcttggccttctctctcctggcgctgcccttctgtgtcctggccagggcccgctgggccttgagcagccgcctctcagcctgcctcaggtgctgggggtttctcaccagggcgctgcttgggtcgtcgacgaccaggggcttggacagggcggccagcaccttcacccccaggtccactcccacggcgcccctctcccgctgccgcctgctgggccgatcgggcacctgcactgtcaccttgcagagcacggaggcgtaccacctgtgtccgcccctactcacagtcacggactgcaccacggcgtcgcctctgtcaatgagcctggcgagccgcttgccgctgtcgtgcagcctcacctcgccaatcctaggcagcctcagccttctgtagccagccagcctgatgctgggcttcttcacatcgtggtgcaatctaaagctatcccgagcccggcccttcttcttaaaccgggggtagcccaccctcctccccactctcttgccgctcaggctgtcgagccagttcttccatgcctggtcggcgtcaataaaggcgctctggaaggcgtaggtgttcacctcgtgccaccatgggcaggccccatccaggcccttccgggaatcccccttcacggcgttcagggccttctggatggctggcttcataggcacggggacccggacctgccgccgggcctgctcctcgggcacgccatcgcccacgagcttggccacctcggcccgccaccgctcgtgggcccccaccttggcggcgagggcgtggttgaaggcccacctggcggccccggcgtgccggctcagggcggccacctggacggaagtaggatcgagggcgaaccgaaaggccttcaggatctctgtctgcaccatgaccttcctcttcttcttaggggccatggtggcggctctccctatagtgagtcgtattagcggccgcggatctctagcggatctgacggttcactaaaccagctctgcttatatagacctcccaccgtacacgcctaccgcccatttgcgtcaatggggcggagttgttacgacattttggaaagtcccgttgattttggtgccaaaacaaactcccattgacgtcaatggggtggagacttggaaatccccgtgagtcaaaccgctatccacgcccattgatgtactgccaaaaccgcatcaccatggtaatagcgatgactaatacgtagatgtactgccaagtaggaaagtcccataaggtcatgtactgggcataatgccaggcgggccatttaccgtcattgacgtcaatagggggcgtacttggcatatgatacacttgatgtactgccaagtgggcagtttaccgtaaatactccacccattgacgtcaatggaaagtccctattggcgttactatgggaacatacgtcattattgacgtcaatgggcgggggtcgttgggcggtcagccaggcgggccatttaccgtaagttatgtaacgcggaactccatatatgggctatgaactaatgaccccgtaattgattactattaataactagtcaataatcaatgtcaacgcgtatatctggcccgtacatcgcgaagcagcgcaaaacgcctaaccctaagcagattcttcatgcaattgtcggtcaagaatcgatagtactaacatacgctctccatcaaaacaaaacgaaacaaaacaaactagcaaaataggctgtccccagtgcaagtgcaggtgccagaacatttctctatcgata

SEQ ID NO: 198 - DNA, 20 bp, synthetic construct
  source 1..20: mol_type = other DNA
ctggcaagtagtaaaatgct

SEQ ID NO: 199 - DNA, 20 bp, synthetic construct
  source 1..20: mol_type = other DNA
gcttcctcaaatcttatgca

SEQ ID NO: 200 - DNA, 22 bp, synthetic construct
  source 1..22: mol_type = other DNA
gatgtactagctgggctgttct

SEQ ID NO: 201 - DNA, 22 bp, synthetic construct
  source 1..22: mol_type = other DNA
ggaagctctgtccaaaccatct

SEQ ID NO: 202 - DNA, 23 bp, synthetic construct
  source 1..23: mol_type = other DNA
gaagagttttctgtggtgtgagc

SEQ ID NO: 203 - DNA, 23 bp, synthetic construct
  source 1..23: mol_type = other DNA
gcctcttataggagactgaaggc

SEQ ID NO: 204 - DNA, 22 bp, synthetic construct
  source 1..22: mol_type = other DNA
ctagtatctcgccaacctgacc

SEQ ID NO: 205 - DNA, 22 bp, synthetic construct
  source 1..22: mol_type = other DNA
gtgaagccaatgaccacagaac

SEQ ID NO: 206 - DNA, 22 bp, synthetic construct
  source 1..22: mol_type = other DNA
tttagtgcagcttctgccgtta

SEQ ID NO: 207 - DNA, 22 bp, synthetic construct
  source 1..22: mol_type = other DNA
acgcaactgacaggaggaattg

SEQ ID NO: 208 - DNA, 24 bp, synthetic construct
  source 1..24: mol_type = other DNA
atcgcatggaaacagacctggcag

SEQ ID NO: 209 - DNA, 24 bp, synthetic construct
  source 1..24: mol_type = other DNA
atcgggatgtggtgcatttggaat

SEQ ID NO: 210 - DNA, 24 bp, synthetic construct
  source 1..24: mol_type = other DNA
atcgcgactcaacctggtaaacat

SEQ ID NO: 211 - DNA, 24 bp, synthetic construct
  source 1..24: mol_type = other DNA
atcgaatcatttccccaagaggaa

SEQ ID NO: 212 - DNA, 24 bp, synthetic construct
  source 1..24: mol_type = other DNA
atcgaggcaagcatggaaacagac

SEQ ID NO: 213 - DNA, 24 bp, synthetic construct
  source 1..24: mol_type = other DNA
atcgtgtttctgccaggtctgttt

SEQ ID NO: 214 - DNA, 24 bp, synthetic construct
  source 1..24: mol_type = other DNA
atcgaagggatgtggtgcatttgg

SEQ ID NO: 215 - DNA, 24 bp, synthetic construct
  source 1..24: mol_type = other DNA
atcgtgtaaggaagctgcagcacc

SEQ ID NO: 216 - DNA, 24 bp, synthetic construct
  source 1..24: mol_type = other DNA
atcgggagacatccgtcggagaag

SEQ ID NO: 217 - DNA, 24 bp, synthetic construct
  source 1..24: mol_type = other DNA
atcgaaggatggagaaagagaaag

SEQ ID NO: 218 - DNA, 24 bp, synthetic construct
  source 1..24: mol_type = other DNA
atcgaggagaagcagtttggaaaa

SEQ ID NO: 219 - DNA, 24 bp, synthetic construct
  source 1..24: mol_type = other DNA
atcgcaaaccttagaggttctggc

SEQ ID NO: 220 - DNA, 24 bp, synthetic construct
  source 1..24: mol_type = other DNA
atcggaatctgcctaacaggaggt

SEQ ID NO: 221 - DNA, 24 bp, synthetic construct
  source 1..24: mol_type = other DNA
atcggagagagatggctccaggaa

SEQ ID NO: 222 - DNA, 24 bp, synthetic construct
  source 1..24: mol_type = other DNA
atcgaggatggagaggtggctaaa

SEQ ID NO: 223 - DNA, 24 bp, synthetic construct
  source 1..24: mol_type = other DNA
atcgagctagcacagactagagag

SEQ ID NO: 224 - DNA, 24 bp, synthetic construct
  source 1..24: mol_type = other DNA
atcggccatcctaagaaacgagag

SEQ ID NO: 225 - DNA, 24 bp, synthetic construct
  source 1..24: mol_type = other DNA
atcgtaccccgtctccctggcttt

SEQ ID NO: 226 - DNA, 24 bp, synthetic construct
  source 1..24: mol_type = other DNA
atcgggggcaaagactggaccctg

SEQ ID NO: 227 - DNA, 24 bp, synthetic construct
  source 1..24: mol_type = other DNA
atcgctcggagctgggaccacgtg

SEQ ID NO: 228 - DNA, 24 bp, synthetic construct
  source 1..24: mol_type = other DNA
atcgacagtggggactagagctca

SEQ ID NO: 229 - DNA, 24 bp, synthetic construct
  source 1..24: mol_type = other DNA
atcgcatctttgctgtgagctcta

SEQ ID NO: 230 - DNA, 24 bp, synthetic construct
  source 1..24: mol_type = other DNA
atcgatgcttcagagacgagatgg

SEQ ID NO: 231 - DNA, 24 bp, synthetic construct
  source 1..24: mol_type = other DNA
atcgcttaagcaaatgccacagct

SEQ ID NO: 232 - DNA, 24 bp, synthetic construct
  source 1..24: mol_type = other DNA
atcgtttaactacttactgtttgt

SEQ ID NO: 233 - DNA, 24 bp, synthetic construct
  source 1..24: mol_type = other DNA
atcgctgtggcatttgcttaagct

SEQ ID NO: 234 - DNA, 24 bp, synthetic construct
  source 1..24: mol_type = other DNA
atcggttgaacaaacagtaagtag

SEQ ID NO: 235 - DNA, 24 bp, synthetic construct
  source 1..24: mol_type = other DNA
atcgagagatgccttactaggtac

SEQ ID NO: 236 - DNA, 24 bp, synthetic construct
  source 1..24: mol_type = other DNA
atcgagctttacaaaagaagggga

SEQ ID NO: 237 - DNA, 24 bp, synthetic construct
  source 1..24: mol_type = other DNA
atcggacaaggttgaacaaacagt

SEQ ID NO: 238 - DNA, 24 bp, synthetic construct
  source 1..24: mol_type = other DNA
atcggtgtcagtttaagaatggtg

SEQ ID NO: 239 - DNA, 24 bp, synthetic construct
  source 1..24: mol_type = other DNA
atcgggtgcagttatgcctcagat

SEQ ID NO: 240 - DNA, 24 bp, synthetic construct
  source 1..24: mol_type = other DNA
atcgtgagggtaaaaagacctggg

SEQ ID NO: 241 - DNA, 24 bp, synthetic construct
  source 1..24: mol_type = other DNA
atcgttcagttagctcccaggtca

SEQ ID NO: 242 - DNA, 24 bp, synthetic construct
  source 1..24: mol_type = other DNA
atcgactgacgcacggaggaacaa

SEQ ID NO: 243 - DNA, 24 bp, synthetic construct
  source 1..24: mol_type = other DNA
atcgggagttttccacacggacac

SEQ ID NO: 244 - DNA, 24 bp, synthetic construct
  source 1..24: mol_type = other DNA
atcggccagggagacggggtactt

SEQ ID NO: 245 - DNA, 24 bp, synthetic construct
  source 1..24: mol_type = other DNA
atcgcatgctgtcctgaagtggac

SEQ ID NO: 246 - DNA, 24 bp, synthetic construct
  source 1..24: mol_type = other DNA
atcgtgtggaggccccactgccca

SEQ ID NO: 247 - DNA, 24 bp, synthetic construct
  source 1..24: mol_type = other DNA
atcgttgagtcttctctcttcttg

SEQ ID NO: 248 - DNA, 24 bp, synthetic construct
  source 1..24: mol_type = other DNA
atcgcagcctcaagatgtggacac

SEQ ID NO: 249 - DNA, 24 bp, synthetic construct
  source 1..24: mol_type = other DNA
atcgaagctatgagggctcacctg

SEQ ID NO: 250 - DNA, 24 bp, synthetic construct
  source 1..24: mol_type = other DNA
atcgtgggcatttgacacagttct

SEQ ID NO: 251 - DNA, 24 bp, synthetic construct
  source 1..24: mol_type = other DNA
atcggtcccaaaatgggcatttga

SEQ ID NO: 252 - DNA, 24 bp, synthetic construct
  source 1..24: mol_type = other DNA
atcgcagatagaataacataaacg

SEQ ID NO: 253 - DNA, 24 bp, synthetic construct
  source 1..24: mol_type = other DNA
atcgccactggatggagaatattt

SEQ ID NO: 254 - DNA, 24 bp, synthetic construct
  source 1..24: mol_type = other DNA
atcgcactatcagctgtggaacac

SEQ ID NO: 255 - DNA, 24 bp, synthetic construct
  source 1..24: mol_type = other DNA
aaaactgccaggtctgtttccatg

SEQ ID NO: 256 - DNA, 24 bp, synthetic construct
  source 1..24: mol_type = other DNA
aaaaattccaaatgcaccacatcc

SEQ ID NO: 257 - DNA, 24 bp, synthetic construct
  source 1..24: mol_type = other DNA
aaaaatgtttaccaggttgagtcg

SEQ ID NO: 258 - DNA, 24 bp, synthetic construct
  source 1..24: mol_type = other DNA
aaaattcctcttggggaaatgatt

SEQ ID NO: 259 - DNA, 24 bp, synthetic construct
  source 1..24: mol_type = other DNA
aaaagtctgtttccatgcttgcct

SEQ ID NO: 260 - DNA, 24 bp, synthetic construct
  source 1..24: mol_type = other DNA
aaaaaaacagacctggcagaaaca

SEQ ID NO: 261 - DNA, 24 bp, synthetic construct
  source 1..24: mol_type = other DNA
aaaaccaaatgcaccacatccctt

SEQ ID NO: 262 - DNA, 24 bp, synthetic construct
  source 1..24: mol_type = other DNA
aaaaggtgctgcagcttccttaca

SEQ ID NO: 263 - DNA, 24 bp, synthetic construct
  source 1..24: mol_type = other DNA
aaaacttctccgacggatgtctcc

SEQ ID NO: 264 - DNA, 24 bp, synthetic construct
  source 1..24: mol_type = other DNA
aaaactttctctttctccatcctt

SEQ ID NO: 265 - DNA, 24 bp, synthetic construct
  source 1..24: mol_type = other DNA
aaaattttccaaactgcttctcct

SEQ ID NO: 266 - DNA, 24 bp, synthetic construct
  source 1..24: mol_type = other DNA
aaaagccagaacctctaaggtttg

SEQ ID NO: 267 - DNA, 24 bp, synthetic construct
  source 1..24: mol_type = other DNA
aaaaacctcctgttaggcagattc

SEQ ID NO: 268 - DNA, 24 bp, synthetic construct
  source 1..24: mol_type = other DNA
aaaattcctggagccatctctctc

SEQ ID NO: 269 - DNA, 24 bp, synthetic construct
  source 1..24: mol_type = other DNA
aaaatttagccacctctccatcct

SEQ ID NO: 270 - DNA, 24 bp, synthetic construct
  source 1..24: mol_type = other DNA
aaaactctctagtctgtgctagct

SEQ ID NO: 271 - DNA, 24 bp, synthetic construct
  source 1..24: mol_type = other DNA
aaaactctcgtttcttaggatggc

SEQ ID NO: 272 - DNA, 24 bp, synthetic construct
  source 1..24: mol_type = other DNA
aaaaaaagccagggagacggggta

SEQ ID NO: 273 - DNA, 24 bp, synthetic construct
  source 1..24: mol_type = other DNA
aaaacagggtccagtctttgcccc

SEQ ID NO: 274 - DNA, 24 bp, synthetic construct
  source 1..24: mol_type = other DNA
aaaacacgtggtcccagctccgag

SEQ ID NO: 275 - DNA, 24 bp, synthetic construct
  source 1..24: mol_type = other DNA
aaaatgagctctagtccccactgt

SEQ ID NO: 276 - DNA, 24 bp, synthetic construct
  source 1..24: mol_type = other DNA
aaaatagagctcacagcaaagatg

SEQ ID NO: 277 - DNA, 24 bp, synthetic construct
  source 1..24: mol_type = other DNA
aaaaccatctcgtctctgaagcat

SEQ ID NO: 278 - DNA, 24 bp, synthetic construct
  source 1..24: mol_type = other DNA
aaaaagctgtggcatttgcttaag

SEQ ID NO: 279 - DNA, 24 bp, synthetic construct
  source 1..24: mol_type = other DNA
aaaaacaaacagtaagtagttaaa

SEQ ID NO: 280 - DNA, 24 bp, synthetic construct
  source 1..24: mol_type = other DNA
aaaaagcttaagcaaatgccacag

SEQ ID NO: 281 - DNA, 24 bp, synthetic construct
  source 1..24: mol_type = other DNA
aaaactacttactgtttgttcaac

SEQ ID NO: 282 - DNA, 24 bp, synthetic construct
  source 1..24: mol_type = other DNA
aaaagtacctagtaaggcatctct

SEQ ID NO: 283 - DNA, 24 bp, synthetic construct
  source 1..24: mol_type = other DNA
aaaatccccttcttttgtaaagct

SEQ ID NO: 284 - DNA, 24 bp, synthetic construct
  source 1..24: mol_type = other DNA
aaaaactgtttgttcaaccttgtc

SEQ ID NO: 285 - DNA, 24 bp, synthetic construct
  source 1..24: mol_type = other DNA
aaaacaccattcttaaactgacac

SEQ ID NO: 286 - DNA, 24 bp, synthetic construct
  source 1..24: mol_type = other DNA
aaaaatctgaggcataactgcacc

SEQ ID NO: 287 - DNA, 24 bp, synthetic construct
  source 1..24: mol_type = other DNA
aaaacccaggtctttttaccctca

SEQ ID NO: 288 - DNA, 24 bp, synthetic construct
  source 1..24: mol_type = other DNA
aaaatgacctgggagctaactgaa

SEQ ID NO: 289 - DNA, 24 bp, synthetic construct
  source 1..24: mol_type = other DNA
aaaattgttcctccgtgcgtcagt

SEQ ID NO: 290 - DNA, 24 bp, synthetic construct
  source 1..24: mol_type = other DNA
aaaagtgtccgtgtggaaaactcc

SEQ ID NO: 291 - DNA, 24 bp, synthetic construct
  source 1..24: mol_type = other DNA
aaaaaagtaccccgtctccctggc

SEQ ID NO: 292 - DNA, 24 bp, synthetic construct
  source 1..24: mol_type = other DNA
aaaagtccacttcaggacagcatg

SEQ ID NO: 293 - DNA, 24 bp, synthetic construct
  source 1..24: mol_type = other DNA
aaaatgggcagtggggcctccaca

SEQ ID NO: 294 - DNA, 24 bp, synthetic construct
  source 1..24: mol_type = other DNA
aaaacaagaagagagaagactcaa

SEQ ID NO: 295 - DNA, 24 bp, synthetic construct
  source 1..24: mol_type = other DNA
aaaagtgtccacatcttgaggctg

SEQ ID NO: 296 - DNA, 24 bp, synthetic construct
  source 1..24: mol_type = other DNA
aaaacaggtgagccctcatagctt

SEQ ID NO: 297 - DNA, 24 bp, synthetic construct
  source 1..24: mol_type = other DNA
aaaaagaactgtgtcaaatgccca

SEQ ID NO: 298 - DNA, 24 bp, synthetic construct
  source 1..24: mol_type = other DNA
aaaatcaaatgcccattttgggac

SEQ ID NO: 299 - DNA, 24 bp, synthetic construct
  source 1..24: mol_type = other DNA
aaaacgtttatgttattctatctg

SEQ ID NO: 300 - DNA, 24 bp, synthetic construct
  source 1..24: mol_type = other DNA
aaaaaaatattctccatccagtgg

SEQ ID NO: 301 - DNA, 24 bp, synthetic construct
  source 1..24: mol_type = other DNA
aaaaaaatattctccatccagtgg

SEQ ID NO: 302 - DNA, 2868 bp, synthetic construct
  source 1..2868: mol_type = other DNA
aggaacccctagtgatggagttggccactccctctctgcgcgctcgctcgctcactgaggccgggcgaccaaaggtcgcccgacgcccgggctttgcccgggcggcctcagtgagcgagcgagcgcgcagctgcctgcaggggcgcctgatgcggtattttctccttacgcatctgtgcggtatttcacaccgcatacgtcaaagcaaccatagtacgcgccctgtagcggcgcattaagcgcggcgggtgtggtggttacgcgcagcgtgaccgctacacttgccagcgccctagcgcccgctcctttcgctttcttcccttcctttctcgccacgttcgccggctttccccgtcaagctctaaatcgggggctccctttagggttccgatttagtgctttacggcacctcgaccccaaaaaacttgatttgggtgatggttcacgtagtgggccatcgccctgatagacggtttttcgccctttgacgttggagtccacgttctttaatagtggactcttgttccaaactggaacaacactcaaccctatctcgggctattcttttgatttataagggattttgccgatttcggcctattggttaaaaaatgagctgatttaacaaaaatttaacgcgaattttaacaaaatattaacgtttacaattttatggtgcactctcagtacaatctgctctgatgccgcatagttaagccagccccgacacccgccaacacccgctgacgcgccctgacgggcttgtctgctcccggcatccgcttacagacaagctgtgaccgtctccgggagctgcatgtgtcagaggttttcaccgtcatcaccgaaacgcgcgagacgaaagggcctcgtgatacgcctatttttataggttaatgtcatgataataatggtttcttagacgtcaggtggcacttttcggggaaatgtgcgcggaacccctatttgtttatttttctaaatacattcaaatatgtatccgctcatgagacaataaccctgataaatgcttcaataatattgaaaaaggaagagtatgagtattcaacatttccgtgtcgcccttattcccttttttgcggcattttgccttcctgtttttgctcacccagaaacgctggtgaaagtaaaagatgctgaagatcagttgggtgcacgagtgggttacatcgaactggatctcaacagcggtaagatccttgagagttttcgccccgaagaacgttttccaatgatgagcacttttaaagttctgctatgtggcgcggtattatcccgtattgacgccgggcaagagcaactcggtcgccgcatacactattctcagaatgacttggttgagtactcaccagtcacagaaaagcatcttacggatggcatgacagtaagagaattatgcagtgctgccataaccatgagtgataacactgcggccaacttacttctgacaacgatcggaggaccgaaggagctaaccgcttttttgcacaacatgggggatcatgtaactcgccttgatcgttgggaaccggagctgaatgaagccataccaaacgacgagcgtgacaccacgatgcctgtagcaatggcaacaacgttgcgcaaactattaactggcgaactacttactctagcttcccggcaacaattaatagactggatggaggcggataaagttgcaggaccacttctgcgctcggcccttccggctggctggtttattgctgataaatctggagccggtgagcgtgggtctcgcggtatcattgcagcactggggccagatggtaagccctcccgtatcgtagttatctacacgacggggagtcaggcaactatggatgaacgaaatagacagatcgctgagataggtgcctcactgattaagcattggtaactgtcagaccaagtttactcatatatactttagattgatttaaaacttcatttttaatttaaaaggatctaggtgaagatcctttttgataatctcatgaccaaaatcccttaacgtgagttttcgttccactgagcgtcagaccccgtagaaaagatcaaaggatcttcttgagatcctttttttctgcgcgtaatctgctgcttgcaaacaaaaaaaccaccgctaccagcggtggtttgtttgccggatcaagagctaccaactctttttccgaaggtaactggcttcagcagagcgcagataccaaatactgtccttctagtgtagccgtagttaggccaccacttcaagaactctgtagcaccgcctacatacctcgctctgctaatcctgttaccagtggctgctgccagtggcgataagtcgtgtcttaccgggttggactcaagacgatagttaccggataaggcgcagcggtcgggctgaacggggggttcgtgcacacagcccagcttggagcgaacgacctacaccgaactgagatacctacagcgtgagctatgagaaagcgccacgcttcccgaagggagaaaggcggacaggtatccggtaagcggcagggtcggaacaggagagcgcacgagggagcttccagggggaaacgcctggtatctttatagtcctgtcgggtttcgccacctctgacttgagcgtcgatttttgtgatgctcgtcaggggggcggagcctatggaaaaacgccagcaacgcggcctttttacggttcctggccttttgctggccttttgctcacatgtcctgcaggcagctgcgcgctcgctcgctcactgaggccgcccgggcgtcgggcgacctttggtcgcccggcctcagtgagcgagcgagcgcgcagagagggagtggccaactccatcactaggggttcct

SEQ ID NO: 303 - DNA, 3430 bp, synthetic construct
  source 1..3430: mol_type = other DNA
gcggccattcggtacaattcacgcgtaaaattttgaatttttgtaatttgtttttgtaattctttagtttgtatgtctgttgctattatgtctactattctttcccctgcactgtaccccccaatccccccttttcttttaaaattgtggatgaatactgccatttgtctcgaggtcgagaattcaaaaaaaatacagaggatactgtcactcgatcgctctttcgagcgtcagcagatcactctgctgaggtgactcaggccgagcgccggagccttcccgcttcgatgcgtcgtgcctaccgccccgagaggtggttggtcttatggatgctccacgggcgtttagcgtctcccgcctatcgcaggcgacgtttcgatcgatcagcactgcggtgtttcgtcctttccacaagatatataaagccaagaaatcgaaatactttcaagttacggtaagcatatgatagtccattttaaaacataattttaaaactgcaaactacccaagaaattattactttctacgtcacgtattttgtactaatatctttgtgtttacagtcaaattaattccaattatctctctaacagccttgtatcgtatatgcaaatatgaaggaatcatgggaaataggccctcggtgaagggggcggccgctcgaggctagtctcgtgatcgataccgtcgagatccgttcactaatcggtacctatcgatagagaaatgttctggcacctgcacttgcactggggacagcctattttgctagtttgttttgtttcgttttgttttgatggagagcgtatgttagtactatcgattcttgaccgacaattgcatgaagaatctgcttagggttaggcgttttgcgctgcttcgcgatgtacgggccagatatacgcgttgacattgattattgactagttattaatagtaatcaattacggggtcattagttcatagcccatatatggagttccgcgttacataacttacggtaaatggcccgcctggctgaccgcccaacgacccccgcccattgacgtcaataatgacgtatgttcccatagtaacgccaatagggactttccattgacgtcaatgggtggagtatttacggtaaactgcccacttggcagtacatcaagtgtatcatatgccaagtacgccccctattgacgtcaatgacggtaaatggcccgcctggcattatgcccagtacatgaccttatgggactttcctacttggcagtacatctacgtattagtcatcgctattaccatggtgatgcggttttggcagtacatcaatgggcgtggatagcggtttgactcacggggatttccaagtctccaccccattgacgtcaatgggagtttgttttggcaccaaaatcaacgggactttccaaaatgtcgtaacaactccgccccattgacgcaaatgggcggtaggcgtgtacggtgggaggtctatataagcagagctggtttagtgaaccgtcagatccgctagagatccgcggccgctaatacgactcactatagggagagccgccaccatggcccctaagaagaagaggaaggtcatggtgcagacagagatcctgaaggcctttcggttcgccctcgatcctacttccgtccaggtggccgccctgagccggcacgccggggccgccaggtgggccttcaaccacgccctcgccgccaaggtgggggcccacgagcggtggcgggccgaggtggccaagctcgtgggcgatggcgtgcccgaggagcaggcccggcggcaggtccgggtccccgtgcctatgaagccagccatccagaaggccctgaacgccgtgaagggggattcccggaagggcctggatggggcctgcccatggtggcacgaggtgaacacctacgccttccagagcgcctttattgacgccgaccaggcatggaagaactggctcgacagcctgagcggcaagagagtggggaggagggtgggctacccccggtttaagaagaagggccgggctcgggatagctttagattgcaccacgatgtgaagaagcccagcatcaggctggctggctacagaaggctgaggctgcctaggattggcgaggtgaggctgcacgacagcggcaagcggctcgccaggctcattgacagaggcgacgccgtggtgcagtccgtgactgtgagtaggggcggacacaggtggtacgcctccgtgctctgcaaggtgacagtgcaggtgcccgatcggcccagcaggcggcagcgggagaggggcgccgtgggagtggacctgggggtgaaggtgctggccgccctgtccaagcccctggtcgtcgacgacccaagcagcgccctggtgagaaacccccagcacctgaggcaggctgagaggcggctgctcaaggcccagcgggccctggccaggacacagaagggcagcgccaggagagagaaggccaagcggcgggtggggagggcccatcacgaggtggccgtccggcggcacgccgccctgcaccagatcaccaagcggctgaccacagggttcgccgtggtggccctggaggatctgaacgtcgccggcatgaccaggtccgccagggggacagtggccgccccagggaagaacgtccggcagaaggccgggctgaaccgggtcatcctggacagcgcccctgccgagctgcggaggcaggtgaactacaaggccacctggtacgggagcgagctggccgtggccgacaggtggttcccctccagcaagacctgcagcgggtgcggctggcagaacccccacttgaagctctccgatagggtgtttaggtgcaccgactgcggcctggtcatggatagagatatgaacgccgctaggaacatcgagaggcacgctgtgttgattgataggaacgtggcctgcgaccggcgggagactttgaacgccaggggggccagcatccggcccaccacaagccggggggggcggcacgacgccagcaagagggaggggagcggggcccggccagagtccccccagcagtctgatctgctcacactccccacactgaacaacgaaaccgccacacccccctctggtggttctcccaagaagaagaggaaagtctaaccggtcatcatcaccatcaccattgagtttaaacccgctgatcagcctcgactgtgccttctagttgccagccatctgttgtttgcccctcccccgtgccttccttgaccctggaaggtgccactcccactgtcctttcctaataaaatgaggaaattgcatcgcattgtctgagtaggtgtcattctattctggggggtggggtggggcaggacagcaagggggaggattgggaagacaatagcaggcatgctggggatgcggtgggctctatgggcggccgc

SEQ ID NO: 304 - DNA, 3430 bp, synthetic construct
  source 1..3430: mol_type = other DNA
gcggccattcggtacaattcacgcgtaaaattttgaatttttgtaatttgtttttgtaattctttagtttgtatgtctgttgctattatgtctactattctttcccctgcactgtaccccccaatccccccttttcttttaaaattgtggatgaatactgccatttgtctcgaggtcgagaattcaaaaaaaggtgctgcagcttccttacacgatcgctctttcgagcgtcagcagatcactctgctgaggtgactcaggccgagcgccggagccttcccgcttcgatgcgtcgtgcctaccgccccgagaggtggttggtcttatggatgctccacgggcgtttagcgtctcccgcctatcgcaggcgacgtttcgatcgatcagcactgcggtgtttcgtcctttccacaagatatataaagccaagaaatcgaaatactttcaagttacggtaagcatatgatagtccattttaaaacataattttaaaactgcaaactacccaagaaattattactttctacgtcacgtattttgtactaatatctttgtgtttacagtcaaattaattccaattatctctctaacagccttgtatcgtatatgcaaatatgaaggaatcatgggaaataggccctcggtgaagggggcggccgctcgaggctagtctcgtgatcgataccgtcgagatccgttcactaatcggtacctatcgatagagaaatgttctggcacctgcacttgcactggggacagcctattttgctagtttgttttgtttcgttttgttttgatggagagcgtatgttagtactatcgattcttgaccgacaattgcatgaagaatctgcttagggttaggcgttttgcgctgcttcgcgatgtacgggccagatatacgcgttgacattgattattgactagttattaatagtaatcaattacggggtcattagttcatagcccatatatggagttccgcgttacataacttacggtaaatggcccgcctggctgaccgcccaacgacccccgcccattgacgtcaataatgacgtatgttcccatagtaacgccaatagggactttccattgacgtcaatgggtggagtatttacggtaaactgcccacttggcagtacatcaagtgtatcatatgccaagtacgccccctattgacgtcaatgacggtaaatggcccgcctggcattatgcccagtacatgaccttatgggactttcctacttggcagtacatctacgtattagtcatcgctattaccatggtgatgcggttttggcagtacatcaatgggcgtggatagcggtttgactcacggggatttccaagtctccaccccattgacgtcaatgggagtttgttttggcaccaaaatcaacgggactttccaaaatgtcgtaacaactccgccccattgacgcaaatgggcggtaggcgtgtacggtgggaggtctatataagcagagctggtttagtgaaccgtcagatccgctagagatccgcggccgctaatacgactcactatagggagagccgccaccatggcccctaagaagaagaggaaggtcatggtgcagacagagatcctgaaggcctttcggttcgccctcgatcctacttccgtccaggtggccgccctgagccggcacgccggggccgccaggtgggccttcaaccacgccctcgccgccaaggtgggggcccacgagcggtggcgggccgaggtggccaagctcgtgggcgatggcgtgcccgaggagcaggcccggcggcaggtccgggtccccgtgcctatgaagccagccatccagaaggccctgaacgccgtgaagggggattcccggaagggcctggatggggcctgcccatggtggcacgaggtgaacacctacgccttccagagcgcctttattgacgccgaccaggcatggaagaactggctcgacagcctgagcggcaagagagtggggaggagggtgggctacccccggtttaagaagaagggccgggctcgggatagctttagattgcaccacgatgtgaagaagcccagcatcaggctggctggctacagaaggctgaggctgcctaggattggcgaggtgaggctgcacgacagcggcaagcggctcgccaggctcattgacagaggcgacgccgtggtgcagtccgtgactgtgagtaggggcggacacaggtggtacgcctccgtgctctgcaaggtgacagtgcaggtgcccgatcggcccagcaggcggcagcgggagaggggcgccgtgggagtggacctgggggtgaaggtgctggccgccctgtccaagcccctggtcgtcgacgacccaagcagcgccctggtgagaaacccccagcacctgaggcaggctgagaggcggctgctcaaggcccagcgggccctggccaggacacagaagggcagcgccaggagagagaaggccaagcggcgggtggggagggcccatcacgaggtggccgtccggcggcacgccgccctgcaccagatcaccaagcggctgaccacagggttcgccgtggtggccctggaggatctgaacgtcgccggcatgaccaggtccgccagggggacagtggccgccccagggaagaacgtccggcagaaggccgggctgaaccgggtcatcctggacagcgcccctgccgagctgcggaggcaggtgaactacaaggccacctggtacgggagcgagctggccgtggccgacaggtggttcccctccagcaagacctgcagcgggtgcggctggcagaacccccacttgaagctctccgatagggtgtttaggtgcaccgactgcggcctggtcatggatagagatatgaacgccgctaggaacatcgagaggcacgctgtgttgattgataggaacgtggcctgcgaccggcgggagactttgaacgccaggggggccagcatccggcccaccacaagccggggggggcggcacgacgccagcaagagggaggggagcggggcccggccagagtccccccagcagtctgatctgctcacactccccacactgaacaacgaaaccgccacacccccctctggtggttctcccaagaagaagaggaaagtctaaccggtcatcatcaccatcaccattgagtttaaacccgctgatcagcctcgactgtgccttctagttgccagccatctgttgtttgcccctcccccgtgccttccttgaccctggaaggtgccactcccactgtcctttcctaataaaatgaggaaattgcatcgcattgtctgagtaggtgtcattctattctggggggtggggtggggcaggacagcaagggggaggattgggaagacaatagcaggcatgctggggatgcggtgggctctatgggcggccgc

SEQ ID NO: 305 - DNA, 3430 bp, synthetic construct
  source 1..3430: mol_type = other DNA
gcggccattcggtacaattcacgcgtaaaattttgaatttttgtaatttgtttttgtaattctttagtttgtatgtctgttgctattatgtctactattctttcccctgcactgtaccccccaatccccccttttcttttaaaattgtggatgaatactgccatttgtctcgaggtcgagaattcaaaaaaatgagctctagtccccactgtcgatcgctctttcgagcgtcagcagatcactctgctgaggtgactcaggccgagcgccggagccttcccgcttcgatgcgtcgtgcctaccgccccgagaggtggttggtcttatggatgctccacgggcgtttagcgtctcccgcctatcgcaggcgacgtttcgatcgatcagcactgcggtgtttcgtcctttccacaagatatataaagccaagaaatcgaaatactttcaagttacggtaagcatatgatagtccattttaaaacataattttaaaactgcaaactacccaagaaattattactttctacgtcacgtattttgtactaatatctttgtgtttacagtcaaattaattccaattatctctctaacagccttgtatcgtatatgcaaatatgaaggaatcatgggaaataggccctcggtgaagggggcggccgctcgaggctagtctcgtgatcgataccgtcgagatccgttcactaatcggtacctatcgatagagaaatgttctggcacctgcacttgcactggggacagcctattttgctagtttgttttgtttcgttttgttttgatggagagcgtatgttagtactatcgattcttgaccgacaattgcatgaagaatctgcttagggttaggcgttttgcgctgcttcgcgatgtacgggccagatatacgcgttgacattgattattgactagttattaatagtaatcaattacggggtcattagttcatagcccatatatggagttccgcgttacataacttacggtaaatggcccgcctggctgaccgcccaacgacccccgcccattgacgtcaataatgacgtatgttcccatagtaacgccaatagggactttccattgacgtcaatgggtggagtatttacggtaaactgcccacttggcagtacatcaagtgtatcatatgccaagtacgccccctattgacgtcaatgacggtaaatggcccgcctggcattatgcccagtacatgaccttatgggactttcctacttggcagtacatctacgtattagtcatcgctattaccatggtgatgcggttttggcagtacatcaatgggcgtggatagcggtttgactcacggggatttccaagtctccaccccattgacgtcaatgggagtttgttttggcaccaaaatcaacgggactttccaaaatgtcgtaacaactccgccccattgacgcaaatgggcggtaggcgtgtacggtgggaggtctatataagcagagctggtttagtgaaccgtcagatccgctagagatccgcggccgctaatacgactcactatagggagagccgccaccatggcccctaagaagaagaggaaggtcatggtgcagacagagatcctgaaggcctttcggttcgccctcgatcctacttccgtccaggtggccgccctgagccggcacgccggggccgccaggtgggccttcaaccacgccctcgccgccaaggtgggggcccacgagcggtggcgggccgaggtggccaagctcgtgggcgatggcgtgcccgaggagcaggcccggcggcaggtccgggtccccgtgcctatgaagccagccatccagaaggccctgaacgccgtgaagggggattcccggaagggcctggatggggcctgcccatggtggcacgaggtgaacacctacgccttccagagcgcctttattgacgccgaccaggcatggaagaactggctcgacagcctgagcggcaagagagtggggaggagggtgggctacccccggtttaagaagaagggccgggctcgggatagctttagattgcaccacgatgtgaagaagcccagcatcaggctggctggctacagaaggctgaggctgcctaggattggcgaggtgaggctgcacgacagcggcaagcggctcgccaggctcattgacagaggcgacgccgtggtgcagtccgtgactgtgagtaggggcggacacaggtggtacgcctccgtgctctgcaaggtgacagtgcaggtgcccgatcggcccagcaggcggcagcgggagaggggcgccgtgggagtggacctgggggtgaaggtgctggccgccctgtccaagcccctggtcgtcgacgacccaagcagcgccctggtgagaaacccccagcacctgaggcaggctgagaggcggctgctcaaggcccagcgggccctggccaggacacagaagggcagcgccaggagagagaaggccaagcggcgggtggggagggcccatcacgaggtggccgtccggcggcacgccgccctgcaccagatcaccaagcggctgaccacagggttcgccgtggtggccctggaggatctgaacgtcgccggcatgaccaggtccgccagggggacagtggccgccccagggaagaacgtccggcagaaggccgggctgaaccgggtcatcctggacagcgcccctgccgagctgcggaggcaggtgaactacaaggccacctggtacgggagcgagctggccgtggccgacaggtggttcccctccagcaagacctgcagcgggtgcggctggcagaacccccacttgaagctctccgatagggtgtttaggtgcaccgactgcggcctggtcatggatagagatatgaacgccgctaggaacatcgagaggcacgctgtgttgattgataggaacgtggcctgcgaccggcgggagactttgaacgccaggggggccagcatccggcccaccacaagccggggggggcggcacgacgccagcaagagggaggggagcggggcccggccagagtccccccagcagtctgatctgctcacactccccacactgaacaacgaaaccgccacacccccctctggtggttctcccaagaagaagaggaaagtctaaccggtcatcatcaccatcaccattgagtttaaacccgctgatcagcctcgactgtgccttctagttgccagccatctgttgtttgcccctcccccgtgccttccttgaccctggaaggtgccactcccactgtcctttcctaataaaatgaggaaattgcatcgcattgtctgagtaggtgtcattctattctggggggtggggtggggcaggacagcaagggggaggattgggaagacaatagcaggcatgctggggatgcggtgggctctatgggcggccgc

SEQ ID NO: 306 - DNA, 6298 bp, synthetic construct
  source 1..6298: mol_type = other DNA
cctgcaggcagctgcgcgctcgctcgctcactgaggccgcccgggcgtcgggcgacctttggtcgcccggcctcagtgagcgagcgagcgcgcagagagggagtggccaactccatcactaggggttcctgcggccattcggtacaattcacgcgtaaaattttgaatttttgtaatttgtttttgtaattctttagtttgtatgtctgttgctattatgtctactattctttcccctgcactgtaccccccaatccccccttttcttttaaaattgtggatgaatactgccatttgtctcgaggtcgagaattcaaaaaaaatacagaggatactgtcactcgatcgctctttcgagcgtcagcagatcactctgctgaggtgactcaggccgagcgccggagccttcccgcttcgatgcgtcgtgcctaccgccccgagaggtggttggtcttatggatgctccacgggcgtttagcgtctcccgcctatcgcaggcgacgtttcgatcgatcagcactgcggtgtttcgtcctttccacaagatatataaagccaagaaatcgaaatactttcaagttacggtaagcatatgatagtccattttaaaacataattttaaaactgcaaactacccaagaaattattactttctacgtcacgtattttgtactaatatctttgtgtttacagtcaaattaattccaattatctctctaacagccttgtatcgtatatgcaaatatgaaggaatcatgggaaataggccctcggtgaagggggcggccgctcgaggctagtctcgtgatcgataccgtcgagatccgttcactaatcggtacctatcgatagagaaatgttctggcacctgcacttgcactggggacagcctattttgctagtttgttttgtttcgttttgttttgatggagagcgtatgttagtactatcgattcttgaccgacaattgcatgaagaatctgcttagggttaggcgttttgcgctgcttcgcgatgtacgggccagatatacgcgttgacattgattattgactagttattaatagtaatcaattacggggtcattagttcatagcccatatatggagttccgcgttacataacttacggtaaatggcccgcctggctgaccgcccaacgacccccgcccattgacgtcaataatgacgtatgttcccatagtaacgccaatagggactttccattgacgtcaatgggtggagtatttacggtaaactgcccacttggcagtacatcaagtgtatcatatgccaagtacgccccctattgacgtcaatgacggtaaatggcccgcctggcattatgcccagtacatgaccttatgggactttcctacttggcagtacatctacgtattagtcatcgctattaccatggtgatgcggttttggcagtacatcaatgggcgtggatagcggtttgactcacggggatttccaagtctccaccccattgacgtcaatgggagtttgttttggcaccaaaatcaacgggactttccaaaatgtcgtaacaactccgccccattgacgcaaatgggcggtaggcgtgtacggtgggaggtctatataagcagagctggtttagtgaaccgtcagatccgctagagatccgcggccgctaatacgactcactatagggagagccgccaccatggcccctaagaagaagaggaaggtcatggtgcagacagagatcctgaaggcctttcggttcgccctcgatcctacttccgtccaggtggccgccctgagccggcacgccggggccgccaggtgggccttcaaccacgccctcgccgccaaggtgggggcccacgagcggtggcgggccgaggtggccaagctcgtgggcgatggcgtgcccgaggagcaggcccggcggcaggtccgggtccccgtgcctatgaagccagccatccagaaggccctgaacgccgtgaagggggattcccggaagggcctggatggggcctgcccatggtggcacgaggtgaacacctacgccttccagagcgcctttattgacgccgaccaggcatggaagaactggctcgacagcctgagcggcaagagagtggggaggagggtgggctacccccggtttaagaagaagggccgggctcgggatagctttagattgcaccacgatgtgaagaagcccagcatcaggctggctggctacagaaggctgaggctgcctaggattggcgaggtgaggctgcacgacagcggcaagcggctcgccaggctcattgacagaggcgacgccgtggtgcagtccgtgactgtgagtaggggcggacacaggtggtacgcctccgtgctctgcaaggtgacagtgcaggtgcccgatcggcccagcaggcggcagcgggagaggggcgccgtgggagtggacctgggggtgaaggtgctggccgccctgtccaagcccctggtcgtcgacgacccaagcagcgccctggtgagaaacccccagcacctgaggcaggctgagaggcggctgctcaaggcccagcgggccctggccaggacacagaagggcagcgccaggagagagaaggccaagcggcgggtggggagggcccatcacgaggtggccgtccggcggcacgccgccctgcaccagatcaccaagcggctgaccacagggttcgccgtggtggccctggaggatctgaacgtcgccggcatgaccaggtccgccagggggacagtggccgccccagggaagaacgtccggcagaaggccgggctgaaccgggtcatcctggacagcgcccctgccgagctgcggaggcaggtgaactacaaggccacctggtacgggagcgagctggccgtggccgacaggtggttcccctccagcaagacctgcagcgggtgcggctggcagaacccccacttgaagctctccgatagggtgtttaggtgcaccgactgcggcctggtcatggatagagatatgaacgccgctaggaacatcgagaggcacgctgtgttgattgataggaacgtggcctgcgaccggcgggagactttgaacgccaggggggccagcatccggcccaccacaagccggggggggcggcacgacgccagcaagagggaggggagcggggcccggccagagtccccccagcagtctgatctgctcacactccccacactgaacaacgaaaccgccacacccccctctggtggttctcccaagaagaagaggaaagtctaaccggtcatcatcaccatcaccattgagtttaaacccgctgatcagcctcgactgtgccttctagttgccagccatctgttgtttgcccctcccccgtgccttccttgaccctggaaggtgccactcccactgtcctttcctaataaaatgaggaaattgcatcgcattgtctgagtaggtgtcattctattctggggggtggggtggggcaggacagcaagggggaggattgggaagacaatagcaggcatgctggggatgcggtgggctctatgggcggccgcaggaacccctagtgatggagttggccactccctctctgcgcgctcgctcgctcactgaggccgggcgaccaaaggtcgcccgacgcccgggctttgcccgggcggcctcagtgagcgagcgagcgcgcagctgcctgcaggggcgcctgatgcggtattttctccttacgcatctgtgcggtatttcacaccgcatacgtcaaagcaaccatagtacgcgccctgtagcggcgcattaagcgcggcgggtgtggtggttacgcgcagcgtgaccgctacacttgccagcgccctagcgcccgctcctttcgctttcttcccttcctttctcgccacgttcgccggctttccccgtcaagctctaaatcgggggctccctttagggttccgatttagtgctttacggcacctcgaccccaaaaaacttgatttgggtgatggttcacgtagtgggccatcgccctgatagacggtttttcgccctttgacgttggagtccacgttctttaatagtggactcttgttccaaactggaacaacactcaaccctatctcgggctattcttttgatttataagggattttgccgatttcggcctattggttaaaaaatgagctgatttaacaaaaatttaacgcgaattttaacaaaatattaacgtttacaattttatggtgcactctcagtacaatctgctctgatgccgcatagttaagccagccccgacacccgccaacacccgctgacgcgccctgacgggcttgtctgctcccggcatccgcttacagacaagctgtgaccgtctccgggagctgcatgtgtcagaggttttcaccgtcatcaccgaaacgcgcgagacgaaagggcctcgtgatacgcctatttttataggttaatgtcatgataataatggtttcttagacgtcaggtggcacttttcggggaaatgtgcgcggaacccctatttgtttatttttctaaatacattcaaatatgtatccgctcatgagacaataaccctgataaatgcttcaataatattgaaaaaggaagagtatgagtattcaacatttccgtgtcgcccttattcccttttttgcggcattttgccttcctgtttttgctcacccagaaacgctggtgaaagtaaaagatgctgaagatcagttgggtgcacgagtgggttacatcgaactggatctcaacagcggtaagatccttgagagttttcgccccgaagaacgttttccaatgatgagcacttttaaagttctgctatgtggcgcggtattatcccgtattgacgccgggcaagagcaactcggtcgccgcatacactattctcagaatgacttggttgagtactcaccagtcacagaaaagcatcttacggatggcatgacagtaagagaattatgcagtgctgccataaccatgagtgataacactgcggccaacttacttctgacaacgatcggaggaccgaaggagctaaccgcttttttgcacaacatgggggatcatgtaactcgccttgatcgttgggaaccggagctgaatgaagccataccaaacgacgagcgtgacaccacgatgcctgtagcaatggcaacaacgttgcgcaaactattaactggcgaactacttactctagcttcccggcaacaattaatagactggatggaggcggataaagttgcaggaccacttctgcgctcggcccttccggctggctggtttattgctgataaatctggagccggtgagcgtgggtctcgcggtatcattgcagcactggggccagatggtaagccctcccgtatcgtagttatctacacgacggggagtcaggcaactatggatgaacgaaatagacagatcgctgagataggtgcctcactgattaagcattggtaactgtcagaccaagtttactcatatatactttagattgatttaaaacttcatttttaatttaaaaggatctaggtgaagatcctttttgataatctcatgaccaaaatcccttaacgtgagttttcgttccactgagcgtcagaccccgtagaaaagatcaaaggatcttcttgagatcctttttttctgcgcgtaatctgctgcttgcaaacaaaaaaaccaccgctaccagcggtggtttgtttgccggatcaagagctaccaactctttttccgaaggtaactggcttcagcagagcgcagataccaaatactgtccttctagtgtagccgtagttaggccaccacttcaagaactctgtagcaccgcctacatacctcgctctgctaatcctgttaccagtggctgctgccagtggcgataagtcgtgtcttaccgggttggactcaagacgatagttaccggataaggcgcagcggtcgggctgaacggggggttcgtgcacacagcccagcttggagcgaacgacctacaccgaactgagatacctacagcgtgagctatgagaaagcgccacgcttcccgaagggagaaaggcggacaggtatccggtaagcggcagggtcggaacaggagagcgcacgagggagcttccagggggaaacgcctggtatctttatagtcctgtcgggtttcgccacctctgacttgagcgtcgatttttgtgatgctcgtcaggggggcggagcctatggaaaaacgccagcaacgcggcctttttacggttcctggccttttgctggccttttgctcacatgt

SEQ ID NO: 307 - DNA, 6298 bp, synthetic construct
  source 1..6298: mol_type = other DNA
cctgcaggcagctgcgcgctcgctcgctcactgaggccgcccgggcgtcgggcgacctttggtcgcccggcctcagtgagcgagcgagcgcgcagagagggagtggccaactccatcactaggggttcctgcggccattcggtacaattcacgcgtaaaattttgaatttttgtaatttgtttttgtaattctttagtttgtatgtctgttgctattatgtctactattctttcccctgcactgtaccccccaatccccccttttcttttaaaattgtggatgaatactgccatttgtctcgaggtcgagaattcaaaaaaaggtgctgcagcttccttacacgatcgctctttcgagcgtcagcagatcactctgctgaggtgactcaggccgagcgccggagccttcccgcttcgatgcgtcgtgcctaccgccccgagaggtggttggtcttatggatgctccacgggcgtttagcgtctcccgcctatcgcaggcgacgtttcgatcgatcagcactgcggtgtttcgtcctttccacaagatatataaagccaagaaatcgaaatactttcaagttacggtaagcatatgatagtccattttaaaacataattttaaaactgcaaactacccaagaaattattactttctacgtcacgtattttgtactaatatctttgtgtttacagtcaaattaattccaattatctctctaacagccttgtatcgtatatgcaaatatgaaggaatcatgggaaataggccctcggtgaagggggcggccgctcgaggctagtctcgtgatcgataccgtcgagatccgttcactaatcggtacctatcgatagagaaatgttctggcacctgcacttgcactggggacagcctattttgctagtttgttttgtttcgttttgttttgatggagagcgtatgttagtactatcgattcttgaccgacaattgcatgaagaatctgcttagggttaggcgttttgcgctgcttcgcgatgtacgggccagatatacgcgttgacattgattattgactagttattaatagtaatcaattacggggtcattagttcatagcccatatatggagttccgcgttacataacttacggtaaatggcccgcctggctgaccgcccaacgacccccgcccattgacgtcaataatgacgtatgttcccatagtaacgccaatagggactttccattgacgtcaatgggtggagtatttacggtaaactgcccacttggcagtacatcaagtgtatcatatgccaagtacgccccctattgacgtcaatgacggtaaatggcccgcctggcattatgcccagtacatgaccttatgggactttcctacttggcagtacatctacgtattagtcatcgctattaccatggtgatgcggttttggcagtacatcaatgggcgtggatagcggtttgactcacggggatttccaagtctccaccccattgacgtcaatgggagtttgttttggcaccaaaatcaacgggactttccaaaatgtcgtaacaactccgccccattgacgcaaatgggcggtaggcgtgtacggtgggaggtctatataagcagagctggtttagtgaaccgtcagatccgctagagatccgcggccgctaatacgactcactatagggagagccgccaccatggcccctaagaagaagaggaaggtcatggtgcagacagagatcctgaaggcctttcggttcgccctcgatcctacttccgtccaggtggccgccctgagccggcacgccggggccgccaggtgggccttcaaccacgccctcgccgccaaggtgggggcccacgagcggtggcgggccgaggtggccaagctcgtgggcgatggcgtgcccgaggagcaggcccggcggcaggtccgggtccccgtgcctatgaagccagccatccagaaggccctgaacgccgtgaagggggattcccggaagggcctggatggggcctgcccatggtggcacgaggtgaacacctacgccttccagagcgcctttattgacgccgaccaggcatggaagaactggctcgacagcctgagcggcaagagagtggggaggagggtgggctacccccggtttaagaagaagggccgggctcgggatagctttagattgcaccacgatgtgaagaagcccagcatcaggctggctggctacagaaggctgaggctgcctaggattggcgaggtgaggctgcacgacagcggcaagcggctcgccaggctcattgacagaggcgacgccgtggtgcagtccgtgactgtgagtaggggcggacacaggtggtacgcctccgtgctctgcaaggtgacagtgcaggtgcccgatcggcccagcaggcggcagcgggagaggggcgccgtgggagtggacctgggggtgaaggtgctggccgccctgtccaagcccctggtcgtcgacgacccaagcagcgccctggtgagaaacccccagcacctgaggcaggctgagaggcggctgctcaaggcccagcgggccctggccaggacacagaagggcagcgccaggagagagaaggccaagcggcgggtggggagggcccatcacgaggtggccgtccggcggcacgccgccctgcaccagatcaccaagcggctgaccacagggttcgccgtggtggccctggaggatctgaacgtcgccggcatgaccaggtccgccagggggacagtggccgccccagggaagaacgtccggcagaaggccgggctgaaccgggtcatcctggacagcgcccctgccgagctgcggaggcaggtgaactacaaggccacctggtacgggagcgagctggccgtggccgacaggtggttcccctccagcaagacctgcagcgggtgcggctggcagaacccccacttgaagctctccgatagggtgtttaggtgcaccgactgcggcctggtcatggatagagatatgaacgccgctaggaacatcgagaggcacgctgtgttgattgataggaacgtggcctgcgaccggcgggagactttgaacgccaggggggccagcatccggcccaccacaagccggggggggcggcacgacgccagcaagagggaggggagcggggcccggccagagtccccccagcagtctgatctgctcacactccccacactgaacaacgaaaccgccacacccccctctggtggttctcccaagaagaagaggaaagtctaaccggtcatcatcaccatcaccattgagtttaaacccgctgatcagcctcgactgtgccttctagttgccagccatctgttgtttgcccctcccccgtgccttccttgaccctggaaggtgccactcccactgtcctttcctaataaaatgaggaaattgcatcgcattgtctgagtaggtgtcattctattctggggggtggggtggggcaggacagcaagggggaggattgggaagacaatagcaggcatgctggggatgcggtgggctctatgggcggccgcaggaacccctagtgatggagttggccactccctctctgcgcgctcgctcgctcactgaggccgggcgaccaaaggtcgcccgacgcccgggctttgcccgggcggcctcagtgagcgagcgagcgcgcagctgcctgcaggggcgcctgatgcggtattttctccttacgcatctgtgcggtatttcacaccgcatacgtcaaagcaaccatagtacgcgccctgtagcggcgcattaagcgcggcgggtgtggtggttacgcgcagcgtgaccgctacacttgccagcgccctagcgcccgctcctttcgctttcttcccttcctttctcgccacgttcgccggctttccccgtcaagctctaaatcgggggctccctttagggttccgatttagtgctttacggcacctcgaccccaaaaaacttgatttgggtgatggttcacgtagtgggccatcgccctgatagacggtttttcgccctttgacgttggagtccacgttctttaatagtggactcttgttccaaactggaacaacactcaaccctatctcgggctattcttttgatttataagggattttgccgatttcggcctattggttaaaaaatgagctgatttaacaaaaatttaacgcgaattttaacaaaatattaacgtttacaattttatggtgcactctcagtacaatctgctctgatgccgcatagttaagccagccccgacacccgccaacacccgctgacgcgccctgacgggcttgtctgctcccggcatccgcttacagacaagctgtgaccgtctccgggagctgcatgtgtcagaggttttcaccgtcatcaccgaaacgcgcgagacgaaagggcctcgtgatacgcctatttttataggttaatgtcatgataataatggtttcttagacgtcaggtggcacttttcggggaaatgtgcgcggaacccctatttgtttatttttctaaatacattcaaatatgtatccgctcatgagacaataaccctgataaatgcttcaataatattgaaaaaggaagagtatgagtattcaacatttccgtgtcgcccttattcccttttttgcggcattttgccttcctgtttttgctcacccagaaacgctggtgaaagtaaaagatgctgaagatcagttgggtgcacgagtgggttacatcgaactggatctcaacagcggtaagatccttgagagttttcgccccgaagaacgttttccaatgatgagcacttttaaagttctgctatgtggcgcggtattatcccgtattgacgccgggcaagagcaactcggtcgccgcatacactattctcagaatgacttggttgagtactcaccagtcacagaaaagcatcttacggatggcatgacagtaagagaattatgcagtgctgccataaccatgagtgataacactgcggccaacttacttctgacaacgatcggaggaccgaaggagctaaccgcttttttgcacaacatgggggatcatgtaactcgccttgatcgttgggaaccggagctgaatgaagccataccaaacgacgagcgtgacaccacgatgcctgtagcaatggcaacaacgttgcgcaaactattaactggcgaactacttactctagcttcccggcaacaattaatagactggatggaggcggataaagttgcaggaccacttctgcgctcggcccttccggctggctggtttattgctgataaatctggagccggtgagcgtgggtctcgcggtatcattgcagcactggggccagatggtaagccctcccgtatcgtagttatctacacgacggggagtcaggcaactatggatgaacgaaatagacagatcgctgagataggtgcctcactgattaagcattggtaactgtcagaccaagtttactcatatatactttagattgatttaaaacttcatttttaatttaaaaggatctaggtgaagatcctttttgataatctcatgaccaaaatcccttaacgtgagttttcgttccactgagcgtcagaccccgtagaaaagatcaaaggatcttcttgagatcctttttttctgcgcgtaatctgctgcttgcaaacaaaaaaaccaccgctaccagcggtggtttgtttgccggatcaagagctaccaactctttttccgaaggtaactggcttcagcagagcgcagataccaaatactgtccttctagtgtagccgtagttaggccaccacttcaagaactctgtagcaccgcctacatacctcgctctgctaatcctgttaccagtggctgctgccagtggcgataagtcgtgtcttaccgggttggactcaagacgatagttaccggataaggcgcagcggtcgggctgaacggggggttcgtgcacacagcccagcttggagcgaacgacctacaccgaactgagatacctacagcgtgagctatgagaaagcgccacgcttcccgaagggagaaaggcggacaggtatccggtaagcggcagggtcggaacaggagagcgcacgagggagcttccagggggaaacgcctggtatctttatagtcctgtcgggtttcgccacctctgacttgagcgtcgatttttgtgatgctcgtcaggggggcggagcctatggaaaaacgccagcaacgcggcctttttacggttcctggccttttgctggccttttgctcacatgt

SEQ ID NO: 308 - DNA, 6298 bp, synthetic construct
  source 1..6298: mol_type = other DNA
cctgcaggcagctgcgcgctcgctcgctcactgaggccgcccgggcgtcgggcgacctttggtcgcccggcctcagtgagcgagcgagcgcgcagagagggagtggccaactccatcactaggggttcctgcggccattcggtacaattcacgcgtaaaattttgaatttttgtaatttgtttttgtaattctttagtttgtatgtctgttgctattatgtctactattctttcccctgcactgtaccccccaatccccccttttcttttaaaattgtggatgaatactgccatttgtctcgaggtcgagaattcaaaaaaatgagctctagtccccactgtcgatcgctctttcgagcgtcagcagatcactctgctgaggtgactcaggccgagcgccggagccttcccgcttcgatgcgtcgtgcctaccgccccgagaggtggttggtcttatggatgctccacgggcgtttagcgtctcccgcctatcgcaggcgacgtttcgatcgatcagcactgcggtgtttcgtcctttccacaagatatataaagccaagaaatcgaaatactttcaagttacggtaagcatatgatagtccattttaaaacataattttaaaactgcaaactacccaagaaattattactttctacgtcacgtattttgtactaatatctttgtgtttacagtcaaattaattccaattatctctctaacagccttgtatcgtatatgcaaatatgaaggaatcatgggaaataggccctcggtgaagggggcggccgctcgaggctagtctcgtgatcgataccgtcgagatccgttcactaatcggtacctatcgatagagaaatgttctggcacctgcacttgcactggggacagcctattttgctagtttgttttgtttcgttttgttttgatggagagcgtatgttagtactatcgattcttgaccgacaattgcatgaagaatctgcttagggttaggcgttttgcgctgcttcgcgatgtacgggccagatatacgcgttgacattgattattgactagttattaatagtaatcaattacggggtcattagttcatagcccatatatggagttccgcgttacataacttacggtaaatggcccgcctggctgaccgcccaacgacccccgcccattgacgtcaataatgacgtatgttcccatagtaacgccaatagggactttccattgacgtcaatgggtggagtatttacggtaaactgcccacttggcagtacatcaagtgtatcatatgccaagtacgccccctattgacgtcaatgacggtaaatggcccgcctggcattatgcccagtacatgaccttatgggactttcctacttggcagtacatctacgtattagtcatcgctattaccatggtgatgcggttttggcagtacatcaatgggcgtggatagcggtttgactcacggggatttccaagtctccaccccattgacgtcaatgggagtttgttttggcaccaaaatcaacgggactttccaaaatgtcgtaacaactccgccccattgacgcaaatgggcggtaggcgtgtacggtgggaggtctatataagcagagctggtttagtgaaccgtcagatccgctagagatccgcggccgctaatacgactcactatagggagagccgccaccatggcccctaagaagaagaggaaggtcatggtgcagacagagatcctgaaggcctttcggttcgccctcgatcctacttccgtccaggtggccgccctgagccggcacgccggggccgccaggtgggccttcaaccacgccctcgccgccaaggtgggggcccacgagcggtggcgggccgaggtggccaagctcgtgggcgatggcgtgcccgaggagcaggcccggcggcaggtccgggtccccgtgcctatgaagccagccatccagaaggccctgaacgccgtgaagggggattcccggaagggcctggatggggcctgcccatggtggcacgaggtgaacacctacgccttccagagcgcctttattgacgccgaccaggcatggaagaactggctcgacagcctgagcggcaagagagtggggaggagggtgggctacccccggtttaagaagaagggccgggctcgggatagctttagattgcaccacgatgtgaagaagcccagcatcaggctggctggctacagaaggctgaggctgcctaggattggcgaggtgaggctgcacgacagcggcaagcggctcgccaggctcattgacagaggcgacgccgtggtgcagtccgtgactgtgagtaggggcggacacaggtggtacgcctccgtgctctgcaaggtgacagtgcaggtgcccgatcggcccagcaggcggcagcgggagaggggcgccgtgggagtggacctgggggtgaaggtgctggccgccctgtccaagcccctggtcgtcgacgacccaagcagcgccctggtgagaaacccccagcacctgaggcaggctgagaggcggctgctcaaggcccagcgggccctggccaggacacagaagggcagcgccaggagagagaaggccaagcggcgggtggggagggcccatcacgaggtggccgtccggcggcacgccgccctgcaccagatcaccaagcggctgaccacagggttcgccgtggtggccctggaggatctgaacgtcgccggcatgaccaggtccgccagggggacagtggccgccccagggaagaacgtccggcagaaggccgggctgaaccgggtcatcctggacagcgcccctgccgagctgcggaggcaggtgaactacaaggccacctggtacgggagcgagctggccgtggccgacaggtggttcccctccagcaagacctgcagcgggtgcggctggcagaacccccacttgaagctctccgatagggtgtttaggtgcaccgactgcggcctggtcatggatagagatatgaacgccgctaggaacatcgagaggcacgctgtgttgattgataggaacgtggcctgcgaccggcgggagactttgaacgccaggggggccagcatccggcccaccacaagccggggggggcggcacgacgccagcaagagggaggggagcggggcccggccagagtccccccagcagtctgatctgctcacactccccacactgaacaacgaaaccgccacacccccctctggtggttctcccaagaagaagaggaaagtctaaccggtcatcatcaccatcaccattgagtttaaacccgctgatcagcctcgactgtgccttctagttgccagccatctgttgtttgcccctcccccgtgccttccttgaccctggaaggtgccactcccactgtcctttcctaataaaatgaggaaattgcatcgcattgtctgagtaggtgtcattctattctggggggtggggtggggcaggacagcaagggggaggattgggaagacaatagcaggcatgctggggatgcggtgggctctatgggcggccgcaggaacccctagtgatggagttggccactccctctctgcgcgctcgctcgctcactgaggccgggcgaccaaaggtcgcccgacgcccgggctttgcccgggcggcctcagtgagcgagcgagcgcgcagctgcctgcaggggcgcctgatgcggtattttctccttacgcatctgtgcggtatttcacaccgcatacgtcaaagcaaccatagtacgcgccctgtagcggcgcattaagcgcggcgggtgtggtggttacgcgcagcgtgaccgctacacttgccagcgccctagcgcccgctcctttcgctttcttcccttcctttctcgccacgttcgccggctttccccgtcaagctctaaatcgggggctccctttagggttccgatttagtgctttacggcacctcgaccccaaaaaacttgatttgggtgatggttcacgtagtgggccatcgccctgatagacggtttttcgccctttgacgttggagtccacgttctttaatagtggactcttgttccaaactggaacaacactcaaccctatctcgggctattcttttgatttataagggattttgccgatttcggcctattggttaaaaaatgagctgatttaacaaaaatttaacgcgaattttaacaaaatattaacgtttacaattttatggtgcactctcagtacaatctgctctgatgccgcatagttaagccagccccgacacccgccaacacccgctgacgcgccctgacgggcttgtctgctcccggcatccgcttacagacaagctgtgaccgtctccgggagctgcatgtgtcagaggttttcaccgtcatcaccgaaacgcgcgagacgaaagggcctcgtgatacgcctatttttataggttaatgtcatgataataatggtttcttagacgtcaggtggcacttttcggggaaatgtgcgcggaacccctatttgtttatttttctaaatacattcaaatatgtatccgctcatgagacaataaccctgataaatgcttcaataatattgaaaaaggaagagtatgagtattcaacatttccgtgtcgcccttattcccttttttgcggcattttgccttcctgtttttgctcacccagaaacgctggtgaaagtaaaagatgctgaagatcagttgggtgcacgagtgggttacatcgaactggatctcaacagcggtaagatccttgagagttttcgccccgaagaacgttttccaatgatgagcacttttaaagttctgctatgtggcgcggtattatcccgtattgacgccgggcaagagcaactcggtcgccgcatacactattctcagaatgacttggttgagtactcaccagtcacagaaaagcatcttacggatggcatgacagtaagagaattatgcagtgctgccataaccatgagtgataacactgcggccaacttacttctgacaacgatcggaggaccgaaggagctaaccgcttttttgcacaacatgggggatcatgtaactcgccttgatcgttgggaaccggagctgaatgaagccataccaaacgacgagcgtgacaccacgatgcctgtagcaatggcaacaacgttgcgcaaactattaactggcgaactacttactctagcttcccggcaacaattaatagactggatggaggcggataaagttgcaggaccacttctgcgctcggcccttccggctggctggtttattgctgataaatctggagccggtgagcgtgggtctcgcggtatcattgcagcactggggccagatggtaagccctcccgtatcgtagttatctacacgacggggagtcaggcaactatggatgaacgaaatagacagatcgctgagataggtgcctcactgattaagcattggtaactgtcagaccaagtttactcatatatactttagattgatttaaaacttcatttttaatttaaaaggatctaggtgaagatcctttttgataatctcatgaccaaaatcccttaacgtgagttttcgttccactgagcgtcagaccccgtagaaaagatcaaaggatcttcttgagatcctttttttctgcgcgtaatctgctgcttgcaaacaaaaaaaccaccgctaccagcggtggtttgtttgccggatcaagagctaccaactctttttccgaaggtaactggcttcagcagagcgcagataccaaatactgtccttctagtgtagccgtagttaggccaccacttcaagaactctgtagcaccgcctacatacctcgctctgctaatcctgttaccagtggctgctgccagtggcgataagtcgtgtcttaccgggttggactcaagacgatagttaccggataaggcgcagcggtcgggctgaacggggggttcgtgcacacagcccagcttggagcgaacgacctacaccgaactgagatacctacagcgtgagctatgagaaagcgccacgcttcccgaagggagaaaggcggacaggtatccggtaagcggcagggtcggaacaggagagcgcacgagggagcttccagggggaaacgcctggtatctttatagtcctgtcgggtttcgccacctctgacttgagcgtcgatttttgtgatgctcgtcaggggggcggagcctatggaaaaacgccagcaacgcggcctttttacggttcctggccttttgctggccttttgctcacatgt